European Patent Specification EP 3 775 184 B1, published December 10, 2025. Title: MODULATING LACTOGENIC ACTIVITY IN MAMMALIAN CELLS. Applicant: GENENTECH, INC. The sequence listing filed with the application follows.

SEQUENCE LISTING (54 sequences)

SEQ ID NO: 1 - protein, 6 aa, Artificial Sequence
  source: /note="Description of Artificial Sequence: Synthetic peptide"
SSYYMA

SEQ ID NO: 2 - protein, 5 aa, Artificial Sequence
  source: /note="Description of Artificial Sequence: Synthetic peptide"
DSYMS

SEQ ID NO: 3 - protein, 17 aa, Artificial Sequence
  source: /note="Description of Artificial Sequence: Synthetic peptide"
DMYPDNGDSSYNQKFRE

SEQ ID NO: 4 - protein, 8 aa, Artificial Sequence
  source: /note="Description of Artificial Sequence: Synthetic peptide"
APRWYFSV

SEQ ID NO: 5 - protein, 11 aa, Artificial Sequence
  source: /note="Description of Artificial Sequence: Synthetic peptide"
RASQDISNYLN

SEQ ID NO: 6 - protein, 7 aa, Artificial Sequence
  source: /note="Description of Artificial Sequence: Synthetic peptide"
YTSRLRS

SEQ ID NO: 7 - protein, 9 aa, Artificial Sequence
  source: /note="Description of Artificial Sequence: Synthetic peptide"
QQGHTLPPT

SEQ ID NO: 8 - protein, 117 aa, Artificial Sequence
  source: /note="Description of Artificial Sequence: Synthetic polypeptide"
EVQLVQSGAEVKKPGASVKVSCKASGYTFTDSYMSWVRQAPGQGLEWIGDMYPDNGDSSYNQKFRERVTITRDTSTSTAYLELSSLRSEDTAVYYCVLAPRWYFSVWGQGTLVTVSS

SEQ ID NO: 9 - protein, 107 aa, Artificial Sequence
  source: /note="Description of Artificial Sequence: Synthetic polypeptide"
DIQMTQSPSSLSASVGDRVTITCRASQDISNYLNWYQQKPGKAPKLLIYYTSRLRSGVPSRFSGSGSGTDFTLTISSLQPEDFATYYCQQGHTLPPTFGQGTKVEIK

SEQ ID NO: 10 - protein, 5 aa, Artificial Sequence
  source: /note="Description of Artificial Sequence: Synthetic peptide"
NYLIE

SEQ ID NO: 11 - protein, 17 aa, Artificial Sequence
  source: /note="Description of Artificial Sequence: Synthetic peptide"
VINPGSGDTYYSEKFKG

SEQ ID NO: 12 - protein, 5 aa, Artificial Sequence
  source: /note="Description of Artificial Sequence: Synthetic peptide"
DRLDY

SEQ ID NO: 13 - protein, 11 aa, Artificial Sequence
  source: /note="Description of Artificial Sequence: Synthetic peptide"
HASQDISSYIV

SEQ ID NO: 14 - protein, 7 aa, Artificial Sequence
  source: /note="Description of Artificial Sequence: Synthetic peptide"
HGTNLED

SEQ ID NO: 15 - protein, 9 aa, Artificial Sequence
  source: /note="Description of Artificial Sequence: Synthetic peptide"
VHYAQFPYT

SEQ ID NO: 16 - protein, 114 aa, Artificial Sequence
  source: /note="Description of Artificial Sequence: Synthetic polypeptide"
EVQLVQSGAEVKKPGASVKVSCKASGYAFTNYLIEWVRQAPGQGLEWIGVINPGSGDTYYSEKFKGRVTITRDTSTSTAYLELSSLRSEDTAVYYCARDRLDYWGQGTLVTVSS

SEQ ID NO: 17 - protein, 107 aa, Artificial Sequence
  source: /note="Description of Artificial Sequence: Synthetic polypeptide"
DIQMTQSPSSLSASVGDRVTITCHASQDISSYIVWYQQKPGKAPKLLIYHGTNLEDGVPSRFSGSGSGTDFTLTISSLQPEDFATYYCVHYAQFPYTFGQGTKVEIK

SEQ ID NO: 18 - protein, 215 aa, Artificial Sequence
  source: /note="Description of Artificial Sequence: Synthetic polypeptide"
DIQMTQSPSSLSASVGDRVTITCKASAAVGTYVAWYQQKPGKAPKLLIYSASYRKRGVPSRFSGSGSGTDFTLTISSLQPEDFATYYCHQYYTYPLFTFGQGTKLEIKRTVAAPSVFIFPPSDEQLKSGTASVVCLLNNFYPREAKVQWKVDNALQSGNSQESVTEQDSKDSTYSLSSTLTLSKADYEKHKVYACEVTHQGLSSPVTKSFNRGEC

SEQ ID NO: 19 - protein, 214 aa, Artificial Sequence
  source: /note="Description of Artificial Sequence: Synthetic polypeptide"
QAVVTQEPSLTVSPGGTVTLTCGSSTGAVTTSNYANWVQEKPGQAFRGLIGGTNKRAPGTPARFSGSLLGGKAALTLSGAQPEDEAEYYCALWYSNLWVFGGGTKLTVLSSASTKGPSVFPLAPSSKSTSGGTAALGCLVKDYFPEPVTVSWNSGALTSGVHTFPAVLQSSGLYSLSSVVTVPSSSLGTQTYICNVNHKPSNTKVDKKVEPKSC

SEQ ID NO: 20 - protein, 694 aa, Artificial Sequence
  source: /note="Description of Artificial Sequence: Synthetic polypeptide"
QVQLVQSGAEVKKPGASVKVSCKASGYTFTEFGMNWVRQAPGQGLEWMGWINTKTGEATYVEEFKGRVTFTTDTSTSTAYMELRSLRSDDTAVYYCARWDFAYYVEAMDYWGQGTTVTVSSASTKGPSVFPLAPSSKSTSGGTAALGCLVKDYFPEPVTVSWNSGALTSGVHTFPAVLQSSGLYSLSSVVTVPSSSLGTQTYICNVNHKPSNTKVDKKVEPKSCDGGGGSGGGGSEVQLLESGGGLVQPGGSLRLSCAASGFTFSTYAMNWVRQAPGKGLEWVSRIRSKYNNYATYYADSVKGRFTISRDDSKNTLYLQMNSLRAEDTAVYYCVRHGNFGNSYVSWFAYWGQGTLVTVSSASVAAPSVFIFPPSDEQLKSGTASVVCLLNNFYPREAKVQWKVDNALQSGNSQESVTEQDSKDSTYSLSSTLTLSKADYEKHKVYACEVTHQGLSSPVTKSFNRGECDKTHTCPPCPAPEAAGGPSVFLFPPKPKDTLMISRTPEVTCVVVDVSHEDPEVKFNWYVDGVEVHNAKTKPREEQYNSTYRVVSVLTVLHQDWLNGKEYKCKVSNKALGAPIEKTISKAKGQPREPQVYTLPPCRDELTKNQVSLWCLVKGFYPSDIAVEWESNGQPENNYKTTPPVLDSDGSFFLYSKLTVDKSRWQQGNVFSCSVMHEALHNHYTQKSLSLSPGK

SEQ ID NO: 21 - protein, 451 aa, Artificial Sequence
  source: /note="Description of Artificial Sequence: Synthetic polypeptide"
QVQLVQSGAEVKKPGASVKVSCKASGYTFTEFGMNWVRQAPGQGLEWMGWINTKTGEATYVEEFKGRVTFTTDTSTSTAYMELRSLRSDDTAVYYCARWDFAYYVEAMDYWGQGTTVTVSSASTKGPSVFPLAPSSKSTSGGTAALGCLVKDYFPEPVTVSWNSGALTSGVHTFPAVLQSSGLYSLSSVVTVPSSSLGTQTYICNVNHKPSNTKVDKKVEPKSCDKTHTCPPCPAPEAAGGPSVFLFPPKPKDTLMISRTPEVTCVVVDVSHEDPEVKFNWYVDGVEVHNAKTKPREEQYNSTYRVVSVLTVLHQDWLNGKEYKCKVSNKALGAPIEKTISKAKGQPREPQVCTLPPSRDELTKNQVSLSCAVKGFYPSDIAVEWESNGQPENNYKTTPPVLDSDGSFFLVSKLTVDKSRWQQGNVFSCSVMHEALHNHYTQKSLSLSPGK

SEQ ID NO: 22 - protein, 453 aa, Artificial Sequence
  source: /note="Description of Artificial Sequence: Synthetic polypeptide"
EVQLVESGGGLVQPGGSLRLSCAASGYDFTHYGMNWVRQAPGKGLEWVGWINTYTGEPTYAADFKRRFTFSLDTSKSTAYLQMNSLRAEDTAVYYCAKYPYYYGTSHWYFDVWGQGTLVTVSSASTKGPSVFPLAPSSKSTSGGTAALGCLVKDYFPEPVTVSWNSGALTSGVHTFPAVLQSSGLYSLSSVVTVPSSSLGTQTYICNVNHKPSNTKVDKKVEPKSCDKTHTCPPCPAPEAAGGPSVFLFPPKPKDTLMASRTPEVTCVVVDVSHEDPEVKFNWYVDGVEVHNAKTKPREEQYNSTYRVVSVLTVLAQDWLNGKEYKCKVSNKALGAPIEKTISKAKGQPREPQVYTLPPCRDELTKNQVSLWCLVKGFYPSDIAVEWESNGQPENNYKTTPPVLDSDGSFFLYSKLTVDKSRWQQGNVFSCSVMHEALHNAYTQKSLSLSPGK

SEQ ID NO: 23 - protein, 463 aa, Artificial Sequence
  source: /note="Description of Artificial Sequence: Synthetic polypeptide"
QVQLVQSGAEVKKPGASVKVSCKASGYTFTGYYMHWVRQAPGQGLEWMGWINPNSGGTNYAQKFQGRVTMTRDTSISTAYMELSRLRSDDTAVYYCARSPNPYYYDSSGYYYPGAFDIWGQGTMVTVSSASVAAPSVFIFPPSDEQLKSGTASVVCLLNNFYPREAKVQWKVDNALQSGNSQESVTEQDSKDSTYSLSSTLTLSKADYEKHKVYACEVTHQGLSSPVTKSFNRGECDKTHTCPPCPAPEAAGGPSVFLFPPKPKDTLMASRTPEVTCVVVDVSHEDPEVKFNWYVDGVEVHNAKTKPREEQYNSTYRVVSVLTVLAQDWLNGKEYKCKVSNKALGAPIEKTISKAKGQPREPQVCTLPPSRDELTKNQVSLSCAVKGFYPSDIAVEWESNGQPENNYKTTPPVLDSDGSFFLVSKLTVDKSRWQQGNVFSCSVMHEALHNAYTQKSLSLSPGK

SEQ ID NO: 24 - protein, 214 aa, Artificial Sequence
  source: /note="Description of Artificial Sequence: Synthetic polypeptide"
DIQLTQSPSSLSASVGDRVTITCSASQDISNYLNWYQQKPGKAPKVLIYFTSSLHSGVPSRFSGSGSGTDFTLTISSLQPEDFATYYCQQYSTVPWTFGQGTKVEIKRTVAAPSVFIFPPSDEQLKSGTASVVCLLNNFYPREAKVQWKVDNALQSGNSQESVTEQDSKDSTYSLSSTLTLSKADYEKHKVYACEVTHQGLSSPVTKSFNRGEC

SEQ ID NO: 25 - protein, 213 aa, Artificial Sequence
  source: /note="Description of Artificial Sequence: Synthetic polypeptide"
SYVLTQPPSVSVAPGQTARITCGGNNIGSKSVHWYQQKPGQAPVLVVYDDSDRPSGIPERFSGSNSGNTATLTISRVEAGDEADYYCQVWDSSSDHWVFGGGTKLTVLSSASTKGPSVFPLAPSSKSTSGGTAALGCLVKDYFPEPVTVSWNSGALTSGVHTFPAVLQSSGLYSLSSVVTVPSSSLGTQTYICNVNHKPSNTKVDKKVEPKSC

SEQ ID NO: 26 - protein, 17 aa, Artificial Sequence
  source: /note="Description of Artificial Sequence: Synthetic peptide"
AIFTGSGAEYKAEWAKG

SEQ ID NO: 27 - protein, 13 aa, Artificial Sequence
  source: /note="Description of Artificial Sequence: Synthetic peptide"
DAGYDYPTHAMHY

SEQ ID NO: 28 - protein, 11 aa, Artificial Sequence
  source: /note="Description of Artificial Sequence: Synthetic peptide"
RASQGISSSLA

SEQ ID NO: 29 - protein, 7 aa, Artificial Sequence
  source: /note="Description of Artificial Sequence: Synthetic peptide"
GASETES

SEQ ID NO: 30 - protein, 12 aa, Artificial Sequence
  source: /note="Description of Artificial Sequence: Synthetic peptide"
QNTKVGSSYGNT

SEQ ID NO: 31 - protein, 123 aa, Artificial Sequence [sequence omitted]

SEQ ID NO: 32 - protein, 110 aa, Artificial Sequence [sequence omitted]

SEQ ID NO: 33 - DNA, 19 bp, Artificial Sequence
  source: /note="Description of Artificial Sequence: Synthetic oligonucleotide"
gtcctttgggcagagacag

SEQ ID NO: 34 - DNA, 19 bp, Artificial Sequence
  source: /note="Description of Artificial Sequence: Synthetic oligonucleotide"
gaccagagtactccctcgt

SEQ ID NO: 35 - DNA, 20 bp, Artificial Sequence
  source: /note="Description of Artificial Sequence: Synthetic primer"
ccagatttggtgaggacgat

SEQ ID NO: 36 - DNA, 19 bp, Artificial Sequence
  source: /note="Description of Artificial Sequence: Synthetic primer"
gaccagagtactccctcgt

SEQ ID NO: 37 - DNA, 30 bp, Unknown
  source: /note="Description of Unknown: Pyruvate kinase muscle WT sequence"
gaccagagtactccctcatgggcacagtgg

SEQ ID NO: 38 - DNA, 29 bp, Unknown
  source: /note="Description of Unknown: Pyruvate kinase muscle WT sequence"
caccctgcctctgtctctgcccaaaggac

SEQ ID NO: 39 - DNA, 27 bp, Artificial Sequence
  source: /note="Description of Artificial Sequence: Synthetic oligonucleotide"
caccctgcctctgcatgggcacagtgg

SEQ ID NO: 40 - DNA, 19 bp, Artificial Sequence
  source: /note="Description of Artificial Sequence: Synthetic oligonucleotide"
caccctgcctctgcagtgg

SEQ ID NO: 41 - DNA, 14 bp, Artificial Sequence
  source: /note="Description of Artificial Sequence: Synthetic oligonucleotide"
catgggcacagtgg

SEQ ID NO: 42 - DNA, 20 bp, Artificial Sequence
  source: /note="Description of Artificial Sequence: Synthetic oligonucleotide"
cccatcacggcccgcaacac

SEQ ID NO: 43 - DNA, 20 bp, Artificial Sequence
  source: /note="Description of Artificial Sequence: Synthetic oligonucleotide"
cttcttcaagacgggggatg

SEQ ID NO: 44 - DNA, 22960 bp, Cricetulus griseus
gagctgcggagggattgcggcgggtcgcagctgggataaccttgaggcccaagaggcgcagtcccgcacacccgtgactcgtcctgagactgcggacgtccgacttaggcatcgctgcaagatccggagtacgcccgaggtgagaggggagagcctacgccatctgggcccagggccgatgcctgcttctgcggagcgcaggcctgcgggcccatgcgggactaaggctcctggcatcgtgcatcccagtacgggttgggggaaaagctacactcgagcacaggtcctgagcttccaaagtcagagggcccagccagccccttcccacgcggtagttctggtccctcttctttccttctcaatctggttccaccctcttatcttactgctgccgtcctccccgccctgttctctcccactcttcgatgctcatcctcctcagccatttactagtggttgttttccctttattttaactctgtgccaccatcccccccaccttcggtgccctctttgtaatctctactcgaaataactctcctgctccccccttgcgccccggcattcatcccccatccaggtcagtatgctcttcgcgtggccctgttggctgctccgcccctccccctccattccagtcacgtccgcgccactgcatcctttcagcatccggatcctcgcccctccccctccgcgctgcttcccccgcccaccgcattctggtcacgtccgcggactcccctcaggccctcgtggtccgcggcctgtaggtagggtgcagttagtggccgtccagggagatacagccaccggttacgtaacatcatcttcccggtggtgtggcaaggagggttggcagctattccttcctattttgtgcggccgcagattcttctggttgccggcgaagcactcgtgctccgggctacccgggccctgtggggtgcctgcaagcgctcacgcggtccatcctgcggtggcgaggctgcgcgtaccgcagggctcctggaccagccagtcacactgctccaacgtgctggcccggggtgggcgatcaaccaagggcggcttccgaatgtagctgcagcccgatgcgaccagaacgctcatagcccacagagttcagtctgattagggaagcaaaatttgtcaagtcagtgctgtgaggaaggatggggctgcacgagctggtccgcacacagggattgagtaagcagtagagcacctagtctgaaggttacttaaaaatacagtcttggaaagatgcctctggatctatctcctcttccaaacccaggagattgataggataaatagagcctcataatgtgggtccagtcctgcgtggaggcagcgggggatatacacaggttttaggaatcttctgaggtggttcagcctcttagacatttgctccagactgctggagttactggcctccgtgtctgtacggacatgactaatctcaggtgaaatgaccacgagggcgtgcacatgtactttttttttgtcaatggatgaaatacagttaccttgaaggccgagtctgtcgcccagttattcctctacacattagtactaagcttggggaggcagggaggcaatgaacacccagtatcccctaggaaacgaattctctctggtccgtgtttacaatgtaactaatgttaacaattgcaactcccaagaaagccagctatctaaagggacaaatgctgcagcttttgtcttcgactgtaacggtagaaacaaaggaacaggtacccggatcagtctcttctgattttctcgtccctgatggttcatgtaagacctttctgctccctggcttgtaggaagttggatttggaagctgttgcagtaagttctgttgccacaatacttagggtggggctactttctagagtacagaagggagggccttgggtcaggattcaaggtaccattgttagcaaacaatttactgtctggtggcctgaggatgttgtaggtaaggcagtgaggctgttctgtgggaaagtgtactgtaatccaccaccgggtctgggcaagatgactcatcctttcacattagcggcattcgagaagattctcatccttgggtgagtggggaaaacttggtactcctaggtttagtaaggcccctgtttagtcagtcaaatactgagctagcgtgcatttccctaagttaaacttctatgtgtcactcagactgagtgtggtggttcagcacttggaggccaggatcgcaggttccagaggggggaaggggcagcaaaatgccggggaccaggccctttgtgctactggagtgctggaagtgtgagtggttggtcctagtctataggtccactcttaattcttgagtgataggcacagcagcttctcatggaacaaccagtatccagaatgacaatttctgtgaactcatttgagttactgcttttaagtggaactatatggatgataattaatcactttctagtacatagctgactccaaacaactcagtctcatgggggttggatataccatctgttttggcaagaaggtatgatcacaggaaaggacatcttatttcttaaagctgttgatttcttaatattgagtagaagaaacgagccatccatgggcaggaaggtagaaaaaaaacctattgcattagactcattacttgggtttttagtgtcttttgcttcagcttttctacaggaagtcaagatgagttggccaagcactaaggtggagattgaggtagaggaaaatgactgattcactttaagtttctgaatcatcccaaatacccacagccaagttaactggtaaactacaaaaatgagttgtcgcctgtgaggttttttacttcgctggtaagagtacataagtactgagtcatccttgcaaacttcactctggtacggatagaaataaatgacagactttttgattaattcctgacatgatactttcttgggtattgcaatttttcccaagagccagacttagactggatatggagtagtcggaagaagtgagcccacgtggtgagcccacgtgggtggtggcctgcaaacctctgctggcctcttaaggcttagtgtaacagctcagctcaggactgggggtggtcttacagacaccaagctgtgcagtgaggccacgcccctaccgtagtttgtgcctgtctgcacgtaggagggaagggggaaggtttgagctgtagtacctctggtggcctctgggacaccttcactgaagggtctggggagctctgaatctttcccaaagccagctaagctctaaaggaagctgcatcccttccaaacatttttttatttttattttttgttgttgttgtgtttgtttttcgagacagggtttctctgtggctttggatgctgtcctgtagaccaggctggtcttgaactcacagaaatccaactgcctcccgagtgctggaattaaaggtgtgcactaccacagcccggctccttccaaacattttcaattaacctacaggtcatattttgactttaaactactggtgttttccagcaatagtgtaaaagattttaaggcatgcccattttggaagagtagggaagcactgggtatggtggtgcacatttttaatctcagcactcaggaggcaaaggcaggcggatcttcaattcaaggacagcccagaagaagctggtaatgtagtgctcgggaaatgtttgcctgttgggcacaaagtctttccatcactagcactacataaaattgacatgcctttaattccaacattcaagatgtggtggcacgaggattggaagtttatattcagcctcagctacttgatgagctcaaggccagtcccagatacatgagaacccatatcaaacaagaaaaaaaagccaacatagggttcaatatagatatagtgattgggtatccaaaattcagggtaggggtggggacaaaggacagcgggagggttagagaagtcagagattgggagaaggaaattatttatggattgaatacaatcagaatactttttatttttggaaagtctaaaaatacaaatcattgttgaagcagagttctaagtggtagaaacacagggtttggggtccctctcccccttgggaaggaatagttgtgatcctataaaggtcactgtagacaggcactcatagtaagtaggtcagtgctcttggacagctggtactgccttccctatttaacaccccccgccccccttggttcaggacagaagctgtgcctccagttggggagaccattgtgcattctgcttacacctggttggtttcctagactcctagccagggtccagagtgggcatcattcccggtaacactggcagcttaagcctgctaaggagggcaccatgtgccagcagaacagaaactttctcccagatcatcttctggctcaaactagttgcaggagatccttggtactaaggactggagagtttctttgtccctggcattctgtcctgaaataaaatggtctttctgcaggatggtcctcataattgcatggcaggatttacagtaggactgttaaagttaaggttaaataaaagatggtttgtgcttgtttctttaattttttttttgaccccacagaaatgagccacccaaacaggtgggctcatattctgaatagccttgtaacaccagacttttctggtacagaatttgctagggttaagaagtagacctccctctggacaaggtagcaaatgccttcaatcccagcattcaggaggtaggggagatggatatcttgagttttaggatagccagggctatgtaataagaccatgtcttaaagaataaataagccaggcagtggtggtgcatggcctgacagtgccagaattagggtggcattggtcagtttttgttgttcttatgccctttgtgccagagatgggagaaggcagaaccagatgacctgagctgagcctgtgcatgcctcaacctgcagcccacactgaagcctgggctgctgtctcctttctcacagaggggcaatggctctgaggaagatactgcttcaggggctcaggctcaagagcagggctcctgtccctgagcatggtgtttaccagtgtcattggacttgccaggcttctgcagctgtctggaggttggctgtgcatgtgggtgcctcctgaggaggaggatggtggcatgggtggggccgcatgacttggcaggcactactgtacaagtagctagccaatagagcaagccctaagggcctaagaaactggggctggaactgctttcctgggccagaaaataacctcagaaagggtattctatatgttatatatagataggtggttggtttgagttgtggggctccataggggtcatgggataggaagaagagtcctgattttgaaggggggcggtgctccaggtatcaatagcctgggaagagaaacgggttagtgagctgggatccagattggtaggggacttgaaacacttgaagttttgtaggaggtctatttaattgtatcgatccattgatacatatttccacttgccactttgtatctggtagcaagataatctgcagactatagtagttctagatggggaagtgggttatatttgaagccaatgaaattttacctgttaaattgcatttccccgccctaagggcagcagcccttgtctaacaaggattgtactgtcaaccctgagaacaggcaaagcaggaaaagaaaattactggactctggcatggaactgataagtttttataatgaaaattttctatgggttatattgtacacttttctttttctttttggctttgagatcaatggatcaagttgttctccaggtcagtgaagcttccctgaggtgcacttgtgactgagggaatattagcagagtcatcctgaagggctcggctgatatatggaaattcactttacatataattcctcccatgagctttatagaatgcatagaaataaatgtgtcattttcagaaactgcgctttttttgtttgttttttggttttggtttcttttttttttttttttttccgagacagggtttctctgtggctttggaggctgtcctggaactagctcttgtagaccaggctggtctcaaacacacagagatccacctgcctctgcctcctgcgtgctgggattaaaggcgtgtgccaccactgcccggataaaggtaaggatttttttttttttttttctcaagacagggtttctctgtgtagctttggagcctatcctggcactcgctctggagaccaggctgctctcgaactcacagagatctgcctgcctctgcctcccaagtgctgggattaaaggcgtgcaccaccacaccagccacttctggttattctttgaacactccatcaggatcatacttgctagattcttggcattttgcatcaactcttgtttttgagctggggtttctttgtgtaacagtgctcccaagtgctggaattaaaggtgtgcgccaccacctggccacatcaacaattttattgataaaggatatgccactgggtgcggtgacacagcattagaaaggcagatttcttttgttttttgtttttctttctttctttttttaatagatttatttatcatgtatacagtgcatgccagaagagggcactagatcacattacagatggttgtgagccaccatgtggttgctgggaattgaactcagaacctctgaaagagcagcagtcagtgctcttaactcctgagccatctctccagccccaggaaggcagatttctgaattggagaccaatctggtctaagtagcacctccagcaggtcagggatgtatagtgagacactgtctcagagaaggaggagggagcattgtagtgaatactgccacccaggtaacaaactgttattttgacatttatcctcttaagctttttatcttaaggtggagaccaggtttttatataaacttagagaatgtggtggtgcacatctgtaacctcaaccttgaggagagaggcaatatgtagtgagttccaggccagccagagctacttagtgagaccctcttaagtaaataggggttgtagtatattacaggtttaaagactgtccaggaaggagtcagtcctagtgactcatgcctgtactcttaacacttgggaagttgagaccggaggaggatctttgtgagtgaagccagcctggggttcattaatattgtgtgtgtgtgtgtgtaacatagctgaatctatctctaagagcaatttctacctggttaaggtgattaccacaaagagctcagctttcgccttaatccttgtacagctctccaaggcaaactgtactcagctctgaacagtctttccaagtgaggccaaggagccactctgagtcaaaaaaacagcattatgtcactggaagcccaggcccagagaaccaaaggtatgacctgattatcagtggcctcaggcaggaatttgcaaggagctttaatgtcttagttggagagaagcacctggtggctcttcaggaaagtgggttcggggtctgtcccactcgtgctgacttcatagttcatagtcctatcatggtcatagccagacttttgtgtcgtgttggtttgatgtaccatctattcctttagcagccaccaaagcatggctgggaggcatgagagtttgccagccctgtttgtttcaaccatgggtagacaaaggacctgactgcctgggacttcctttgtgaggacttctcagatttggagaggggaaacaagcagaactgatcttggcagagagaccttaatgagactgagagctcatttaacaaatactacaaggtgccttagcaccttgtagaccccaaaggagaggttgaacagtgttggccaatggcagtagttagaggtctgattcctcctttaaaagttttccgttctgcagtgaaaatagtggtgcacccctggaatccagcacccagaagcccggaactcgtgggtggccagccttcttttccattgcatcactagtaggttacaggggtccccaggtctcaagaagcagagatgaattttagtgatcaagaaatccatggttgttgagtgagggtcctttactaggagtcagggcagagcaaggatgcagaggggtttattgtagatgagccccttggcctgagaactcagatgagaaggacacccagcttcattcaagcctctcaacttttgtaaaacacaaagcttctacagagttatgtcctctaaccagctcagtgagcatttagttgtgagtcggtaataaagttaaagcaaaggtcaggcggctgttgggattgtgacctgggtggttaattacctggaacagatgctcaggcttctgagagtgctctacctacctatcagacatagagagggattccagatgcttagaactggggctgggaaagccatgtctaacgtcagcacgtggaaagatcgaagagtgagttcaaggtcagcctaggttatagagtggattctaggtcatctgagactagctactgtgcaattctgtttcctaggttacagacgactccttggtgtaatgactttggagctattccagtgctcttgcgagcaaaatttgctttgtgtgtcttttaattgttgctgttgttttattgctaaagcattctgggattttgcttcctgcctagaagaactacttttttgccgcctatcatttggatcttatgctcttatgtctaataaaataagcttaggcaacgaggccagtgaaaacctagaactctggagctaaagggggcttgggacccttgtgtttgtctccttgatctgtgggaccatttgagtttgggtgaacatggtaaagaggctgttgggtaccaaagcacatacttgtagattcagtgcctcatcatggtagacttcccaaggtaccaggtgtttgtatgatgatagattagttgtaactttgggggaggatagttcttacaacttttgcaagtttcttcaagtatgtaaagtgatgtccttcctagggtggtgtgaaagctatccgtagcagctcttgtgatactcctgcttttactgccccctgggacaatatatgctttggatgggaagttacttttgttcatcaaggtctttgctgtttgctcacagtcacattgagccctttgcccaatttgaggagcacccacagaaccagcacaggccaggcctctgtgtgacttgtgcacaaagcaatcgtattaggttaatgtgtaatcgggagacagctgcctacgccaagtggctcattaagcactgcccaatctaattgcactcttcaactccccgggacccaggacctcagaaaccatgccgaaaccacacagtgaagcagggactgccttcattcagacccagcagctccatgcagctatggctgataccttcctggaacatatgtgccgcctggacattgactccgcacccatcacggcccgcaacactggcatcatttgtaccattggtgagtgagtgtggcgctcccctagatggaggcttcccacctgatgatctgctaaagagcatagcaattacaaggctaacctaggttctgagtgaggcactgtacacatttcttggaatggaggtcataagaaatggccataaagaattagtatgttttgccgggcggaagtggtggcacacagctttaatcccagcactcatgacacagaggcaggtggatctctgagttcgagctagcttagtctacagagcaagttccaggccagccagggctacacacaaagcctatttcaaaacaaaaacaaaaaagtgcactttgttttctgtgataggtagaattcaggggttcttccttagataatcgttgtaggagtatttctgagatctcaggtctttttcatatggattgtatcaccaacattcagtagttggacaacttgagggcaagggaaactgcttaattctaccctccacttccctgattatgtgggggccctaaagaatttagagagtggcagggtttccccctcgtatacgtaggttaggaaagttgactggcataatgctttgtgttcatttttggagttgattttaaaaacaattaaaggatgaagaatttgctgagaaaattacacacgttttcttgtatcatgcttttttacctgtggttttaaatatttattaataggtcctgcctcccggtctgtggagatgctgaaggagatgatcaagtctggaatgaatgtggctcgtttgaatttctctcatggaactcatgaggtaggcctcagctagagcaatttattggaaacaggaggtgtggtgataattagcgctactcccggcagatatgaaccccagttcagtgggacattgtcctagccctagcccatcctggattccctctttccctcctgtcaccttcataggcctaaacaaacaaggccagctttgtcaaggaccagggctgtcctacccttaaccttcacaaaagaaggcaggaaggatttagctggtaacccctctaggccatcaactgtcttagctctgcacttgggaacaatgcctcagggtttctctagtggctcctgtgagtctggtgaccaaaaggtcatgcagaaggttgattccggcttagttcaatcctgagatgattagctagttccatagataggggtttccacttgagcctgagtcgagtgcccaaagtctgtgatggatcatactcccctctccattggcattgtcttcctagcatcagttccctccataaggtgaggtaggaatgcatttgagctgggtctgttcattagaaattccaactgatggagaggcaatatgcaggagccagatggcagctgtgagttagaaaaacccatgtgtgccagtgctctcaagtttagaacaacccattctagcagtcgggcagataaagaaaccttaaaagtttcaaatactttcaaactggattttctactgggatcaatggaggtgggcacagacctcttcccacatcttggtttctttatgttctataaaagtattaccctgtgctctattctgccctctgacctttggaagttgtttagactaaaaatagaggaggaagagcagtccaagaaaatgaaccccctccttctcagaacatgagactcatcatagattccatagcccatattccataaacagcctggtggaggcttgcccccaaatgtcatagtacctaggatagtctagttgtacctaagcagtatatgacacctccttgctagatgtggtggtacagaactgccttgggatacatagcaggttggagacaagcctcaggaacataacaagagcctattgcaaaccaaaaagaggaagcttgttgctttccaagctctgttgccgtcggcaggaactgctaagaataaacacaagggtaagaccaactcaggcaagattggatccacttgccatggtccttgcaagtagaatctgcatggtctccgatttgcaggacagtcagaaaataaatttggggacatgacctttcatggctcttgaatcctgtaaaataataccatgcaactctgccatggcagtgaccagtgaggttcagacctgctggacaattggccagctccagcttgactttttaactataagaagcatttggagattatctgtacttttcctagattggacttgggctttattttattcatttatttgttcttgtaagtttatttttaggtttttagaatgagatgaggttaatcccagaaggttttgggaagctggtctgttaatggcatgtcgtgcacacagtttggccatgtgttaggtctcttatttcatgtgctgtctccatgaggagctggggtgtttttgctgggcttgatgtgatggttttaagttcttccggagacactgggatggcattccctccctctgacaggaacatctaccagctgcatctgatcctttcccatccttggcagtcttgtaattacacctcttgctggtcacatgggcaagatgagtattcttgctgaacaggcaatgctgtcctgctgtactgacttttaaatggcctaaatttagagcctctacaaggatggcactcatggattccagtcttcgttcaccatttggtaatgcgccagcaaagccatagctgtgacagaagacacgatctaccttccaaaagtgtaccataggttggccatacaaagaattttaataatgggccacccagtgttctaacctttgggattataatgcagttttatatacacggtgccaaatatgtgtttgtttagagcacttgtgaatgggctgaggtgtgtagctcagcaagaacaaatccctgggttcaaacctcacacatacttataaagatacattaggccagagggaaggattttaactcctataaagtagaaattattcagctgtaattcttctatgggaattaagggcaacctccaaaaaaaaactattatgagtacctctctaaaatgaatcaagcagtcagtagttactgtcagaaaagattagctctcaggccgcctgtggatgaaggacagattcaggcttccaggtgtcttaactgggcacagtggttaaaagacaaagcccttaaaatgatgaattatatatatgtcctgtgatcagtggcgtcacacagatctgcactatccacagattctatagctgtcttggctctgactcccaggtagaaaaaggaaaaggcctttgggggtactattgcaagtgaagtatagtgaacggtagttctatcagagataggccactaatcaccggttcctctccttttctaatcagacctaagaaagtgattgtgaaaggaggtgtctgcatatgaccaagcaatgagctgtttagcttggaccattgttaccttaagtcaacaactttgggtttgaattgactttgggatcgatagtggaaacagactgccagggcagacttcaaacacaaatcctgggtcctttacctgccccagttgttaggcatctttgagtcctagggatactaggacaactgaagggacacatagctgctttaagagtagggctttagtgacagtgtttcagaatgttcttgggatttgctattggagttagttctgtggtggggagaatggatgctgatgagattagtgggttggggatgaggatggaattcagacccttttctttcataagtgattggtcaactttggctcacaggtagggaatgggaactgaagtcaggtgtggggcacctgtcagtcaatctcccttctttccccagtatcacgcagagactatcaagaatgtgcgaacagccacagaaagctttgcatctgaccccatcctctaccggcctgttgctgtggctctggacacaaagggacctgagatcaggactggactcatcaaaggcgtgagtatcctaggaagtgctctgagggcaggcaaaccctccctccctggtagctttctctagtttctgactgggtaagttttagagtttaagtctaccaatgatagtgtttttattaatgcatatgggtgtgggtggtttttttgtgtggctatgcaccacatgtatgctgtgcactgcagttatggatgtctatgagacccaccatatgggtgctagatcttctgcatgaacagtaagtgctctaaaccactgcaccatctccagtcccggcatgagaatgttttttgtcattgctcttttcatctgcatagctaggaaacatgggggttggtccttaattttttttaactacttaagtctcaatggtgaacggagcttagaatttcttcaaaggaagaaggttgcttagtactccgaaccagggtttgagcatccccattaggggtgtggcttctgcagttcacacacccacgggctgtcttgaatctacagagcggcactgcagaagtagagctgaagaagggagccaccctgaagatcaccctggacaacgcctacatggagaagtgtgatgagaacatcctgtggctggactataagaacatctgtaaggtggtggaggtgggcagcaagatctacgtggatgacgggctcatttcactgcaggtgaaggagaaaggtatgcatggcgcatggtccatcgccaattcccatctccagcgctctcaagttgaatcttttttttaagattttatttatttattacgtatacaacattctgcttccatgtttatctgcacatcggaagagggcaccagatctcataacagatggttgtgagccaccatgtggttgctgggaattgaactcaggacctttggaaaggagtcagtactcttaacctctgagccatctctccagcccccaagttgaatattttaactccttttggtatagcactcgcctgcatgtatagggcctgggttcaatctccagaggatcagatttaaaaaaaaaaaaaaaaaaaactccccaaagggccaggagggtggggcgagcctttagtgtttagtcctaacacttgggagtcaatggcaggtgggtctctcaatatggcatgtagaatatttctatgtgcctttcaagtttttgttatgttcacattgttctgcctgaatgtccacctgcatgacggaagagggcaccaaatctcattacagatggttgtgagccaccatgtggttgatggcaattgaactcaggatctctgtaatagcaaccagtcagttctcttaacctctgagcaatctctccagtccctcctgtgtgcctttgaatgccagttaaatcttacctgtttaaatggtttatgtgttcgtttcattttggttttatgagagggtttttttgttgcctgtgctgggctttactatgtaactgaggccaaatgaggctgattcactagcttagctatttattttgagacaaggtctcactttgtagcgctggctgacatcactgtgtagatcaccttagtcttgaacacagatttttctgcatctgcatcttgagtgttggggtaattaacctgtgctaccacacccaaaattcaaaacatcttagcaacttgtacatgggtattgtttataggttcggaaactgacagtgtcaaattgactcagcctgaggtcttgtaatctggctttcacgtggctctagttgcctcagtgatgtgacctcctgcaagaagaggcaggtcctcatcactgatccttcacttacacaggtgctgactacctggtgacagaggtggagaacggtggctccttgggcagcaagaagggggtgaacctccccggagctgctgtggatctccctgctgtgtcagaaaaggacattcaggacctgaagtttggagtggagcagggtgtagacatggtgtttgcctctttcatccgcaaggcagaagatgtgcatgaggttaggaaggtcctgggagagaagggccagaacatcaagatcatcagcaaaatcgagaaccatgaaggcgtccgcaggtgagtcctgtggccccttttcatggtccagccatggttatgagtcctggatccctgcccagcaagtgcagcctgccaagcctggtttccgtggatgtagcattgtagtcttcacttggaaaacaatgattctgatgagtggtccatttagctcaccataggaaagaaagcatatgaagcttcgttaagttggtgttcataagaatgaggcaaagcagggtgactcgtttgacgtctgttctatgttgataagccataggtgctattggaccttggtgttacgtcagccctgtaggcactctgggcgggacacctcacctcaagggtcagcactcagaatcattagctaagtgaagccatgcgcaccttctggcctcactcttgctttgttggaagcgccaattagagaagtaagatacaagaggctataagagcaagacggaagagaagtcagcccacgcaactaaatctcatccccctcatctttcaatgaagtagtcatggtggtattgaagaagcccagcaagcaagattgctcggttgcttggatgctttgttttgttctttgcttcctattgaatatcatctttctcttctgaatcaggtttgatgagattttggaggccagtgatgggatcatggtggctcgtggtgacctgggcattgagattcctgcagagaaggtcttcttggctcagaagatgatgattggacgatgcaaccgagctgggaagcctgtcatctgtgctactcaggcatgtactgtgtactctgtttaggagctgcccatgtactgtgtactctgtttaggagaactttgggtcttgtcccatggtccctgttgtacagacatgttaacctatacatagctgtcctctggtcctacaaaatatccagggagtcatcttagcaactgcttgtcactgaacgtggcccatagtctcacacaggtctcactgaatgctcatctgtcccctcttagatgctggagagcatgatcaagaaacctcgccccacccgtgctgagagcagtgatgtggccaatgcagtcctagatggagctgactgcatcatgctgtcaggagaaacagccaagggggactaccctctggaagctgtccgcatgcagcatctggtatgttcttccgagcatggggtggaaacaagctctgccacagaggcttctgcatcctctacatggtctcttcccattctcctgttgtagtaacagtggcgtagtgtgaaagagtgcttctttatttttttttttccctgtggtgctttcactgcctctaccccagccctctttctcctaccctggaggttgccactttcattacataggccacatttgataaaagatttaagtcataggatgcagtcaaaggatgccttagacctccccctggacagtccagaagacctggtacctctgctctattctaaaagagccaagagtttgttcccagctggtctttttggtgtttggcttccaatttgatgccctactagtccctaggacagatgcttgtacccacactgagctgttttgagctggccttgcatggtgcctgtgtcctgggactgcctcccttgctgtgccacacccaaaccagggctacaaatagagctgggggtggagggagagtgttaaactcagcaggccctgggccaggaatatagaggaactgtgaagacttttctctgggaatatgttctttaagacttctaactttggtcagatatggtgatgagtcatgcctgaagtccagtattcagaggatggggcaggaggatagctaagagtttgaggctaggcaggattacaataagactctatcttatagggacaatagactccaagcagcaacgtcttctgctgcttacggatgaggacccagttcatgagccctgtgttttgccctggaacttactgagcttttacttttgactgatgaaagagtattagaaattaacttcttgagcttttctattccattttcagccagcaaaggacccctgtcctttttagccccagtccccaaatttaagccaactgaaaaaagaaagaatagcccccctctggattagtcgtcattcctttcttcccttcatctgtctgattattgagtttgcaaaaattccaaggtgaactgtattctggctgtgtgaaattttctgtggccttattatttgtgcctcctatattgaaactgtcagacaagccctgttgctgttctggttggtaatgtgggctctcatagctgcccatggcaggtagttgctttttctcccagaaagccatgtgccttcagtcaccttcacagttgctgcctttccacttttataccacatagcccttatctagttacctgcttagttgtgtcatctggccacagcgtggtcaggaacaggttaagggcatctttgaccgggtattctgaaccatgtatccacatagatgtatgtatagctgggggcaagttatatgacctcaagaccttgccctaagatgggtttgatgagatattaattatagccttagcattaaacatttactgccgtcattaaattttagataagcctctaaacacattggtgtaatcttcgtgaccccaatctgtgaatgagtcacatgatgtgataaatgtgggtttgagcccaggtttgctttctgtagtgcctgccaccggcccatttgcattatgctggaacagcagatgtggacaggtctccatgtcctacttccatgccctgttctttcctatggtcagacaccttagaacctcgaggcttgggactgcatggcgctgctcagaagatgaggcacagagtctaggttaaactggctgcctctccagggggtacaagcctttccctctgttaacacctcagcttctccccttacctgtcggctgtttcctcccttgtctaactgatgcagttcatgacctggaatttagagctaggcaccctagctatggttgttggtcctttgcactgcatgcattccattcttaacaaaaggaatacttttctgcttgtgaacctgcttatactgtcaaattagtgaaatgatttgctggttccttctcatccttcccatactaagatgccggtgattatggcattctaattttctgaaacttaaaatttcctttctgatgcctggtcttacctgaacaggtgtgtctgtaatgtaacacacttgctatcttgcaacggttttaattgctaagttttaatcagtattttgacgtgcatgcatgctttcacgggcatcattctcttcacatggttgttaagtgagccagagttttcactattttctttagaactggtatgctgtgggactttggctcttttgaccccagctttccagagctgcctcaatgtttccactgtaaacactgggctgtgtctatgtaagctgggctggaagccctgttgtagtcagacagccatgtgaagagggaagggcctattctattccttcctgtaagctgtgttgtgaggcattgtggtcagatggaagtgatttggcatccttccatgtcaaggtcctagggcctaacactttgtccctttcttagcttcgatttaaagaaaaagggaaacaaatttatagccagatattgatggtacatgcccattatcccaaagaattactttgagggcaatgggggcaagttcacacccagtaagggccattatgtaagatcttatctaaaaaactcaaatgggggcaggggggaggataaaaaaaaaataaattggagggggaaatcacaagtgggtaaataaagtctttccagaaaggaaaaaactttccttgtattagaaccaaaaaagagcacgtggactttgaccaccctgcctctgtctctgcccaaaggacagatttaactgtaccttcctctctgattaatcccctctgtcttcccatgtgttgtctctcctgttttttccttcatcccttctaccctaacccttacagatagctcgggaggctgaggcagccatgttccaccgtctgcagtttgaagaacttgtgcgagcctccagtcactccacagaccccatggaggccatggccatgggcagcgtggaggcgtcctataaatgtttagcagcagctttgatagttctgacgacatctggcaggtagggccctgagggcaggtatcgctataggataaccacttcttacttcagaaaaaaaaagccttgtgcctgagcttgggcacagcttctctccttcattcaggaaggtagccaaggaggtcatgatagggcaggaccagagtactccctcatgggcacagtggaagtcacaggcaccagtgaggatggtttctgtggagtttttgattttgctcaatttagaacagttcagtgactgttcctcctggacctttttttgcccaggacatcttcccagttgtctgtgactcatcctccctctccatttgtgacaaagctctgacaaagccctgtcccccctcccttcgtccctctggacggatattgctcccctagattgcccgtgaggcagaggccgccatctaccacttgcagttatttgaggagcttcgccgtctggcacctattaccaacgaccccacagaagctgccgccgtaggtgccgtggaggcctctttcaagtgttgcagtggggccattatcgtcctcaccaaatctggcaggtaggaggcggcagtggctccctggggatgcccacctcaattggcagccctccttagggatcccaagagtggctctgggccaagttttgctgccactaaaggactccaggcaccactcacaggtataccaaacaaaccatgtggttccaataaagttcagcttgcctcacaatgggaagcaaatacccagttttgcctagtttagctaccatgtggtcttgaaaaagggagcaagctgactcctgatctcacatgcatgtcagcagatacactaatagtgataagcactttaaaattccacttggactgggtggtggtagcgcacatgcctttactcctagcacttgggaggcaggcaggtggatatccatgagtttgaggccagcctagtctacagagagagttccagaacaggctccaaagctacacagagaaaccctgtctcaaaaataaataagtaaataagtaaataaataaatattgtgcttggaggggttggagataacatctcagtgagtaaagtatttgttgcacaaacatgagggtccgaattggaatccagcacctatggtaagaatgcatgcagacaggacagtactcggggcttcccatcaagccagtcgagtttcagactccataagagatcctgtctcaaaaaattagatgagtgtcttggcctctgaggtccctggcttacaaaggctcacaactgtctgtctagtcctagaggaatccaatgcccccttctaactccccacaggcagtacatgtatgtggtgcacaaatgcacttatggaaaatacccttacacataagtaaaaacatccagatgtgatagcccatatctgtaatcccagcactcatgaggcagaggaagaaaggtgggctacagctttgctcttaggagctctaagatataagatcaatgcagggcttttgcctcagcctctgcactttggcgaggagttcctgattacagcaactacccacttcaaggccttgtgaatgcaggccagcatgaagaagggtagtctctgctgtgttttttctggtttccacagtacttgtgtgttttcagagcttgttcagttaattcagcaaacctgagacacacctgctagaagtagacattatcacttgtcacaggtagttttgagaagggggggtcactacattcccaaaggttctagatgggctaagcattgctatataatgcctggtcactgtccggattttgtggcaccaagtgtgttttgggctctagagttaggcttctgggactgccatgggaacagcatactactgcagtccttaatattgttggctcccaggagctaggtgtatgctgcttggttgcaaatgttgctagcagttgtggatgctggtgagattggccaaagctgtctccctgctacatggaagggttcatgatatgggagggattctagccatgggccctgagggactgctgctcctattgaaggagcagttaagaaaggacagaggacaggatgtggggggtggccagtccttggaacagagtaagctctcagtgggcaaggcctgtgcctcacttgtgttagtgagctcctgctgaaggtgcttcctgtctcctgggtcttgtgacacgtttcatagtctatcctatttcccatctcaggagtgctcaccaggtggccaggtaccgcccacgtgctcccatcattgctgtgactcgaaatccccagacagctcgtcaggcccatctgtaccgtggcatcttccctgtgctgtgtaaggatgcggtacaggatgcctgggctgaggatgtagacctccgtgtgaatttggccatgaatgttggtatgtagctggaagcaagaagatggggtgctgagcaatggcttttctgggaattctgaaactgtcattctctgaagacttgggctaagcctttttgtccacaccctcccaatttggggcccaaggcaaaattaaggtgggacacacagattatgtactgctgctatagcctttgttcctctataaggttggacattggggtgggaggaggccgctggctctgtgatctccaaaggtccctacagtcttgagttcagccattgtttggtctaggaggcttgcaccaccttgtggtagaaagaagaattggttcaggcagactggtccccttatcataggcaatgggattgtaggtagctctttgggcatttgccctggaatgcccatgcctgggtggcctctgggctaggagggaagtgccaccttgtggtaggagagagtaatggttgttcaatttggggcagttaccccaagtgtttacttctattcacaacctttctattctttcaggcaaggcccgaggcttcttcaagacgggggatgtggtcattgtactgactgggtggcgccctggctctggctacaccaacaccatgcgtgtcgtgcctgtgccttgatggccctctggagcccctcttctagcccctgtcccatcccctcccccatgccatccattaggccagcaacgcttgtagtgctcactctgggccatactgtggcgctggtgggctgggacacccaggaaaatttactggctttgaaatatggactagagcccagctgtctcatggccctacccaagctagggatgaaggaggaatgcagaattgtaaaccctctgcctttatcacaaaaggg

SEQ ID NO: 45 - DNA, 32596 bp, Homo sapiens
aacccataaatctgggccctgcccaggtaggccgggacagctggggtggcctgggccgagagccaagaaaagacaccccatctggcagcccaacttggcggcaacaggtggcccggcgcccgggggtctgggaggaaagtcgctccgggggcgggccccgttgccccgccgcgtccccattggtcatcaggtttcttaaaatgtgactctgaatctgtgtccttccgccgcagaatttagtcccaccgaaagggcaacctgcccgcgcgttccgccgccgccgccgcgcttcctcctgaaggtgactgcgcccgcggggacgcagggggcggggcccgggtcgcccggagccgggattgggcagagggcggggcggcggagggattgcggcggcccgcagcgggataaccttgaggctgaggcagtggctccttgcacagcagctgcacgcgccgtggctccggatctcttcgtctttgcagcgtagcccgagtcggtcagcgccggaggtgagcggtgcaggaggctacgccatcagtccccaccaagggccagtcgcccggctagtgcggaatcccggcgcgccggccggccccgggcacgcaggcagggcggcgcaggatccagggcgtctgggatgcagtggagctcagagagaggagaacggctcctcacgcctggggcctgctcttcagaagtccccagcgccgttccttccagatcaggcgggtccgccggctcctttcccgccccagccctaccccctcattctggtcccatcctcttcctcctgccccaatcctcaatgcgcctccatcctcgcctgccttctctcggtccctcgtgattgattccacccttgcttcccctttctccgcgccgcctgttccgtgctcgttttcccctcttcctccttaagtctggtccttccaccccctcctcttcaagctgtgcgtgtcccctgattctaatgctttctgtgtaactcattgaaactgcgttctggttcccctcccgcgtccattctccattcatgcgcgaccgcccttcccgcgccccagttccctctcgccgcccctccccctgcttgctggtcacgtccgctcccccgcatccccttcctcgcctggcgtgtccgctccctccctccctctctgctctggtcgcgcccgcccacttgctccggtctccgagcgcggtcccaccccccttttccatcaccgcctcccagctcccagcaggctcgggcggtgctgaggccccgtgtccggggcgggcgggcggagggctgggctgggtgccccgcgcggcgggcgggatgcggcggcccgggggcagctggagacttacgtaacgttggcctgccccgctgccgggaggcagggcggttgcccctgcggcgcggtgccgtcccctgtggccgggattagatgggcggcctgcgagggcctgggaatggctcggggcccgagagctcgaccggcccttgccgggtggccgccagggaccacgctccatctcgccgcggccgggctgcacgtagcggccgcgcccagggcccaccccgcttcaccgggcgatggccttgggcctcgtaacgggcgggataaacctctgcaggctttgctggggcctcctggccctcgcccgttccgcgcctctccggcacgtttctttcttttcctttcttttttctttcttttttttttttttaattatccggcacattttttaacaaatgcgtcctgattgtggaacgcggaggccgcggggtggggtggggatctggttacggagggggcaggaaatctgtcgcgttcactgaacgcaaacggtgtgggtcaagggctgtttgggggtcagagttagagaccaggatgactagacgagtcatagcccaccgagctcacaatcttaaaatgtatctcctgtaatgctgggagtggggtacgagcttcctgctgtgggagggagggggacaggaagcctcgtaaggtctcaccaggtggcaagcacactggattagaagatgcaggaaagcaccttccagtctgaagatcatttaaagactcagtcatgtaagggcatcccttggcttcttaatctacgtactccagacccagggcttggacctttgctggtacgggttaaagtgaggccgacagtgaaggtccacgtggagagagacattgggaagttgtcaaaaaggcgtttagaatcaggtttgactcattaatttcctgagactctgaaggagttcagcctctacacctcagtttcccctgggaaaactgggagtaacattttcctcatgatggttgaaaggattcatgcttacgtggatgtggcacactcagtaagtgtctaatctctggcgaaatacccagaagaaaagcctgtgactgaatatattatttttgagcacaattacttagtccacaattgagcataagggccttgatccattgtcttcctactgtccccaaacgcctacagctaatcgtgaggaatcaggctctctgaataaccacgtgtctcctggaaaccagttccccaagggatctggtttaatattgacaaagtaactgataatgtaactttccaactctctgcttggagcagatgctttttggtcatctgagattgggacctgtagacaaaggcaggcaaggaggggctgagttaagcctttggtgttccgctgtaagtagaatactacctaccagaggaacattccagcccttgacttgctctgcctgctggtgagattaggattggagccagggtcagtagcccccagttggccgtcttgagggtgtggccactccctaggtcacagaggagatggaggtcaggactcccctgctgcagcgttgttagcaaataatttgccctttggtggcctgaggtgctgtgggggcaggagtgggctgtcttgtggggaagggaaatgtaacgtatcaccaaatctgtgggggagtggggctctgtggggaagatgactcaacctttcaattattctgcttttgagagaattatcttcgctgggtgagtggggaaactacattgtggttcttgcaggcttaaaaagtcccttctcccctttcagtgagtcagataatgaagcatgcatttcccctaattaaaaatgcctcaactacggagcttgcagtgagccgagatcgcgccactgcactccagcctgggcgacagagcgagactccttctcaaaaaaaaaaaaaaaaaaagccacaactaattaaaaaatgattggtccgggtcacctggttctctgtactgccttaagagcttaagtgtagactggcagagcccggtgcccagctaatgccgtctgtgcagcttcattcctggcccttttgtagcgggcacagccgcctctcctgggacttgattaatgatgacttaaagaaggttcttgaactcatttctcagttactgacttgagccaaaatgtatggatgttggtctcctgtctagcacaactgctttcattttaagcattgcattagaaataatgttgtattcatattttagcaaagagcatcattagctctttaagaaccgtacccccagtgacttagcaaatttggtggcggtgactctaaacagctagcactttatgggagttgcttctgtgccttgaatgttgtgacactgatgtggggtcacaggaaaaaccattttatttcctaaagctgtttatttcttaatattgaggcaatggaagaaatgaggaaacggccgtgggcaggaaggtagaagaaaatgcagcacttacattacaaactcactttacttgggttttagtttattttgcttcagttttttgttttttttttttttttttttttttttttttgagatagttttgctcttgttgcccagtctggagtgcaatggtgtgatctcggctcactgcaacctccacctcctgggttcaagcaattctcctgcctcagcctcccgaagtagctggaattacaggcacttgcaccacgcccagctaatatttttgtatttttagtagagatggggtttcaccatgttggccaggctggtcttgaactcctgacttaggtgatccaccggcctcggcctcccaaagtgccgggattacgggcgtgagccactgcacctggcctgcttcagcttttatgaaggcaagtcaggatgtgttatcttggccaagagctaagactgagaccggagtagaggaaaatgactcatttgacattacccttctttctgaatcactccaaaagtccacagtcaaatctcaattagctggtataacacaagaatgcgttgaccctgtgagcagagttttattgcatcttcaagggtcttcgtgagattggtttatttggtatgaggtcttaaggattttaagttgtccctttaagcatcagttctgatacagatgggaatagagctaaacaaccagatatatgaagaccatttttgataccaccatacttgcggggagcttgcatttttttaccaaggggcagactggataattgagtaatttaaatacttgggactttgttaaagaagctgttgggggaaggtgagcctgggtgagtggtggagggtgatgtgcagcatctgctgggccttcctgcctcttggtatgactgctcagctcaggagttgggtgctttagggcccctaccatgcagtgcggtgaagccccgcccctgcagtggtttgtgcttgtctgcacgtaggagggaacaagccggctgcagtaccttcggtggcctctgagactcacctcccccacttctgtccatagacaaagctcctggggagccctaagcctctttcctcatgccagcaagcagtcttggaagcaggctggggctgcagtgggagagatgccaagaccagttattcaagggcagtgaggttgccagtcctagcatttcacactgtggaccagcacagctgctggctgaatactgcagtcaagattctctgaagggagtcctatcccttccaaacatcttcagtttacttgcagataatgtttcttcattttttattttattttattttattttatttttttgagacggagtctcgcaccatgacccaggctggagtgcagtggtgcaatctcagctcactgcaagctccgcctcccgggttcatgccattctcctgcctcagcctcctgagtagctgggactacaggcaaccgcaaccacgcctggctgattttttttgtattttttagtagagacggggtttcactgtgttagccaggatggtctcagtctgctgacctcgtgatccacctgtcttggcctcccaaagtgctgggattacaggcatcagccaccgcgcctggccatgtttcttcaattttaaacaactgatatctcccttggccatgaacgaaaaagaactgcccatcagtggagtcagtcagggcacataagacacactgtgtccaccatgccatttcagaggagatttgattgagttaagcagggaaatagagatgttgtaaacgttgaaactatctgggtatccctctttggttattaacattagatgagcagaaaaacaaatgtcaccgatgggcaaacatttaaaaagtctggcagtaccaagtgtggaaaaaggtgtggaaggcagcaactcagcgttcattgatatagccactttggagagcaattcagccttatttagtaaaaatagaaataaacatactccatgacctaagacttcaatttctggatatatagaaactcacacagtacagggagacatgtactacaagagtattgattaatagaagaaacttagtttaacggggagggagagtggccaccagtaagacagtccataaataaaatggtctgttgtacagtggactagtgtaacagcttaaatgaattagctagatccatatacccactggatggatcttaaatgtgctgctgagtgaaaaacaagttactcagtgatatatacagtataccacttagggcattaagaaaaccacaatattatagggttcagtatagacatagatacactgtacatagacttcagtgaactggaaggatatagagttcatgacagtgattgggtgtcaaaatgcatgatgtggctgggagcagtggctcacacctgtaatcccagcactttgagaggctgatgcaggaggatcacttgaggccaggaggtcgagaccagcctgggcaacatcgcaagattcccatctctatttaaataaataaaatagaaaaaaaagtttaagatggaggtggaaagggttggaggagcttggggatggagaaaaaatgaactgtataaaattaaaattcttgtttttgtttttagaaagtaaagagggccgggcacagtggctcatgcctgtaatcccagcactttgggaagctgaggtgggcggatcacgaggtcaggagattgagaccatcctggctaacacggtgaaaccccgtctgtactaaaaatacaaaaaaaaaaaaaaaaaaaaattagccgggcctggtggcgggcgcctgtagtcccagctactcaggaggctgaggcaggagaatggcctgaacctgggaggtggagcttgcagtgagctgagatcgcgccagtgcactccagcctgggcaacagagcgagactccatctcaaaaaaaaaaaaaaaaagaaaaaagaaattaaagaaaatacagctcagcctttatttgtgtttttttttttttcctttttttctgagacagagtttttcactctgttgcccgggctggagggcagtggtgcgatctccgttcactgcagcctccacttcctggattcaagcaattctgtgtctcagccacccaagtagctgggattacaggtgcgcgcctggctaatttttgtatgtttagtagtgatggtgtttcaccatattagccaggctggtctcgaactcttagcctcaagtgatctgcccgcctcagcctttcaaactgttgggattacaggcgtgagccaacacagccagccatggctcagtgttaatggtcagttctgggtggtagagaggcagatgttaaaacttttttttctttaattcgtaacatagaagcaaacctataaaggctgccgtaggaagaccagtcatagtaactagttcagtgctcttggagagttggcactgcctttcctcctttatccccccgactagaatgcagggcagcccttccagtaaatgttgagccagtgcctcactttgctgaggccatcacccaccttagttgcacttaagaggaccctaaatcagggtcccaggtcccttgctgattttagagtgtggatatcatacccagaaacaccgccctacttttaatcctagtaaggaggcaccatgtcccaggacaactaatgcttcccccaaaccacctccttcaggctgaaaccagttctctgcactgagcagctgggatggaaccaggaaatcctcggcatctgaggacattgaggggtctctgacttagggcttcttcacctgaagttgagtggtctttgagggaagtaggcccatttagcatcagctgctcttccctattccacactctagttggaaataggaccttaggttcctgttgacaagtcatttactttcagccccgaagaaataaaagagccaagattttttttttttttttaaagccagggaattttactagaacctacaagtgggctcattttgttctgtgtagcctggtaacaccatactgctttctgctgtggggcctcctggggttaaagtgtgggcttaagacccaggtctcttagctagaagatatcttatcctctgtatcctgcacccatatgcaaatacattattgtcattacccttaactatagatgaagatgaacagtgcctattccagaccttactaggttctgctggcccgtcacccattttgatcatgttgctggcctagtttgattagggcaaatcttagaaactccatttccattgttgaggaagagaactagagagcaggctgacctgaatgccagcgtatcatgatgcagactttctaacggatgcaggtgttcggaagagttgtggatcgaaacgccttcatgatggcttggaggtgtaggtagcaaactgacgtcacaggaaggaacacaatcttgggtacctactggcaacgttggagggagaaagtgagcatcaggtgccatcattttatagttgatctatgtgatgaggttggtatcggagcataattggtacaaaggaaaaatgacttaggcagatgcagactcacgggccaggctattttattagggcagaatgatttggtcctttgtggaagaattggtggagtgaagcgtgaatctttcccagcacaacccaacaacagtcctggccctaagaagtggagcatgggagttgggtgtggttcgtgcctgtagtcccagctacttgggatgctgaggctggaggatcgtttgagggtgcagtgagctataatataatataatcacaccactgcactccagcctgggtgacagagtgaaaccctgtctgaaaaaaaaaaaaaagaaaaaaaaaaagttggagggaggagtgttgggtattttttatgatttttgtctcctggtttctgaagaatggccaaaaaattgtgtctgacacaaaggaaactaatataaaaagccaggagctgtctgagatgagaaaggaaagggagaatagggcacttggagctgagctgtgattgtgcctgttccaacctgtcactccagactaaggcctcttagagatggtgtctcctttctcacagaggagacatggctctgaggaagatcttactgcaggggctcgggctcaagaataaggctcctggacctgggcatggtgtgtgctgctatcagtggatacgccaggcttccactgctggctggaggttggctctgcatgtctgtgccttcctaggaggaggatgcaatagtgagtcagactggcatgggtggggccacatgtcctggcaggcactgtccaggcagctggcatgagggagaggagtctttcccagaagtccgccctgagaaaccaaggctgggctgctctcctggagccaggggagtccagtgagtgttttacatacaactctaggtacgtggttggtgggatgggcagtttgtgctgggaagaggcttgtggaggattttggagaaggcaggagagctctggccctccctgcaagggaggcttcaggtcagagcctgaggaaagacctgggcatgagatatgaggtctctggctgggtagagagcatgaaggacacatgagatctggagtctggatgaacttgctgacaagcaagctttttttgactgctaatgcgtaaatccactatagaaattttcatttgtcatttttgtacttattggcaaaaaattagagcttataggcatcagatttaatttgagatagttgaaatagggtttgtgtttgaggccaatataattttatctgctaatggcatctcgtggacttggaggcagcccttctgtaccagaacattgtcaaaagcttttactgtaaagcttgagaacaaactagtttgctggatttgggcatgtaactaacaggtttgaggcatgggattatcctgtggacttttttttttttttttttgctttgaggttctgaatgtattaaggttgaccttcttaagccgttgaaactgttctgcagtacatttgtgatgtagggcctaagacttgtatcgttttttttttttaatcacaacccagtgtacagaacttgagacatgcgtcttttctctgccaccttttaaaagcagattattcttgaagtgcatagagcagcaattgattaatggaattggtgtcttcacatttcatttacttcctcccaacaattttataggatgcatataaatatttccaaaagaggtacacataatttcttactataaaagtatttttatatttatatcagtaaatttgttaataaagaggatttttttttttctgtaatcctaccaccccaatgacgtcctattaaaatttcagtatatatcctcccaggtcttttaggtatgtttaatttggtgtcccttccccgctcccaaaaggggagggaccaggttcttgtatagaatagtggaatgttagtaaatcacaggtttaaagagacataacagtggaatctctagagcagctgtcacctggatacctggttattaaggtaatttttccattaccccaaagagctttagttacactcagctttttccttaatccttgtgcagctctccagggcacaccgtattcagctctgagcggtctttgctagtgaggccaaggagccaccctgagccaaaaggggagcattatgtcaccggaagcccaaccccagagaaccaaaggtatgacctgatattcagtggccccagccaggtctttacaggaagaccctcatatctcaggtctaagaagagccagctgatggtttttaaaaagagtggaattagttactccaacccacttattcagatcttattttgttcacaatacagtccctagattgtaggcccattggaggccacagcaaagcctttgtgttccagttggcctgatgtgccatctctcagtaatgttcccttaacagccagacttccctaagcccagctgggagctctgaaggtatgcgagccctccctcaaccatgagtgtagggaaagggaccaggggccccaggctttcctgtcagtaatgcagaagttcctcagatttagggaagggggagcagaggcataactttgattctgacaaagaggcattcagagagactgaaaggtcatttaacaaacactggaatgcttccacatactaggtgctaggagatacaaaaccatataggtcctggaagggaggattgattttttcattttggtacgtagtagatattaggggcttaggaaatacacatcgaaatgaagagtgcatttgccatgttgaaccgttagccggtatcttatttccccattttaaaagttttagaatctgtggttgaggacttgtggccatcagttttccatagccaacagactgttcactactgccttcagagctccttggacctcagcgggccttctttggagatggcagagatggatttagatgtatactctactcgagccacccagagagcccacaaagtcagagatggaacagggtaaaggagtaagggtcatatgtgtgagatgccttgatttggaactttgagatttaggatgaggtggggaagggctaaagaggagcttgttcctgagccttgcttggccgaagcatttaggctcaagcgttttagaaagagtagcccttggtctgagaactcaaggaaacagctttctgatgagacgtgtagcaagcttctggttcacatccttacctgatagttcttcaaacactgcctggtctggttcacatccttacctgatagttattcaaacactgcctggaagcttctcctgagtttttgtctctaatcagctaactaacaggctgagtgagtttagttgtaagtcattaatgaagaaagcaaaggttggggccattgtcagggttgtgacctgggctagttaattacctggaactgatggtctgtgttacagagtggtggtatacttgtcaggcttagaaaagaaatcaggatgtgtatcaaaaatcatttggggaaaagatttgaccagcaactttaatttctctatgtttgcaactatcctgttaatgtagttgtgataatttcagaattataccagtgcccttatgttatccttgctttgcaaattgcaaattgctttgcgtgtcctgacatccttctggccaacagtagatgtggttttaggtttagactcctgggatggaagcttttgcattcaggggaatgactttgggtttgggtgaggattgtaaagaggcaatatgggtgccccacgacaaagcagctatttgtagctttgtgacagcttgacatgcagagatctaggcttatcaaggcactaagctaggagtcagttgtttgtatcactggaagattggttacaacttccttcattggaagctccttcagtgcatgttaaatgatgttatttatagatagggtggtgagaaagctgtctaggtagatgtcagtcagcccagtgtaagagagacctgcttactgtgggtgcttgggactatgtggagtgggtgggaggttttaacttgttcagtaaggtcctttccattgttcacaatctggtgaaccctttttctaacatgaggagcacccacataaccagatcatgtctggcttccctgtggcttgtgtacaaagcgtgcttattgagttaatgtgtaagcaggagacagccttctgtgctaaatggtatattaaccacttctcagtcttaccactctctttcaatttgtctcgacccaggacctcagcagccatgtcgaagccccatagtgaagccgggactgccttcattcagacccagcagctgcacgcagccatggctgacacattcctggagcacatgtgccgcctggacattgattcaccacccatcacagcccggaacactggcatcatctgtaccattggtgagtgggtgtgccccttcccccaaaaaagggcttcatgggcagtgacctttctctcctgaaaagagtaactaaatgtcctaacaaacctaggtgctacatgggatactacacagattcttatgaaaggactcaggtcataggaagttgcagtaaagaattagtatgtgcataggatggcaaatacagttaataagagagtattagacatttcaaaattgctaagatggcgaggtatggtggctcccagcactttgggaggccaacgtgggaggattgcctgagcctcgaaatttgagaccagcctgagcaacttagaccctgtctctccaaaaagtgaaaaaaaaaaaaaaaaaattagctgggcatggtggcatgcacctgtagttctggctacatgggaggctgagacaaagatcacttgagtccaggagattgaagttgcagtgagccatgatcacaccactgcactccagtctaggcaacagagcgagatcctgtcttaagaaaaaaaaattgtccgggcgcagtggcacatgcctgtaatccagcacttcgggaggctgaggcaggtggatcacctgaggtcaggagttcgagaccagcctggccaacatggtgaaatcccatctctactaaaaatacaaaaaaattagccgggggtggtggcgggtacctataatcccagctacttgggaggctgaggcaggagaattgcttgaacctgggaggcggaggttgcagtgagctgagatctgaccattgcactccagccttggcaacaagaacgaaactctgcctcaaaaaaaaaaggaagaaaaaagaaaaaaacatcgctaagagtaaatttcaaatgttctcaccacaaaaatgttaagtatttgaagtcatggatatgttaactaacctgatttaattattccacattgtatccaaactgtatgtattggattacataactttgtaacccaaattataaattaccagtttataataaaaaataatttgttgcaaaaagaatccatatggtttaggttttatgctataggcaaaatttagaagatgttttccttagcaggtctttgtaggagcaacttaaagacctaggaaagatctttctaacatgttctgtgctaccaagattctgtggttggacatctggctgggtttcagtgagggtggagaaggctggccaagtcttaacctaggcttttctgatacagtgggagcctgcagaacttgaaggaaatggtcgaagtgtcccagtagatcaagaaagtaagctggcacggtagtagccttccatgcactttttaaagacttttgagctatttgggagaggaaaagttttcagggaaaaaaattctttaaacttaagcaaacttaaatgtttttccttctttgaataattaatacttgtggctttaaaacttttcctaataggcccagcttcccgatcagtggagacgttgaaggagatgattaagtctggaatgaatgtggctcgtctgaacttctctcatggaactcatgaggtgagctgtggctggaccctatggccattgtgatggcctgtaggaaacagggagggggtgcagtgttcgtttagccacagtggactagacaaggatgagtctgagtttcacagtcagtgtgaagtttgtctttactagcccatccctactctccttccctcttgtcctgacaaagcaactggctgagtctcttttagcaaaaaggaccccctttgttgctggctgtggttctcccacacacctctcctacccttagcttttacaaaggaagatatggaaaggttctactggaaaaccctctaagccttaggtgtcctggccacagcgcttgactctcctgtcccagggtttctgcttcaccttgtgttgccatggtaaaccatctagcagattgattctagcttagaaccaaaataactgggcaggtccatgagaacggtttccactattctaagttttgagggactgagcctaatgcataagcactatctggggtgtaataccccacttcctcagcactgtattctcagcctgtgccttcccaggggttctggtacattaaaataacaccagttagcactcttccccaggagcctagtaggactgtatttgtgctgggctctttattagctggctttacctatggacagaggccttgcccaggagccaggtagcagctgttgggatggctccattcctgcctccattgccagatttagaattaacccattctgaggagcttggggttccctgaggtaccatgacttatttatttttttattttataaaacaaaattttgctctgtcatccaggctggactgcagtggtatgattatggctaactggatccttgacctcccaggttcaagtgatcctcttgcctcagcctcccgagtagctgggaatacaggcatgcaccaccacacctggctaatttaaaaatttttttgggggaaatgaggtctcactatattgccttggctggtctcaaactcctgggctcaagtgattctctcaaatgttgggattacaggaatgagctaccatgctcagcctgggattgtgcctttttaaaaccttcagacttaaccataggtttcccatagatcatgggatttcgtaatggcattgataagaggaattacagaagaggcaaactttgcacctgtcttggcttctgtatttcctgttgagagtaaagaaaatgctatcctgtaaggccaattgccttacagaggttgccctctggcatttggaagttggtattaagtttggactaaaaataaagcctcaggaaatgcaatccaagagtgaattcctccttttgggaaacacaagactcttcatcatagattccctaacctgtgttcataaacagcctatggcctggctagtggctggcccttaaatgtcatggggacctgaccaagtccagcagacataccatgtaggttaagacatgtccctgtaccttttggaaaattctgtagttttccaaaagcaaggggtccttagcaggagtcaccgagaattacttgttagagaattaagtgttagcttagcttagagagagctgaagacaatgctggaggtctgttcgctgttgatccctgctgctgtagtctgccatgggctcctgcattcaggggaaggagcagaaatagatttttaagaagttgacctttaagtaggctttatggttccttcatccagtaaaataacaccacatagctctaacatggcaagggcgagtgatacctgccacacctgctggatgagagctggctccgattttggtattttaaactttaagaggcttttggagattatctctactttcactcctattcccagattataattaagatttattttttattttttatctatttattttttaaagatgtccctcttgtgtgttcattttgaagttttagaccaagatgaggttgtgtgtgggctcagcttggaaactgatctgaaattattctaatttatataatgtaatgtaaacagtttcagccttaccatacgtcagggctatcgtttcatgtgcacctttgactaggggctggggcgtacttttccagtttctgactattttaaatgctcttctgagcagaacgttgagattactgtcttccctctcactctgacagagggacatcaaatgtctgcatctgatcttttaacagctttttttttttgagacagaatcttgctctgttgcccaggctggagtgcactggcacaatctctgctcaccacaacctctgcctcccaggttcaagcaattctcatacctcagcctcctgagtagctgggattacagacctgtgccaccacgcccagctaatttttttatatttttagtagagacggggtttcgccatgttggccaggctggtcttgaacttgtgacctcaggtgatccgactgcctcggcctcctaaaggcgtgagccaccacgcccagccctcttttaacagctttggcaactagtcttcagccctcacttttggcagttcacatgggcaagatgcattcttgctgaacatgtggttccatatgccatgttttccagatttatttatttatttatttatttatttagagagggagtctcgctctgtcatccaggctggagtgcagtggcacgatcttggctcactgcaacctctgcctcctgggttcaagagattcttctgcctcagcctcctaagtatctgagattacaggcacctgccaccacacccgactaatttttgtattttagtagagacttggtttcaccttgttggccaggctgatctcgaattcctgacctcaagtgatccatccgccttggcctcccaaattgctgggattacaggcgtgagccaccacacctggcctagaaataatgacttttaaacaacctaaatgtagagccttccacaggacagcattgatggatgctttaccacataacatcccaataaagccacagctgaagtggaagactcagtacacctcccagagatgctctaagagattatgatatatgacatagatttgaataatatacctaataattggtatgtttataatatatggttttacatccccaagaccaaaaatgcatgtttgcatgaaacactcatggttacaaaaatatattaggccaccaaaaaaacccccacgtttcataaagtagaaattatacagacacattctctgataaaattttttagtggaaattaagaacaaagtcaagaaaactgaagtgtgcttactttagaaagcaaagatctcaaggtagatgaaataaatatttaactcagaacactaggggaggaaaaccctaaaaagggtgaagaaaataattttgtaagattatagctcaatgaaatgaaaataaatttgacagattaagctaagagctgattctttgtggggaaaaaatagtaaaatagaaagttctgagaagccaggtgaagaatgcgaggatgtgcaaataagagtatgaatagaaaagagaatatttcctacacattggagattttaaaagtcaagaaagacttataacttaattcctatatagagagatgactctggctattttcaaagaaaagataaatatccaaaagatagaaaatatgaatagaccagtggccataagaagttgaaaaagtgggctgggcgtgcggtggctcacacctgcaatcccagcactttgggaggccaaggcggagggatcacttgaggtcaggagttcgagaccagcctggccaacatggtgaaaccctgtctctactaaaaatacaaaaattggctgggcatggtggcacatgcctgcagtcccagctactcgggagcctgaggcaggagaatcgcttgaacctgagaggtggaggctacagtgagccaagatcgcgccactgcactccagccaaaaagttgaaaaagtgattaagatctggttcacctcagaacacttaagtccaaatgattttagtggctgaattgtctccccttcaaagttcagttacattgttaaactgttccagagcctagagaaatatagaaatcttcccactgtgttctttgaaaccaatatacgctgatactgagatcaaacaaggacagtaccaaaaccaggcaggtactaacagttagtgtgctagaccagtctcacttagatgcagaaaacaaataaaatttaataatccaaatccagtagtgattgaaaggaatgtcttgatccatgaccaagtagattttattctaggagaacaaaattctacatcgggattaagtagagttaaggttgacatttttttttttttcttctgagacggagtctcgctctgtcacccaggctggaatgcagtggcacgatctcggctcactgcaacctctgccttccgggttcacaccattctcttgcctcagcctcccgagtagctgggactacaggcgcctgctaccacgcccggctaattttgtttttgtacttttagtagagacggggtttcaccatgttagccaggatggtctcgatctcctgaccttgtgatcccccctcctcggcctcccaaagtgctgggattacaggcgtgagccactgcgcctggcctgagttaaggttgacttttaaacaacctaaatatagctaaatatagagccttccgcaggacagcattgatgtgtggaactcttatccacgtgataacatcccaacaaagccacagctgtagtggaactcagtacacctgagtcttatcattataagatgataataggtaacatttattagataattaccatgtactttgtcctaatacttcatgtattcttttactcctcacgtcaactctgaaggaaaggcaccacctatccccttaaaagaaaacaactattactattcttttttttttttttcttttagagacggaatctcactctgtctgtcgcccaggctggagtgcagtggcacgatctcggctcactgcaacttctgcctcctaggttcaagtggttctcttgcctcagcctcctgaatagctgggactacaggtgcacgccaccacgcccagctaatttttgtattttaagttgagacgaggtttcaccatgttggcctggttgttgtcaatctcttgatctcatgatccacccgccttggccttccaaagtgtttagatgacaggtgtgagccaccgcgcccagcctctattctattctattttgttctatttctattacaagccagtaagcaagaaaatatcataatttataaggaaccctataaaaaacagacaagccaagggtctgtcattaggaagtatgcctgaataagaagctgaagatttttagacacaggtttcaggcaacactgtctttagaggctaggctctggctccagctccctccagcctcctgtgaataacaggcaggcttacttgcaggtgccactttcctggacagtggtggttaaaggacaaggcccagaaagtgctgaattaggtgcccttgttaccgctaatgtcttattgatgacactatcttagagctcttttgacatcttggctctgcgtcttttttttttttttttcttgagatagggtgttgctttgttatccaggccggagtgcagtggtgtgatcatggctcactgtagccttgacctcctagacataacccacctcagcctcacaagtagctgggaccccaggcacgcaccatcatgcacagttaatttttgtgttttttgtagagacgaggtttcgccatgttgcccaggctcatctcaaactcctggcccaaactgtcctcccaccttagcctcccaaagtgtttggtttataggcatgagccactgtgcttagcctgagtccctcttttaaacaaacaaaatggtaaatggaaaggaggaaaggcttaagaaaaaagattgaagccaggatttgttgtaagcaaggagtaataaagggcagttcatttagagaaaggcatatgaccacctttccccctccaatcagaatctagaaagtgattgaggccgggcgcagtggctcacgcctgtaatcccagcactttgggaggccgaggtgggcggatcacgagatcaggagatcgagaccatcctggctaacatggtgaaaccccgtctctactaaaaatcgaagaagttagccaggcgtggtggtgggcgcctgcagtcccagctactcgggaggctgagaggcaggagaatggcgtgaacctgggaggtggagcttgcagtgagcctagatagtgccactgcactccagcctgggcgacagagcaagactctgtctcaaaaaaaaaaaaaacaaagcgattgagaaaatcaggtctgtgtgaccttagcaatgagttatttagcttgggccactgttagcttaagtcaataacttcaagtttgcgttgtagttggaatcaatagaggaaaagctctcagcattaccacatatatcagaatgtgacattgattgccagaccagccttatccaaacacaagtcctaggctttttgccctgtttatgagctttatatgctgagggtatttgatgagtcttagggaaaaaagaacagccctggggacacagctgcttttatgatgagacatgtttgcacccataccttaatgggttttggtggcaatattctgaaatttgccacctacatttcaaagatttgccctttgggtgaattagtgctgtagtagaagtgggtggaggctgaggaggttggattaagcaggtagaggatttctcagtgcatggatcgtgctgaggatggagatagagctctaagacatccacgggcctttcctgagtgatcagctttggctcctgggcaggggaattggagctggattctagtgtgggagcacgcttgtcatcttccttcttttcccccagtaccatgcggagaccatcaagaatgtgcgcacagccacggaaagctttgcttctgaccccatcctctaccggcccgttgctgtggctctagacactaaaggacctgagatccgaactgggctcatcaagggcgtgagtattctgcggagagcgaggggaaggctcagtaggcaatatgccccagagacatgtcctccaaagcgctgggttgccatgtttcttcccagtactatgaaggactgcagaggagttgaggtctacaaatgaggatttattcatcactgtaaacaatgttgatttgatctactttgctaggaaatggtaccacaaaggaaccttttttttttaccctaaaaacctaaactttaggctttctaacttggagaaccatctctttgtatctttttccccatcattaagtagcataactgaaacatattcttttcttggattatttccgtgaagtatacagagttagagaataagagcaaaaaactgtattacttttagcagtgacttgagcattgttcccgggaggaaagagcttttccattccttctgaggtgatgctgctactggtgtctccagtttggactcttgcttactctcttgtccctagagcggcactgcagaggtggagctgaagaagggagccactctcaaaatcacgctggataacgcctacatggaaaagtgtgacgagaacatcctgtggctggactacaagaacatctgcaaggtggtggaagtgggcagcaagatctacgtggatgatgggcttatttctctccaggtgaagcagaaaggtacgtatgggagctggagtccagttgtctaaaacagtcttttgtctctaaacttccttgacacaaggaagatgggaaggttggttgcctggcagtgagattgagtctgtgtgttctcaggaatcccttttataactcatttatcctcaaagataggctttaatccagcatagttacattcttctggttctggagaacacaggaacatacatacatatatatatatatatacatatatatatatatatatatatatatatatatatatatatatatttgtttcgctgtgttttgttttgttttcaagacagagtctcgctctgttgcccaggctggagtgcagtggcatgatcttggctcactgcaacctctgcctccagagttctagctattctcctacctcagcctcctgagtagctgggattacaggcacccgccaccacacccggctaatttttttgtatttttagtagagatggcgttttgccatgttggccaggctggtctcaaactcctgacctcaggtgatctgcctgccttggcctcccaaagtcagaacagtcttaattatccttatttatgggtgaggaaagtgaggtacagagaggttaaatggcttgcccaggattacacagtgtagtaggttttcaactctggtaaaacagctccagcacccataatgcaccacttcccagctcactgtccttgcgggaaaggtgcctgcttcctgttgacctgtgccctcgtgctctgcctcccctacttaccctttttcatacaggtgccgacttcctggtgacggaggtggaaaatggtggctccttgggcagcaagaagggtgtgaaccttcctggggctgctgtggacttgcctgctgtgtcggagaaggacatccaggatctgaagtttggggtcgagcaggatgttgatatggtgtttgcgtcattcatccgcaaggcatctgatgtccatgaagttaggaaggtcctgggagagaagggaaagaacatcaagattatcagcaaaatcgagaatcatgagggggttcggaggcaagtccccgttgtccctgctccagtcccagcgcagctctccgaagggcatggtccatcctgtgaatgtctgattcccagcccctagcccatcagaatgtagactcccaagccagttccaaacctgctgaatcagaatatcttaggagagtagaaggcattatgtttttttgtttttgtttttttgttttttttaaaaaaaagcttcccaggtaattgagatgctggcagcttgacattgttccctgggcctggggaccaacatttgagagaacagggtcactgctcacaggaccaggggccatgatgttctgttcctgatcagaaacactaccagtgtttgctggaatggggggaccagggggaaagatgacagcagacacttaagaaagggctctttttggcccttcctggggagccatgtggaatttcagggcctggtgtccatgttaaagcttatggcctcctggtcttcacttagaatgcagctggctcagtgatcatgctaactctggtatggtccattccactctcagaggaagatgtgtggttcttctccagtttcagattgccccaacttagcttaccccctccccaatgctcacaaagtagagcccagtgggcatggccaccatttttggcatcctgctaggaatacaactcagcacaactaagatgctagacacactcttgtggattagaagtgtgtttggggagggtgggggagcaaccctgtgcacccactgtagtggccttactgtctgagctttgtgtagatatcctctgtaccaggcaatttggggtcctcccctttgccatcctgataagccataggctagctgaacttggccctaggccaggcaaagccacattccctcttgccttcagcaggttggagtgggccacctcaaagggcagtcctcaagtgtccttgactagatgaggccatgggtctttgtggtggaagcagtcatcaggcctcaggttccctgtcttgaagtgctgattggaaaatggaggccctagagagacccctaacatgcatgggatttggagaggagaccttgggaatgagcccatttggatttgccctctcccctttcttccgtcaatgaagcatccatattggtgttgaagcccagcaggcagaattgttggcccactctgggggcctaaggtagctggactgccttgccatctgtgtgcacccatgatgatatcatggatgtctgtcctggtacaaggacatctaagttagggaatcccagggaaacttcttgtctactgccatacttgtggcctctgttctatataacctctctccccccaactttgtccatcaggtttgatgaaatcctggaggccagtgatgggatcatggtggctcgtggtgatctaggcattgagattcctgcagagaaggtcttccttgctcagaagatgatgattggacggtgcaaccgagctgggaagcctgtcatctgtgctactcaggcatgtgcccacccttccccacattctcatgtgcacactcgcatgtttgtatgggaaagctctggaggctgtctgatctcttcccatggaattgtcgcacgtaacacacagataatccccttcccccatgtacctacacaaagccatactctgtgtacctactcactatccagaggatcagcttgctgtcatttgtctctgaagacagctcaagctacatctcactaatgctctgtcccctcccagatgctggagagcatgatcaagaagccccgccccactcgggctgaaggcagtgatgtggccaatgcagtcctggatggagccgactgcatcatgctgtctggagaaacagccaaaggggactatcctctggaggctgtgcgcatgcagcacctggtgagttctggggcctgccccatcccccagggcttcggactgggcctgggatggatgcaagctctggtgcagagctttttaggtttctccatcctcttatgcacagcctttcattatcctccaagttacagcagcaagagggtgggggtggaagtggaggtggcttttttttttctcctgttctgcattcctgcccacacccccacccctccatttccttctgctctggaggcatcctccttcattggacaccacacagtttatttcacttctgacttcaaggttgtgaattcttcccatggcttaagtcctgggatacttctgcagtgaaaggaggtcttgtacctcttcctcagagtcagaagttctgagtacctttgccctattctgaaaagggctaggggctcctgctcccagctgccctcttcctttggcttccaattcagttccctctgccccgcatcctgcagacaggcgctcccgcagggggcccttgtggacctgcactggagtctgttgccttcactgagctgcctgtgctggccttgcatggtgcctgtagggggatttgctttgctgtgccattggggtacagctgctgctcttactctagaccaaaaagtcgggttgagtgactggtggcagggccacagatagagacagcggggagggtggctgaccctggcggccctggactgagcgtctggaggagtcgtggaggctctttcccttctttctcctctgagagctcgttcttcaggctcttccagcttgtcatgtcgagtgcctggccactgctcagggttggaggctcagtccctttgccctgtctgttccagctctggagctaactcagggatccctgatcagggttacataggtttggtaaaatgagtgctggaaattaactttctcccagtagtcttaggtcatgctcagtgaacttaaactttatccagatatggttttccttcagcctttctattccctttctagccagtgaaagacccgctgccctttgacctcagcccctccaagcccccaagtttaaaacgccaccccctgccaccagaaaaaacagaaaaaaaaaaaaaaaaaaaaaactaaaacacccatctggtctgggcatcttcctttcctttttcactatgtatcctgttactgggcttaaacagctttcagagaagagatgtcatttctattaaatgctctttcagtagcgaactgagttcacacttgactaaggatattttccggactgtctgtcatcagcatccttagtgggtttccccatatttaaattggtagaggccagggatggtggctcacacctgtaatctcagtactttgggaggccaaggtaggtggattgcttgagctcagaagaccagcctgggcaacctggtgaaaccctgtctctactaaaaattcaagttagctagctgggcatggtgatgcacttctgtagtcccagctacttggagagggggtgatgctggggcagcaggatcgcttgaacccaggaggttgaggttgcagtgagccaagatggtaccagcctaggtgacaaagtgacaccctgtctcaaaaaagaaaccaaacaaacataaaaaaaaaaacaaaaaaatcggtagagagtgatttctctcccaggcccacttaatgtagactgggcctggctgacacctcaccattcgtgtgatgtgattgctgttctgatgcttagatactcttggcgcagtctcacaattgccaccatggtaggaaggtgtcccaggagacggtgcaccttgaaccagtcaccactaaagtggctgcctttctgggtctctccacacatcccctctctctaatttccctacttaatcgtgtgacttcatggtctcaaaggaggaacagaggctgatcttgacttagatatactgaaccatgaaatcactgcatagaatgtggggacttgaatgtgtctttgggcaagtcatttaacctcttaagacctcatctgtaaaatggattagatatgtttaattatagccttagcattaaatattcattgctgttattattaagtgtctgataagtctctgtgtacatggatgtaatcttcctaactcccattacctccatttatagatgagggttatatggccaataaagcctgggtttgaatctaggtctactgcctccaaagccagtcttctctcctgcaacatcatgctctgtctagcaggagatgagaacaggtctccatttggagcctgtcagtggggtcagagactaagattcaggctcagggtctaaattccatatcctttcttccataccctggtgtttcctatgaacagatagatactttagggctgcaaggtttggattgcatggcactgctcagaagataagttacaggtctgggctaggctgtagctgcccctccaggtggctagacctttcctttctgtgtcaccagttaacactggccaacagttccttccattaactgttcactgctttctcctgtgtctaactgatgcagtttatgacccataactaagagcagtaccaggtatggctctgtttcctgttcatgtcccctgtcctctgggctgcatgcattccgttcttacagaaagaatacctttaacctagtacatcctgccacacatctgcttctactgtgaaattgatgagggggtattaccgattcttccctcacccatcatttactgagatgctggtgattgcattataatcctctaaagcttacattgtctttctgattcttggtcttatctgagcaagtgatctataaataactcagtggctttctcatgactgttttaattattagattttaatcaagtgtcttattaaatatatctgcatgcttccacaggcatctgtctcttcacatggctgttcagtgtgcctctcacaagttagcccacgttttctgttctcctgcttcaaactcagttgagctgccttgctttggctttgatcccagctttccagcgctgctcaatctgttgccatggcaggccattggaaaggctcagtgcatccccgtgcctgaagccaagtgagcgctcactccatgcatgcatggaggctgggcaggagcctgcctaatcaaccagccatgtgaggagggagggcctgttccttcctgtaagctatgtcatgaggcagcgtggtcaagtcctctgccagggagtggcctgggcccagcctgggcatgttttcatgccagggtgctagagcctactgccagattgtctccctccacccccaatgaaaaaatccttccagaagggaagagccaatttcccctgtattggaggggaagtggcagcacctcctgaagcagttggactttcatcaccctacctctgcatctgcctgaaggacagatttagccaattaacctaaggttaccttcctctctgataaattccccattctgtcttcccatgtgttgtgtctcgtttttttcctcctccttccctcttccttgccccctcttcccctaaaccttacagatagctcgtgaggctgaggcagccatgttccaccgcaagctgtttgaagaacttgtgcgagcctcaagtcactccacagacctcatggaagccatggccatgggcagcgtggaggcttcttataagtgtttagcagcagctttgatagttctgacggagtctggcaggtagggccctaagggcaggtaacactgttaggataaccagcctcttgctccacctgctctaggagaagacagccaggcccaacctggcatctgggcacagagcctcttctcgtctgtaggaacaccgccagggaggtcatggcagggcaggaccaaagggtcctgtggctcagtaggcacagtagatgtcacaggcacttggtgaaggactggtttctgtggagtcttgatcttggctcagctcagaatctccagtgattgggctcctcttggcctttgttcccaggaacatgttcctcaccagctgtccggtgactcttcccctccctctccttttgtgacaaagctctgacaaagctctgtccccctctcgtccctctggacggatgttgctcccctagattgcccgtgaggcagaggctgccatctaccacttgcaattatttgaggaactccgccgcctggcgcccattaccagcgaccccacagaagccaccgccgtgggtgccgtggaggcctccttcaagtgctgcagtggggccataatcgtcctcaccaagtctggcaggtaggaggcggcagcggctccctggaatgccctgctcagtggtacctcaccttgggggtcctgggagcagtccattgaacaatgctcaggtggcactgagccaaggtaagacccctctgcctgccaccttgggcctgcagggaaggattgagcagagccccttccctgggcccaaaggactctaggtagcactcataaggaatgtcagaacatttggatcaaaagcaaatttatgctggagatttattacataacagtgcacaggctgactacaaatggttatttgatattgaaaatttagtcctctaaaattgtaaaagataaccacttttgcttattccagttactatgtgctctttaaaaatttcagttgggaaatgaatttatttaaatgctgtttactgtgcctccatttggcacactagtccctgctgtttttgagccctaaagacaaattgggttccagctcaggagaggttgctgtgctatcttggctgacattctgtggggcctggcagccaggctgaggactgtgtggcctatgctgggcctccaacttgggatcccttccttggcccaggacattgagttaatgtccttcactctcctagttagggagtatgctccttgtccctgtccacagggcagcaagggtttcctggaagaggggagcaaacaggcagtgcccatgcactgaggagcagcagatgggcgtgggcagcccagagaaccaggacacaagctctgtgcagatgccctcagcagagggctccagcctcccactcttggctgaacagctccaacccgtagggttgacctttcttaaaaggtccagttcttgctgtttggctattttaagctctagtcttctggggtttcactcagctggtcctggcttcagcaattgcttccctctgaaggccttgcatagaggccaagcgtgaagtgcagggacttctctgctgtgatgtggcttaagtttccctgacacctgttgagtgtcctcataacttcccttctggtgcccctccccagctcctgagacacagctgcagctacaagtgtgcagtgtcagtgttcaagaaagtgcctggcagaggggctttagaagggtcccctgccttccaaaggagctttggcaggcagagctgctcctgcagcaacactcccatttcctgttcttgcctgctgagtagcacctagatttctaagcctcatctagatactcagatttgattctgggcctttatagcccagttgctgggactgtttcaggagctaggggccatgtggggcagggagagggcacaaaagtagagaagcctgatgttgattcccagggggctggtcagctctgctactgctccttgcagatgtcaagagtcaggtgctagtcacgtgctgcttggcttgtcactgtcattggcagcgagaggaatgggtgctggtgacattgggccagggctgcctctctgtgtcagagttcagggtgtaggaggggttctgccaaccatgggctgtgtggggtaagtgggtgaggctgatcttgctgggtcaaggtgatcctgagcccttggcctgtggaatgggggtagagggcaaatggtaacctagcatgctgtgggggatataggatgaggggctgcccgagcctcgggaggggtcctagggagcagatgttgaagaggccagagccctcagtgagctggatgagagggtgagctgtttgaacgccctgagggtacttcctggggcctcgtgtaatggtctcttctgtatgtcccccatcccatctcaggtctgctcaccaggtggccagataccgcccacgtgcccccatcattgctgtgacccggaatccccagacagctcgtcaggcccacctgtaccgtggcatcttccctgtgctgtgcaaggacccagtccaggaggcctgggctgaggacgtggacctccgggtgaactttgccatgaatgttggtacgtggctggagcaggggctagagcctagaggagcttggggatgcttgagcattggcttctgtgggaccccgaaagtttggggaatagaaaggggaacacacagaccttagtggggcaaaaggcccagcgactgttcctctcccttattgggaatgttcattctgaatctctcattctccgaagtcctaagctgagccaggagggaaaagggtcctttgagttgtagggctgagcaattcagttcctcttctcttctagtctggggctcaaagcaaaattgtccattttttggcatctgctcattactgagagttttttttgttttttgttttttttttaaataaaattggccacagctcctgtgctgtggggtggcatacacagattacgtactgatgtggccattgtccctgtataaggtagggtatcatcagatgacaggaagcagctagctctgaccctgggcaaggctttgcaccctctccaggatagtgaatgatgtccaaaggtccctgccaaccctgccatctgagtgataaggacatttcagggccttcctcctgtttgcctgggctgtgagtttggtgccaccttgtggtgtgaggaagtagtggtcagccagcctagttcagtactcaggctatggggcagctgcccaggtgcaaacctgcctggcttggcttttactcaccaacctcccttctcttcctccaggcaaggcccgaggcttcttcaagaagggagatgtggtcattgtgctgaccggatggcgccctggctccggcttcaccaacaccatgcgtgttgttcctgtgccgtgatggaccccagagcccctcctccagcccctgtcccacccccttcccccagcccatccattaggccagcaacgcttgtagaactcactctgggctgtaacgtggcactggtaggttgggacaccagggaagaagatcaacgcctcactgaaacatggctgtgtttgcagcctgctctagtgggacagcccagagcctggctgcccatcatgtggccccacccaatcaagggaagaaggaggaatgctggactggaggcccctggagccagatggcaagagggtgacagcttcctttcctgtgtgtactctgtccagttcctttagaaaaaatggatgcccagaggactcccaaccctggcttggggtcaagaaacagccagcaagagttaggggccttagggcactgggctgttgttccattgaagccgactctggccctggcccttacttgcttctctagctctctaggcctctccagtttgcacctgtccccaccctccactcagctgtcctgcagcaaacactccaccctccaccttccattttcccccactactgcagcacctccaggcctgttgctatagagcctacctgtatgtcaataaacaacagctgaagcacc

SEQ ID NO: 46 - DNA, 34218 bp, Macaca mulatta
agcatttccttctcaacaacagctaaagtgaccaggaaggcttacagaagaaagtgaaaaatttttatctcacttcaaacagaaatttacttttaggctgtcactgtctcatcccagcttatctgagctaacaggaagcgaatgaaggcctgtgattcagctgcaggcagcgggtaagcctgagcaggtcacactcatttggtctcttttgccaggaaaagaaaaaaagaacctgagagaactgtcttcacattttgaatgcgcaacattgtatctgtgaatgaaggcaagagttaacagctgtttaattgataactgctcgcatcattggttgctggctaacaattgggaaatcggaaaatgtcttgtagaaaaatgtaagaaaagttccaacaatattgacttaaattcatgacaaggtgaaaacagaaatgctgactcctgcataggttatcggctctaatgttctgacttgattatttccagatgcccagctctgcgctaatatcaacgccgtctatttgctttttactctcaggcattcgctctgcaggattccagaccctactaaattattcacatggccccaacctgtccttccttgttccgcggttctaagacaacaaatggtcctaagaggaaaagggcctcgcgctcccgctccaggcccacttcgcagtccctagttctccctactgccgctccagtgccagagcccctccgaaggcggtcgagacctccaaccacgcacaagtctgcagctctccccaacttcccgttcagctcagtctccgagggtgcgccagggcagacacccggaggagtggggagtggcagggcggggccgggagaatgctgccccggaacccataaatctgggccctgcccaggtaggccgggacagttggggtggcctgggccgagagccaagaagagacctcatctggcagcccaacttggcggcaacaggtggcccggcgcccgggggtctaggagggaagtcgctctaggggcgggatccgctgccccgccgcgttcccattggccgtcaggttctttaaactgtggctctgaatctgtgtccttccgccgcagaatttagtccccccgaaagggcaacctgcccgcgctctctgccgccgccaccgcgcttcctcctgaaggtgactgcgcccgcaaagacgcagggggcggggcccgggtcgccgggagccgagattggacagagggcggggcggcggagggattgcggcggcccgcagcgggataaccttgaggctgaggtccctgctactcgcacagcagctgcacgtccctgggatccacatctcttccaatttgcagcgtagcccgagtcggtcagcgccagaggtgagcggtgcaagaggctgcgccatctgtccccaccaagggcctgtgcacccggctagtgcggaatcccggcgcgccggccggccccgggcacgcaggcggggcagcgcaggatccggggcatgtgggacgcggtggagttcagagactggagaacggctcctcagaagtccccagcgccgttccttccagatcaggcgggtccgccggctcctttcccgtcccagccctaccccctcattctggtcccatcctcctgccccaatcctcaatgcgcctccatccttgcctgccttctctcggtccctcgtgattgattccacccttgcctcccctttctccgcgccctctgttccgtgctcgtttgttccacttcctcctcaagtccggtccttccacccactcctcttaaacctgtgcttgcctcttcgttctaatggcttccgtgtaacttactgaaactcggttctggttcccctcccgggtccatgctccattcatgcgcgaccgcccttcctgcgccccagttctctcttgccgcccctccccctgctcgctggtcacgtccgctctcccgcatccccctcctcgcctggcatgtcgcctccctccctctctgctctggtcgcgcccgcccacttgctccggtctccgagcgcggtcccgcgccccttttccatcaccgcctcccaactcccagcaggctcgggcggtgctggggccccgtgtccggggcgggcgggcggagggctgggctgggtcgcccgcgcggcaggcgggatgcggcggcccgggagcagctggaggcttacgtaacgttggcctgccccgctgcctggaggcagggcggctgcccctgcggcgcggtgctgtcccatgcgaccgggattagatgggtggcctgcgagggtctgggaatggctcgggacccgcgagctctcccggcccttgccgggtggccaccagggaccacgctccatctcgccgcggccgggctgcacgtagcggccgcgcccagagtccaccccgcttcaccgggcggtggccttgggccgcgtaacgggccgtagaaacgtctgcaggcttcgctggggcctgccggccctcgcccgctccgcgcctctccggcacgttttttttttttttcttttcgttttttcttttttctttctttctttcttttttttttttttttattatccagcaggttttttttaacacatgcgccctgattgtggaacgcggaggccgcggggtggggtgggggtgggctctggttactgagggggcaggaaatctgtggcgttcactcaacgcaaacggtgtgggtcaagggctctttgggggtcggagttagagaccagaatgactggacgagtcatagcccaccgagctcacaatcttaaaatgtatacccggtaatgctgggagtggggcacgagcttcctgctgtgggagggagggggacaggaagcctcgtaaggtctcaccaggtggcaagcacactggattagaagatgcaggaaagcaccttccagtctgaaggtcatttaaagactagtcatggaaaggcatccctgggcttcttaatctgcatactccagacccagggcttggacctttgctggtacgggttaaagtgaggccgacagtgaaggtccacgtggagagagacatcgggaagttgtcagaaaggcttttagaatcaggtttgactcattaatttcctgagactgattgaaggagttcagccgctacacctcagtttcccctgggaaaactgggagtaacattttcctcatgatggttgaaaggattcatgcctacgtggatgttgcacactcagttaagtgtctaatctctggcgaaatacccagaagaaaagcctgtgaatgaatatattattttcgagcacaattacttagtccagaattgagcataagggccttgattcattatcttactgctgtccgcaaacgcctgcagctaatcgtggggaatcaggctctctaaccacgtgtctcctggaaaccagtccccccagggatctggtttaatattgacaaagtcactgataatgtaactttccaactctctgcttggagcagatgctctttgatcatctgagattgggacctctagacaaaggcaggcaaggaggggctgagttaagccttcggtgttcccctgtaagtggaatacctcttaacaggggaacattccagcccttgacttgctctgcctgctggtgagattaggattggagccaggatcagtaacccccagttggccatcttgagggcgtggctactcccgaggccacagaggagatagaggtcaggactccccggctgcagcattgttagcaaataatttgccctttggtggcctgaggtgctgtgggggcaggagtgggctgtcttgtggggaagggaaatgtaacgcatcaccaaatctgtgggggagtggggctctgtggggaagatgactcaacctgtcaattattctgcttttgagagaattatcttcgctgggtgagtggggaaactacgtagtggttcttgcaggcttaaaaagtcccttctctttcagtgagtcaaataatgaagcatgcatttcccctaattaaaaatgcctcaacttcggagcttgcggtgagccgagatcgcgccactgcactccagcctgggcgacagagctagattccgtctcaaaaaaaaaaaaaaaagtgcctcaactaagtgaaaaatgattggtccgggtcacctggttctctgtactgccttaagaacttaggtgcagagtggcagagcccggtgcccagctaatgcagtctgtgcagcttcgttcctggcccttttgtagcgggcacagcagcctctcctgggacatgattaatgatgacttaaagaaggttcttgaactcatttctcagttactgacttgaaccaaaatgtatggatgttggtctcctgtctagcacagctgctttcattgtaagcattgcgttagaaataatgtattcatattttagcaaagagcatcattagctctttaagaactgtacccccagtgacttagcaaatttgttggctgtgactctaaacagctagcactttatgggagttgcttctgtgccttgaatgttgtgacactgatgtggggtcacaggaaaaaccattttatttcttaaagcggtttgtttcttaatattgaagcaatggaagaaatgaggaaatggccatgggcaggaagatagaaaaaaatacagcagttacattacaaactcactttacttgggttttagttcattttaaagcttcagggtttttttttttttttttgagacagttttgctcttgttgctcagtctggagtgcaatggtgcgatcttggctcactgcaacctccgcctcctgggttcaagcgattctcctgcctcagcctcctgaagtagctggaattacaggcacctgccaccacgcccagctaatatttttgtatttttagtagagatggggtttcaccatgttagccaggctggtcttgaactcctgacttaggtgatccactggcctgagcctcccaaagtgctgggattacgggcatgagccaccacgcctggcctgcttcagcttttatgaaggcaaatccggatgtgttatcttggccaaaagctaagactgagaccagagtacaggaaaatgactcatttgacattacccttctttctgaatcactccaaaagcccacagtcaaatcccaatttaactgatataccacaagaatgcattgcccctgtgagcagagttttattgcaacttcgagggtctttgtgagattggtttatttggtatgaggtcttaaggattttaagttgtccctttaagcatcagttctgatacagatgggaatagagctagacaaccagatatatgaagaccatttgtgataccaccttacttttggggagcttgcatttttttaccaaggggcagactgaataattgagtaatttgaatacttggggcattgttaaagaagctgttgggggaaggtgagcctgggtgagtggtggagggtggcgtgcagcatctgctgggctttccggcctcttggtatgactgctcagctcaggagttgggggctttagggcccccaccacccagtgcggcgaagccccgcccctgcagtggtttgtgcttgtctgcacgtaggagggagcaagccggctgcagtaccttcggtggcctctgagactcacctcccccacttctgtccgtagacaaagctcctggggagctctaagcctctttcctcatgccagcaagcagtcttggaagcaggctggggctgcggtgggagagatgccaagaccagttatacaagggcagtgaggttgccagtcctagcatttcagactgtggaccagcacagctgctggctgaacactgcagtcaagattctctgaagggagtcctatcccttccaaacatcttcagtttacttacagataatgtttattcatattttattttatttttttgagatagagtcttacactgtaacccagggtagagtgcagtggcacgatctcagctcactgcaagctccacctcccaggttcacgccattctcctgcctcagcctcctgagtagctgggactataggcgcccaccaccacgccaggctaatttttttgtattttttagtagagacggggtttcaccatgttagccaggatggtctcggtctgctgacctcgtgatccgcctgtcttggcctcccaaagtgctgggattacaggcatgagccaccgcgcccagccatgtttcttcagttttaaacaactgatgtctcccttggcaatgaataaaaaagaactactcatcaatggaatcagtcagggcacataagacccactgtgtccaccatgccatttcagaggagattcgattgagttaagcagggaaatagagatgtcgtaaacattgaaactatctcggtatccctctttggttattaacattagatgagcagaaaaacaaatgtcacccatcagatgggcaaacatttaaaaagtctggcagtaccaagggaagaaggtgtggaatgcagcaactcaacgttgattgatacagccactttggagagcaaatcagccatatttagtaaaaatagaaataaacataccccatgacctaagacttcaatttctggatatatagaaactcatacagtacagggagacatgtactacaagagtattgattaatagagaaaaactagtttaatggggagggggagtggccaccagtaagggagtccataaataaaattgtctgttgtacagtggactagtgtaacagttcaaatgaattagctagatccatatacccactggatggatcttgaatgtgctgctgagcgaaaaacaagttactcagtgatatatacagtgtaccacttagggcattaagaaaaccacaatattatagggtttcagtatagatatagatatactgtacatagacttcagtgaactggaaggatacagagttcatgacagtgattgggtgtcaaaatgcatgatgtggctgggtgcagtggctcacgcctgtaatcccagcactttgggaggctgatgcaggaggatcacttgaggccaggagatcgagaccagcctgggcaacatcacaagattcccatctctatttaaataaataaaatagaaaaaagagttcatgatggaggtggaaagggttggaggagcttggggatggggaaaaaatgaactgtataaaattataatttttttttttttaagaaagtaaagagggccaggcacagtggctgacgcctgtaatcccagcactttgggaggctgaggcgggcggatcacgaggtcaggagattgagaccatcctggctaacacggtgaaaccccgtctgtactaaaaatacacacacacacacaaattagccagacgtggtggcaggcgccaaaacgacgccccgtagacacgccgatccgatatcatcccccccgtggtggaattcccgattgcagtgaaccgagatcgcccagcagcccccccgcctgggcaacagagtgagactccatctcaaaaaaaaaaaaaaaaagaagaagaagaaagtaaagaaaatacagctcagcctttatttgtgttttttttttttttttccttttttttctgagacagagtttttcactctgttgcacaggctggagtgcggtggtgcgatctctgttcactgcaatctgcacttcttgaattcaagcaactctgtgcctcagccacccaagtagctgggattacagatgcgcgccaggctaatttttgtatgtttagtagtgacagtgtttcgccatattagccaggctggtctcgaactcctagtcccaagtgatctgcccacctcagcctttcaaactgttgggattacaggcgtgagccaccacagccggccatggctcagtgttaatggtcagttctgggtggtagagatgcagatgttaaaactttttttttctttaattcataacaaaatagaagcaaacctataaaggctattgtaggaagaccagtcatactaactagttcagtgctcttggagagttggcactgcctttcctcctttattgccccaactagaatgcagggcagcccttccattaaatgctgagccagtgcctcactttgctgaggccataacccaccttagttgcacttaagagtcctaaatcaggattcctggttctagagtgtggatatcatacccagaaacaccaccctacttttaatcctagtaaggaggcaccatgtcccaaggcagctaacgcttcccccaaaccacctccttcaggctgaaaccagttgtctgcaccgagcagctgggatagagccaggaaatactcggcatctgaggatactgagggttctctgacttaggacttcttcacctgaagttgagtggtcttttggggaagtaggcctgtttagcatcagctgctcttccctattccacactgtagctggaaataggaccttaggttcctgttgacaagtcatttacttttagccctgaagaaataaaagagccaagtgttttttatttttatttttatttttttttaaagcaagggaattttactagaacctgtaagtgggctcattttgttctgtgtagcttggtaacaccatactgctttctgctgtggggcctgctggggttaaagtgtgggcttcagacccaggtctcttagctagaagatatctcatcctctgtgtcctgcacccatatgcaaatatgctattgtcattatccttaactgtatatgaagacggacagtgcctactccagaccttactaggttctgctggcccatcacccattttgatcatgttgctggcctagtttgattagggcaaatcttagaaattccatttccattgttgaggaagagagctagagagcaggctgacccgaatgccagaatatcatgatgcaaactttctaatggatgctggtgttctgaagagttgagggttgaaaggccttcatgatggcttgaagatgtaggtagcaaactgacgtcacagcaaggaacgcaatcttgtgtacctactggcaacgttggagagagaaagtgagcatcaggtgccaccattttacagttgatctgtgtgaggctggtatcggagcataattggtacaaagtaaaaatgacttaggcagatgcagactcacgggccaggctggtttattagggcagaatgatttggtcctttgtgaaagaattggtggagtgaagcgtgaatctttcccagcgcaacccaacaacagttctggccctaagaagtggagcatgggagctgggtgtggttcgtgcctgtagtcccagctacttggggtgctgaggctggaggatcgttttgagggtgcagtgagctataatatataatgtaatataatataatataatcataccactgcactccagcctgagtgacagagtgaaagcctgtctcaaaaaaaaaaaggttggagtggggagtgttgggtattttttatgatttttgtctcctggtttctgacgaatggccgaaaaattgtgtctgacacaaaggaaactaatacaaagagccaggaactgtctgagatgagaaaggaaagggagaatagggcacctagagctgagctgtgattgtgcctgttccaacctgtaactccagactaaggcctcttagaggtggtgtctcctttctcacagaggagacatggctctgaggaagatcttactgcaggggctcgggctcaagaataaggctcctggacctgggcacggtgtgtgctgctatcagtggatacgccaggcttccactgctggctggaggttggctctgcatgtctgtgccttcctaggaggaggatgcagtagtgagtcagactggcatgggtggggccacatgtcctggcaggtactgtccgggcaactggcatgagggagaggagtctttcccagaagcctgccctgagaaaccaagactgggctgctttcctggcgccaagggagagtccagtgagtgttgtacatacaactctaggtaggtggttggtggtgtgggcagcttgtgctgggaagaggattttggagaaagcaggagagctctggccctccctgcaagggaggcttccggtcagagcctgaggaaagacctgagcttgaggtatggggtctctggctcgaagagagcattaaggatgcatgagatctgaagtctggatgaacttgctgacaggcaagcttttttttttgactgctagtgtgtaaatccactatagaaattttcatttgtcattcttgtacttattggccaaaaattagagcttataggcatcagatttaatttgagatagttgaaatagggtttgtgtttgaggccaatataattttatctgctaatggcatcttctggacttggaggcagcccttctgtaccagaacattgtcacaaagcttttactgtaaagcttgagaacagactagtttgctggatttgggcatgtaactaacagatttgaggcatgggattatcctatggacttttttttttttttttgctttgaggttctgactatattaaggttgaccactttaagccattgaaactctcctataatacatttgtgatgtagggcctaagacatgtttgtttggtttttttttttgagacatgtatctttgctgtcttttaaaagcagattattttttatttatttatttatttttttgagacggagtctcgctatgtcgcccagggtggagtgcagtggccggatctcagctcactgcaagctccgcctcccgggtttttacgccattctcctgcctcagcctcccgagtagccgggactacaggcgcccaccacctcgcccggctagttttttgtattttttagtagagacggggtttcaccgtgttagccaggatggtctcgaaccctgacctcgtgatccgcccgtatcggcctcccaaagtgctgggattacaggcttgagccaccgcgcccggccaaaaaagcagattattcttgaagtgcatagagcagcaaccgattaatggaattggtatcttcacatttcatttacttcctcccaacaattttataggatgcatataaatatttccaaaaaaggtgtacataatttcttactataaaagtatttttattttatatcagtaaatttgttaataaagaggaatttttgttgttgttgttgtaatcctaccaccccaatgacatcctattaaaatatcagtatatatcctcccaggtcttttaggtatgtttaatttggtgtcccttccccactcccaaaaggggagggaccaggttcttgtatagaatagtggaatgttagtaaatcacgtgtttaaagagacataacagctgaatctgtagagcagctgccacctggatacctggttattaaggtaatttttccattaccccaaagagctttagttacactcagcttttaccttaatccttgtacagctctccagggcacactttattcagctctgagcggtctttgcaagtgaggccaaggagccaacctgagccaaaaggagagcattatgtcaccggaagcccaagcccagagaaccaaaggtatgacctgatattcagtggccccagccaggtctttacaagaagaccctgatatctcaggtctaagaagagccagctgatggtttttaaaaagagtggaattagttactctgacccacttactcagatcttattttgttcacaatgtagtccccagattgtaggcccattggaggccacagcaaggcctttgtgttccaactggcctgctgtgccatctctcagtaatgttcccttaacagccagacttccctaagcccagctgggagctctgaaggtatgccagcccccccttaaccatgagtgtagggagagggaccagggcgccccaggctttcctgtcagtaatgtagaagtttctcagatttagggacgtgggagcagaggcataactttgattctgacaaagaggcattcagagagactgaaaggtcatttaacaaacactagaatgcttccacttactaggtgctaggaaatacaaaaccatataggtcctggaagagaggatacatagtagatattagaggcttaggaaatacagttgaaatgaagaatggatttgccacgttgaatagttagttggtatcttatttccccattttaaaagttttagaatctgtggttgaggacttgtggccatcagttttccatagccgacagactgttcactattgccttcagagctctttggaccttaataggccttctttggagatggcagagatgggtttagatgcatactctgctggagccacccagagagcccacaaagtcagggatggaacagggtaaaggagtaagggtcatatgtgtgagatgccttgatttggaactttgagatttaggaagagatggagaagggctaaagagggacttgtttctgagccttgcttggctgaagcatttaggctaaagcgttttagaaagagtagcccttggtgtgagaactcaaggaaacaactttctgatgagaaatgtagcaagcttctggttcacatccttacctgatagttcttcaaacactgcctggaagcttctcctgagcctttgtctctaatcagctaactaagaggctgagcgagtttagttgtaagtcattaatgaagaaagcaaaggtcggggccattgtcagggttgtgacctgggctagttaattacctggaactgatggtctgtgttacagagtggtggtatacttgtcaggcttagaaaagaaaacaggatgtgtatcaaaaatcttttggggaaaagatttgaccagcaactttaatttctctatgttgcagctatcctgttaatgtagttgtgataattttagaattataccagtgcccttatgttatccttgctttgcaaattgctttacgtgtcctaacgtccttctggccaacagtagatgtggttttaggtttagcctcctaggatggaagcttttgcattcaggggaatgactttgggttgggtgaggattgtaaagaggcaatgtgggtgccccacgacaaagcagctatttgtagctttgtgacaacttgacatacagatatctaggcttatctaggcactaagctaggagttagttgtttgtatcactggaagattggttataacttccttcgttggaagctccttcattgcatgttaaatgatgttatttatagatagggtggtgggaaagctgtctaagtagatgtcagcctagtgtaagagagacctgcttactgtgggtgcttgggactgtcagcagtaggtgggaggttttaacttgttcagtaaggtccatttccattgttcaccatcttgtgaaccctttgtctaacatgaggagcaaccacataaccacagcatgtctggcttccctgtggcttgtgtacaaagcgtgcttattgagttaatgtataagcaggagacaccctcctgtgataaatggtatattaaccacttctcagtcttaccactctgtttcaatttgtctggacccaggacctcagcagccatgtcgaagccccatagtgaagccgggactgccttcattcagacccagcagctgcatgcagccatggctgacacattcctggagcacatgtgccgcctggacattgactcaccacccatcacagcccggaacactggcatcatctgtaccattggtgagtgggtgtgccccttccccaaaaaaagggcttcatggaaagtgaccctttctctcctgaaaagacttaactaaatgtcctaacaaacctaggtgctacatgggatgctacacagattcttataaaaggactcaggtcataggaagttgcagtaacgaattagtatgtgcacaggatggcaaatacagttaataagagagtattagacatttcgaaattgctaagatggccaggtatggtggctcccagcactttgggaggccaaggtgggaggattgtctgaggctagaaatttgagaccagcctgagcaacttagaccctatctctccaaaaagtaaaaacaaaagaaaaaaaaaattagctgggcatggtggcatgcacctgtagttctgactacatgggaggctgagaaaaagatcacctgagtccaggagattgaagttgcagtgagtcatgatcacaccactgcactccagtctgggaaacagagcgagatcctgtcttaggaaaaaaaaaaaattgtctgggtgtggtggcacatgcctgtaatcccagcactttgggaggctgaggtgggcggatcacctgaggtcaggagaaccagcctggccaacatagtgaaatcccatctctactaaaaataaaaaaaaatagccgggcgtggtggcaggtgtctataatcccagctacttgggaggctgaggcaggagaatcgcttgaacctgggaggtagaggttgcagtgaaccgagacctgaccattgcactccagccttggcaacaagaatgaaactctgtctcaaaaaaaaagaaagaaaaaagaaaaaaacattgctaagagtaaatttcaaatgttctcaccacaaaaatgttaagtacttgaagtcatggatatgttaactaacctgatttaattattccacattgtatccaaactgtatgtattggattacataactttgtaacccaaattataaattaccagtttataataaaaaacaatttgttgcaaaaagaatccatatgctttaggttttacgctataggcaaaatttagagggtgttttccttagcaggtctttgtaggagcaacttacagacctaggaaagatctttttaatatgttctgtgcaaccaagattctgtggttggacatctggctgggtttcagtgagggcggagaaggctcgccaagtcttaacctaggcttttctgatacagtgggagcctgcagaatttgaaggaaatggtcgaagtgtcccagtaaatcaaaaaagtaagctggcacggtggtagccttccatacactttttaaagacttttgagctatttgggagaggaaaagttttcagggaaaaaaattctttaaacttaagcaaacttaaatgtttttccttctttgaataattaatacttgtggctttaaaacttttcctaataggcccagcttcccgatcagtggagacgttgaaggagatgattaagtctggaatgaatgtggctcgtctgaacttctctcatggaactcatgaggtgagctgtagctggaccctgtggccattgtgatggcctgtaggaaacagggagggggtgcagtgttcatttagccacaacagattaggcagggatgagtctgagtttcacagccagtgtgaagtttgtctttactagcccatccctactctccttccctcttgtcctggcgaagaaactggctaagtctcttttagcaaagaagaccccttttgtcactggccatgtttctctcacacacctctcctaccgttagctttcacaaaggaagatatggaaaggttctcctggaaaaccctctaagccttagatgtcctggccacagcgcttgactctcctgtccccaggtttctgctacagcctgtattgccatggtaaaccatctagcagatcgattctggcctatcttagaaccaaaataactgggcaggtccatgagaagagtttccattattctaagttttgaatgactgagcctaatgcacaagcactcgctggcgtataatacccctcttcctcagcactatattcccagcctgtaccttcccaggagttctgtacattaaaataacaccagttagcactcttcctcaggagcctagtaggactgtatttgtgatgggctctttattacctggctttacctatggacagaggccttgcccaggagccaggtagcagctgtcaggatggctccattcctgcttctgttgccagatttagaataaacccattctgaggagtttggggttccctgaggtaccatgacttatttatttttttattttataagacaaaattttgctctgtcatccaggctggactacagtggtatgatcatggctcactggatccttgacctcccaggttcatgtgatcctcttgcctcagcctcccaagtaactggtaatacaggcatccaccaccgtacctggctaatttaaaaaaaaaattttgtgtaaatgaggtctcactatattgcctaggctggtctcaaactcctgggctcaagtgattctctcaaatgttggaattagaggaatgagctactacccccagcctgggattgtgcctttttaaaaccttcagacttaaccatagatttcccatagatcatgggatttcgtaatggcattgataagaggaatcacagaagaggcagactttgtccctgtcttggcttctgtatttcctgttgagagtaaagaaaatgctaccctgtaaggccaagtgccttatagaggttgccctctggcatttggaagttgatattaagtttggactaaaaataaagcctcaggaaatgcagtccaagagtgaattcctccttttgggaaacttgagactcttcatcatagattccctaacctgtgttcataaacagcctatggcctggctagtggctggcccctaaatgtcatggggacctgaccaagtcctgcagacataccacgcaggttaagacatgtccctgtaccttttggaaaattctgtagttttccaaaagcaaggggtccttagcaggagtcaccgagaattactacaagtgttagcttagcttaaagagagagagctgaagacaatggtggaggtcagttcactgttgatccctgctgctgtagtctgccgtgggctcctgcgttcagggaaaggagcagaaatagatttttaagaagttgacctttaagtaggctttgtggttccttcatccagtaaaataacaccacatagctcttacatggcaagggggagtgatatctgctgcacctgctggatgagagctggctccgattttggttttttaaactttaagaggctttttggagattatctctgctttcactcctactcccagattataattaagattttttttaaattttttaatttattttttaaagatgtccctcttgtgggtttattttgaagttttagaccaagatgaggttgtctctgggctcaatttggaaactgatttgaagttattctaatttgtgtaatgtaacataaacagtttcaaccttaccgtttgtcagggctgttgtttcatatgcacctttgactaggggctgggatgtacttttctagttcctgactattttaaaggctcttctgagcagaacattgagattactgtcttccctctcactctgacagaggaacatcaaatgtctgcatctgatcttttaacagctttctttttttgagacagagtcttgctctgttgcccaggctggagtgccctggcacgatctcggctcaccacaacctctgcctcccaggttcaagcaattctcatgcttcagcctcctgcatagctgggattacagacctgtgccaccatgcccagctaatttttaaatatttttagtagagacagggtttcgccatgttggccaggctggtcttgaactcgtgacctcgggtgatccaactgcctcggcctcccgaagtgttgggattacaggcgtgagccacacgcccagctctcttttgacagctttggcaactagtcttcagccctcacttttggcagttcacatgggcaaggtgcattcttgctgaacatgtggttccatatgccgtgttttccagatttatttatttatttagagagagagtcttgctgtgtcacccaggctggagtgcaatggcacgatcttggctcatcttggctcactgcaacctccacctcctgggttcaagagattcttctgtctcagcctcctaagtagctgagattacaggcatctgctaccatgcccggctaatttttgtattttagtagagatggggtttcaccttgttggccaggctgatctcgaattcctgacctcaagtgatatgtctgccttggccttccaaagtgctgggattacaggtgtgagccactgtgcctggcctagaaaaaatgactttcaaacaacctaaatgtagagccttccacaggacagcattgatggatgaaactctttaccatgtaacatcccaacaaagccacagctatagtagaagactcagtacacctcccagaaatgctctaagagattataatatgtaacatagatttgaataatacacctaataattggtatgtttataatacatagttttacatccccaagaccaaaaatgcatgtttgtgtgaaacactcatggttacaaatatatattaggccaccaaaaaaaacccccaagtttcataaagtagaaattatacagacacattctctgctaaaaattttttaatggaaattaagaacaaagtcaagaaaactgaagtgtgcttactttagaaagcaaagatctcaaggtagatggaataaatatttaactcagaacactaggggaggaaaaccctaaaaagggtgaagaaaaataattttgtaagattatagctcaatgaaatgaaaataaatttgacaaattaagctaagagctgattatttgtgggtaaaaaatagtaaaatagaaagttctgggaagccaggtgaagaatgcaaggatgtacaaataagagtatgaatagaaaagggaatatttcctacacattggagattttaaaagtcaagaaagacttataacttaattcctatagagagagatgacactggctattttccaagaaaagattaaatgccaaaaagatagaaaatatgaatagaccagtggccataagaagttgaaaaagtgggctgggctcacacctgcaatcccagcactttgggaagccaaggaagagggatcacttgaggtcaggagttcgagaccagcctggccaacatggtgaaaccctgtctctactaaaaatacaaaactggcggggcatggtggcacatgcctgcagtcccagctactcaggagcctgaggcaggagaattgctagaacctggggaggtggaggctacagtgaactgagattgcaccactgcactccagccaaaaagttgaaaaagtggctaagatctggttcatctcagaacatttaagtccaaacgattttagtggctgaattgtctccccttcaaaattcagttacattgttaaactgttccagagcctagagaaatacagaaatcttcccactgtgttctttgaaaccaacatactctgatactgagatcagacaaggacagtaccaaaaccaggcaggtactaacagcgtgctagaccagtctcacttagatgcagaaaacaaataaaatttaataatccaaatccagtagtgattgaaaggaatgtcttgatccatgaccaagtagattttattctaggagcacaaaattctacattaagattaagtagagttaaggttgacttttttttttttttttttttttttttttttttgagacggagtcttgctctgtcacccaggctggagtgcagtggccggatctcagctcactgcaagctccgcctcccgggtttacgccattctcctgcctcagcctcccgagtagctgggactacaggcgcccgccacctcgcccggctatttttttgtattttttagtagagacggggtttcaccgtgttagccgggatcgtctctcgatctcctgacctcgtgatccgcccgtctcggcctcccaaagtgctgggattacaggcttgagccaccgcgcccggccgacttttttttttttttttaagacggagtctcactctgtcaaccaggctggaatgcagtggcacgatctcggctcactgcaagctgtgcctcccgggttcacaccattctctgcctcaggctcccgagtagctgggactacaggcacctgccaccaacgcctagctaattttgtttttgtatttttagtagagattgggtttcaccgtgttagccaggatggtctcgatctcctgaccttgtgatcccccctacctcggcctcccaaagtgctgggattacaggcgtgagccactgcgcccggcctgagttaaggatgacttttaaacaacctaaatgtagctaaatatagagccttctgcaggacagcattgatgggtggaactctttaccacatgataacatcccaacaaagccacagttatggtggaactcagtccacctgagtcttaccattataagatgataataataggtaacatttgttaaataattaccatgtactttgtcctaatacttaatgtattcctttactgctcacatcaactctgaaggaaaggtaccacatccccttaaaagaaaacaactatttctattctattcttttattttttttagagacagaatctcactctgtcacccaggctggagtgcagtggcacgatctaggctcactgcaacttctgcctcctaggttcaagtggttctcttgcctcagcctcccgagtagctgggtctacaggtgcatgccaccattcccagctaatttttgtattttaagtcaagatggggtttcaccatattggcctggatggtcttgatctcttgatgtcatgatccacctgccttggcctcccgaagtgttgggattataggcgtgagccaccgcacccagcctctattcaattctattttgttctatttctattacaagccagtaaggaagaaaatatcataatttataaggaaccctataaaaaacaaacaagccaacggtccctcattagggagtatgcctgaataagaagctgaagattttcagatacaggcttcaggcaacattgtctttagaggctaagctctggctccagctccctccagcatcctgtgaataacaggcaggcttacttgcaggtgccgctttcctggacagtggtggttaaaggacaaggcccagaaagtgctgaattaggtgcccttgttatcagcaatgtcatattgatcacgctgtcttagagctctttcgacatcttggctctgcatctttttttttttttttttttaaatcttttttcttgagatagggtgttgctttggatagtagggtatccaggccagagtgcagtggtatgatcatggctcactgtagccttgacctcctagacataagtgatcctcccacctcagcctcacaagtagctgggaccccatgcacccaccatcatgcacagttaatttttgtgttttttgtagagatggggtttcgccgtgttgcccaggctcatctcaaactcctgggcccaagctgtcctcccaccttagcctcccaaagtgtttggtttacaggcatgagccactgtgcttagcctgagtccctcttttaaacaaacaaaatggtaaatggaaaggaggaaaggcttaagaaaaaagattgaagcacagatttgttgcaagcaaggaataataaagggcagttcatttagagaaaggcatatgaccacctttccctgtctccagtcagaatctagaaagtgattgaggctgggcgcagtggctcacccctgtaatcccagcacttttgggaggccaaggtgggcggatcacgaggtcaggagatcgagaccatcctggataacatggtgaaacccagtccctactaaaaatccaaaaaattagccaggcctgctggtgggcgcctgcagtcccagactgaggcaggagaatggtgtgaacctgggaggcggagcttgcagtgagctgagattgtgccattgcactccagcctgggcggcacagtgagactgtattcccccaaaaaaaaagtgattgagaaaatcaggtctgtgtgaccttagcaatgagttgtttagcttgggccactgttagcttaagtcaataacttcaagtttgcgttgtagttggaatcaatagaggaaaagctctcagcattaccacatatatcagaatgtgacattgattgccagatcagccttatccaaacacaagttctaggctttttgccctgtttatcagctttatttgctgagggtatttgatgagtcttagggaaaaaagaacagccctgggaacacagctgcttttatgatgagacatgtttgcacccataccttaatgggttttggtggcaatattctgaaatttgccaccaacgtttcaaagatttgcccttagggtgaattactgctgtagtagaagtgggtggaggctgaggagattggattaagcaggtagaggagttctcagtgcatggatcgttctgaggatggagatagagctctaagacatccacaggcctttcctgagtgatcagctttggctcctgggcagggaaattgagctggatcctagtgtgggagcacgcttgtcatcttccttctttttccccagtaccacgcggagaccatcaagaatgtgcgcacagccacggaaagctttgcttctgaccccatcctctaccggcccgttgctgtggctctggacactaaaggacctgagatccgaactgggctcatcaagggcgtgagtattctgtggagagcgagggaaagactcagtaggcaatatgccccagagacatgtcctccaaagcgttgagatgccgtgtttcatcccagcactatgaaggactgcagaggagttgaggtctacaaatgagggtttattcatcactgtaaacaacgttgatttgatttactttgctaggaaatggtaccacagaggaaccctttttttaccctaaaaacctaaactttaggctttctaacttggggaaccatctctttgtatctttttccccatcattaagtagcataactgaaacattatattctattttcttagattatttctgtgaagtgtactgagttagagaataagagcaaaaaactgtattatttttagcggtgacttgagcattgttccctggaggaaagagcttttccattgcttctgcggtgatgctgctactggtgtctccagtttggactctggcttactctcttgcttactccctagagcggcactgcagaggtggagctgaagaagggagccactctcaaaatcacgctggataacgcctacatggaaaagtgtgacgagaacatcctatggctggactacaagaacatctgcaaggtggtggaagtgggcagcaagatctacgtggatgatgggcttatttctctccaggtgaagcagaaaggtacgtatgggagctggaatccaattgtctaaaacccatcttttgtctctaaagttccttgacacaaggaagatgggaaggttggttgcctggcagtgagattgagtctgtgtgttctcaggaatcccttttataactcatttatcctcaaagacaggctttaatccagcatagttacattcttctggttccggagaacataggaacatatatatatacacacatatatttcttttttgagacagagtctcgctctgttgcccaggctggagtgcagtggcacgatcttggctcactgcaacctctgcccccagggttctagcgattctcctacctcagcctcctgagtagctgggtttacaggcacccgccaccacgcctggctagtttttttgtatttttagtagagacggggtttcaccatgttggccaggctggtctcaaactcctgacctcaagtgatctgcctgccttggcctcccaaagtcaaaacaatcttaattctccttttttatgggtgtggaaagtgaggtacagagaggttaaatggcttgcctaggattacacagttagttgtagtagggtttcaactctggtaaaacagctccagcacccatgatgcaccacttcccagctcactgtgcttgggggaaaggtgcctgcttcctgttgagctgtgccctcggtgctctgcctcccctgcttaccccttttcaaaacacaggtgctgacttcctggtgacggaggtggaaaatggtggctccttgggcagcaagaagggtgtgaaccttcctggggctgctgtggacttgcctgctgtgtcggaaaaggacatccaggatctgaagtttggggtcgagcaggatgtcgatatggtgtttgcgtcgttcatccgcaaggcagctgatgtccatgaagttaggaaggtcctgggagagaagggaaagaacatcaagataatcagcaaaatcgagaatcatgagggggttcggaggcaagtccccattgtccctgctccagtcccagcgcagctctctaaagggcatggtgcatcctgtgaatatctgattcccatcagaatgtagactcccaaacctgttccaaacctgctgaatcacaatatcttagtagagtagaaggcattgtgtgtgtgtgggttttgtttttttgttttgttttgttttgtttttaaaaagcttcctaggtaattgagatgctggcagcttgacattgttccctgggcctggggaccaacatttgagagaacagggtcactgctcatagtaccaggggccatgatgctctgttcctgatcagaaacactaccagtgtttgctggaatgtggggaccgggggaaagatgacagcagacacttaagaaggggctcgttttggcccttcctggggagccatgtggaatttcaggggctggtgtccatgctaaaacatatggcctcctggtcttcacttagaacgcagctggctcagtgatcatgctaactctggtatggtccattccactctcagagtaagatgtgtggttcttctccggggtcagattgcctcaacttagcttaccccctccacagtgctcatgaggtggagcccagtgggcatggccaccatttttggcatcctgctaggaatacaacttagcactactaagatgctagacctacgcttgtggattaggagtgtgtttggggagggtgggggaacaaccctctgcacccactgtagtggccttactgtcttagctttgtgtagataccctctgtaccaggcaatttggggccctcccctttgccatcctgataagctgaacttggcgctaggccaggcaaagccacattccctcttgccttcagcaggttggagtgggccacctcacagggcagtcttcaagtgtccttgactagataaggccatggggctttgtggtggaagcagtcagcaggccttgggttccctgtcttgaagtgctgattggagaatggaggccctagagagacacctaacatgcatgggatttggagaggagaccttgggaatgagcccatttggatttgccctctcccctttcttctgtcaatgaagcatccatattggtgttgaagcccagcaggcagaattgttggcccgctctgggggactaaggtagctggactgccttgccatctgtgtgcatccatgatgatgtcatggatgtctgtcctggtatgaggacatctaagttagggaatcccagggaaacttcttgtctaccggcatacttgtggcccctgtctgtataacctctctccccccaactttgtccatcaggtttgatgaaatcctggaggccagtgatgggatcatggtggctcgtggtgatctaggcattgagattcctgcggagaaggtcttccttgctcagaagatgatgattgggcggtgcaaccgagctgggaagcctgtcatctgtgctactcaggcatgtgaccacccctccccacattctcctgggcacactcacatgtgtgtatgggaaagctctggaggctgtctgatcttttcccatggaattgtcccatgtaacacacagataatccccttcccccatgcacctacacaaagccatgctctgtgcacctactcactatccagaggatcagcgtgctgtcatttgtctctgaaaacagcccaagccacatctcactaatgctctgttcctcccagatgctggagagcatgatcaagaagccccgccccacccgggctgaaggcagtgatgtggccaatgcagttctggatggagccgactgcatcatgctgtctggagaaacagccaaaggggactatcctctggaggctgtgcgcatgcagcacctggtgagttctggggcctgccccatcccctgggctgtggactgggcctgggttggatgcaagctgtggtgcagagctttttaggtttccatatcctcttaggcacagccgttcattatcctccaagttacagcagcaagagggtgggggtggaggtggaggtggctttttttttttttttttttaattctgtttttcattcctgccgacacccccacccctccatttccttctgctctggaagcatcctccttcactggacaccatacagttcatttcacttctgacttcaaggtggtgaatccttcccatggcttaagtcctgggatacttctgcagtgaagggaggtcttgtacctcttcctcagagtcagaagttttgagtacctttgccctattctgaaaagggctcggggctcctgctcccaactgccctcttcctttggcttccaattcagtcccccgacccccacatcccgcagacaggcgctcccccagggagcccctgtggacctgcactggagtctgttgcctgcactgagctgcctgtgctggccttgcatggtgcctataggaggatttgctttgctgtgccattggggtacagctgctgctcttacaacagaccaaaaagtcaggttgagtgactggtggcagggccacagatagagacagcagggaggggggctgaccctggtggccctggactgagcgtctggaggagtcgtggaggctctttcccttctttctcctctgagagctccttcttcaggctcttccagcttgtcatgttgagtgcctggccactgctcagggttggagactcagtccctttgccctgtctgttccagctctggagctaacttggggatccctgatcagggttacataggtttggtaaaatgagtgctggaaattaactttctcccagtagtcttaggtcaggctcagtgaacttcaactttacccagatatggtttttcttcagccattctattccctttctagccagtgaaagacccgctgccctttgacctcagcccctccaagcccccaagtttaaaacgccaccccccgccaccaaaaaaaaaaaacaactaaaacacccacctcgtctgggcatcttcctttcctttttcactatgtgtcctgttactgggcttaaacagctttcagagaagagatgtcatttctattaaatgctctttcagtagcgaactgagttcagacttgactaaggatattttctgggctgtcatcagcatccttagtgggtttccccatattggaattggtagaggccggggacggtggctcacacctgtaatctcagtactttgggaggccaaggtaggcggatcgcttgagctcagaagaccagcctaggcaacatggtgaaaccctatctctactaaaaattcaaaagttagctagctgggcgtggtgatacacttctgtagtcccagctacttggagagggggtggtgctggggcagcaggatcactgaacccaggaggttgaggttgcagtgagccaagatggtaccagcctaggtgacaaagtgacaccctctctcaaaaaagaaaccaaacaatcataaaaaaaggaaacacaaaaaatcagtagagagtgatttctctcccaggcccacttaacgtagcctgggcctggctgacacctcaccgtttgtgcgatgtgattgctgttctgatgctgagatcctcttggcgcagtctcacaattgctccatggtaggaaggtgtcccagagacagtgcaccttcaaccagtcaccactaaagtgactgcctttctgggtctctccacacgtcccctctgtctaattcccttacttaattgtgtaacttcatggcctcaaaggtgggacagaggctgatcttgacttagatttactgaaccatgaaatcactgcatagaatgtggagacttgaatgtgtcttttggcaagtcatttaacttctcaagaccttatctgtaaaatggattagatatgtttaattatagccttagcattaaatattcattgctcttattattaagtgtctgataagtctctgtgtatatggatgtaatcttcctaactcccattacctccatttatagccgagggttatatggccaataaagcctgggtttgaatctaggtctgctgactccaaagccagtcttctctcctgcaacatcatgctcttaggtctagcaggagatgagaacaggtctccatttggagcctgtcagtggggtcggagactaagaatcaggctcagcttctaaatttcatgtcctttcctccataccctagtgtttcctatgaacagacagataccttagagctgcaaggcttggattgcatggcagtgctcagaagataagttacaggtctgggccaggctgtagctgcccctccaggtggctagacctttcctttctgtgtcaccagttaacactggccaacagttccttcccttcactgttgattgctttctctgtgtctaactgatgcagttaatgacgcataactaagagcagtagcaggtatggctctgtttcgtgttcctgttccctgtcctctgggttgcatgcattccattctgataaaaagaatacctttaacctagtacatcctgccacacatctgcttctactgtgaaattcatgaggggctattaccgattcctccctcacccatcatttacttagatgctggtgattgcattataatcctctaaagcttacattgtctttctgattcttggtcttatctgagcaagtgatctgtaaataacccagtggctttctcatgactgttttaatcattagattttaatcaagtgtcttattaaacatatctgcatgcttccacagacatctgtctcttcacatggctgttcagtgtgtctctcacgagttagcccaagttttctgttctcctgcttcaaactcagttgagctgccttgctttggcttggatcccagctttccagcgctgctcaatctgtttccatggcaggccattggaaaggctcagtgcatccctgtgcctgaagccaagtgagcgctcactgcgtgcatgcatggaggctgggcaggagtctgcctaaccagacagccatgtgaggagggagggcctgttcctttctgtaagctatgtcgtgaggcagcgtgatcaagtcctctgccagggagtggtgtgggcccagcctgggcatgttttcatgccagagtgctagagcctactgccagattgtctccctccatccccaatcaaatccttccagaacggaagagccaatttcccctgtgttggaggggaagtggcagcacctcctgaagcagttggactttcatcaccctacctccgcatctgcctgaaggacagatttagccaattaacctaaggttaccttcctctctgattaattccccattctgtcttcccatgtgttgtgtcttgtttttttcctcctccttccctcttccttttcccctcttcccctaaaccttacagatagctcgtgaggctgaggcagccatgttccaccgcaagctgtttgaagaacttgtgcgagcctcaagtcactccacagacctcatggaagccatggccatgggcagcgtggaggcttcttataagtgtttagcagcagctttgatagttctgacggagtctggcaggtagggccctaagggcaggtaacactgctaggataaccagcctcttgcttcagctgttccaggagaagacagccaggcccaacctggcacctgggcacagagcctcttcttgtctataggaacaccgccagggaggtcatggcagggcaggaccaaagggtcctgtggctcagtaggcacagcagatgtcacaggcacttggtgaaggactggtttctgtggagtcttgaaattggctcagctcagcatctccagtgactgggctactcttggcctttgtccctaggaacatgttcctcaccagctgtccgggtgactcttcccctccctctccttctgtgacaaagctctgacaaagctctgtccccctctcgtccctctggacggatgttgctcccctagattgcccgtgaggcagaggccgccatctaccacttgcaattatttgaggaactccgccgcctggcgcccattaccagcgaccccacagaagccaccgccgtgggtgccgtggaggcctccttcaagtgctgcagtggggccataatcgtcctcaccaagtctggcaggtaggaggtggcagcggctccctgggatgccccgctcagtggcacctctccttgggggtcctgggagcagtgcattgaacaatgctcaggtggcactgagccaaggtaagacccctctgcctgccaccttgggcctgcagagaaggattgagcagagccccttccctgggcccagaggactctaggcagcacacataaggaatgtcagaacatttggatcaaaagcaagtttatgctggagatttattacataatagtgcacaggctgactacaaatggttatttgatattgaaaatttagtagccaggcgctgtggctcactcctgtaggccgggcgcggtgacttgtgcctgtaatcccagcattttgggaggccgaggtgggcggatcacgaggtcaggagattgagaccatcctggctaacacggtgaaaccccatctctactaacaatacaaaaaattagctgggcatggcggcgggcgcctgtagtcccagctactctggaggctgaggcaggagaatggcgtgaacccaggaggtggagcttgcagtgagccgagatcgcaccactgcactccagcctgggcgacagagtgagattccgtctcaaaaaaaaaaaaaaaaatttagtcctctaaaatagtaaaagataaccacttttgcttattccagttactatgtgctctttaaaaatttcagttgggaaaatgaatttatttaaatgctgtttactgtgcctccatttggcgcactagtccctgctgttttcgagccctaaagacaaattggtttccagctcaggagaggttgctgtgctatcttggctgacattctgtggggccaggcagccaggctgaggactgtgtggcctatgctgagcctccaacttgggatcccttccttagcccaggacattgagttaatgtccttcactctcctagttagggattatgctccttgtccctgcccacagggcagcgagggtttcctggagaagagcaaacaggcagtgcccatgcactgaggagcagcaggtgggcatgggcagcccagagaaccaggacacaagctctgtgcagatgccctcagcagagggctgcagcctcccactcttggctgaacagcttcaaccagtagggttgacctttcttaaaaggtccagttcttgctgtttggctattttaagctctagtcttctggggtttcactcagctggtcctagcttcagcagttgcttccctctgatggccttgcatataggccaagcgtgaagtgcagggacttctctgctatgatatggcttaagtttccctgacacctgttgagtgtcctcataacttcccttctggtgcccctccccagctcctgagacacagctgcacctacaagtgtgcagtgtcagtgttcaagaaagcgcctggcacaggggcttcagaagggtcccctgccttccaaaggagctttggcaggcagagctgctcctgcaccaacactcccatttcctgttcttgcctgctgagtagcacttagatttctaagcctcacctagatactcagatttgactctgggcctttatagcccagttgctggactgtttcaggagccaggggccatgtgggacagggaagagggcacaaaagtagagaagcctgatgttgattcccatggggctggtcagctctgctactgctctacatgctacttggcttgtaggtgtcaccggcagcgagaggaatgggtgctggtgacactgggccagggctgcctgtctgtgtcagagtgtaggaggggttctgccaaccatgggctgtgtgagataagtgggtgaggctgaccttgggtcaagataatcctgggtcaggataatcctgggcccttggcctgtggagtgggggtagagggcagatggtagcctagcctgctatggaggatataggatgaggggctgccctagccttgggaggggtcctagggagcagatgttgaagaggccagagccatcagtgagctgggtgagaggatgagctgtttgaataccctgaggtacttcctggggccttgtgtgatggtctcttctgtatgtcccccatcccatctcaggtctgctcatcaggtggccagataccgcccacgtgcccccatcattgctgtgacccggaatccccagacagctcgtcaggcccacctgtaccgtggcatcttccctgtgctgtgcaaggacccagtccaggaggcctgggctgaggacgtggacctccgggtgaactttgccatgaatgttggtacgtggctggagcaggggctagagcctagaggggtttggggatgcttgagcattggcttctgtgggaccctgaaagtttggggaatagaaagggaaacatagaggggcaaaaggcccagctgactgttctctccctcattgggaatgttctttctgaatctgtcattcccggaagtcctaagctgagcccaggagagaaaagggtcctttgagttgtagggttgagcagttcctttcctcttctcttctagtctgggactcaaagcacaattgtccattctttggcatctgctcattactgagggttttgtttttgtttttgttttttaaataaaattggctacagctcctgtgctgtggggtggcatacacagattatgtactgatgtggccattgtccctgtataaggtagggtatcaccagatgacaggaagcagctagctcttgaccctgggcaaggctttgcaccctctggaggatgaagtgaaagatgtccaaaggtccctgccaaccctgccaaccctgccatctgagtgataaggacatttcagggcctccctcctgtttgcctgggctgtaagtttggtgccaccttgtggtgtgaggaagtagtggtcagccagcctagttcagtgctcaggctatggggcagctgcccaggtgcacacctgcctggcttggcttttacttaccaatctcccttctcttcctccaggcaaggcccgaggcttcttcaagaagggagatgtggtcattgtgctgaccggatggcgccctggctccggcttcaccaacaccatgcgtgttgttcctgtgccgtgatgaacctgagagcccttcctccagcccctgtcccacccccttcccccaacccatccattaggccagcaacgcttgtagaactcactctgggctgtaatgtggcactggtgggctgggacaccagggaagaagattagtgcctcgctgaaacatggctgtgtttgcagcctgctctagtgcgacagcccagagcctggctgcccatcatgtggccccacccaatcaagggaagaaggaggaatgctggactggaggcccctggagccagatggcaagagggtgacagctttctttcctgtgtatactccgtccagttccttgagaaaaaatggatgcccagaggactcccaaccctggcctggggtcaggaaacagctagagagttaggggccttagggcaaggggctgttgtccccttgaagctgactctggccctggcccttacttgcttccccagccccctgggcctccccagttcgcacctgtccccgccctccactcagctgtcctgcagcaaacactccaccctccaccctccaccttccattttcccccactactgcagcgactactgcagcgcctccaggcctgttgctatagagcctacctgtatgtcaataaacaacagctgaagcacc

SEQ ID NO: 47 - DNA, 31207 bp, Chlorocebus sabaeus
  modified_base (30235)..(30244): a, c, t, g, unknown or other
atgaaggcctgtgattcagctgcaggcagcgggtaagcctgagcaggtcacactcatttggtctcttttgccaggaaaagaaaaaagaacctaagagaacggtcttcgcattttgaatgcgcaacattgtatctgtgaatgaaggcaagagttaacagctgtttaattgataactgctcacatcattggttgctggctaacaattgggaaatcggaaaatgtcttgtagaaaaatgtaagaaaagttccaacaatattgatttaaattcataacaagggtgaaaacagaaatgctgactcctgcataggttatcggctctaatgttctgacttgatatttccagatgccgagctctgcgctaatatcaacaccgtctatttgctttttactctcaggcattcgctctgcaggattccagaccctactaaattattcacatggccccaacctgtccttccttgttccgcggttctaagacaacaaatggtcctaagaggaaaagggcctcgcgctcccgctccaggttcacgtcgcagtccctagttctccctactgccgctccagtgccagagcccctccgaaggcggtcgggacctccaaccacgcacaagtctgcagctctcctcaacttcccgttcagctcagtctccgagggtgcgccagggcagacacccagaggagtggagagtggcagggcggggccgggagaatgctgccccggaacccataaatctgggccctgcccaggtaggccgggacagttggggtggcctgggccgagagccaagaaaagagaccccatccggcagcccaacttggcggcaacaggtggcccggcgcccgggggtctaggagggaagtcgctctaggggcgggctccgctgccccgccgcgttcccattggccgtcaggtttcttaaactgtgactctgaatctgtgtccttccgccgcagaatttagttcccccgaaagggcaacctgcccgcgcgttccgccgccgccaccgcgcttcctcctgaaggtgactgcgcccgcgaagacgcagggggcggggtccgggtcgccgggagccgggattggacagagggcggggcggcggagggattgcggcggcccgcagcgggataaccttgaggctgaggcccctgctactcgcactgcagctgcacgtccctgggatccacatctcttccagtttgcagcgtagcccgagtcggtcagcgccggaggtgagcggtgcaagaggctgcgccatctgtcctcaccaagggcccgtgcacccggctagtgcggaatcccggcgtgccggcgggcccgcgcaggatccggggcgtctgggacgcggtggagctcagagacgggagaatggctcctcagaagtccccagcgccgttccttccagatcaggcgggtccgccggctcctttcccgtcccagccctaccccctcattctggtcccatcctcctgccccagtcctcaatgcgcctccatccttgcctgccttctctcggtccttcgtgattgattccacccttgcctcccctttctccgcgccctctgctccgtgctcgtttgttccacttcctcaagtcctgtccttccacccactcctcttaaacctgtgcgtgccccttcattctattggcttccgtgtaacttactgaaactccgttcttgttcccctcccaggtccatcctccattcatgcgcgaccgcccttcccgcgccccagtcccctcttgtcgcccctccccctgcttgctggtcacgtccgctctcccgcatccccctcctcgcctggcatgtcgcctccctccctctctgctctggtcgcgcccgcccacttgctccggtctccgagcgcggtcccgcgccccttttccatcaccgcctcccagctcccagcaggttcgggcggtgctggggccccgtgtccggggcgggcgggcggagggctgggctgggtgccccgcgcggcgggcgggatgcggcggcccgggagcagctggaggcttacgtaacgttggcctgccccgctgccgggaggcagggcggctgcccctgcggcgcggtgctgtcccatgcgaccgggattagatgggtggcccgcgagggcctgggaatggctcgggacccgcgagctcacccggcccttgccgggtggccaccagggaccacgctccatctcgccgcggccgggctgcacgtagcggccgcgcccagggtccaccccgcttcaccgggcggtggccttgggccgcgtaacgggccgtggaaacgtctgcaggcttcgctggggcctgccggccctcgcccgctccgcgcctctccggcacgtttttttttttttcttttcgttttttctttttttttttttattatccagcacgtttttttaacaaatgcgccctgattgtggaacgcggaggccgcggggtggggtgggggtgggctctggttacggagggggcaggaaatctgtggcgttcactcaacgcaaacggtgtgggtcaagggctgtttgggggtcggagttagagaccagaatgactggacgagtcatagcccaccgagctcacaatcttaaaatgtataccccgtaatgctgggagtggggcacgagcttcctgctgtgggagggagggggacaggaagcctcgtaaggtctcaccaggtggcaagcacactggattagaagatgcaggaaagcaccttccagtctgaaggtcatttaaagactagtcaaggaaaggcatccctgggcttcttaatctgcatactccagacccagggcttggacctttgctggtacgggttaaagtgaggcctacagtgaaggtccacgtggagagagacatcgggaagttgtcagaaaggcttttagaatcaggtttgactcattaatttcctgagactgattgaaggagttcagctgctacacctcagtttcccctgggaaaactgggagtaacattttcctcatgatggttgaaagggttcatgcctacgtggatgttgcacactcagttaagtgtctaatctctggcgaaatacccagaagaaaagcctgtgaatgaatatattattttcgagcacaattacttagtccagaattgagcataagggccttgattcattatcttactgctgtctgcaaacgcctgcagctaatcgtggggaatcaggctctctaaccacgtgtctcctggaaaccagtccccccagggatctggtttaatattgacaaagtcactgatgatgtaactttccaactctctgcttggagcagatgctctttgatcatctgagattgggacctctagaggggctgagttaagccttcggtgttcccctgtaagtggaatacctcttaacaggggaacattccagcccttgatttgctctgcctgctggtgagattaggattggagcctggatcagtaacccccagttggccatcttgagggcgtggctactcccgaggccacagaggagataaaggtcaggactccctggctgcagcattgttagcaaataatttgccctttggtggcctgaggtgctgtgggggcaggagtgggctgtcttgtggggaagggaaatgtaacgcatcaccaaatctgtgggggagtggggctctgtggggaagatgactcaacctgtcaattattctgcttttgagagaattatcttcgctgggtgagtggggaaactacgtagtggttcttgcaggcttaaaaagtcccttctcccctttcagtgagtcaaataatgaagcatgcatttcccctaattaaaaatgcctcagcttcggagcttgcggtgagccgagatcgcgccactgcactccagcctgggcgacagagctaggttccgtctcaaaaaaaaaaaaaaaagtgcctcaactaagtgaaaaatgattggttcgggtcacctggttctctgtactgccttaagaacttaggtgcagagtggcagagcccggtgcccagctaatgcagtctgtgcagcttcattcctggcccttttgtagcgggcacagcagcctctcctgggacatgattaatgatgacttaaagaaagttcttttttttttttttttttgagatggagtctcgctctgtcgcccgggcgggagtgcagtggccagatctcggctcactgcaagctccgcctcccggattcaagcgattctcctgcctcagcctcccgtgtagctgggactacaggcgcccgccactttgcccggctatttttttgtattttttagtagagacggggtttcaccgtgttagccaggatggtcttgatctcctgacctcgtgatccgcccgtctcggcctcccaaagtgctgggattacaggcttgagccaccgcgcccggccttaaagaaagttcttgaactcatttctcagttactgacttgagccaaaatgtatggatgttggtctcctgtctagcacagctgctttcattgtaagcattgcgttagaaataatgtattcatattttagcaaagagcatcattagctctttaagaactgtacccccagtgacttagcaaatttggttgctgtgactctaaacagctagcactttatggtagttgcttctgtgccttgaatgttgtgacactgatgtggggtcacaggaaaaaccattttatttcttaaagctgtttcttaatattgaagcaatggaagaaatgaggaaatggccatgggcaggaagatagaaaaaaatgcagcacttacattacaaactcactttacttgggttttagtttattttaaagcttcagggtttttttgttttgtttttgtttttttttttttttttgagacagttttgctgttgttactcagtctggagtgcaatggtacgatcttggctcactgcaacctccgcctcctgggttcaagcgattctcctgcctcaacctcctgaagtagctggaattacaggcacctgccaccacgcccagctaatatttttgtatttttagtagagatggggtttcaccatgttggccaggctggtcttgaactcctgacttaggtgatccactggcctgagcctcccaaagtgctgggattaccggcatgagccaccacgcctggcctgcttcagcttttatgaaggcaaatccggatgtgttatcttggccaagagctaagactgagaccagagtacaggaaaatgactcatttgacattacccttctttctgaatcactccaaaagcccacagtcaaatcccaatttaactggtataccacaagaatgcgttgcccctgtgagcagagttttattgcaacttcgagggtctttgtgagattggtttatttggtatgaggtcttaaggattttaagttgtccctttaagcatcagttctgatacagatgggaatagaactagacaaccagatatatgaagaccatttgtgataccaccttacttttggggagcttgcattttttttaccaaggggcagactgaataattgagtaatttgaatacttggggcattgttaaagaagctgttgggggaaggtgagcctgggtgagtggtggagggtggcgtgcagcatctgctgggctttccggcctcttggtatgactgctcagctcaggagttgggggctttagggcccccaccacccagtgtggcgaagccccgcccctgcagtggtttgtgcttgtctgcacgtagaagggagcaagcccgctgcagtaccttcggtggcctctgagactcacctcccccacttctgtccatagacaaagctcctggggagctctaagcctctttcctcatgccagcaagcagtcttggaagcaggctggggctgtggtgggagagatgccaagaccagttattcaagggcagtgaggttgccagtcctagcatttcagactgtggaccagcacagctgccggctgaacactgcagtcaagattctctgaagggagtcctatcccttccaaacatcttcagtttacttacagataatgtttcttcatattttattttatttttttgagatagagtcttgcactgtaacccagggtagagtgcagtggcacgatctcagctcactgcaagctctgcctcccgggttcacgccattctcctgcctcagcctcctgagtagctgggactataggcgcccaccaccatgccaggctaatttttttgtattttttagtagagacagggtttcaccatgttagccaggatggtctcggtctgctgaccttgtgatccgcctgtcttggcctcccaaagtgctgggattacaggcttgagccaccgtatccggccttgtttcttcagttttaaacaactgatatctcccttggcaatgaatgaaaaagaactactcatcggtggaatcagtcagggcacataagacccactgtgtccaccatgccatttcaggggagattcgattgagttaagcagggaaatagagatgtcgtaaacgttgaaactatctcggtatccctctttggttattaacattagatgagcagaaaaacaaatgtcacccatcagatgggcaaacatttaaaaagtctggcagtaccaagtgtggaaaaaggtgtgcaatgcagcaactcaacgttgactgatgcagccactttggagagcaattcagccatatttagtaaaaatagaaataaacataccccatgacctaagacttcaatttctggatatatagaaactcatacagtacagggagacatgtactacaagagtagagtgttgattaatgaggaaaactagtttaatggggagggggagtggctaccagtaagggagtccataaataaaattgtctgttgtacagtggactagtgtaacagttcaaatgaattagctagatccatatacccactggatggatcttgaatgtgctgctgagtgaaaaacaagttactcagtgatatatacagtgtaccacttagggcattaagaaaaccacaatatttatagggtttcagtatagatatagatacactgtacatagacttaagtgaactggaaggatacggagttcatgacagtgattgggtgtcaaaatgcatgatgtggctgggtgcagtggctcacgcctgtaatcccagcactttgggaggctgatgcaggaggatcacttgaggccaggagatcgagaccagcctgggcaacatcacaagattcccatctctatttaaataaataaaatagaaaaaaaagttcatgatggaggtggaaagggttggaggagcttggggatggagaaaaaatgaactgtataaaaatataattttttttatttttagaaagtaaagagggccaggcgcagtggctgacgcctgtaatcccagcactttgggaggctgaggcgggcagatcacgaggtcaggagattgagaccatcctggctaacacggtgaaactccgtctttactaaaaatacacacatacacacaaaaattagccaggcatggtggcaggcacctgtagttccagctacttgagaggctgaggcaggagaatggcatgaacctgggaggtggagcttgcagcgagctgaggtcatgccactgcactccagcctgggcaacagagtgagactccatctcaacaacaacaacaaaaaggagcagaagaaagtaaagaaaatacagctcagcctttattatttgtgggttttttttttttccttttttttctgagacagagtttttcactctgttgcacaggctggagtgcggtggtgcgatctctgttcactgcaatctgcacttcttggattcaagcaactctgtgcctcagccacccaagtagctgggattacaggtgcgcgccaggctaatttttttatgtttagtagtgacagtgttttgccatattagccaggctggtctcgaactcctagtcccaagtgatctgcccacctcagcctttcaaactgttgggattacaggcgtgagccaccacagccggccatggcttagtgttaatggtcagttctgggtggtagagatgcagatgttaaaacttttttttttctttaattcataacaaaatagaaggaaacctataaaggctattgtaggaagaccagtcatactaactagttcagtgctcttggagagttggcactgcctttcctcctttattgccccaactagaatgcaggacagcccttccattaaatgctgagccagtgcctcactttgctgaggccataacccaccttagttgcacttaaggggaccctaaatcaggattcctggttctagagtgtggatatcatacccagaaacaccaccctacttttaatcctagtaaggaggcaccatgtcccaaggcaactaacgcttcccccaaaccacctccttcaggctgaaaccagttgtctgcactgagcagctgggatagagccaggaaatactcggcatctgaggatactgagggttctctgacttaggacttcttcacctgaagttgagtggtcttttggggaagtaggcccatttagcatcagctgctcttccctattccacactgtagctggaaataggaccttaggttcctgttgacaagtcatttacttttagccctgaagaaataaaagagccaagtgtttttgtttgtttgtttgtttgttttttaaagcaagggaattttactagaacctgtaagtgggctcattttgttctgtgtagcttggtaacaccatactgctttctgctttggggcctgctggggttaaagtgtgggcttcagacccaggtctcttagctagaagatatctcatcctctgtatcctgcacccatatgcaaatatgctattgtcattacccttaactgtatatgaagacagacagtgcctaccccagaccttactaggttctgctggcccatcacccattttgatcatgttgctggcctagtttgattagggcaaatcttagaaattccatttccgttgttgaggaagacagctagagagcaggctgacccgaatgccagaatatcatgatgcaaactttctaatggatgctggtgttctaaagagttgaggattgaaaggccttcatgatggcttgaagatgtaggtagcaaactgatgtcacagcaaggaacgcaatcttgtgtacttactggcaacgttggagagagaaagtgagcatcaggtgccactattttacagttgatctgtgtgaggttggtatcggagcataattggtacaaagtaaaaatgacttaggcagatgcagactcacgggccaggctggtttattagggcagaatgatttggtcctttgtgaaagaattggtggagtgaagcgtgaatctttcccagcgcaacccaacaacagtcctggccctaagaagtggagcatgggagctgggtgtggttcatgcctgtagtcccagctacttgggatgctgaggctggaggatcatttgagggtgcagtgagctataaaatatactatactatactatactatactatactatactatactataatcataccactgcactccagcctgggtgacagagtgaaagcctgtctcaaaaaaaaaaaaggttggagtggggagtgttgggtattttttatgatttttgtctcctagtttctgaagaatggccgaaaaattgtgtctgatacaaaggaaactaatacaaagagccaggagctgtctgagatgagaaaggaaagggagaatagggcacctggagctgagctgtgattgtgcctgttccaacctgtaactccagactaaggcctcttagagatggtgtctcctttctcacagaggagacatggctctgaggaagatcttactgcaggggctcgggctcaagaataaggctcctggacctgggcacggtgtgtgctgctatcagtggatacgccaggcttccactgctggctggaggttggctctgcatgtctgtgccttcctaggaggaggatgcaatagtgagtcagactggcatgggtggggccacatgtcctggcaggcactgtccgggcaactggcatgagggagaggagtctttcccagaagcccgccctgagaaaccaagactgggctgctttcctggatccaagggagagtccagtgagtgttttacatacaactctaggtaggtggttggtgggatgggcagcttgtgctgggaagaggattttggagagagcaggggagctctggccctccctgcaagggaggcttcaggtcagagcctgaggaaagacctgagcttgaggtatggggtctctggctcaaagagagcattaaggatgcatgagatctgaagtctggatgaacttgctgacaggcaagcttttttttttgactgctagtgtgtaaatccactatagaaattttcatttgtcattcttgtacttattggcaaaaaattagagcttataggcatcagatttaatttgagatagttgaaatagggtttgtgtttgaggccaatataattttatctgctaatggcatcttctggacttggaggcagcccttctgtaccagaacattgtcacaaagcttttactgtaaagcttgagaacagactagtttgctggatttgggcatgtaactaacagatttgaggcatggaattatcctatggacttttttgtttttttgctttgaggttctgaatatattaaggttgaccaccttaagccattgaaactctcctataatacatttgtgatgtagggcttaagacatgtttgtttggttttttttttttttgacacgtgtatctttgctaccttttaaaagcagattattcttgaagtgcatagagcagcaactgattaatggaattggtatcttcacatttcatttacttccaacaattttataggatgcatataaatatttccaaaaaaggtatacataatttcttactataaaagtatttttattttatatcagtaaatttgttaataaagaggaatttttgttgttgttgttgtaatcctaccaccccaatgacatcctattaaaattttagtatatatcctcccaggtcttttaggtatgtttaatttggtgtcccttccccactcccaaaaggggagggaccaggttcttgtatagaatagtggaatgttagtaaatcatgtgtttaaagagacataacagctgaatctgtagagcatctgccacctggatacctggtaattaaggtaatttttccattaccccaaagagctttagttacactcagcttttaccttaatccttgtacagctctccagggcacactttattcagctctgagcggtctttgcaagtgaggccaaggagccaacctgagccaaaaggagagcattatgtcaccggaagcccaagcccagagaaccaaaggtatgacctgatattcagtggccccagccaggtctttacaagaagaccctgatatctcaggtctaagaagagccagctgatggtttttaaaaagagtggaattagttactctgacccacttattcagatcttattttgttcacaatgtagtccccagattgtaggcccattggaggccacagcaaggcctttgtgttccaattggcctgctgtgccatctctcagtaatgttcccttaacagccagacttccctaagcccagctgggagctctgaaggtatgcgagccctccctaaaccatgagtgtagggagagggaccagggcgccccaggctttcctgtcagtaatgcagaagtttctcagattgagggacgggggagcagaggcataactttgattctgacaaagaggcattcagagagactgaaaggtcatttaacaaacactagaatgcttccacttactaggtgctaggaaatacaaaaccatataggtcctggaagagaggatacatagtagatattagaggcttaggaaatacaattgaagaatggatttgccacgttgaatagttagttggtatcttatttccccattttaaaagttttagaatctgtggttgaggacttgtggccatcagttttctgtagccgacagactgttcactattgccttcagagctctttggaccttaacaggccttctttggagatggcagagatgggtttagatgcatactctgctggagtcacccagagagcccacaaagtcagggatggaacagggtaaaggagtaagggtcatatgtgtgagatgccttgatttggaactttgagatttaggaagagatggggaagggctaaagagggacttgtttctgagccttgcttggctgaagcatttaggctaaagcgttttagaaagagtagcccttggtctgagaactcaaggaaacaactttctgatgagaaatgtagcaagcttctggttcacatccttacctgatagttcttcaaacactgcctggaagcttcccctgagtctttgtctctaatcagctaactaagaggctgagcgagtttagttgtaagtcattaatgaagaaagcaaaggtcggggccattgtcaggattgtgacctgggctagttaattacctggaactgatggtctgtgttacagagtggtggtatacttgtcaggcttagaaaagaaaacaggatgtgtatcaaaaatcttttggggaaaagatttgaccagcaactttaatttctctatgttgcagctatgctgttaatgtagttgtgataattttagaattataccagtgcccttatgttatccttgctttgcaaattgcaaattgctttacatgtcctaacgtccttctggccaacggtagatgtggttttaggtttagactcctgggatggaagctttcgcattcaggggaatgactttgggttgggtgaggattgtaaagaggcaatgtgggtgccccacgacaaagcagctatttgtagctttgtgacaacttgacatacagagatctaggtttatctaggcactaagctaggagtcagttgtttgtatcactggaagattggttataacttccttcgttggaagctccttcattgcatgttaaatgatgttatttatagatagggtggtgggaaagctgtctaagtagatgtcagcccagtgtaagagagacctgcttactgtgggtgcttgggactatcagcagtaggtgggaggttttaacttgttcagtaaggtccatttccattgttcaccatcttgtgaaccctttgtctaacatgaggagcaaccacataaccacagcatgtctggcttccctgtggcttgtgtacaaagcatacttattgagttaatgtataagcaggagacaccctcctgtgataaatggtatattaaccacttatcagtcttaccactctctttcaatttttctggacccaggacctcagcagccatgtcgaagccccatagtgaagccgggactgccttcattcagacccagcagctgcatgcagccatggctgacacattcctggagcacatgtgccgcctggacattgactcaccacccatcacagcccggaacactggcatcatctgtaccattggtgagtgagtgtgccccttccccaaaaaaagggcttcatagaaagtgaccctttctctcctgaaaagactgaactaaatgtcctaacaaacctaggtgctacatgggatgctacacagattcttataaaaggactcaggtcataggaagttgcagtaaagaattagtatgtgcacaggatggcaaatacagttaataagagagtattagacatttcacaattgctaagatggccaggtatggtggctcctagcactttgtgaggccaaggtgggaggattgtctgaggctagaaatttgagaccagcctgagcaacttagaccctctctctccaaaaagtaaaaacaaaagaaaaaaaagaattagttgggcatggtggcatgcacctgtagttctgactacatgggaggctgagaaaaagatcacctgagtccaggagattgaagttgcagtgagccatgatcacaccactgcactccagtctgggaaacagagcgagatcctgtcttaggaaaaaaaaaattgggtgtggtggcacatgcctgtaatcccagcactttgggaggctgaggtgggcggatcacctgaggtcaggagaaccagcctgaccaacatagtgaaatcccgtctctactaaaaataaaaaaaaaatagccgggcgtggtggcgggtgtctgttatcccagctacttgggaggctgaggcaggagaattgcttgaacctgggaggtggaggttacagtgaaccgagacctgaccattgcactccagccttggcaacaagaacgaaactctgtctcaaaaaaaaagaaagaaagataaaagaaaaaaacattgctaagagtaaatttcaaatgttctcaccacaaaaatgttaagtacttgaagtcatggatatgttaactaacctgatttaattattccacattgtatccaaactgtatgtattggattacataactttgtaacccaaattataaattaccagtttataataaaaaacaatttgttgcaaaaagaatccatatgctttaggttttatgctataggcaaaatctagagggtgttttccttagcaggtctttgtaggagcaacttacagacctaggaaagatctttttaatatgttctgtgcaaccaagattctgtggttggatatctggctgggtttcagtgagggcggagaaggctggccaagtcttaacctaggcttttctgatacagtgggagcctgcagaatttgaaggaaatggtcgaagtgtcccagtaaatcaaaaaagtaagctggcacagtggtagccttccatacactttttaaagacttttgagctatttgggagaggaaaagttttcagggaaaaaaattatttaaacttaagcaaacttaaatgtttttccttctttgaataattaatacttgtggctttaaaacttttcctaataggcccagcttcccgatcagtggagacgttgaaggagatgattaagtctggaatgaatgtggctcgtctgaacttctctcatggaactcatgaggtgagctgtagctggaccctttaggaaacagggagtgggtgcagtgttcatttagccacaacggattaggcaaggatgagtctgagtttcacagccaatgtgaagtttgtctttactagcccatccctactctccttccctcttgtcatggcgaagaaactggctaagtctcttttagcaaagaagaccccttttgtcgctggccatgtttctctcatacacctctcctaccattagctttcacaaaggaagatgtggaaaggttctcctggaaaaccctctaagccttagatgtcctggccacagcgcttgactctcctgtccccgggtttctgctacagcctgtattgccatggtaaaaccatctagcagatcgattctggcctatcttagaaccaaaataactgggcaggtccatgagaagagtttccattattctaagttttgaatgactgagcctaatgcacaagcactcgctggcgtataatacccctcttcctcagcactatattcccagcctgtgccttcccaggagttctgtacattaaaataacaccagttagcactcttcctcaggagcctagtaggactgtatttgtgatgggctctttattacctggctttacctatggacagaggccttgcccaggagccgggtagcagctgtcaggatggctccattcctgcctctgttgccagatttagaataaacccattctgaggagtttggggttccctgaggttccatgacttatttatttttttattttataagacaaaattttgctctgtcatccaggctggactacagtggtatgatcatggctcactggatccttgacctcccaggttcatgtgatcctcttgcctcagcctcccaagtaactggtaatacaggcatccaccaccgtacctggctaattaaaaaaaatttttttgtgtaaatgaggtcttactatattgcctaggctggtctcaaactcctgggctcaagtgattctctcaaatgttggaattagaggaatgagctactacccccagcctgggattgtgcctttttaaaaccttcagacttaaccatagatttcccatagatcatgggatttcgtaatggcattgataagaggaatcacagaagaggcagactttgtccctgtcttggcttctgtatttcctgttgagagtaaagaaaatgctaccctgtaaggccaagtgccttatagtggttgccctctggcatttggaagttggtattaagtttggactaaaaataaagcctcaggaaatgcagtccaagagtgaattcctccttttgggaaacttgagactcttcatcatagattccctaacctgtgttcataaacagcctatggcctggctagtggctggcccctaaatgtcatggggacctgaccaagtccagcagacataccacgcaggttaagacatgtccctgtaccttttggaaaattctgtagttttccaaaagcaaggggtccttagtaggagtcaccgagaattactacaagtgttagcttagcttaaagagagagagctgaagacaatggtggaggtctgttcactgttgatccctgctgctgtagtctgccgtgggctcctgcgttcagggaaaggagcagaaatagatttttaagaagttgacctttcagtaggctttgtggttccttcatccagtaaaataacaccacatagctcttacatggcaagggggagtgatatctgctgcacctgctgcatgagagctggctccgattttggttttttaaactttaagaggctttttggagattatctctgctttcactcctactcccagcttataattaagattttttaaaaatttttttatttattttttaaagatgtccctcttgtgggtttattttgaagttttagaccaagatgaggttgtctctgggctcaatttggaaactgatttgaagttattctaatttgtataatgtaaggtaaacagtttcaaccttaccgtttgtcagggctgttgtttcatatgcacctttgactaggggctgggatgtacttttctagtttctgactattttaaatgctcttctgagcagaacgttgagattactgtcttccctcttactctgacagaggaacatcaaatgtctgcatctgatcttttaacagctttctttttttgagacagagtcttgctctgttgcctaggctggagtgcactggcacgatctcggctcaccacaacctctgcctcccaggttcaagcaattctcatgcttcagcctcctgaatagctgggattacagacctgtgccaccatgcccagctaatttttaaatatttttagtagagacagggtttcgccatgttggccaggctggtcttgaactcgtgacatcgggtgatccaactgccttggccccccaaagtactgggattacaggcgtgagccacacgcccagctctcttttgacagctttggcaactagtcttcagcccttacttttggcagttcacatgggcaagatgcattcttgctgaacatgtggttccatatgccgtgttttccagatttatttatttatttagagaggcagtcttgctgtgtcacccaggctggagtgcagtggcacgatcttggctcactgcaacctccacctcctgggttcaagagattcttctgtctcagcctcctaagcagctgagattacaggcatctgctaccatgcccggctaatttttgtattttagtagagatggggtttcaccttgttggccaggctgatctcgaattcctgacctcaagtgatatgtctaccttggcctcccaaagtgctaggattacaggtgtgagccactgtgcctggcctagaaaaaatgactttcaaacaacctaaatgtagagccttccacaggacagcattgatggatgaaactctttaccatgtaacatcccaacaaagccacagctgtagtagaagactcagtacacctcccagaaatgctctaagagattataatatataacatagatttgaataatacacctaataattggtatgtttataatatatagttttacatccccaagaccaaaaatgtatgtttgtgtgaaacactcatggttacaaatatatattaggccaccaaaaaaaaccccaagtttcataaagtagaaattatacagacacattctctgataaaaaattttttaatgcaaattaagaacaaagtcaagaaaactgaagtgtgcttactttagaaagcaaagatctcaaggtagatggaataaatatttaactcagaacactaggggaggaaaaccctaaaaagggtgaagaaaaataattttgtaagattatagctcaatgaaatgaaaataaatttgacaaattaagctaagagctgattatttgtgggtaaaaaatagtaaaatagaaagttctgggaagccaggtgaagaatgcaaggatgtacaaataagagtatgaatagaaaagggaatattttctacacattggagattttaaaagtcaagaaagacttataacttaattcctatagagagagatgacactggctattttccaagaaaagattaaatagccaaaaagatagaaaatatgaatagaccagtggccataagaagttgaaaaagtgggctgggctcacacctgcaatctcagcactttgggaggccaaggcggagggatcacttgaggtcaggagttcgagaccagccaacatggtgaaaccctgtctctactaaaaatacaaaactggcggggcatggtggcacatgcctgcagtcccagctactcaggagcctgaggcaggagaatcgctagaacctggagaggtggaggctgcagtgaactgagattgtaccactgcactccagccaaaaagttgaaaaagtggctaagatctggttcacctcagaacatttaagtccaaatgattttagtggccgaattgtctccccttcaaaattcagttacattgttaaactgttccagagcctagagaaatacagaaatcttcccactgtgttctttgaaaccaacatactctgatactgagatcagacaaggacagtaccaaaaccaggcaggtactaacagcatgttagaccagtctcacttagatgcagaaaacaaataaaatttaataatccaaatccagtagtgattgaaaggaatgtcttgatccatgaccaagtagagtttattctaggagcacaaaattctacattaagattaagtagagttaaggttgactttttttttttttttttaaagacggagtgtcactctgtcaaccaggctggaatgcagtggcacgatctcggctcactgcaagctgtgcctcccgggttcacaccattctctgcctcaggctcccgagtagctgggactacaggcgcctgccaccaacgcctagctaattttgtttttgtatttttagtagagattgggtttcaccatgttagccaggatggtctcgatctcctgaccttgtgatcccccctacctcggcctcccaaagtgctgggattataggcgtgagccactgcgcctggcctgagttaaggatgacttttaaacaacctaaatgtagctaaatatagagccttctgcaggacagcattgatgggtggaactctttaccacatgataacatcccaacaaagccacagctatggtggaactcagtccacctgagtcttaccgttataagataataataggtaacatttattaaataattaccatgtactttgtcctaatacttaatatattcttttactgctcacatcaactctgaaggaaaggtaccacatccccttaaaagaaaacaactatttctattctattcttttatttttttttagagacagaatctcactctgtcttccaggctggagtgcagtggcacgatctcggctcactgcaacttctgcctcctaggttcaagtggttctcttgcctcagcctcccgagtagctgggtctacaggtgcacgccaccattcccagctaatttttgtattttaagtcaagatggggtttcaccatattggcctggatggtctcgatctcttgatgtcgtgatccgcccgcctcagcctcccgaagtgttgggattacaggcgtgagccaccgcgcccagcctctattcaattctattttgttctatttctattacaagccagtaagcaagaaaatatcataatttataaggaaccctataaaaaacaaacaagccaacggtccctcattagggagtatgtctgaataagaagctgaagattttcagatacaggcttcaggcaacattgtctttagaggctaagctctgtctccagctccctccagcatcctgtgaataaccggcagacttacttgcaggtgccgctttcctggacagtggtggttaaaggacaaggcccagaaagtgctgaattaggtgcccttgttatcagcaatgtcatattgatcatgctgtcttagagctcttttgacatcttggctctgcatctttttttttttttttttttttaaatcttttttcttgagatagggtgttgctttggatagtagggtatctaggccagagtgcagtggtatgatcatggctcactgtagccttgacctcctagacaaaagtgatcctcccacctcagcctcacaagtagctgggaccccatgcacacaccatcatgcacagttaatttttgtgttttttgtagagatggggtttcgccatgttgcccaggctcatctcaaactcctgggcccaagctatcctcccaccttagcctcccaaagtgtttggtttacaggcatgagccattgtgcttagcctgagtccctcttttaaacaaacaaaatagtaaatgaaaaggaggaaaggcttaagaaaaaagattgaagcacagatttgttgcaagcaaggaataataaagggcagttcatttagagaaaggcatatgaccacctttccccctctccagtcagaatctagaaagtgattgaggctgggcgcagtggctcacccctgtaatcccagcactttttgggaggccaaggtgggcggatcaccaggtcaggagatcgagaccatcctggataacatggtgaaacccagtccccactaaaaatccaaaaaattagccaggcctgctggtgggcgcctgcagtccccgactgaggcaggagaatggtgtgaacctgggaggcggagcttgcagtgagctgggatagtgccattgcactccagcctgggcggccagtgagactatctcaaaaaaaaaaagtgattgagaaaatcaggtctgtgtgaccttagcaatgagttgtttagcttgggccactgttagcttaagtcaataacttcaagtttgcgttgtagttggaatcaatagaggaaaagctctcagcattaccacatatatcagaatgtgacattgattgccagatcagccttatccaaacacaagttctaggctttttgccctgtttatcagctttatttgctgagggtatttgatgagtcttagggaaaaaagaacagccctggggacacagctgcttttatgatgagacatgtttgcacccataccttaatgggttttggtggcaatattctgaaatttgccaccaacgtttcaaagatttgcccttagggtgaattactgctgtagtagaagtgggtggaggctgaggagattggattaagcaggtagaggagttctcagtgcatggatcgttctgaggatggagatagagctctaagacatccacaggcctttcctgagtgatcagctttggctcctgggcagggaaattgagctggatcctagtgtgggagcacgcttgtcatcttccttctttttccccagtaccacgcggagaccatcaagaatgtgcgcacagccacggaaagctttgcttctgaccccatcctctaccggcccgttgctgtggctctggacactaaaggacctgagatccgaactgggctcatcaagggcgtgagtattctgtggagagcgagggaaagactcagtaggcattatgccccagagacatgtcctccaaagcgttgagatgccatgtttcatcccagcactatgaaggactgcagaggagttgaggtctacaaatgaggatttattcatcactgtaaacaatgttgatttgatttactttgctaggaaatggtaccacagaggaaccctttttttaccctaaaaacctaaactttaggctttctaacttggggaaccatctctttgtatctttttccccatcattaagtagcctaactgaaacattatattctattttcttagattatttctgtgaagtgtactgagttagagaataagagcaaaaaactgtattatttttagcggtgacttgagcattgttccctggaggaaagggcttttccattgcttctgaggtgatgctgctactggtgtcttcagtttggactctggcttactctcttgcttactccctagagcggcactgcagaggtggagctgaagaagggagccactctcaaaatcacgctggataacgcctacatggaaaagtgtgatgagaacatcctatggctggactacaagaacatctgcaaggtggtggaagtgggcagcaagatctacgtggatgatgggcttatttctctccaggtgaagcagaaaggtacgtatgggtgctggaatccaattgtctaaaaccatcttttgtctctaaagttccttgacacaaggaagatgggaaggttggttgcctggcagtgagattgagtctgtgtgttctcaagaatcccttaatattttttttttttttttttttgagacggagtctcgctctgtggcccagactggagtgcagtggccggatctcagctcactgcaagctccgcctcccgggtttacgccattctcctgcctcagcctcccgagtagctgggactacaggtgcccgccacctcgcctggctagttttttgtattttttagtagagacggggtttcaccgtgttagccagaatagtctcgatctcctgacctcgtgatccgcctgtcttggcctcccaaagtgctgggattacaggcttgagccaccgcgcccggccaggaatcccttttataactcatttatcctcaaagacaggctttaatccagcatatttacattcttctggttccggagaacataggaacatatatatatatacacacatatatttcttttttgagtgagagtctcgctctgttgcccaggctggagtgcagtggcacgatcttggctcactgcaacctctgcccccagggttctagcgattctcctacctcagcctcctgagtagctgggtttacaggcacccgccaccatgcctggctagtttttttgtatttttagtagagacggggtttcaccatgttggccaggctggtctcaaactcctgacctcaagtgatctgcctgcctcggcctcccaaagtcaaaacaatcttaattctccttttttatgggtgtggaaagtgaggtacagagaggttaaatggcttgcctaggattacacagttacttgtagtagggtttcaactctggtaaaacagctccagcacccataatgcaccacttcccagctcactgtacttgggggaaaggtgcctgcttcctgttgagctgtgccctcggtgctctgcctcccctgcttaccccttttcaaaacacaggtgctgacttcctggtgacggaggtggaaaatggtggctccttgggcagcaagaagggtgtgaaccttcctggggctgctgtggacttgcctgctgtgtcggaaaaggacatccaggatctgaagtttggggtcgagcaggatgttgatatggtgtttgcgtcgttcatccgcaaggcagctgatgtccatgaagttaggaaggtcctgggagagaagggaaagaacatcaagataatcagcaaaattgagaatcatgagggggttcggaggcaagtccccattgtccctgctccagtcccagcacaactctctaaagggcatggtgcatcctgtgaatatctgattcccagccccctagcccatcagaatgtagactcccaaacctgttccaaacctgctgaatcacaatatcttagtagagtagaaggcattgtgtgtgtgtgggttttgtttttttgttttgttttgttttgtttttaaaaagcttcctaggtaattgagatgctggcagcttgacattgttccctgggcctggggaccaacatttgaggaacagggtcactgctcatagtaccaggggccatgatgctctgttcctgatcagaaacactaccagtgtttgctggaatgtggggaccagggggaaagatgacagcagacacttaagaaggggctcgttttggcccttcctggggagccatgtggaatttcaggggctggtgtccatgctaaaacttatggccttctggtcttcacttagaacgcagctggctcagtgatcatgctaactctggtatggtccattccactctcagagtaagatgtgtggttcttctccaggttcagattgcctcaacttagcttaccccctgcgcagtgctcacgaggtagagcccagtgggcatggccaccatttttggcatcctgctaggaatacaacttagcactactaagatgctagacctacgcttgtggattaggactgtgtttggggagggtgggggaacaaccctctgcacccactgtagtggccttactgtcttagctttgtgtagatatcctctgtaccaggcaatttggggccctcccctttgccatcctgataagctgaacttggcgctaggccaggcaaagccacattccctcttgccttcagcaggttggagtgggccacctcacagggcagtcttcaagtgtccttgactagataaggccatgggtctttgtggtggaagcagtcagcaggcctcgggttccctgtcttgaagtgctgattggagaatggaggccctagagagacacctaacatgcatgggatttggagaggagaccttgagaatgagcccatttggatttgccctctcccctttcttctgtcaatgaagcatccatattggtgttgaagcccagcaggcagaattgttggcccgctctgggggactaagctagctggactgccttgccatctgtgtgcatccatgatgatatcatggatgtctgtcctggtacgaggacatctaagttagggaatcccagggaaacttcttgtcttccggcatacttgtggcccctgtctgtataacctctctccccccaactttgtccatcaggtttgatgaaatcctggaggccagtgatgggatcatggtggctcgtggtgatctaggcattgagattcctgcggagaaggtcttccttgcccagaagatgatgattgggcggtgcaaccgagctgggaagcctgtcatttgtgctactcaggcatgtgaccacccttccccacattctcctgggcacactcacatgtgtgtatgggaaagctctggaggctgtctgatctcttcccatggaattgtcccatgtaacacacagataatccccttccaccatgcacctacacaaagccatgctctgtgcacctactcactatccagaggatcagcgtgctgtcatttgtctctgaaaacagcccaagccacatctcactaatgctctgttcctcccagatgctggagagcatgatcaagaagccccgccccacccgggctgaaggcagtgatgtggccaatgcagttctggatggagccgactgcatcatgctgtctggagaaacagccaaaggggactatcctctggaggctgtgcgcatgcagcacctggtgagttctggggcctgcccccatcccctgggctttggactgggcctgggatggatgcaagctctggtgcagagctttttaagtttccatatcctcttaggcacagccattcattatcctccaagttacagcagcaagagggtgggggtggaggtggaggtggcttttttttttttttaattctcctgtttttcattcctgccgacacccccacccctccatttccttctgctctggaggcatcctccttcactggaatcatacagttcatttcacttctgacttcaaggtggtaaatccttcccatggcttaagtcctgggatacttccgcagtgaagggaggtctcgtacctcttcctcagagtcagaagttttgagtacctttgccctattctgaaaagggctcggggctcctgctcccaactgccctcttcctttggcttccaattcagtcccccgacccccccatcccgcagacaggcgctcccccagggagcccctgtggacctgcactggagtctgttgcctgtactgagctgcctgtgctggccttgcatggtgcctataggaggatttgctttgctgtgccattggggtacagctgctgctcttacaacagaccaaaaagtcaggttgagtgactggtggcagggccacagatagagacagcagggagggtggctgaccctggtggccctggactgagcgtctggaggagtcgtggaggccctttcccttctttctcctctgagagctcattcttcaggctcttccagcttgtcatgttgagtgcctggccactgctcagggttggagactcagtccctttgccctgtctgttccagctctggagctaacttggggatccctgatcagggttacataggtttggtaaaatgagtgctggaaattaactttctcccagtagtcttaggtcaggctcagtgaacttcaactttatccagatatggtttttcttcagccattctattccctttctagccagtgaaagacccgctgccctttgacctcagcccctccaagcccccaagtttaaaacgccaccccccgccaccaaaaaaaaaacaacaaacaactaaaacacccacctcgtctgggcatcttcctttcctttttcactatgtgtcctgttactgggcttaaacagctttcagagaagagatgtcatttctattaaatgctctttcagtagcgaactgagttcataatttgactaaggatattttctgggctgtcatcagcatccttagtgggtttccctatattggaattggtagaggccagggacggtgccttacacctgtaatctcagtactttgggaggccaaggtaggcagattgcttgagctcagaagaccagcctaggcaacatggcgaaaccctatctctactaaaaattcaaaagttagctagctgggcgtggtgatacacttctctagtcccagctacttggagagggggtggtgctggggcaggaggatcactgaacccaggaggttgaggttgcagtgagccaagatggtaccagcctaggtgacaaagtgacaccctctctcaaaaaagaaaccacacaatcataaaaaaaggaaacacaaaaaaatcagtagagagtgatttctctcccaggcccacttaacgtagcctgggcctggctgacacctcaccgtttgtgcgacgtgattgctgttctgatgctgagatcctcttggcgcagtctcacaattgcccccatggtaggaaggtgtcccaggagacagtgcaatttcaaccagtcaccactaaagtgactgcctttctgggtctctccacacgtcccctctctctaattcccttacttaattgtgtaacttcatggcctcaaaggtgggacagaggctgatcttgacttagatttactgaaccatgaaatcactgcatagaatatggagacttgaatgtgtcttttggcaagtcatttaacttctcaagaccttatctgtaaaatggattagatatgtttatagccttagcattaaatattcattgctcttattattaagtgtctgataagtctctgtgtatatggatgtaatcttcctaactcccattacctccatttatagataagggttatatggccaataaagcctgggtttgaatctaggtctgctgactccaaagccagtcttctctcctgcaacatcatgctcttaggtctagcaggagatgagaacaggtctccatttggagtctgtcagtggggtcagagactaagaatcaggctcaacttctaaatttcatgtcctttcctccataccctagtgtttcctatgaacagacagataccttagagctgcaaggcttggattgcatggcagtgctcagaagataagttacaggtctgggccaggctgtagctgcccctccaggtggctagacctttcctttctgtgtcaccagttaacactggccaacagttccttcccttcactgttgattgctttctcctgtgtctaactgatgcagttaatgacgcataactaagagcagtagcaggtatggctctgtttcctgttcctgttccctgtcctctgggttgcatgcattccattctgataaaaagaatacctttaacttagtacatcctgccacacatctgcttctactgtgaaattcatgaggggctattaccgattcctccctcacccatcatttacttagatgctggtgattgcattataatcctctaaagcttacattgtctttctgattcttggtcttatctgagcaagtgatctgtaaataactcagtggctttctcatgactgttttaatcattagattttaatcaagtgtcttattaaacatatctgcatgcttccacagacatctgtctcttcacatggctgttcagtgtgtctctcacaagttagcccaagttttctgttctcctgcttcaaactcagttgagctgccttgctttggcttggatcccagctttccagcgctgctcaatctgtttccatggcaggccattggaaaggctcagtgcatccctgtgcctgaagccaagtgagcgctcactccgtgcatgcatggaggctgggcaggagtctgcctaaccagacagccatgtgaggagggagggcctgttcctttctgtaagctatgtcgtgaggcagcgtgatcaagtcctctgccagggagtggtgtgggcccagcctgggcatgttttcatgccagagtgctagagcctactgccagattgtctccctccatccccaatcaaatccttccagaacggaagagccaatttgccctgtattggaggggaagtggcagcacctcctgaagcagttggactttcatcaccctacctccgcatctgcctgaaggacagatttagccaattaacctaaggttaccttcctctctgattaattccccattctgtcttcccatgtgttgtgtcttgtttttttcctcctccttccctcttccttgtcccctcttcccctaaaccttacagatagctcgtgaggctgaggcagccatgttccaccgcaagctgtttgaagaacttgtgcgagcctcaagtcactccacagacctcatggaagccatggccatgggcagcgtggaggcttcttataagtgtttagcagcagctttgatagttctgacggagtctggcaggtagggccctaagggcaggtaacactgctaggataaccagcctcttgcttcagctgttctaggagaagacagccaggcccaacctggcacctgggcacagagcctcctcttgtctataggaacaccgccagggaggtcatggcagggcaggaccaaagggtcctgtggctcagtaggcacagcagatgtcacaggcacttggtgaaggactggtttctgtggagtcttgaaattggctcagctcagcatctccagtgactgggctactcttggcctttgtccctaggaacatgttcctcaccagctgtctgggtgactcttcccctccctctccttctgtgacaaagctctgacaaggctctgtcctcctctcgtccctctggacggatgttgctcccctagattgcccgtgaggcagaggccgccatctaccacttgcaattatttgaggaactccgccgcctggcgcccattaccagcgaccccacagaagccaccgccgtgggtgcnnnnnnnnnnggatgaagcaaaagatgtccaaaagtccctgccaaccctgccatgtgagtgataaggacatttcagggcctcaatcctttttgccttggctgtaagtctggtgccacattgtggtgtcaggaaggagtgttcagtcagcctagttcagtgctcgggctatggggcagctgcccaggtgcacacctgcctggcttggcttttacttaccaatctcccttctcttcctccaggcaaggcccgaggcttcttcaagaagggagatgtggtcattgtgctgaccggatggcgccctggctccggcttcaccaacaccatgcgtgttgttcctgtgccgtgatgaacctgagagcccttcctccagcctctgtcccacctccttcccccaacccatccattaggccagcaacgcttgtagaactcactctgggctgtaatgtggcactggtgggctgggacaccagggaagaagattagtgcctcgctgaaacatggctgtgtttgcagcctgctctagtgggacagcccagagcctggctgcccatcatgtggccccacccaatcaagggaagaaggaggaatgctggactggaggtccctggagccagatggcaagagggtgacagcttcctttcctgtgtatactccgtccagttccttgagaaaaaaatggatgcccagaggactcccaaccctggcctggggtaaacagctagagagttaggggccttagggcacggggctgttgttcccttgaagctgactctggccctggcccttacttgcttccccagccccctgggcctccccagttcacacctgtccccgccctccactcagctggcctgcagcaaacactccaccctccaccttccattttcccccacttctgcagcgactactgcagcgccttcaggcctgttgctatagagcctacctgtatgtcaataaacaacagctgaagca

SEQ ID NO: 48 - DNA, 24791 bp, Canis lupus
gaaatgcagtggggctgtcctgaggggaagggtatgtagcccatcaccaggtttgtggatgagtggggaggcctctgggggaagatgactcaacctttcaacctctctgcttttgagagaattctctttgttgggtgagtgggaaactgcattgtggtcttcacaggtttaaaaagtcccttctcttcatttagtgagtcaaatagtgaaacacgcattttccccagttaagtgaaaagtggttgtccaggttgtcccggctctctgtactcccctaagagcttaggtgcagcgtgacacaggcctgtgcccaagtaacgtagtctatgcacctgcattcctgagacttccccaggggacacggcagtcctttgtgggaggggggcctgttatggttatgaataatgatgactgaaagaatgtccttgaactcacctctgacttgagtcaaaatagatggacattagtctcttccagtcttagtttagctgctctcattctaagcactgcgttaggagtaaataattttgatgttgaattcatagtttaacagcatttttgggtgtctaataatttgccagtgacctggccaatttggtaggggggactccagacagaactgggaccttgtacaagttgtttctgtgccttggatgttgtgacattaatggggtggggggtgtcacgggaaaagccattttatttcttaaagctgtgtgtttcttaatgttgaggcagtggaagaaatgaggaaatgactgtgagctaggaaaaacccaactcttgcattatcaactcacactaccctggttctaatttatgttgcttcagcttgtatgaaggcatgtcaggatgtgttattttggccaagagctaagactgagctcaaggtaggggaaaatgactcatttgacattttatttctgaatcattccaaacgtctacagtcaaatctcagttaggtggtaccccacaaggatgagtcgcccgtttgagcaaagttttcttgcagccttgttgaggacgttgggaaatgtagaagtggtttactcggtgggagatcctgtaggaggggagcctggctggctcagccagtagaaagggcgactcttgatcttggggtcgggagtttcagcctcatgttgggtacagagattactttaaaaaagaaacattttttaaaagttctccaggactgtgagtcatcactttaaacctcagttctggtccagctaggactagagctaaaggaagagcgttcttaatgcgagcatgctctgggaacttgggtttttcaccacgagcccgtctcagactagaccaatgaatagtctgcttgtttggggctttgttaaggaagctgtttgggggaaggtgagccagggtggctagtggatgggggtgtgcaacatctggtgggcctctctctcggcctcccggtgtgactgctcagctcaggggagggggtgttggcagagccaccgagtggtgtggcgcccgcccctgcagcggtctgtgcagttctgcacgtaggaaggagggcctgcaggaaggagggccagccgggctgcagtacctccggcggcctctgagacttacctcccccacttctgtccatagcaaagcttctggggagctctaagcctctcttccctgacgccagcaagctatgtttggaagttaggcaggggccgtggtgggggagatgccaagccaagctgtgacagtgccagcttagctgatatagttcgaaaaggtctctggaaaggcgcccattccttccgagcctttgaagtcgacctacagctagtacttctttaacttcaggtaattagtgtcttccgtgtttccagcgacgagggcaaaagaattaacccggtcagtgaatcagtcacggtataggagacaaaaccacgggcaacttgaaggagccctgggagttttaatctcgttagaggtagggaagtagaggcttttgataactggtatctctcttttgttatgacattagaaaacaggttaatgtcccctatccagagggtctacattttaaagctctgacaatattgaatgctggcagaagtgttagagggcaagaactcacattgctggatggttgtaaatggatataacctcgttagggcccttcagcaatatttagcaaaatagaaaataaacataccctgtgacttaggaatttcatttctggatatatatagaagctcacacttgcacatagagccgtgtaccaggagaattgttgattgcattgaataatagggggaaaattgattgggttgccaaccagtaagggaatgcgtaaataaccgatgtagtcgtgcagcggatcggcatagtcgttcgtatgaattaactagatctgtgtacccgcaggatagatcttacatgtgctgaaaaaaagcaagatgtttatttgtacagtattgtactgagggcattttagaaaaccggtgtcataggaatcagtatagatatagatgcttaaatggattagaaggatacaaaattcctgacagtggctgggtgtcaaagttcgtcgaaaggttggagggccctggggatggagggaaaataaactacaaaattgtaatggttaagaaaaaaaagtctacaggaattctggctaaatgttagtagtcagttctgggcggtagaaatacggatgttaatattcctttttttttttcttcaattaaaaataaagcaaaatagaagcagatctgtgaaagtcactttaggaagaccagttgtactaactaggtcagtgttcttggagagctgggactgcccttcctcctttcatcctccccttctctccctccagctatggtgcaggacaacccctcctttaaatgctgagctagaacacctcactttgcggaggctgtcacccatcctggttgtgtatcggactttgaagggccctaacctagagtcccaggtcccttgctacttccaaactatgcatatcatgccctaaaacactgcctcactattttaggcctagtaaggaggcgtggtaacacaggacaacaacagtttcctccaaacttccttcttcaggctgaaaccacttctctgctttgagcttctgtggtcaaacaaggacatctgaggtttctctgacttgggacttcctgctctggagtggagtggttctttggaggctgggcccgtgttgtatctacttttgtgccctaatcccactttgaaatatgacttgagactcctgcttgtaaagccacgtccctgaataaataaaagcaagggaattttacttgaacctgcaagtgggctcattttgtttcctgtaagcaggtgagctagactttgctgtctgctagggagcatgctgagggttggaacctcagctccctcctccgtatctcgctccatatataaatgcacaatatcattactctaactgtttatcagggcaaacagtcattcggtgcagaccttactaggttctgtgggtggcctggcacctgttttgatcgtgttgtcagattggggtcagtcttgggaattgggaattctattgctccatcatctaggaactctctagagagcacactggcccgaacgccttgtctgttctgaagattagaggcctgaaaggccttcatcatgctagcttggagacttggaggtgtaggtagcatattgatgacagagccaggaccacagttgtgggcatcaggtgccatcatcgttgggttactctgtgtggcgaggtcagcgtcagaggaaacttggtgcggagagccctggctggttaaaaattggcttgtgtgcatacagctcacgggccaggctggtttactagggcagaatgatttgggcctttgtgaaagaatcagtggagtgaagcgtgaatctttcccggcacaaacttgccaacagtactggccctaagaagtggcacgtcgtatcttttatgtgattccctcccactgtggtttctggagcgtggccgaagacctgtgtctggcacaaaggaaactatagttttggagaaccaggagctgcttaagatgagaaaggaaaggtgggccggggacctggggagctcaggtgtgaccgtgcccaccccatccccttggcctggtagggcttctcacggtgtctcctttctcacagaggagaaatggctctgaggaagatgttactgcaggggctcaggctcaagaataaggttgccgtacctgggcatggcatttgccaccatcagtggatacgccgggcttctactgtaggctggaggttggctctgcatgtctgtgcctcccgggaggagggtgcaagagtgagtcagcggggcacccgctggctgcgtgtcccggcaggcgctgtccagacggccagcatgagggagggagctcttcgcagaggcccgcgggaaaccagggctttggctgctgccctggggccaggggagagtcctggggggttttggcaagaacttgaggtagtggtggttggcaggacgggaaactggtgctcaggaggacctgagaggcaggcagcagagccctgacttccagcaaggggggctcagaggctgggagctgagtgctctggtttggtagacgtgtctaagggcactttgagatcttgtaggagtttggacaagcaagcttttttttctttttttttctttttttctgattactggtgtggaaatccactcaaatgccagataagtgttcattattattattattttttacatttcataggctgggtgagcagaaaatcagcttgcaaaacctcagatttaaattgagatggtaaaatagggttgttgtttgagcgcaatataattgtatttgctaatggcatctcctggccttggagacagcccttctgtaccagaatatccttgtcacaaagattatgctgagaagtttgaggacagactaaacaggcaaagaagtttgctggatttggatgcataactaacaggcttggagcatagaattgtcctgtggtctatgtcaactttttttttttttttccttttctttctttttttttttttttttaatttttatttatttatgatagtcacagagagagagagagagagaggcagagacacaggcagagggagaagcaggctccatgcaccgggagcctgacgtgggattcgatcccgggtctccaggatcgcgccctgggccaaaggcaggcgccaaaccactgcgccacccagggatcccttttttttccttttctttctttggggttctaagtggatcagagttggccttcttaagccagtggaatggtctggcaatgcttttgtgatctggggcctgagacgtgttatctcgcctctgccacatttaagcagagtattcctgaagtgcatagagaggcggttgattaatgaaaccagaagttaagcttcatttttgttttgattccaacatttttaccaggaaacttataaatgtatcatttttggaagaagtacatttgtgatttttcttaatacaaaaatatttccattagtaaatttattagtaaagcgaagaaaacattttgctgtaatcctaccacctaggtgacctgccattactttatgggtaaatagacttccaggcctattatgcatgtttagtttagtagcccttctccctcaaaaactgggaattgaccaggttcttgtatagaatagtgaaatgttaattaaccacatatttaaagggaatttagagcgaaaataatctgggtattcaggaggagataaagcatcatagagctagcaagaatttcctttacctgcaaattttctgttaccattttcttggtatttccttggaggtatctgtgtgtgtgtgtgtgtgtgtgtgtgtgtgtgttttaagattttatttatttattcgagagagagagagaggcagagggagaagcaggctccatgcagggagtctgatgtgggacttgatcccgggcccctgggatcatgccctgagctgaacgcaggcgcttaaccgctgagccacccaggagtcccatatctatgtttttctctgtaacatagcagagtctccgggagcagctaccatctggttacctagttactaaggtcatatttccattgccccaaagaacttcagttacactcagcttctaccttgatccttgtacagctctgcagagcaaaccttactcagctctgagcggtctttgcaagtggggccaaggagccaccctgagccacaaaaaggacattatgtcaccggaagcccaagccccgagaacacaaggtatgacccaacaacctgtggccccggccaggtctttgtttgcaaggaaacactcttgtctcgggtctagagaagagatagctgactatgtttttgtgttttttatgtttctgtttttggtttttgtcaggtgtttttttttttttttttttattttaaattttatttattcaggacagacacagacagacagagagaggcagagacacaggcagagggagaagcaggctccatgcagggagcccgatgtgagactcgatctcgggtctccaggatcacgccctgggctggaggcggtgccaaaccgctgggctatcagggctgctccagctggtgatttttaagaagatgcaggttaattattccaatccactttttgagatcttgttttattcatgatgacagtcctcagactggatgatgattccacttggaggccacagctaggcctttgtgttccagttggctgggtgtgccacctggtgccatctcttcagtcatgttctcttaacaggcagacttacctcagccctgccatgtgctccgaaggcacaggagccctgactccacgcgagtgccaataaagaaaccctggctgccgaggcaggccctctagtaattcataaattcttcagatttggggaaggagggaagagaggtataactttggttttgacaaagaagctttgaggtacacggaaaggtcgttcagcaaacactggaacactccccagtactaggtgctaacagagaacaggtaggtcacagaggagaggacctccaaacattttcgttttggtgcctggtgtgtattagggagttacgaaacacacgttgaaaggagcagcgcatttgccgtgtggaatagttagccaacatcttatttccccatttttgaagtatcagcctctgtagctgagcatgggtagccatccgttttcactagctgacaagttttgctcacaactggtcacggaacttcttgggcgtgtatcagaattcttgaaggtagcagatatgggctgagatgcaagctaccccgagaggccccaaagtcaagggcggggggaggaggaagtaaaagtggcatgtatggcgtgcctggattcagagccctgagagttaggaggagctgggacaggcctgaggagaggcttgttcaggagcctgggctgaagccttgaagctcccagggtgttaggagtaacccttggtccaagaacttgaagaagggacagccttgtgatgaggagggtcgagcttctgactcacatccttacctgatggtccttcagaccagcctggaagcttcttaggtctctataatcagcaaactaaccggctgagtgagtttagctgtcagtagtgaaggaagcaaaggtcgggacagttgtcaggattgtgaccgggtctgtttaattacctgtaacaggtggtctttgcggtgtgcttgtcagaaagggaatcgggatggtgtatcagaaaatcaggtgggggagagggtttggccagcagtctggatggatttcctcaggtgtaactgtcctgttaaagtaggtgtaatacgtctagaacctgaccagtgccattggggttatctggttttatgcaaattgctttgcacgtccctaaagtcctgctgaccacaagtagctgtggttttcaggtgcagactcctggggtgaaagtgcgctcgggattttgggtcagctctgcttcctgtccaaggagtggttcttactatctgtcagtgaactgggatcggctctcctgccagagcaagccaaggaatgaacttacatgttgctctggcttagagaaaatctaggattccagaggtcaaaggactgcctggatgatgattgtctttacaaccaggaaaatcactttgagtttgggtggggattattaaaaaccactatggatgccccaccccatagcggacgtttatagcttgagatagcttttcatacaaagatttatatttgccaagatactaaactagcagttagtgctttctgtcgctggaaggttggtcacgccttcctttggaggtagcttccttcgatgcctgtgagatgttgtttggaggaggacgaggaaagctgtcaaagcggatactagcccgttgtaagggagatctgcttacagcggatgcttgggaagcacgtgtgttggggacgaggttttaaattggtctttgaggtcctttccacttgctcatggtcacgtgaaccctttgcccgacttgaggagtgcccacgccaccagagcatggtggggctccctgtggctcgtgcagagtgtgcctattgagttaatgtgtaagcaggaaacagcctcttgtgctaagagatctattaaccacctgggcttctcagactgatgactctctcttcaattcccctggatccaggacctcagcagccatgtcaaagccccatagtgacgtcgggaccgccttcattcagacccagcagctgcacgcggccatggctgacacgttcttggaacacatgtgccgcctggacatcgactccccacccatcacggcccggaacactggcatcatctgtaccattggtgcgtgggtgtgtcccccgctgcgccccccccccccccaaaaaaaaaacaggggcttcatatgaccgtgatcttccctgaaaagacaaaagaaatgtagcaaacctgggtgctgagcgagatgctacacaggttctttgggaactctggactccggtcctaggaagttgcaataaggaattttgcgtgctctgtgtttgctgctaaaggcagaatatagacagtgtgttgttccatagcacatcttttaggagcatctcagaaatctagggaagatcctttttttttttttttttttaagattttatttattcatgagagacacagagggaggcagtgacacaggcagagggagaagcaggctccatgcagggagcccagtgtgggactcaatcctgggaccccaggatcacgccctgagcctaaggccgacgctcaaccactgagccacccggggatccctagggaagatctttttgacttgctgtgtgcaaccaagattctgtggttggacatctggctaggcttcagggccaagtcttacttaggccttcttagttagatgggggcctgtaggatttcaagggcatagcaaaagcatccccttagctcagggaagtgggtaaacataatattagtcatgtatatgcttttgaaagaattttgagctgtttctgggaggaaaatttaagggaaaaggatatcaagagttcttcaaacttgaaagtgttattccacctttgaatatttaacactttggctttaaaactttttttccccctccactaggaccagcttcccgatcggtggagacgttgaaggagatgattaagtctggaatgaatgtggctcgtctgaacttctctcatggaactcacgaggtaagcctcagctggacagcctggccataggggcagcctgtaggaaattgggtggcagtgtggttcatttagtcatagtgaattaggcaagaggaagtctggggtttacagccagcgggacgagtgtcttcactggcctatcctatcatcctttccccatctcctgccatcccagttggccaagtcttcttacccaaagatgacctatttggttattggccatggttttctcacactcgtgtactgactaaagtgtggaaggtttggggcacctggctggctgaggcagaggagcgtgcaactcttgatctcagaggtgaacatttggggcccacactgagtgtagagcttgctgggaaaataactttaaaaaaagagtgtggaagggttctactggaaaaccctgtaagccgttaggtagcatggcctcagtgcttgacacctcctacccctgggtttctatagctgttcatattgcagtgatgaaccaaaaagtcaccctgcagattgatttctggccgaatgtagacccaagataactgagcaggtccaagagaagagtttctataccattgcaagttaaggaccgagtccgatgtaatcacactatccagcatacagtaccccacttcatcaacactgttcctagcctctctcttcccatgggttctagcatgttaaaatagagtcagcacactccccagcagcctggtaggaaaggatctgtactgaggctgagtatgagctgacttgacctgtggacagagacttgacccagggaccaggtggcaactcttgggacatgctccatcccccctcctgttcccaaactaattttgagggaggagtggaggttccctgagggacaattccttttaaaacccatcgggttccatcataagctgtgggatttcaaagtggtatcgataaagaatgaaggcgccagacttagttccttctttcgacttctgatactttctgttcagaataaagaaaaagctgccctgtaaggacaagtggtgaggggttgccctctggcatttggaagctgctgtttagactaaaaataaagcctcaggaagtacagcccaagaggtgaacttctccttctggaaacgtgagactctccagcatgggttccctaacccagtttcataaacagcctatggcctggcaggcagctggcctccaaatgtcatgggggcctgactgagttcagaggagctgggctcagccggcacttcaggcaggttaagacacgttcgtggtgacattctgcaattttccaaagtcggggtccttggcaagagtccccaggaattcttgcaagggttagctcagcccagagagagagctaaagatatcagtggggatcagttcaccattgatccctgctgccggaccatgccagggtctgctgggtgcagcagaagcagcagaaatagatgtgaagaagttgacctttaacaaggcttgatatggcctctcccatccagtaaattaacaccacagcagctccaaaatggcaaggctgtgtggtgtccgctacacgtgctggacaggggggctggcttggggatttggactttttaaaacaagagccatttggagataatctctgcttaaatacttattcccagattagaattgggatttggggaaaaaaaacaaaaacacccaagttcctgttgtttgaggtttttgactagaataaagttgtctctgggatcaagggtttaaaaactcctctgaaattgttctgatatcctataatgtcacataagcagtttgaccgcatatccgagctcttacttaatacccacctttggttagtggctacaatctgctttcccagctcttgacaatttttaaatactcttctaaacagagcattgaaatagttttctctccctcacactgaagggacgtctattgtctgcatctgatcttttctgacagctttgcctgccacactgtccctaacccccttgggcagttcatatgtgcaagaggtattcttactcaatgtgtggtcccagagacacagacctttttctttttaagattttatttattcatgagagagactgacaggcagagaaacaggcagagggaggaacaggctccatgcagggagcccagtgcgagacttgatcccggaactctgagatcacggcctgagccaaaggcaaacgctcaactgctgagccacccaggcgtccggagacactgacttttaaacagcctaaatttagaaccttccacagggacagtattgatggatggaactctttaccatttggtaacatccaacaaaaccacagccatagtggaagactcagtacacttcccagaaatgcaccaaaagatgacagtatagaggatctgaatgatgtaagacctaataatctcatttgtttatacatagccgatgattttatgccccccccaagaacaaaaacacgtgttgatttagaatgtttatgattaagtaagttattaggccaccaaaacccctcaagttccataaaatggaaattatatagaccatattttctgggatatctttttatgcaaattttcagtctccggaaaactttcaggggcatgggcacacagtaggttaatcatcttactcttgatttcagctcaggtcatgacctcagggttgtgagatcaagccccacatcagactccgtgctgggcatggagttttcttaggatcctccctttccctcagtcactcccctacttcatccacaaacaaaacttacaggcttaaatgtactttttggaaaacaaaagtcttaatgaaagttaatgaaatacttaaaatactaggagccaaataatctaaaagggataaaagaaaagcactgatcttcaagcataacttgataaaacaaaatgaatttgacaaaccgaaaataacttcctgtgaaacaaacttctggaaagtctggtcaagaatgaggatgcataaaaagaccatgaaaagggactatttcccatatattaggagagagtttgaaagtcataaaaagacttctctaatttctgtaagttgagatgaagttgactatcctccaagaaaaggtaagtccaagaggtagaaagtgtagattaacagcctgaagaaatcggaaaggtgggcagcccaggtggctcagcggtttggcaccgccttcagcccagggtgtgatcctggagacccgggatcgagtcctacgttgggctctctgcatggagcctgcttctccctctgcctgtgtctctgcctctctctctctctctctgtgtgtctctctcatgaataaataaaaaaaaaaaaaaagaaaaaaagaactcgaaaaggtgactgtgggctctagctccatcccaggtcaagaggacttgatggcttacttctgtctcccctcaaaggaactttgtcatgctgttccagagcctagaagtcttcccaatatgttctttgaagccaacacacaccctgatagtgaagtgagatgaggacagtaccgcaaccagacaggttagctcttggggcctgtctctcacttagaagcagaaagcaagggtaaaattcaacagtccacatccactcatctgttaaaggaatttcttcccccgtgaccatgtgaattttattctaggaacataaagtccacactgggatgaaatagagtggccagcatgaggtgatggtgataactaggtgctcacctctgttctaaggacttcgtggattcttttacttttcacatcagctctgaggaaaaggcatctgacaacaacgaaacacctactcctttaaaataaattacctctatattctgttctatacagaatatttttattctgtttcacaagctagcaatagaaagacatattttcataactcctagtacggacatctgcccccagagaacaagccatggtcctcatcagagactataatagaagctgaagattctcagacacagcttcaggcagcaccatccttggagatgagactctggttccagctcccccctcagctgccttatgggtgctgctctcccgggcaggctgaaggacagacaaggcctgtcaagtgctgaactgggtgcccctgttaccagcaatgtcctggtggctacactaagaacttggtgacgtcttggctttgagtccctttttcagtcgtcagtcgtggcgagtggaaagggaaaaggctggaagccagggcgcgtggttcagagagaggcgcattttcctgttccctagaccactccagaaagtgattgtgaaaaccaggtctgtgggcccctaggcgatggcttatttagcttgagctattgtaagcttaagtaaataactctggagtttgaattgtagttggaatcaataggggaaaagctcagaactgccaactctcccaccggactctgacactgattgcccggccagtatcacccacacacacgttagtgcaaggtctttttctcccgcggtctgctttatttgccaagggagcatgagcgtaagggagacagacttctttcatgctgacaccgtgtttacatcatccctgtagtgggctttggtggccgtattctcgggtttctaagctttggccttgagtgagtgagtgagtgagtgccacggaaggagtgggtggcaacgaggcgattgaaatgagcaagtggggggtgctcagtgagtggatgaccctgacgccagacacaggagggtagaggtctggaacatcacaggcctttgcggagtgatctgcttcagccgcggctccagatcttgggtgggagcacagctgtcctcttccttcccccagtaccacgcagagaccatcaagaacgtgcgtgcagccacagaaagcttcgcttctgaccccatcctctaccggccagtggctgtggccctggacaccaaaggccctgagatccgaactggcctcatcaaaggcgtgagtatcaggggccagtgggagggaaggtgcaggaggcagtgggccctagagagccgtcctcggtggcgtgtgtcccggttggaggccgtgttcctcacagtgcagatctggaaattctattcatcatggctaaaaaagttgatttggtgtactttgctaaaaaatggtacaaagaagaatcttttttttactttactctgagaacctccttccaagtctgtccgttgcttttcctctatcgttacatagcgagacgatgatgttgtaggacgttgtaagtctttcttgggtcacttccttgagaaaagattgtttatttccaaagccagaagctttattgttcctcatggctgggattggagcatgttccctggaggaaagagcttttcttttccttcggagcgggcccggctcctgtggtttggactcgtggcttattctcttgtctgtagagcgggactgcagaggtagagctgaagaaaggagccactctcaagatcaccctggacaatgcctacatggaaaaatgtgacgagaacatcctgtggctggactacaagaacatctgcaaggtggtggaagtgggcagcaagatctacgtggacgatgggcttatttctctgcaggtgaagcagaaaggtatgtactggaggcaatgtctcggtgtctagaaccagccctaaatttcctttgacccaaggaaagtgggaagtttggctgacagcaaggttaaggctggtttttctcaggatttctttctgtaattccttgtcctttacaatagactttggctcaacttaatcaccttcttggggagcataggagaagatttctttttccccatcctgtttgtgtctttgtggttttcttccttccatcgctcagtgtgatacgtgtcaggcactatcccaagtattttacatggtaatttgttcacgttttataacaaccttatgagtgggtattatgatctctgacaggtggggaaacaggcacagagaggttagttgacctttcccagactttacgattagtgagttaggatctgagttctggacatagtggctccagcacccacaatgtgctgctttccagttcaccctgctggggagagcctgcttcctgttggacattgtgcttccatccctccatccccatttcgcacaggtgctgacttcctggtgacggaggtggagaacggtggctccttggggagcaagaagggtgtgaacctccccggggctgctgtggacctgcctgctgtgtcagagaaggacatccaggatctgaaattcggggtggagcaggacgtagatatggtgtttgcgtctttcatccgcaaggcagctgatgtccatgaggtcaggaaggtcctgggagagaaagggaagaacatcaagataatcagcaaaattgagaatcatgagggagttcggaggtgggtgtcctgaccgccccctgcccctcagccccagcccggcattccagaaagcagactgtatcccgtggatacccaggtcccaaacctggcgacctacccatcagagtgcaaactcccaagcttaggctagacccactggggaggagaaggcattggcatttttaattatttacataagggttttttttttttttttaatttgatgtatttattcatgagagacacaggcagaaggagaagcaggctccatgcagggagcccaatgtgggacttgatcctgggattccaggatctcgccctgagtcaaaggcagatgctcaaccactgagccacgcaggtgcccctatttacttagttttttgttgaattttatttaagtaatctctatacccgatgtggggcttgaacccacaatcctgagatgaagagtcacatgttctttcaagtgggccagccaggggccccaaggaatgggtatttttaagaaaatacatatatcatatatatcttcccaggtgattggcatggcgatgcaccccagaagtgactgacattgttctgtaggcccaggcccagtgttgggagtggatggggagggtcactgctcacaggggccctcatgctgtcctcctgatgagcgctacctgtgtttgctggaataagaggacgtttccccccatcctacacctccaccccatttttcccagtggaaggaagaagatggcaggctgttaggaaggtgctcttgtttggcccctcacttgggagataggtggaagctcatggtgtccttgtcttcacttaaaaggcagttggcctgctgactgggccggttctggcatgttcccagcttcctggaggaaagcatgtggtcctagctgtacttcacctccttcccagtatccccaagtagagctaaaagagtatggccagcttggtgacatctgttcctctgcagctccctgctaggaacataagtcaccagaactaaaaccccagacctacttgggtggattaggcctgtgcttggagagggcagaggggcagccctacttgatcttgccatccttagctttgtgcgggtggcctttgtaccaggcaatatggagtctaccttctgtcctgataaaccatgggtgatagctgtccttggccataggccaggccaagccacatgtcctcatgccttcagcaggttggaggggcccccctcaaggaacagccctcaggtgtccttggctggaaggccacagacctttgtgtcaggagcagtcagctaaccttggaagtgctggcggcagtgggggtggtagagaggtgccttaggcggggcctcatgacctgcagggggagaggaaacaaacccagggggcttcggaggaaaccttgtcttttcccttaccccttggtggaacctccatacgagtgctaaagcagcccagcaagcagtactgttagcccaccttgggagaccaggtagctggaacaccccatcccctttgtgcccacggcgaggtcctggacagctgtcctggtgaagggctgctgagtcagagtccaggagaacctctgtgcgtcactgcacttgcggccttgttccatagaacctctctctccctgccctctttgtcaggtttgatgagatcctggaagccagcgatggcatcatggtggctcgaggtgatctaggcattgagattcctgcagagaaggtcttccttgctcagaagatgatgattgggcggtgcaaccgagcgggcaagcctgtcatctgtgcgacacaggcatgtgcctctccccacactcacacactcacaggcgggtgctgcttggtctcttcccaggaccctgccccacgcctctcaaacacacgtgcaccctcccttcccctcgtgcatgcacacaaagccttactctgtgcacgaacacaggatccagggaatcagcctgtagtccttcctttctggagaccgcccaggccacatctcactaatgctctgtccccgcgcagatgctggagagcatgatcaagaagcctcgtcccacccgggctgagggcagtgatgtggccaatgcagtgctggatggagctgactgcatcatgctgtctggagagaccgccaaaggggattaccccctggaggctgttcgcatgcagcacctggtgagttcctcgggcctccccgccgatgtctgtaggctcgggctgggtggaagcaggctctggtacgaggcaacacctttcaggcttctgtgcccacaaccttttatgatcctctaataagtcacagcaagactgcggaggtgtgtgctggggaggagagggtgtcttggttttcgttctcttctgtcttcactgtccacgctccatctcctgtctcctcctgtcctggaggcatcctccttcatcagcctacacggttcacttctggcctcgaggttgtgaatctgtcccatgattcaagtactgaggtacttgtccctcttcctctggacagcccagaggacccagaagaggccgtgggctcctgctccctgccagcctgtctggcttccgtttgcatccccacctggccacatcaggtgtctccccccgcccccaggggccccgggcctgcactggagactgtcgtgtgtgtgaggggaccgagctggccttgcatggcgcctgcagcggggcctgcttcgctgagctgctgaacggtggggtttagtgactggcagcaagtccacaagtagaggcaggtggaaggcgactgagcctgctggggcgtggagggagagcctccggaagagtcctggaggcagctttttcccaccctggcagctagctagctctgacgctcttgggcttgtccacgtgcccctgcctggctccttctcagttccttggccctgtctggtcctgctctagacacacggaagacttcacccagggttcacttaccagggctcctgaggcctgggaggcagaggcctgcacattcactttcttaacagtagtccagtgtcagcacttaacgtgtgtggagctctgcaaacttgcctctgatcctgaagtggtttttccttgacctattccttttcccatcagcagagggaccctgtgccctttgcgtgatgccgcctcccccgaactctcccagatgtaaccccccaatacacaaagtctcttcctttcctcgttcactttttgtgtgtccagttattagcctgtgtagattgatgtaatctttgtatatcccctgtgtgatagatgtcaccccaatttacggatgaggattacgtgatgataaagccttagtttgaacccagaactgctggctgcagggccagtgttgtcctgtatgtagtgttctgtctagcaggcgataaggccacgtctccatcaggggcctgtactgggctcagagattaagactctccctctggcctctgaattccagctatttttccataaccagtttctcctctggacagacagacacaccttagagagaaccccagggcttggatggcactgctcagaagataagtgatgaggtgtaggtgaggtggcctctcctcacgtccccagttaacgccgagcttctcttaaccgttcactgctttctctcgtgtgttgtgtaaatgaggcaattaaccacccataactcagggctaggccgtctcaggtacgtcccgtttcctgctcggtctcctgtcctttggattgcatgcactccgttcttagagaagaaagaaaacctttaacctagtgaatcctgtacctgcctttaccgtcaaattaatggaacgttctgatttttctcgcacccatcattctctaagattccaatcttccgaagcttaaattttctttctacttcctgatgttatccgagcaggtagtctgtgactataacggaacggctttctcatgactgtgataatccttaatgttgtaatcaagcgtctctgttaaactcacccgtgtgcttccacaggcttctgtcccttcacatggctgttgagtgtgcccctcgcaagtttgccatctccccacctttgtgcttggacctcggttaagctgtgtggctttggcttcatctgaccccagctttccagcgctgctccgcgcgtttccatggcaggccatcggaaaggctcctagcagccgcatgcggaggccaagcaagtgctccatgtgtgcatggaagccaggcaagacgccccgtggtaaccagacagccatgtgaggagggagggcctgttccttcctgtaagctgtgtcttgaggcagcatggtcaggtcctgccagggagcggcgtgggcccagcctgggcatgtttctatgccaaggcgccggtgcctgccgccatcttgtctccctctacccccccacccccaatcagaaaatccttccagaatggaaaaccccatttttcctcttttggagaggaaacagcagcagttgatgctggaaattctccagccatccctgagcagttgggctttcatcatgctgcctcttcgcatctgcatgaaggacagatttagccaattaacctaaggttaccttcctctgattaattccccattctgtctttccatgtgttgtctctcgtttttctccctcctccttccctcttcttgcttctcctcccccctccaaaccttacagatagctcgtgaggctgaggcagccatgttccaccgcaagctgtttgaagaacttgtgcgaggctcaagccactccacagacctcatggaagccatggccatgggcagcgtggaggcttcttataagtgtttagcagcagctttgatagttctgacggagtctggcaggtagggccccaagggcaggtaactccgtaggataaccagcctcttgctccagctgatctagaagacggctggggcgcagccctgcagctggggcccggctccagtcctctcctcgtctgcaggaagccagccagggagtcagggcagggcaggaccgcaagggcctccggctcggtaggcacagtggctgccacaggcacctggtgatgggccagttcccatgaaccttggtcttgcgcgggtctgcggctccagttgtccgccgcctcttggcctcctgtccggggacacgtccctcaccagctgtctgtgagcctcttcccctccgtctcccgtgcgacaccgctctgacagtcctgtccccctcctgtccctctggacggatgttgctcccctagattgcccgtgaggcagaggccgccatctaccacttgcaattatttgaggaactccgccgcctggcgcccattaccagcgaccccacagaagccgccgccgtgggcgccgtggaggcctccttcaagtgttgcagcggggccataatcgtgctcaccaagtctggcaggtaggaggtggcagcggctcccagggcacgccctgctcggggcaccttccctgggcgtcccgagagccgtgcgttgatcggggctcagatggccctgagcccaggtaagcccctctgcctgccacctgggcctgaggacccgaggttagactagagacttcgttgccgaacgacagactgcacatgctcacttgagtatgtgaaagttcatcttttaagaaagtaattgatgaccagttttgttcattccagccactacatgccctttaaaagttcagtttgggagattagtgctgttcactgacgtgctgttgggttggtgcacctgtctctgtctgtctttgagccccaaaggcaagcagattcaggcctaggaaaggtcaccacgtcatcttgctggcaccctagtgtcgggccgccgagctgaggctgctgattggccttggcttgggatctcctcctcatctggacatggagtcagcctctgtcattgccccagtctgggagtgtgctcctcatccctgcctgcagggccacaggaattcctggaaggggaagggatggggtcaggctggtggtccccgagcatggaggtgcggcaggtggggttgcgtgtagaaccgggacatgagatctgtgcagattacctcagcagagggctccggataaacagctccaaccatcagggttgacctttgtggaaaggtccagcctttgctctttggctatttttagctccagtcttctgggatttcactctaaccagtcccgacttcagcacttgcttccctctgaagccttgtatgggggccaggcctttagcagggcagcctctgctgtgacatggcttaagtttccctgacacctgtcggtgtccttagggcttgccttccgacgcccagtgcctcctgcaagcaagcccctccccagctcctgagacccgtctacagccacaagtgtacaatgttcaaggaagcatgtggcactggggcccaggggggccctctaccctccaggggactctgcacagacagagcctcccacattaaccttcccatctcctggtctagcctcctgggtaatacccaggtttggctctagagctgggttgctaggactgttttagggacttgggggccatgtaggctgggggagagggcacagcagtagagggctggctttgtaggttccctggggggctggtgagctctgctgctgttctttgcagatgccaagagtcaggtgctattcacatgctgcttggcttgtagctgctgctggcagcaggaggaatgggtgctggtgaggttgggcagggctgtatctgtgccaggatgggaaagttcagaggaggggcttctgccaactgagtcgtgtggggtgagtgggtgagactgaccgggccgggtcggtgtgatcctggggccctgggctgtggggaggggggtaagaagccaagtggacagatagcataggaagaagagtcggattctgttcctcggaaggtggaggacgaggggcagccctggcatggggagcagatgctaaagtggccagagtctgatgctggcagaatgagttggattagaggctgagttgttgctgaaggccctgtggggggctctgggaggctctggaacactgtttaatggtctcttctgcttggccgtcatcctgtcgcaggtccgctcaccaggtggctagataccgcccccgcgcccccatcatcgctgtgacccggaaccaccagactgctcgccaggcccacctgtaccgcggcatcttccctgtggtgtgtaaggacccagtgcaggaggcctgggctgaggacgtggacctccgggtgaacttggccatgaatgttggtgcgtggctgggagcaaagggctagcacctgcctggaggggtggggacggtgcttgggcactgatctccctgggatcctagagaaaggggaacatgctgaccttggagtgtgcaagagtcctagctgtcttcccagggaacgttctctgactcctccttcccattccctgaagttctgggctaagcccaggagggaggaggagccttggagttctggggctgagctgcccacttctctgtcttcccatccggggcccaaagcaaaggatcctggatagtcaggaatgtcccttcttgggcatctgctccttgttgagggttaagaaaagattagagcgttacatcatggggtgtcctacacacagatcacgtactcatggcctttgtccctaataaaagtaggatgtccgtgcatgagagggactactccaccctctagagtataaaatgatgtccaaaggtccccggcagctgccatttcaattgatgaggaagagtcggggcctccctggtccctgggctgggcggcttgcgccaccttgtggtgggaggcagtaagggtcacccagtctggctacctcggcgggcgggtcagacaggtgctctcctgcctggcttgctttttctcaccgacctttcttctcttctttcaggcaaggcccgaggcttcttcaagaagggagatgtggtcattgtgctgaccgggtggcgccctggctccggcttcaccaataccatgcgtgtggtgcctgtgccgtgacgggccccagagtccctcctccagcccctgtcccacccccttccccaacccatccattaggccagcaatgcttgtagtgctcactcgggggttgtcatgtggcactggtgggctgggatgccagggaagatgaacgcctctgtaaaacatgacttttttaggaccctgttcagtgcaggtggcccagagctgggctgcacatcaggtgacctcaccgcagcaacggacgagggaagggtgcaggactggaagccccagagctttaacacggagggcaacagctcctgcttctcctcctctgtgtactccattcggttcctatagaaaatggatacgcagagaactcccaaccctggcctggctgggtctagagaccaccgcaagaatcgcagcccagggcagtggttccagttacactggctcaggcccttactcgcttctccacccccctgtctcccccactcccacctgcccttctgttcctaggctcagctgcaggcaaacactccaccctccatttcccccactcctgcagctgcctccaggcctgttgctatagagcctacctgtgtgtcaataaacaacaattgaagcaccca

SEQ ID NO: 49 - DNA, 23008 bp, Mus musculus
cgatgtccttccgccacggaaggtagtcctcctcaaaagggcaacctgcttgtcccgcctaccctgagcttctctcaggaggtgcgggcgccccgttgagaggcggggcgccgccggccgcagcccggattgggcgaggggcggggctgcggagggattgcggcggcccgcagctgtgataaccttgaggcccagtcggcgcagccccgcacagcagcgactcgtcttcacttgactgacgtccgctctaggtatcgcagcaggaaccgaagtacgcccgaggtgagcggggagaacctaagccatctgtccccagagccgatgcccactggtgtgtaacgcaggcctgcctgcccacgcgggactcaggcgccaggcatcgagcatcccactccgggttggggaggagccacacttgagtccaagtcttaatcctccaaattgagggtggccggctagctcctttcccacggtctcattctgctctctcttccatctcaatctggttccagcctcttatcttactattgctatcctcgccaccctgttctcgccctgctccgatgctcgtcctcctacatccactacgacttacgaccttcctcttagctctgtgccctcataattcggtgccctcctcttaatctctacttgaaataattcccctactcaccccacccccaccccccattcagcctccgcgttcatcctcctttcaggtcagcgttctcttcccgcgccagtgttcgcagctcttcgtcgcccctcccccctccgatccggtcacgtccgcgccgcagcatcctttcaacctccatatcctcgcccctccccctcgcagcttttcccctccccccgcattctagtcacgtccgcggactcctcgtggtccggtgcatggaggtaggatgcagtcactagcggtccttggtaatgcagctacaagttacgtaacttttgtattcccggtggcctggcaagaaaggttggccgctattgctgcctgttttgtgtgcccgcagatttttggtggtgggcacgggccctcattgctctcgcgctccatcctgcggcggaggggcggcacgtactgcgatgcgtctgattaatcggtcatgctgctcccacgtgctggcgagggggagggtgggcgatcaacccatacccgttcccgacagaaactggagcccgacgctaccagaacacacatagcccacagagctcggtctaattagggaagcagattttgtcaagtcagtgctatgaggaagatggggctgcatgcacaaggtggccggcatactggttttgaaaaagccgggcatcttctagtctgaaggctataaagacccagtaaatacccagtcatagtaagataagagctcgaccactttttccaaatccaggacactggtagtttggaaaaagtgaaccttatagtgaaaatccagtcgtgcatggaggcagctaggttttggaatccggtgtgatctattaatattcttaggtttggcctctggtcctgtgtcactccaggctgctaaattactggtctccttgtaagtacgggccatcctcgatgtagtgactaacctcgggtgaaatatccagaagggcatgcattatatccttttggtcaatgaatgaagtagttaccttgaaggctaccaacttgattctgtctccttactatttttatgcacattaggggtaagcttggggaggcaggtaggctctgaatacccagtatgcccatggaaacaaattctctctggaatcccgtcagtgtttacaaagtaattaatgttacattgcagctctcctgagaaagagctatctaaagggagaaatctgtgcagcctttgtctttggctgtgagggtagaaacaaagaaacaggtacccagatagaagccttccggtcctctttgttcaagtaagccttttatgccttctggcttgtaggaagtttggtactgttgccccaacagtggggtgggggggctcagatcaagactcaaggaagcattgttagcaaataatttgccctctgatggcctgattatgctgtaggaaaggcagtgagggtgttctttgggaaagtagtgtaaaccatcaccgggtctgggcaagatgactcaacctttcaactttgcggcttttgagaaaattttcttccttgggtgagtgaggggaccacacttgttctctgaagtgttgtaaggttccctcttttttagtgagtcaaatagcgtgcattttccctgaattaaacatgtctcactcagactgagtgtggtggttcagctttaatcccagtacttgggaggaaggcctgtgagcttgagaacatggagcgggtgataccctgtttccagaggtggcgggtatcacctaaatgaaggtgaccataagagtggaaatgtggagtggctgcttctagacggcatattttcattcttgaatgattggcacagcagcttttcatagaacaaccagtatccagattggcagtttctctcgaggcatttctgaattattgcttaagccaaactatatgaatactaatcacttatttagtacatagctattttcattttaagcattatattttaaattatttaatttgtagggaaatttgttaagaactgtttgccagcactcaggaggcagaggcatgcagatctgagtttgaggccagcctactctacaaagtaccaagacatccagagctacacagaaaccctattttgggagtgggctttggtggaaatgtatctcaaccaggtataatggcccttgatccctttattcccggtgttctggaggcaaactggcaaatgactttgagtttagtccagccagtgagtgacttggcacatttcatagctgactccaaacagatttatgggggctgggtatgccatctgtgttatatgaacgtgttggtcacaggaaacgctattttatttcttaaagctgttaattgcttaatattgagtggaagggatgaggaagcggctatggacagaaaggtagaaaaagcgtttcttgccttaaactcacattgggtttttagcatctttagcttttttgcagcaagtcgacacgagttgggcaagaactaagctggagattgaggtagaggaaaatgactcatttgtctttcagtttctcaatcatctcaaatacccacaggcaagttaactggtgagtttttttttttttttttttttttactgcttctggtaaaggaccgagtcatctctgtaaactgcactcatggagactataataggagtagatgactgtatgacgaagaacattcttcctgccctggaactttcgtgcgtcttgaaatttttaaccaagagccagacttactttggctatgtagtaatcaggagaggtgagccccacgtgcatcgtggcctgcaaaactgctggatcttaaggcctagtgtagctactcaggtttggaggtggtcccagggcaccaccagctgtgctgtgaggccacacccctactgtggtttgtgcctgtctgcacgtaggagagaggtctgggctgcagtaccttaagtggcctctagggagctctgagcatctcctgaggcctgcctccaaaggaagctgtattccttctaaatgtgtgaataacctttaggccatattttggccttaaagtactggtgtctccagtgtaaaagactttaccctttgccatgcccactttggaggagtcaaaggtttgatttgatgtagagaagggctgggtgtggtggaatgtatttttaatctcagagagacaggacagtcaggatttgtagagtccttgtctcaaaaaaacaaagtagggaaggggctggcaatgtagatctgatacaaagccatggtccatccctactactacataaaatgcacatagtagcacgtgtctgtaatcatactgagcaaaggacagtgggattggagaagttgtgagttggaaaaaacaaaatggactatgaactgaataaagtcagaatgctatttaattaagttttggaaactataaagataaaaagtcagtgttgatgctaagttctgggtgggagaaatggagtctttagatcccactccttggggaaaaggcggtcgtgcaagcctgcgggcagaagtagtaagtaggtcagtgctcttggacagctggtgctgccttccttccgactttaatcaccctgcccccaactgtggctccgggctgagccggtgcctcctgttgctgagaccattgtgcattctgcttacacctggttctctgggcttctgagccagggtccagagcatgggcagcattcccggaaacactggccttgctaaggaagaccgcatgtgccaaccggacagaaacttctgcaaagtcacctccttcctgctctggctagttctccgctctgcacagctgagctagaagccaggaaatcccttgctttgaggaaagtaagaccttgtcttaaaaatcaaataagctgggccgtgaggcaggcagatctctcagtttgaggccagcctggtctattgagttccaggacagccagggctacacagagaaaccctgtctggaatctgactctcaacccccaaaatctctgctcaagtgatctgtacccttgataccgcacatttaattttgttgtatgctgggtactgtgctccaggccttaccactttctggggatagaactgtcacctgctttgaccctggtgttggcttctcattagggtcactgatagctggacagcagcctttctgatggatgaagtgagatgatcttgggtactggggaaagtaggcttggggtgacatcagagaaaggttgctacaaagccctgttcctaggccaggctgctttattagggcagcaatgatttggacctacgtgacgatgtcattggtggggtgaggcatgaccttccaagagtgttggctctaagaagcagggtggcaccaggcatttttggtttggggattttttttttttaatgacctttgttcctgacacgagggagatgaatgtgaagggccgaggagaactgcctgagacaggaaagggcagaaccaggtaatcagagccaagctgggcctgtgcatgctccaacctacagcccaactgaggcctgggctggtgtctcctttctcacagaggggcaatggctctgaagaacatcctgcttcaggggctcaggttcaagagtaaggcttctgccccagggcatggtatctactgctgtcgtgggacacaccgggtttctgctgccggctggaggttggctgtgcatgtgggtgcctcctgaggaggaggatgctgtagtgagttggctggcatgggtggggccgcatgtcctggcagtcactgctatctatacaagtatttggccaataaggcaagtcctgcccaggggcccaccttaccctaaggaacaaggctggagctgctgtcctgggccagaaaagacttctaaaagggtgttctatttatactatactatagataggtggttggctggagttgtggggctctggaggccatgcaatgggcagaagagctgtgggagggagggaggggctccaggtcagagccttgggagtgaaaatagctgggttctaaggatgaggttggtaggggacttgaaacccctgtaaggtttgttagaagtctgtttaattgtgtccatccattggaacacatgtattttcatttgtcactttgtatatggtagcaaggtaagtctactctgcagactttaggtttaattctagatagagaaatgggttgtgtgtgaaattttacctgctaaattgcatcctgagccctggagggcagcagtgcttgtctgttggaacatccttgttgcacaacaaagttctgtcaagcctgagaccggtcaaaacaggagaagaaaattgcatggaactgataggttgtggtcatgaaatttttccatggattagccacacacttttgggaaggtgacttttaaagtcagtggattaagttgcccttcctgggtcagtgaagctgccctgctgagcacttttgagggcatagagaacacacatctatcactatattttagcagggtaattctgaaggacacggctgatgtcacagtgagctttatagggtgcatagagataaatgtgtcattttcaaagactacttaattaacagttttattaataaaggacacgctgggcagacagaagtgtagtaagatgctgtctcagaagagtagggcagtaacgtgatacaggctatcatccaaggtggagcagcgagggtcagtgagatagcttggaaacacacacaggagcttgcttctgatggctccagtgcttctgtccccagaacctgagtggtaggaggggagagcacagttgtggtcctctgatccctgcaaggtgcccaccaggtaccccctaaaactaaatagtgaaatttgtgtattgggggaataaagtacttcaagggatccagtaaagggtcacttttaccactgggtttttttatttatatcttctccactgtatatctgttttaatgtagttaacagcaactttttgccttgttattaaggtcgttaccacaaagagcttagtcatattcagctttcaccttaatccttgtagctcttcagggcaaagcatactccactctgagcgatctttccaagtgaggccaccaagccacactgagtcaacaaaacagcaatatgccatcagaagcccagacccagagaaccaaaggtatgacctgatcactgggcctcactcaggcagggatttgcgagggcacactcgtgtctcagatgggaagaacggcctggtggctggctttttcagtagttttcagacactgtcctggtgtctgtcccgctcacttgtcccatctcggacacagcaaggcctttgtgtctcattggcttggtgtaccatctgtactgtcccttagcggccacttatcctaagcctggctgggagccgtgagtttgccagttgtgtttgtttcggccatgagtagaccaaggacctggctgcctagggacttctcacatttggggagagggaaaaccaggcagaattgatcttggcagagacccggagctcatttaacaaacaaggtgctgggaggcaaggagctaagactctggagaagttgacatcttggtgtctgatgtgtcttgtagagttaggaatgaacaatgttggccactggtttcttccttcctttaaaggttctcaattctgcaaagaatgtagtggttgcacccctgtaatcccagcacccaagagctggaacatgagactgtcatcagttcaagaccagcctgtgctacatatgataactttgtcttaaagtttttcatatctgcatttgaagacttacaggtgtctggtacttggtcactagtgggtggctgaagtctcaggttgcagagacagacttaggtacatactctccaggcgtccagaaaagccagagttccgggaagagtgggggtcctcagctgaggagacaggggagagcaaggatatggagatactgtggagcacaggctgaagactttatgttcaggagtttgagaggagccttgtggcctgaaaactcagatgagaaagaatgtcagcttcattcaagtctcagatagtctgcgagctatagcccagagctctcccgagagttctgtcctctaatcagctgactatccagctcagtgagcacttagttgtaatgaagtaaaagcaaaggtcaggacagctgttggaattgtgacctgggtggttaattacctggaacagatgttcagactactgggtgctatacctatcagacagagaaagaggctccaaatagccagacctcgggctggggaagctaggtctaatgtcagcccttggaaagattaaagatggtaacttcaaggtcagcctaggttgcacagtggatttcaggccagtgtagagtagctgctgtgattccatctcctaggttacagaagactccttggtgaggttataatgactttggggccatttcaatgcccttgtgcaaaatttgctttgtatgtcttgtaggtggtactgtgtttttgtttttgcttttgtttattttttgctaaagaattatggacttttgcttcctgcccagaagaactgttttgttccctgtaatttggaccttactcttgtgtctgataaaagctaaagaatacatttagatagacctgggactttgggagtaaaagaaaggctttgggacagggtttctcttgtttgcaggaccactttaggtttgggtgaatgagagagtgagaccatgctgagtgcctaccaaagccaatactggagattggacatcatgataggcttcccaagatgtttgtgtgctgacatactagttagaacatgcgctggggggtgtttcttactgtaactttggaggtttccttgtgtggggaaagtgatgttctttctagggttgatgagaaagctcttaagacaaggtgacagcccatgtgagaagcctgcttaaactggctcccagggtgtgtgcagtgggtagggagttactcttgttcaccaaggtctttgctgtttgccaatagtcacaagagccctttgcccaatttgagtagcacccacataaccagcacgtgccaggcttttatgctgcttgtgcacaaagcaatcttattgggttaatgtgtaagcaggagacagcttcctatgccaagtgcctcattaagcagtgcctaatctaattgcactcttcaaatctccgggacccaggacttcaggaaccatgccgaagccacacagtgaagcagggactgccttcattcagacccagcagctccatgcagccatggctgacaccttcctggaacacatgtgccgcctggacattgactctgcccccatcacggcccgcaacactggcatcatttgtaccattggtgagtgtggccctccttcctctaaatggaggcttctacctgatttgaaaggcatagtaaccattgcagagctagcctaggttctgagtgaggcacggtccacatttctaggggagtagaggtcttgggaattggccatcaagaagaattagtgtgctttttctgtagttggtgaggttcaggggtggtctttttcatgtgctgtcaccaacagcattcggtagacagacatcttgaaggcagagaaaactgttgccctccacttttctggctgaatgaggccctgcagaatttgtagagaatgttagtgttcccacataattaagaaagtgactagtacaatagtcttttctgtactttggaaagacctttctcttaatttgtgaaggtaattaaaagcaaaggatgaagagttgtttaaatgttgagcaaatttcagacattttcctacctgagtcatgattttcttcctgtggatctaaatgtttcttgatagggcctgcttcccgatctgtggagatgctgaaggagatgattaagtctggaatgaatgtggctcggctgaatttctctcatggaacccatgaggtgagcgtcaacgagatccaggagactcagcgattccttaacagtcgtactgcaggcaggtgtgagtccaggggtcccagtgaacggaacattgccgtttctctcttctaacttcactggaatagaaacctggcctgctttgtcacccaccgaccagggttagccctaccgtcaacctttatgaaagaaggcacgtaagggtttagctggaaaccctaggccatcagatgtcttggcccccatgcttcagggtttttacagtggttcctgtgtgtgaaccaaaaggttctgagcagatggatagctggagtcattttaagatctaccttttaaatacttctctctccccctccctccctctcgacagggtttctctgtatagccctggctgtcctggaactcactttgtagaccaggctggcctcgaattcagaaatctacctgcctctgcctcccgagtgctgggattaaaggcttgtgccaccaccgcccagctttttaaatactttctaacttgactgtggatttcctactggtattggtgaaggagggaaggagactcctctctgcctcttggtttctgtgtcctatttagagtaaaagcattaaccctgtgctgttttgccctctgacctttggaagttgtttggactaaaaatagatggagaagaatggtccaagaagtgaaccccagaacatgagaatcttcatagattccctaacccatattccataaatagcttggaggctagtgcccaaatgtcatggaacctgagatagttcctcaggcacctaagcaatatttgacacattcttgctgggtgtggtggtacaagattgtggttttgaggccagaatggggactatcctcagtaacatagtaagatcttattgcaaaccaggagaggtccttattttccaaactctggctttccacaggagctcccaggaagaaggtgagcctagttcagagacagaactagggccacttgccatggtccttgcgagtagtgtgtttagtcaggcaaaaatagatttggaggtgctgacctttagggctcttgagtccagtaaaataacaccatgcagcaggtctaagagggcaggggacagtgagactgtccagaccactgggcaggccagctctgccttgatttcagactaaggcattagagattggctgtactttgaacctttttatatcacaatataaagcttcacaagtcagggctcttattccatgtgcaccttcagtgaggctctgggtgatggtggtgctggtcttggtgattccctggagaccgtggaaaccaagctccttccctctgacaggaacatcagccacctagctgcacctgatcttgacagctttggctgtgtctctaattcccatctcttgcttttcacatattcaagatgtgtcattcttgctgaacaggcagtactgtactcccacactggcttttaaacagcctaaatttagagcctctacaaggatagcactgatggctgccagtcttccccatttggttacatgccagaaaaaccacagctgtgataatggatagcacgacccagctcccagcagtgttaccatgcagagaaggctaattcaccaccagatactccaatcacaatgcagctttatatatacgaagctgaagagtgtttattatgctcgtgaatgtgctgaggtgtgtaactcagtgtgtacagccataattcttcagtggaaattaagggagaaatccaaacttctagaggatctctaaagcaaatgaaggcagtcggtagtcaatattttgggatatctggagctgggttaccgggtggtggtcagcctttgggcagcttcggtccttgtggatgaatggtggttccagctctgccctaacaaacaggcttgcaggtgttttgctgtgctcagtggttcaaggaccagactcataaagtgctgaattgaatggtccattgtcaccagtgtcacaaggatatgcactggcaacaaactattttgctatcttggctctgagtcccagataggaaagggaaaaggtttggggaaactttattacaagtgaagaaagcaatggcggttgcaccggggcaggctcctggtcggaggaagtggttatgaaagcagggtctgcgtgactagagctgtttagctcggccattgctcactaagtcaacagctttgagtttgaattgcagttgggatcgatagtgaaaacagatagaggctgccagggcagaaatcttcaaacacaaatcctgggtctttgcttgtcctgattagcatcccttggtgagtcctagggacactgggacaacagaagggtcccacaggatgggtttatagtcttccctttaattgattttggtggcagtattctggaactgtatgagagttggagttgatgctgttgtgtagagggaagaatggatattgctaaggttaggagatgggtgaaggtcaggagtcagacatacttttttttttttatttgctaattgatcatctttagctccagggtggggattggaaactggacagggacacctcacctgccaatctgcctttctttctccagtaccatgcagagaccatcaagaatgtccgtgaagccacagaaagctttgcatctgatcccattctctaccgtcctgttgcggtggctctggatacaaagggacctgagatccggactggactcatcaagggcgtgagtatctagaatagcctggtagggggtcacacttttgctatgtaaataacctatttagtctcactctgggaaacgggtattttgtttgttttatttcttcctcaatatacaaattcaggctttatagaaaggtgagaggtttctttggactttgagccagagttgagcgcccccatcaggggcattggcttcttcagttcacactcccatttcctgctttaatccatagagcggcaccgctgaggtggagctgaagaagggagccactctgaagatcaccctggacaacgcttacatggagaagtgtgacgagaacatcctgtggctggactacaagaacatctgcaaggtggtggaggtgggcagcaagatctacgtggacgatgggctcatctcactgcaggtgaaggagaaaggtatgtctggtacacagtccgtggccaatgccaactccaatccccagagctctggcaagcacagacctcgaatgtatgaagatctgggtttaatctccagaggatcaaaagtctaaggttattgttggtctgcgtccctgacctgtctgaaatactgtctcagaaaaaaggcagatggggctggagagatggctcagtactgactgatcttccgaagatcctgagttcaaatatcccagtaaccacatggttgctcacaaccatctataatggttgtgatgccctcttctggtgtctaaagagagctacagcgtgtataaaaggtctttgggccggagcaagtgggggatcctaaattcaattcccagtagccacatgatggctcacaaaccatctctacagatacagtgtacagataaaacacattaagtaaataaataaataaataaataaatataaaaggtctttgggccggagcaagtgggggatcctaaattcaattcccagtagccacatgatggctcacaaaccatctctacagatacagtgtacagataaaatacattaagtaagtaaataaataaataaataaataaataaataaatttttttaaaaaagaaaagggcaaataacccacaaaggtccaggtacctttagtcctccgtcctagcgttcgggaatcaggaaggtggagatgtctcggtgcagcatatgttagactactattatatgccttagaatgagagttaaagttacttattctaaatactttgtgacagtttgagagggtttcctatagctagccttgaactcttgattcttctgtttccacctcccaaatgctcacattaagaatatacaccaccagctgggcatggtggcgcacgcctttagtcccagtactcgggaggcagagacaggcagatttctgagttcgaggccagcctggtctacaaagtgagttacaggacagccagggctatacagagaaaccctgtctcgaaaaccaaaaaagaatgtacaccacctcgtgtggctatttatttgtttattcattaatttgaggcaaggtttccctttgtagccctgcctgacttggaattaactgtgtgtgtagaccaggctggtcttgaactcaaaggtctgtttgcatttgcctcttgtgctaccatacctaaaactcaaattttcttagcagtttgtaagtaagtatttataggtgagaaaactgacttggctttcctgaagtgttttgtttggtttggtttttgttttgtgtgtgttggagtcttaattatggctttagagtcctcctccctctgcttcttgtaaattgaggtggtcttctgtgatccctttcacacaggcgctgacttcctggtgacggaggtggagaatggtggctccttgggcagcaagaagggcgtgaacctgccgggcgctgctgtggatctccccgctgtgtcggaaaaggacatccaggacctgaagtttggggtggagcaggatgtggacatggtgtttgcatctttcatccgcaaggcagccgacgtgcatgaagtcaggaaggtgctgggagagaagggcaagaacatcaagatcatcagcaaaatcgagaaccatgaaggcgtccgcaggtgagtcctgagacccttccattgcccagcccttgagaggggtgtggccatggtgtgtcctggatacctgctcagcaaaatacagcctgctgggattggtccaggcggacatctgaatcagcattagggaggccaagtatttttagtcatcattttgggacccggctggatactcaagggcctcagatgtccatgctaaagcttgaagccttagaaatcttctggtctgataatggtgctgatgaggagtggcccattcagcttcccatagagaagcatgatgcctacgtaaatggaaattaattaaggtggcattcataaggatgagtggtttattgacaaatgttcatacttggctttctccctactgcttcccctagaactgcttctgtgggttacagtgggcttggctctgtgtcctttgtactgggcaactgggagtctctttctatcttgataagccataggtgctgatggccttggtatttggggctggggagtgggtcagctcaaagggcagcagtcagtgcccttagctaaatgatgatccactttgtagaagatccactggcctcattctgtctttgaagtgtcgattagggaagtacaaaacggggtggggggtgagatgcagaccaaaacctccctgaaatatttattatggtgtttaagaagtccagccagtaaaattgttgtgctgtgagtattatcatactgtgctgtggatgccccctcgcctgtgtgcccctgggtgtgacctttgaaagcatctctgtcgggatcccaggtactttggttgtgcttcctgtcctctattatctttctcttctttaccaggtttgatgagatcttggaggccagtgatgggatcatggtggctcgtggtgacctgggcattgagattcctgcagagaaggtcttcctggctcagaagatgatgatcgggcgatgcaaccgagctgggaagcctgtcatctgtgccacacaggcatgtgctatttcattccttctgcattctccacctaggagacctggccttgtcctgtcctttgggcacacatagctgtgatctgtgcacctgcacaatcttaagggaattatcttggcaattatcactgaagatggcctaggatctcatttagtgatggtcttttaccgagagcccttgtctgtcccctcctagatgctggagagcatgatcaagaagccacgccccacccgtgctgaaggcagtgatgtggccaatgcagtcctggatggagcagactgcatcatgctgtctggagaaacagccaagggggactaccctctggaggctgttcgcatgcagcacctggtaagtcctccaagcctaccaccaaggcctctgcatcacccagtcttttacctccctccgaccacggccagaagagtgaggtgtgtggagcatgctctgcttcttgattttcacgttgtgctctcgctgcctgcgccccaccacgttgtcctgctctggcgattaccttttccattacgtaggccacatctggctaaaatattaaagtcctaggacttagtcaagggataccttcctccctcctgaacacccagacggcggggcggcctctattctaaaggagccaagagtgtgtattcttggctgttcgcctggtttggcttctaatttgatctcttgatggtcccatgagcagatgcttctctgcactgcaggctgtagccatactaagctgctttgagctggccttgcatggtgcctgtcacatgggacgtctcttgctatgccaaacccaatgtagggctagaaatagctctgggcgtggggaatgggtgctgaatttagcaggttctggactggagattataaagactttctctgggcaaatctatgctctttttgactaagtcttctggtttcagtaagatagggtctggaggtccagcattcagagcctgaggcaggaagatagcttgaggctaggctgggctagaataaggcattatcttacagaaacaacagacttccagctgacctgactcctgctgactgtgatgggtgaggacccagaacttcctgagcagagcagttagctagggcgccagttaggacctttccttgcctcatgaaagcattgttggctaactttcttggagcttttctattcccttttcggccagcaaagaaccactgttctttttgtgtctccagtttccaataagcccccaaactgaaagaaaaaaaagcccccttcaggattagacatcttaccttgcttcatttgtgtacagctgttaagtagattccatgatctacccatggtttatctgaattgtagctgtagccagatgtgtgcctatattgaaacagaccagccgttttgtagaagcttgaactcagcttgtctcagctggtcacctcctgatctgattggtattgggagctgatcttcacagcttctcagtagctagcatgcagacattccttctccagcagtctgtgtgccttcctgatctacaccaaacccccttcttttctagtcacctgcttagttgtcttatcacctcagagtggtcaggaacaagaccaggtagtctaaaccatgcagtcacatacatggatttatctttgtatagctctgggtgacttatatgaccgcaagaccttgcccaaggtggcatttgatgagattaattataattaattagtcataacattaaacaatttactgccataatgaaatgttagataaccctctgggctcattgatgtaatctttgcattctcattttctttttaaagggaatcacatgtgatagtgtgtttgagcacagatttgctatcctcatagggccagccagctgtctgtttgcaccctgctgtagcaggtgtgggcagagtaggagttagttctcatgtcctgccctctctcatgccctgccctttcctatgaacagacaccttagaacctcgaggctgggattgcatggccctgctcagaagatgagtcacagagtccgggttagactgtggctgccccttcagggggtgcaagcttctctctcatcagttaacactcaggatagcttctccccttcatctgttcgctgcctcctcctctgtctaactgatatagttcatgacctgtaattaagagctagacatcccagctatggtcgtttcctgttcatgtcctttgggctgcatgcattccatttatttgtaactaaaagaatactttccacttgcaaatctgctaatactaccaataaatgtgagttattggttttacatcttctctatactaaaatacttgggattgcactctctaaaacttagattttcattctaatgcctggttttacttgaacagatagtctatatataacacatttgctgttttgtaacagttttaattgctaagttttaattggtgtcttaaggcatgcatgctttctcaggcatctgcctcttcacacggctgtccactgtgttcaagtgagccagagttggccactgttctgtttagaactggcgcaccatgtaactttggctcttttgacctttgaccccagctttcagagctgcccagatgtttctattataaaccaggtgcaaggactcgctcttgtatgtaggctaagctagatgtcttgtaaccacacagccgtgtgtggaggggaggcctagttcttcctgtaagctgtgtcatgaggcagtgtggtcaagtggaagtgtggttggctccaccttggcatctttccatgccaaggtcctagggcctaacaatatgtccctgtcttagcttcaatcaaaaacaaaagaaattgatggtgcctgcctgttatcctagcacttgggaggctgaggcaaagaaaatagtgatttttgaggataactgtggcaagttcaaggctgataggggctatggtaagatcccatctcaaacacatgggggtgagtcccatctcataaacacatggggatggggttttttttaagaaacaaaggggaaagtcccaaaaggataatatctttctagaacggaaggaactttccttgtatttgaacagtaaggggaaaaggagcagcccaaaatcccacgcaaccattccaggagcatatgggctttgaccaccctgcctctgcatctgcctctgcatgaagaaaagattaaacctaaacctaagggtgccttccttcctctctgatgtagttccctgtctttccatgtgttgtctctcttgtttttgcctttatccctcttccttatccctcctaccctaaaccttacagatagctcgggaggctgaggcagccatgttccaccgtctgctgtttgaagagcttgtgcgagcctccagtcactccacagacctcatggaggccatggccatgggcagcgtggaggcctcttataagtgtttagcagcagctttgatagttctcacggagtctggcaggtagggccctaagggcaggtatcattataggataaccagcttctcgcgcaactaggtccgctatgtgcctgagcctaggcacagcctctctccttcaggaagacagccaaggtcaccatagggcaggaccaaaggattcccttgggcacagtggaagtcacagcacctggtgcaggatggttcctgtggagtttctaatcttgctcagttcagaacatggagtggctcaccttctcctggccatttttgtgcccagggacatgttccttcccagttgtctgtgactcctttcctccctctccatttgtgacaaagctctgacaaagccctgtcccccgtcctcgtccctctggacggatgttgctcccctagattgcccgagaggcagaggctgccatctaccacttgcagctattcgaggaactccgccgcctggcgcccattaccagcgaccccacagaagctgccgccgtgggtgccgtggaggcctccttcaagtgctgcagtggggccattatcgtgctcaccaagtctggcaggtaggaggcggcagtggctccctggggatgcccacgctcagttgacacctctccttgaggatgccaagagtgagtggctctgggccagtttaaggcccctggctgccactagaggattccaggcagcactcacagatagaccaaaccaactggctggctccagtgcacgttcaaagcctgcctcacagagagctggaacaaacacccagtttcaccgtgattagtactgtggggccttttgacagaacactgcgtggcagctgggcatggcggagcatgcctctaatctcagcacttgggccaaagaggtaggcgaatgtctggatttgtagcctgtctagtctacaaagtgagttccatccaggacagagccctactcacaaaatagctcagctggtaaagttgcttgctacacaagcttgacccatatttggtccccagaaaccatggaggacggagaaggctggccctgggtatgcgcaagggtacacacttggaggggtcttggtggataaaggatttgcacaatcatgactatctgaatttgaatctggcaccttaaaggttttttattattactttttatttttttaaagtgcacacagaggtcaccaggaaaggtggtctggcctttaggagcactgtcagttctttcagaggcccaacacctgcctatatatggcagctcacaactgtctgactccagtcctggggaaatctaatgcatgtggtcagaatacccaggcagctgtagtgaatgtacggtggagggagagagtgaggtgcccagtgtctatctatctatatagcacaatagatagataaaaaatacccaagtgtggtggtgtgtgcctgtagccccagtgctcatggtgcagaggaagaaagagcaagttgtatcacagcctagctacagaaagccaaacacatgtaaaatcagtgtggaggactaggcactggtctgtctccctaaggcagtgttcatgaactaagtagcagaaagctacttaggcctgggctgaggatggtggcctctgtgtaagcttggccatgaatgttggtatgtagctggaagccagggatgatggggtactgagaaatggggacactaaaactatcatttttagtcctggagttttgaaagctctaaaatacaaggtctatgctaattctggggtttctctgaagagttcctggttccagcagctacctccttccttcaaagcctatgtatgcaggctagcatgaagctctgctgtggaattcctcagtcccccgtgcctagctaattgagtaatctgatagagatagacactatcatttgttacaggttgagaataggggttccctacattcccaggggatcttgaatggccagatattcctcttaccacacctgatcaccacccagatttctttttctttcttttttttttaaatttatttatttatatgagtacacgtacttcagacataccagaagaggacattggtatcggatcccattacagatggttgctgggatcccatgtggttgctgggaattgaactcaggccctctggaagagcaatcagtgctcttaactgctgagctatctctccagcccccagatttctttttctttctttttttttttaaagattgatttattattatatctaagtacactgtagctgtctgcagatgcaccagaagagggtgtcagatttctttatggatagttgtgagccaccatgtggttgccgggacctgaactcaggaccttctgaagagcagtcagtgctcccaaccactgagctatctctccagccctaccacccagatttctaaaaccatagaaattctgaggtttcttttaacattagctgctaggactcccataggagaacagtatagtgttatggtgaacattgttggcttccagggcctggtaactctgctgctgttctttgcagaagaagtcaggagctaggcacatggtacttggattgtaaaagttgctggcagctacaggagtgggttctgctgagattgggccaaagctgcctcactgccagatggaagggttcatttgtgggaagaattctaccagccatgctcctataggactgcccatactgagagcaggataatcatcttagaaaagacaggacaggtctgaggggcaggccagaccttgaaacagttgtcagtgggcaaagcctgtggtccagagttgaattagagggtattacttttggcttaggcttactgaaagggtcttatgacatgtttaacggtcagtctttccaacctgtttccatctcaggagtgctcaccaagtggccaggtaccgccctcgggctcctatcattgccgtgactcgaaatccccagactgctcgccaggcccatctgtaccgtggcatcttccctgtgctgtgtaaggatgccgtgctgaatgcctgggctgaggatgtcgaccttcgtgtaaacttggccatggatgttggtatgtagctggaaacaagggaatgatgaagtgctaataaatggggaccctaaaactaccacttcctgaagtcatgggctgggcctatctgttttatcacccagttgtaagattagctggagctactgtcctgagcagggtggggttagagggtggggaacacaagcttttgtggccttattcctatatagagacaaggaggcagctgaccctgactctctagagtataaactgaatggtgtccaaaggtctctgcattctgagttcagcctcagcccttgtttaggctaggaggcttgcaccatcttgtggtgagaagaagtaactgtcaacctgctcccctacccagacgaggattattagggcagttatctgcacctgccttgttggatttgtgtctgggttgggaaaagtgccactttgtgtgatcaattaggactgtggggctttgcagttttcctcaagtgtatacctctactcaccaacctccttttccccccaggcaaggcccgaggcttcttcaagaagggagatgtggtcattgtgctgaccgggtggcgccctggctctggattcaccaacaccatgcgtgtagtgcctgtaccttgatggccctctggagcccctcttctagcccctgtcccttcccctcccctatcctttccattaggccagcaacgcttgtagtgctcactctgggccatagtgtggcgctggtgggctgggacaccagggaaaattaatgcctctaaaacatgcaatagagaccagctattattcagggccctacctgagccaggggtggaggaggaatgcaggactggaaaccctgactttatcacagaagggcggcagcatctctgggctttgcttctgtagaaagttgtcagaattcccagccctagcctggagtcaggagacagcaaaagagtaggggctgagggtgtggggcccagggtcccagtgtagatgacgacttctggccctggccctgacctgctttcccaacagctttggcctccccacttcttgtgcactccacttctgtcactgcagacactccactctccaccttgtattctgcagagtctccaggcctgttgctatagtgcccacctgaatgtcaataaacagcagctgaagcacctgt

SEQ ID NO: 50 - DNA, 21995 bp, Rattus norvegicus
  modified_base (20158)..(20161): a, c, t, g, unknown or other
aatgtccttccgccacggaaggtagtccccctcaaaagggcaacctgcttgtcccgcctaccctgcgactctctcagaaggtgcgggtgcctgttgagaggcggggctctgctagctgctgcccggattgggcgaggggcggggctgcggagggattgcggcggcccgcagcagtgataaccttgaggcccagtctgcgcagccccgcacagcagcgacccgtcctaagtcgacagacgtcctctttaggtattgcaacaggatctgaagtacgcccgaggtgagcggggagaacctttgccatctgtgcccagagccaatgcccactagtgcgcaacgcaggccttcttgcttgcccacgctggacccaggcgcctggcatcgagcatcccattccgggttgggggagaagctacacttgagtctaagtactaatcttccaaattgaggcgcggggtggggggcggctagctcctttcccacgtactcgttctgctctcctttctcaatctggttccaacttcttattttattattgctatcctcgccaccttgttccaatgctcatcctcctacattcactagtactttcgaccttcatcttagctctgtgcccttatcattcggtgctctccttgtaatctctccttgaaataactcccctgctcacccccctcccgcttcagcaccgacgttcatcctcctttcaggtcagcgtgctcttcccgcgcctgggttagcagctccttgtcgcccctcccccactcctttctggtcacgtccgcgccatagcatcctttcagcctccctatcctcgcccctccccacagcttttcccctccccctcattctagtcacgtccgcgaactcccctctggccctcgtggtccgttgcatgtaggaagaatgcaatcactagcaatcctaggtgatgcagctacaaattatgtaatttttgtaattccggtggccaggcaagaaaggttggccctattgctgcctattttgtgcgcccgcagatttctgtggtcgtgggctaggctcctcgcgcaccggggtcctgcgtgctcccgtgctccatcctgcggcggcgggcctgcacgtactgcggggcgtcggctcccacgtgctggagaggggaaggtgggcggtcaactcatacctgctccctacagaagctggagccggacgcgacccgaacgcacacagcccgcagagctcagtctaattagggaagcagaatttgtcaagtcagtgctatgaggaagatggagctgcatgcacaaggtggccggcatactaggtttgaaggagccgggcatcttctagtctggaggctatataaagacccattcatagtaagatatctctcgatcaccttttccaaatccaggacattggtagttcggaaaaagtgaacctaatagtgaaaattcatttgtatgtggcggcagctgcgttttagaatccgctgtcatttattaatatctgaggtttttggtcctgtgtcatgagtggaaacatttactccaggctgctaaattacttgtctccttgtgtgtacgacatcctcgacctactttctggtgaaatgcccaaaagggaatgcatatatcctttttgtcaatgaagtagttacattgaagaccaccaacttcagtctgtctctgctatttttacgcaggttaaggttatgcttggggaagcccgtaggctccgaatacttattcacatggaaacaaaatctctctggaaccccatcggtgtttacaaagtaactaatgttacattgcaactctcctgagacaaccatctaaaaggagaaatctgtgcagcctttgtctttggctgtgagggtagaaacaaagaaacaggtatccagatagccttccgagtctggtctctgttcatgtaagactttcatgctttctggcttgcaggaagttacatttggtactactgttgcagtactgttgcctccaaattcagggtgtggctacattctagggtacagaggggaggccttaggtcaacactgaaggtagcattgttagcaaataatttgccctctgctggcttgagtatgttgtagggaaggcaatgagaatgttctgtgggaaagtgtaaaccatcaccgggtctgggcaagatgactcaacctttcaacttagaggcttttgagagaattttcttccttgggtgagtggggaaaccacacttgttctccaaggtgttgtaagatcccctcttaagtgagtcaaatactatagttcatttccctaaattaaacatgtctcaccgggactgagtgtggtgtgcatttggctttaatcccagcactgaggaagaagggctagacctgtgagcttgagaccatgtaggtggtgggtatcaagtaaatgaaggtgacctttgtgctgccataagagtggaagtgtggagtggctgcttttagtctgcatatcttcatttttgagtgacacagcagcttctcagaaccaccagtatccagaatggcagtttctgggaatgcgtttctgagttattgcctaagccaaactctgaatgctagtcacttatttagtacatagctattttcattttaagccttatattttaaattagttgtagggaaatttgttctataatgaggagatctttgccagcaatcaggacgtagaggcatgcagatctgagtttaaggccagcctagtctacacagccagagctacacaggaaccttgttaaagctgttgattgcttaatattgagtggaagaaatgaggaagcagctatggacagaggggtagaaaaacttttttttttttagcatctttagcttttctgcagcaagtcgagatgagttgggcaagaactaagctggagattggggtagaggaaaatgactcatgtctttcagtctctgaatcattccaaatacccagagccaagttaacttgttgtccccccccccctaccacttctggtaaaagaccgagtcatctctgtaaactgcgctcatagaaactataataggagtaaatgacagactatatgacaaagaacattcttcctgctgtggaactctcgtgagtcttgaaatttttaccaagaggcagacttagtagtgggagaggggagcctacatggtcatggcctgcaaacctctgcctgatcttaaggcctggtgtaacagctgaggattggggagtggtcttagggccaccactagctatgcagtgaggccacacccctgctgtggtttgtgcctgtctgcacgtaggagggaggtctgggctgcagtaccttcagtggcctctcgggagctctgagcatctcctgaggcctccaaaggaagcagtattccaaatgtgtgactaacctgcagtcatattttggctttaaactactggtgtctccagcaatgagtgtaaaagattttaccccataccatgcccattttggaggagtcaaagttttgaccttaagtaaagaagggctgagcttggtggcatgtgtttttaatctcagagacaggaggaactgagttcgaggacagtccgggctatgtagagagtccttgtctcaaaaaaaaagtagggaaggagctggtaatctctatggaattccattctgatggaatgtttgcctatggtgcataaagccttgctccatccctagtactacatagtatgctcatagtagcacgtgtctgtaatcaagctgagggtgggagcaaaggacaatgggattggagaagttatgagttggaaaaaaacaaatttgtgtgtgaatttattaaaatcagaatcctttttcgtttttggaaaatgtaaaaacaaatctgtgataatgctaagttctaggtgggagaaataggttttggattccactcctccttgggaaaaaggcaaccctgtaggcagaagtagtaagtaggtcagtgctcttggacagctggtgctgtcttctttaatcacccccacccccaactgtggctcagggcattttaaatgctgaaccagtgcctcctgttgctgaggccattgtgcattctgcttacacctggtcctccagggtctggaggagcacaggcatcattcccagaaacactggtccttctaactgctaaggaagacagcatgtgccaacagaacagagacttctgcaaatcccctccttcctgctctagctagttctctgctctgcacagctgagctagaagccaggaaatccctctctttgaggaaagagtttaaagtagaactgttcaggttaaggttaaataaaagttggtttttgcttatttttctctctagttgttttgaccacaggagtttaacttgacttcaccaggtggtagctagcctagtaagccaggcctttctgagagaatatactcttctttggacatggtagcatatgcctttaatcacagcactcaggaggcagaggctaaccagggctagatagtaagacctggtcttaaaaaatcataatctgggccgtagtgacacacgcctggaatcccagcacctagcagatctctgagttaaaggccagccttgtctattgaattccaggacaaccaaggctacacagagaaaccctgtctagaatctgacccccaacctaatctctgcttaagtgatctgtacccccaataccatatatgacttaattttgttgtattctgggtactgtgttccagaccataccaatttctgggggtggaattgtcagctgcttggaccctggtgtagcctgtgggttagggtcacttctgtagatctgtgctccagaggaagctcctagagagcagggtgaccagcatgttgcgtgtcatcttgcagcctttctgatggatgaaactaggtgatcttgggtactggaaaaagtaggcttcagatgatatcaaaaaaatggtggctacaaagccccgtccctaggcagcagtggttcggggcccgtccctaggcagcagcagttcgggccccattcgtccctaggcagcagtggttcgggccccgtccgtccctaggcagcagcggttcgggcccacatgaagatgtagttgttgtcggagtgaggcatgaccttacaagagttggctctataaaaagcagggtggcactgggcatttggggttttaagtgacctttgttcctgacacgagggaaatgaatgtgaagggccaaggaactgcctgagacaggaaagggcagaaccaggtaatcagccaagccaggcctgtgcatgctccaacctgcagcctgcactgaggcctgggctggtgtctcctttctcacagaggggcaatggctctgaggaacatcctgctgcagggcctcaggttcaagagtaaggctcctgcctctgggcatggtgtctgctgctgccgtgggacacaccgggcttctgctgctggttggaggttggctgtgcatgtgggtgcctcctaaggaggaggatgctgtagtgagttgcgctggcatgggtggggccgcatgtcctggcagtcacagctatcaatctatgcaggtaattagccgatagtgcgagccctgcccagagggccccctactctaagagacaagggtggaccaggaaaagacaccaagagtagggtgttctatttttatactatactataggtaagtgattggctggagttggggctctggaggccatgggacaggcagaagagctatgggtgggtgagagtggggggtcagagccttgagtgaaaagaactgggttctagggataaggttagtaggagagttggaacgcttgtgagttttgttagaggtctattttgtatcagtccattgaaacacatgtatttccatttgtcactttttatctggtagcaggataagtccactctgcagacttcaggtttaattctagagagagaaatgggttgtatatttgagattttacctgctagattgtgccctgagccctggaggcagcagtgcttgtctatcagaacattcttgtcagcacaacaaagattgttctgtcaagcctgagaccagtcaaaacaggaaaagaaaattgctggactctggcatggaactgataggttgtggtcatgaaatttttccatggattagacacactttggggaaggtggctttttaaatcaatggattaagttgcccttcccaggtgaatgaagctgcccagcttgagcacttgggagggcaaagagaacacatctgttactgaatcttagggtagtttcgaaagacacagggctgatgtgtggaacttcgcaatgagtttataggatgcatggaaataaatgtgcatttccaaagactgttcttaatttcacatcaacagtttctttattaataaggatatgctggttggattttgctggagaccactctggcctatgttgtaccttacataataagaaacagtctcagggggttggggatttagctcagtggtagagcacttgcctaagaagcgcaaggccctgggttcagtccccagctccgaaaaaaagaaccaaaaaaaaaaaaaagaaacagtctcagaaggggggagggaatgtcataatacatgctaccactcaggtaatgaagaagggggaaacaaagcaacgagggtcagtgagacagatggctgggaggacacggaaacttgcttctgatgactcaggtacttctatccccagaacctgagagatagaaggaatgagaagacttgtggtcctctgatctctatacggcgtccaccatgtaccccctaaaactaaatagtaaattttaggtgttgggaataaagtacttcaggggatccagtgaggggtcacttaccaccgggtttttgtcttctccagtatacatctattttaatgtagttgaatctctaaaagcaacttttaccttgtcattaaggtcattttcacaaagagcttagtcacattcagcttttcccttaatccttgtagctcttcagggcagagcatactcagctctgagctgtctttccaagtggggccatcaagccaatctgggtcaaaaaaacggcaatatgtcaacagaagcccagacccagagatccaaaggtatgacctgatcacctggccctgagcaggaatttgcaaggatacacttgtctccggtggagagaagggcctagtggctggcttttcagtacttttcagacactcttctaatgtctgtcccactcatttggacttcatagttcatagtcccatcgtggtcacagcaaggcctttgtgtctctttggctttgtgtaccatctgtactgtcccttagtggccacttaacctaagcctggctgggagccatgagggtttgccaaccatgagtttgtttcaaccatgagtagaccaaggacctggctgcctaggatatcctgttgtatacaggacttcctcagatttggggagagggaaaactagtagaccctggagaagaggttgacttgacgtcttggtacctaatgtgtcttgtagagttaggaatgaccaatgttggccgctggtttcttcttcctttaaaagttctcaattctgcaaggaatgtagtggtgtacctctaatcccagcacccaagagctggaatatcaggactgtcatgagttcaaggccagcctgggttgtatatgagaacttgcctcaaagtttttcatctccaggcctctgatttttgatcactagtgggtggctgcaatgtcaggtggcagagccaggcttgggtgcatgttctttaggtatccagaaaagccgatgtccagggtagagtgcgggtctttgggaaggcagggaagagcaaggagatgtggagtgcaggctgtgtgctcaggagtttgaaaggagcctcgtggcctgaaaattgattcaagtctctggtattctgtgaggtacatcccaggttctcgcttactcagccaactatccagctcagtgagtgcttagctgtaagtcgtaataaagtaaaagcaaaggtcaggacagctgttgggattgtgacctgggtgattaattgcctggaacagatgttcagactactgtgtgtggtccctatcagacagagaaggagactctagatagccagaactggggctgggaaagctgggtctaatgtcagcccttgggaagagtagtgactttcaaggtcaacctcggttgcacagtggatttcaggccagcatagactagctactgtgtgtgattccatctcctaggttactgaagactccttggtgaggttgtaatgactttggagccatttcaatgtccttgtgcaaaatttgctttgtgtgtcttgtacatggtgctgttttttgcttcttgtccagaaaaaaacttgttgcctgtaatttggaccttattcctgtgtcggatagaggctaaggaatacatttaggtgatacctcaaacctaggactttaaaaagaaaggacttgggacagggttcgtctcttggcagcaggatcgctttaggtcatggcgaacatgataaagaggctatgtcagtgccaaagcaggtttgacattgtcgtgataggcttcccagatgttcgtgtgctgacacattagctacgtgctctgcaggagtggggaggtttccttgtgtgggaaggtgatgttctctctagggttggtgtgaaagctcttcaaatagatggcagccgttgtaagaagcctgcttaaactggcttccagggtgtgtatgtgcactgggaaggaagctacttttgttcaccaaggtctttgctgttcgttcatagtcacaggagccctttgcccaatttgagtagtacccacataaccagcacgtgccaggcctctgagtgacttgtgcacaaagcagtcttattgggttaatgtgtaagcgggagacagtctcctatgccaaatggttcattaagcactgcctagtctaattgaactcttcaaatctccgggatccaggatctcagaaaccatgcccaagccagacagcgaagcagggactgccttcattcagacccagcagctccatgcagccatggctgacaccttcctggaacacatgtgccgcctggacattgactccgcacccatcacggcccgcaacactgggatcatctgtaccattggtgagtgagtgtggcccccttcgcagggcttctgcctggtttgaaaggcgtaataaccattgcagggctaacctaggttctgagagacactgtccacacttttagaggaagtattggtgtacttcttctgcagttggcgaggttcagggtggtcttagtgggcctttgcaggagtagttcagggacttcagatctttttcctgtgctgtcactccactttctgcagaatttatagaaaatgatagtgtccttccttacatataaattaagagagtccttccttacatataaatcaagagagttgactagcacagtagtctttctggactttggaaagacctttctctaaatttgtggaggtgattaaaaacaaaggacaaggagttgctttgatagtgagcagatttcatatactttcctacctgagaatcatgattttcttcctgtggctctaaatgtttcttggtaggccctgcttcccgatctgtggagatgctgaaggagatgattaagtctgggatgaatgtggctcggctgaatttctctcatggaacccatgaggtgagtggcagcttgatccaggaggttcgggacttgctgctgctgtgctccaggcttctcagtgaatggagcgttgctctagctagcatttacatccctctctccctcttcccctctggccaacttcattggcatcaacaacctggcctgctttgtcgccggccagggttatccctaccatcaagctttgtgaaggaaaccctttatgtaagggtttggctggaaactctaggccatcatgtgtcttgactgcacttggcacccacgcctcgggctttctacagtggctcctgtgagtccggtgaaccaaaaggtcatgcagaagacttagttcaggccccagatggctaggtaggtgcagatggttttcccgtgagaccgagtctaacgcacaaatgcagtgcggtctggggatatcccacttactcctgctgcactgtctgcccatcatcagtgcccctccctaggagtgaggtagggatgacctgggctgtttattattaggtggccccactgatggagaggctgtgcctaggaagcaggtggcagctgttagaagggtccattcctgcccctgctcactttgagaacaacccgctctgagcagatgggtaggtgggggcgtccaacgatccgccttctgactttctaacttgacagcctttcctactggcactgatgaaggagggagagactccttcctgcctcttggtttctctgtctatttagagtataagtattaaccctgtgctattttgccttctgacctttgaagttgttttgactaaaaatagatggagaagaacagtccaagaagcgaacccttccttcccagaacataaggatcttcatagattccctaacccatattctataaatagcttgtagactagcccccaaatgtcatgggagtgcaatggtccctcaggcacctaagcagtacttgatacattcttgcttgggtgtggtgctacagaatgtgggttcaaggccagcgtgaggtaacataccaagatcctattgcaaaccaagagaggtcgttgctttccgggctctgttgctctccatcagagctcccaggactaaacgcaaaggtaagcatagctcagagtcagaactagatccatttgccatggtcctcaggtctgttcagccaggcaaaaatagatttggagacactgacctttagggctcttagatccagtaaaataacaccgtgcagcagcccggacatgacaggggacagtgagacagttcagaccactgggcagctcagctctgccttgattctaactctaaggcattagagattagctgtcctttgaacctttttatgtcacataattaaagcttcaccagggctttcttattctatgtgcaccttcgatgaggggctgtggctgtctgtcttggatgaggggctgtggctgtctgtcttggttttaaccattcctggagacggtggaatgaatcgagctccttcgagctccttccctctgacgggaccatcaattagtcagctgcacctgatccctgggcagttttggcagtgtctctagttcccgtctcctgcttttcacatggtcaggatgtgtcccttttgctgaacaggcagtgctgcactcccacactgacttttaagcagcctaaatttagagcctctacaaggacagcaccgatggctacccgtcttcaccatttggttgtgtgccaggaaaaccattgctgtgatagtggaaagcacggtctacctcccagaagtgttcccgtgtagagaaggttgctggaccatcagacactcgaatcttttttttttttaaagatttattcatttattatatataagtacactgtagttgtcttcagatacactagaagagggcatcagatctctctacagatggttgtgagccaccatgtggttgctgggaattgaactcatgacctctggaagagcagccgggtgctcttaaccactgagccatctctccagccccagacactcgaatcttaatgcagttttacatacatgcggtagaaagtttgtcattgctgaattgaatggtctgctgtcagctgtgtcacttggaggcacattggcaacagactattttgccatcgtggctctgtgtcccaaagaggaaagggaaaaggttttgtttgggggaactttattgcaagtgaagaatagcaaaggcagttccactggggcacgctactggtcagagaaagtgattgtgaaagcaatgtttgcacgaccagagcaatgggctcttcagctccggccattgttcaaagtcaacagctttgagtttgaattgaggttgggatcgatagtgaaaacagatacagacagccagggcgcaaatcttcaaacacaagtcctaggtctttgcctgtcctggttgttagcattctttggtgagtcctagggacactagaacaacagaagacacacagtaggacaggcttaatactcttcgagttggagttgatgctgttatgtggaggggagaatggataaggtgaggttcaggacttggacatacttttcttggctaattgatcatctttggctccagggtggctcagggcatgggaactggacttgggtgtggagaacacctacctgtcaatctccccttctttctctccagtaccatgcagagactatcaagaatgtccgtgcagccacagaaagctttgcatctgatcccattctctaccgacctgttgcggtggctctggatacaaagggacctgagatccggactggactcatcaagggcgtgagtatccaggagtttaggtctttaaatgagaatatttttcatctgcctggtaggaattattatagatgcacatttttggtatgtgaataacatacttaagtctcactctggggacctggtttgttgtttgttttgtttgtttccctcaataaacaaattcaggatttacagaaaggtgatcggtttcttggggctttgagccagagtttgagcgccgccatcagggtgttggcgtccacagtcacacgcctctgctgtctttaatctagagcggcaccgcagaggtggagctgaagaagggagccacactgaagatcaccctggacaacgcctacatggagaagtgcgacgagaacatcctgtggctggactataagaacatctgcaaggtggtggaggtgggcagcaagatctacgtggacgatgggctcatctccctgcaggtgaaggagaaaggtatgtgtggtgtacagtccacggcccaatgccactcccatccccagaactctggtaagcacttaacctagcatgtatgaattggtctcccaaggatcaaaagtttaaggtggttgttggtctgcatccctggcctgtctgaaacactgcctgagaaaaaaaagacaaataacctacaaaggcctatgtgtacacctctaccctttagttccagcactcgggaatcagcaggtgtgtgagttctcatgtgtaagactactcctgtatgccttagaatgatagttaaaatttaccgaatctaaacactttgatagtctaagacagcgttttcagtagctagccttggactcctgcttctccggtttccacctctcaaatgctagcattaaaaatacacatcaccattcatggctgtttgtttattcatttattttgaggcaaggtttcactcttttgacttggaattaactgtgtgggccaagctggttttgaacttgatctgtttgcgtgtgcctcttgtgctaccaccccaaaaactcagattttcttagcagcctgtgggcaggggtttataagtgaggaaactgatttattggcttgcttaatcatggctctagagttctcttggcttctcacaaactgagatagatggtcttgatccctttcacacaggtgctgactacctggtgacagaagtggaaaatggtggctccttgggcagcaagaagggcgtgaacctgcctggtgctgctgtggacctccctgctgtgtcagaaaaggacatccaggacctgaagtttggggtggagcaggacgtggacatggtgtttgcgtctttcatccgcaaggcggctgacgtgcatgaggttaggaaggtcctgggagagaagggcaagaacatcaagatcatcagcaaaatcgagaaccatgaaggtgtccgcaggtgagtcctggtggagacctttttcacattacccagccatcgagagagagagaaaggtgtgtctgtgctgtgtcctcagcaaaataaagcctgccaggactggtccagaatatctgggtcagcatcggaaaggcaaagtagtgttagtcattattttggaaactcgggcctggtgtccacctagatagagccttggaagtcgtctggcctgacaatggtgctgaggaagactggcccattcagcttcccatagggacgcatgctttagttaagatgtcattcataaggatgagtggtttagtgatacatacttggcattctctcacttcccctagacctacttctgtgggttacgagtgggcttggaagagttagggcggtaattgttaacacacacacacacttgtccttggctctgtgtccttttatactgggcaatttttccctcttgataagccataggtgctggtggccttggtatttgttcagccctggaggaggtggggagtggaacagctcaaaggacagcactaaggaccctagtaaggacccttagctaaatggagcatgggcctttgtaggtctgtgggcctcaatttgtctttgaagtgctgattagggaagtatgatacaaggggttgtgagatgtagaccgaagaacccatggaactgaacctcatccccttgacgtatccccgcaagtaaaatggttattgtgctgtgggtatcatcaaggtggtgggtgcccactccctcaccgtgtgcctgggggtgtggccttggagggcacctctgtcagggccccaggaaagctctgtccattctttggttgtacttcctgttctatagcatctttctttttatcaggtttgatgagattttggaggccagcgatggaatcatggtagctcgtggtgacctgggcattgagattccggcagagaaggtcttcctagctcagaagatgatgattggacgatgcaaccgagctgggaagccagtcatctgcgccacccaggcatgtgctatcccttccttctgtgttctccacctaggagacctggtcttgacctggcctttaggtacacgtacccgcacatagctatgacctgcgtacctgtgcaagcttcggggaattgccctggcaatcatcactgaagatgtcctgctcttccattatttagtgactttcatttagcggtggtctcttacttaataaaaacccttgtttgtcccctcctagatgctggagagcatgatcaagaagccacgccccacccgtgctgaaggcagtgacgtggccaatgcagtcctagatggagctgactgcatcatgctgtccggagaaacagccaaaggggactaccctctggaggctgttcgcatgcagcacctggtgagtaagtcctcagagcctggggtagaagcagctctgctggagaggcctctgtccagtcttgttacattgctcccgtcacagcaaggagagtgaggtttgtggaggtgtgcttgagtttcattgtgctttcactgcctgcacctgcccctttgtcctgctctggggattacataggccacatctggctaaaatatcaaggtcctaggatgcagtcaagggatgccttccttgtggacacccagagggcctgggtacctctattctaaaggagccaagagtttgttcagctattctccttgtttagcttctcatttggtctcctggtggtctgtcccatgggcagatgcttctctccactgcaggctgtagccatactgagctgctttaagctggccttgcatggtgcctgtgacatgggacttcctcccttgctgtgccagacccaactcggggctacaaatagctctgggggtggggaatgggtgctgaatttagcaggttctgtctggtctaggaattataaagacttctcaggcatattatgtgctcttttgattaagtcttctggtttcagtaagatagggtctggcgcaagcttgtaattccaacaatcaaatcagcctgcggcaggaagatggcttgagattaggctggactagaatgagacatcttgtagaagcaacaggcgtcagctgacctgtccctgcggactttccacccaggcctccgtcttctgtgttctgctccagaacttcttccggagcagaacaattatctggggcatcagttagggaccgttgcctgataaaggcatggtggattagctttttgggggttttctattcccttttcagccaacaaagaaccacagtatcttttgtggctccagtttcccacaagcccccccaaacttaagacaagtgaaagaaaagaaggaagccccttctgggttaggcatcttaccttgctttatatgtatatgagagttgagtagattccatgatctttccatggtttatctgaattatagctgtagccagatgtttgcctatattgaaacagaccagcgctttgactcggctggtcatgacctgttctgattggaattgtgagctggtcctcatagcttctcatagcatgcaggcattctctcccagaagacttttcccttccttcaatctcccccacagtagctgccttcctggtttacaccaaaaccccttttctacttacctggcctcacagtggtcaggaacaggactttgaccaggtattctaaagcatgtagtcacataaatgtatttttggatagctcaagaagaccttgcccaaagtggcggttgatgagattaattacaattaattatatgtgtatgagttagttttggtgtcctgtccttttctcatgccctggtctttcctatgaacagacaccttagaacctcgaggctgggattgcatggccctgctcagaagatgagtcacagagtccgggttagactgtggctaccccctcaggggatacaaatttctctatcagttaacacttaggacagcttctcccctttctttatctgtttgctgtttcctcctgtgtctaactgattcagttcaaaacctgtaattaaaagctagacatcccagctgtggttgcttcctgtccatgcctcttgtcctttgggcttgcctgcattccatgcttaaccaaaagattactttccacttgcaaatctgctaatgctaccaataaaatcgagtgctggtttcatatcattcctggaattgcactctctaaaactttatttctttatttctaatgcttggttttacttgaacaggtggtctgtatataacacatttgctatcctgtaaccgttttaattattgagtttgaatctgtgtcttgaaaggcctgtgtgctttcccaggcgtctgcctcctcacatggctgttcagtgtaccgtgttcaagtgagccagtcgaccactgttctgtttagaacttgtgcactgcaactttggctcttttgaccctcacccccagctttcagagctgcccgagtgtttccactgtaagccaagtgcaagcgctcactcttgtgtgtaggcggagttggatgccttgtaaccacatagccatgtgaggaggggacgcctttttcttcctgtaagctgtgtcaggaggcagtgtggtcaagcggaagtgtagttggctccaccttggcatctttccatgccagggtccctttctcagctttaatcaaaaacaaaagaaatgatggatggtgcatgcctagcacttgggaggctgaggcaaagaaaatagtggtgttttgaggctgaccatggcaagttcaaggccagtaggtgctatggtaagatcctatctcaaacctgtgtggggttgagaattggctttttttgtttgtttgtttttagaaacaggaaaatcccaaaaggatactatctttccagaagggaaggaaggatctttccttgtgtttgaacagaaaagagagccacccaaaatcccacatataataccattccaggctttgaccaccctgcctctgtatctgcatggagaagaaaagattaacctaagagttccttcctctcattagttccctgtctttccatgtgttgtctcttgtttttgccttcatccttcttccttatccttcctaccctaaaccttacagatagctcgagaggctgaggcagccgtgttccaccgcctgctgtttgaagagcttgcgcgagcctccagtcaatccacagaccccctggaggccatggccatgggcagcgtggaggcctcttataaatgtttagcagcagctttgatagttctgacggagtccggcaggtagggccctgagggcaggtatcattataagataaccagcttctcacacaactagggcccactgtgtgcctgagcctgggcatagccctctctcctgcaggaaggcagccaaggaggtcacgatagggcaggaccaaaggattccctagtgggtacagtggaagtcacaggcactggttcaggatggttcctgtggagtttctaatcttgctcagttcagaacgtgtagtgactcatcttctcctggctttttgtgcccagggacatgttccttcccagttgcctgtgactcctttcctccctctccatttgtgacaaagctctgacaaagccctgtcccccttcctcgtccctctggacggatgttgctcccctagattgcccgagaggcagaggctgccatctaccacttgcagttattcgaggaactccgccgcctggcgcccattaccagcgaccccacagaagctgccgccgtgggtgccgtggaggcctccttcaagtgctgcagtggggccattatcgtgctcaccaagtctggcaggtaggaggcggcagtggctccctggggatccccagagcaactctgggctgatttaagacccctggctgccaccaaaggactccaggcagcactcccaggtacaccagattaggtggctccagtgccagtcagtgcacggcctgcctcagggcctgaagcatatatacagttttgcttagttacggtgtggaagctgggcatgggtacatgcctttaatcctcccagcattcgggcagaagaggtgggcaaatgtctgcattcgtggacagtctggtctacaaagcaagttccaggacagagccctagctcacaaaaataactcagctggtaaatactacttgctacacaagttagaccatggaggagggagaaaggtaacttacaagcgtgcccaaggacatatacagtaacactttttctcatcccacttggagggagctcaatggataaagtgttggcaatctggatttggatctggcacctgtgggtttttgttgttgtttgggtttttgtttttttttttttttttaagtcacctggagaagtagttaggcctttaggagcactggggttttggtttttaagatttatttattatatatgaatacactgtccctatcttcagtcgcaccagaagagggtgattacagatgattgtgtaagccaccatgtggttgctgggagttgaactcaggacctctggaagagcagttagtgctcttaaccactgagccatctctccagccagcactgttctttcagaagcccaacacatacatgacagctcacactatctaactgcagtcctggggggaatctaatgccctcttctaacttccagccgtacatgtttatatgatgcatgtggtcaggatacccagacagctggagggaaaggaaggtgcccaacacacctgtgtgcctgtaatcccagcactcatggtacagaggtagaaagatcacaagataggtctaatctgagcaaattctgcaacagcctagatacagaaagccaaacacataaaaatcagtgtgggctgaggatgttgacctttgtgtgaacttggccatgaacattgtatgcagctggaagcaagggatggggtgctgaaaaatggggaccttaaaactaattttctgaagtcctgaagtttcgagagctccaagatacaagttctatgctaatcctggactttctctgaagagttcctggttccttcaaagcccatgtaggccagcatgaagcagggtattttctgctgtggaatgccacatcccctaataccttgtgtgtcctcaagatgcctagttaattcagtaagcctgaaacagatctgatagaagtaaacatatcatttgctatcggttgaggagagaggggctccctacattcccaaaggatcttgattggccagatattaaccatgcctggtcacacctagatttccaaaaaccataggnnnnagatttccaaaaaccatagaaattcagaggtttcttttagcaccaagttcagctgataagactcccaaaggagcagtatagtactgctctggcaaatactgtccactccagggtctctgcagataccagaagtcaggagctaggcacatggtgcttggattgtaaaagttgctggcagctacaggatggttctggtgagattaggccagagctgcctcactgcctgatggaagggttcacagtgtgggagggatcctgccagccgtggtcctatgggactgcccacactgagatcaggacaatgagttaaaaaggacaggacaggtctgagggggtggccaggcactgaaacagtaagttgtaagtgggcaaagcctgtggcctagaggtgaattagagggtgctgcctttggctgactgaaagggtctcgtgacacaatggccattcttcccaccttctcaggagtgctcaccaagtggcccggtaccgcccaagggctcctatcattgctgtgacacgcaatccccagacagcccgccaggcccatctgtaccgtggcatcttccctgtgctgtgtaaggatgccgtactggatgcctgggctgaggacgttgatcttcgtgtgaacttggccatgaatgttggtatgtagctggaagcaagggatggggtgctgggaaatggggagcctaaaactaccatttcctgaagccctcacccaattttgggcccaaggcaaaattaattgcctcattaggctcttgtaagattaattggagctactgccctgtggggtggggcacacaagctgttgtggtctttgttcctatataaggttggatatcaagagacaaggaagcagctgaccctgaacttgggcaaggctggccactctagagtctaaactgaatggtgtccaaaggtccctgcagtctgagttttgcctcagcccttgtttaagctaggagacttgcaccaccttgtggtaaaaagaagtaactggcaacctgctctcctacctgaattagaagcaatagggcatttgtacctgcctggttaggcttgtgtctgggctgggagaaagcaccaccttgtggtaggagagagtactggttgctcagttaggactgggtagggctttgcagttatccccaagtgttgtatatacctctactcaccaacctccttctcccctcaggcaaggcccgaggcttcttcaagaagggagatgtggtcattgtgctgactggatggcgccctggctctggcttcaccaacaccatgcgtgtagtgcctgtaccatgatgatcctctggagcttctcttctagcccctgtcccttcccctcccctatcctatccattaggccagcaacgcttgtagtgctcactctgggccatagtgtggcgctggtgggctgggacaccaggaaaaattaatgcctctgaaacatgcaatagagcccagctatttttcatggccctacttgagccaggggtgaaggaggaatgcaggattggaaaccctctgactttatcacagaagggcagcattatctctgtgttctttgctcctgtagaaagttttccagagaattcccagccctggcctggaatcaggagacagcaagaacagaggctgggggcccagggttcccatgtagatgacttttggccctgtccctgacttgctttcccaacagctttggcctctctcctcgtgcactccactgctgtccctgcagatgttccactctccacctcgtactctgcagcgtctccaggcctgttgctatagtgcccacctgaatgtcaataaacagcagcggaagca

SEQ ID NO: 51 - DNA, 13748 bp, Oryctolagus cuniculus
  modified_base (6934)..(7189): a, c, t, g, unknown or other
atgtcgaagtcccacagtgaagccgggtctgccttcatccagacgcagcagctgcacgcagccatggcggacacattcctggagcacatgtgccggctggacatcgactccgcgcccatcacggcccgcaacacgggcatcatctgtaccatcggtgagcctcggggaccgagtccgggaaggagcgcgcattgtgcgttctgctgggggtgagcgtccccagctcagaggcctaggcctatgccaccaagatgggcagagggctggccaagctcttaacctgggctttcctgactgtagggggctacagacctgtgcagggcgtggggagaggtgttcccctaaatcaagaaagcaggctagcacatcgacggccgtgagtgtgctctctgaaagacttgcgttatttgggggaggaaaccgaggaagcgtttctttgagtcactgacgctgtgccgcaatatgtaacaggccctgcctcccgatcggtggagacgctgaaggagatgatcaagtctgggatgaacgtggcgcgcatgaacttctcccacggaactcacgaggtgagcctcggctgcacattggccgcgggggcggctgtaggcgacagggaggagtgccttgttcacttagggtgggctccacagattccagtctgggtgtcccagccctaggctcctgccctgagctctctgcagcttggttctggcccagttcaggctgcagagagctgggcaggcgcccagaggtttccactctggcaggcgagtgccccgcccgtcagcactgtgcccccagcctcgccctctccagaggttctgctgcacggacagaaaaccagccggcgagtgtttgcgctggagctgttggccgtggcaggaagcggcgctctgagggtgctggggttccctgaggggccgcagtcgtggggcttcatttcggcattggtagaggagtaatgggcaggctgacgttgccctctcttgccctctgtcctttcctcctctgaggtcagtggtgagggtcactctctggcatttggaagctggtgttaagtttggactaaaaataagccctcgggcagtgcaaaccgcggggtgaattcttgctttctggaaacatgagacttgactctccatggtaaatgctgcagcccctaactctggggcccagccagggccagcaggcacctcgggcagcctgaggcgcatcctgggctctcaccaggaattgctgcgtgtgtcaccctgcccagagggccaaggcagcagtgaggatcagttcacctttgacccctgctgccggagtctgccgtgggccctgcgtgcgggtgaggagcagaaatagatttggaggcgctgacctttcagccgctgcgcgctccctccaccagtaaaacaacaccgccccgctcggaaatggcaagggctgcacctgtcgcacgagggcgtgggtctgtgcttctgattctcattcccagattaaaagtgggatgaaaaaggaaagaagcgcagtgcctctggtggtttagggtcaggcccaggtgagcttccagggtcagcatctgggaagcgggcctgaggtgctgaggtgtggactgacgtgaccgccttccccctcctcacctgacagaggcacggctgcttctgtgtctgggcttttgtgttgttttttgtttttgttttgttttgtttttttttttttttttaatttatttaattctatttgaaaaacaaacagattttcccactgatttattctccaaatgcctgcagcagccaggaggcaggactcggttcaggtctcccgcatgggtggcaggggcccgcacacttgagccccgtcacctgctgccatccaagcgtgacgagaaccaggactcaaccccaggccctccggtatgggatgcacacatcccaggtgctgtctccagtgctcagtcctacaccttgtctctggcagctctgaccgtgtccctagcccccgccctggcagctcatgtggaccatctgtgcttgctgaacatgcagttccacaacgccaggctggccagaactgactctgacataatctaaatttagagccttccacagggcagcagtaatggtggggtgggcaccactccgcagataataagcagcccagccccaccccagccagcaccctgtcaaccatttagaatgtttatgacataagattttacatccccaagaccaaaaatggcatgtttatatactttgagttgcaaaaagtattttctgtcactcaccaaaaaacttcaagttccataaaagtagaaattttacagacacatgacctgacataattttttagaattgtttgaaaggtagaggcagagcgacatctctgatcttcccaaatgtccatagcagctggagctgaaccaggccagagctgggagtccggaactcactctgggtctctgtacaaggcaggcagggacccaggcacttgaaccatcacctgctctgtccatgcactgtgttgtcaggaggctggatcggaagtgcacctgggactcaggcgtgtcttcagtggattcttgactgctgtgccacactcagccctgactttttttcatggaaatcaagatcagtatagagtgtgatgatcaggagagcttcaaaactcgttctagaaccagaagccgtggcaccggcaataaataaatctttaaaaaaaagttaaagaaaaagaatttgtaagaccatggcttgatgaaatagaagattgaaaaattaagctgagatctgattctttgtgggaaacagtaaatcagaaatctcaggaaggcctggtcaagaatacgaggatgggggccggcgctgcggctcactgggctaatcctccaccttgcggtggcggcacaccgggttctagtcccggttggggcgccggatcctgtcccggttgcccctcttccaggccagctctctgctgtggccagggagtgcagtggaggatggcccaaatgcttgggccctgcacctgcatgggagaccaggagaagcacctggctcctgccatcggatcagcgcggtgcgctggccacagcgcatcggccgcggcggccattggagggtgaaccaacggcaaaggaagacctttctctctctctctctctcactgtccgctctgcctgtcaagaaaaaaaaaaaaaaaagaatacgaggatggggagggaattgtggcgcagaggcttaagcctccactgggacccagacacctcatatcagagcactggtttgggtctcactggctctacttttttctttatttatttttaaagatttattttatttgtttgaaagagttacagagagaggtagaggcagaagaagagaggagtctttcatctgctggttcactctccagatggccacagtggctggagctgagctgatcccaagctgggagccaggagcttccgggtctcccacgtgggtgcaggggcccaagcacttgggccatcttcactgctttcccagatgcaccagcagagagctggatctgaagtagagcagctgggactcgaaccagtgcccataggggattctaacactgcaggccagaaatttaacccactgcaccgcagcgccagcccctggccccacttctgatccagtttcctgctggtgtgcctgggagtaatggcctcagtacttgggtcctggtcacccacatagagacccaggatagagtgaggttcctggcttcagcctggaccagccctagccattggagccacttggggagtgaaccaatgatgaaagatctcccactccctctcctctgttaaaggaatttcttgactggtggccaagtaaattttattgtgggaacatagagttattaaataattcctgtgtgcttgactcttctgagtttcatgttattttagtcctcagaacaaaaggtatttggtaatattcagcacccctccctccctccctgcctctctctctttctttctttaccggcagagttagagagagagacagagaaaggtctttcttttccattggttcacctccaaattggctgctgtggctggcgtgctgccccaatctgaagccaggagccaggtgcttctcctggtctcccatgcgggtacagggcccaagaacttgggccatcctccactgccctcctgggccacagcagagagctggacaggaagaggagcaaccaggactagaactcggcgccccaaccgggactagaactcagggtgccggtgccacaggcagaggattagcctagtgagctgtggcgccggccaatccgttccttttttacatactgcaggatcaaaaaacaccacaccagaactatctccagactgggtgtctggtcagaggttaagttgctccttggaatgtccacatctcatatctaagtgcattgttcaagtcccagcttctctgcttccaactgtttattgttagtgcatatcctgggaggcgacccatgcgggagacctggatggagttgtaggctcctgacaattgcaggcatttggggagtgaacccagcagctgcaagataatctctctctctgcctttgaaataaaaagtgaaaataaattaattataagtaaatgatttctattgcaaaccagcaatacgaagaatgtagaacctctgtggaatagaaagtggagccagtggtcgctccttgcagagagtgcctgagttagaagctcatggtggtcagacagctttgggcagtgtcgtccctggagacggctctggctcctggtaccttccagcgtcccaggcctgctggcagctgctgttgcccagacagtggtggttaaaggccaagcccatgaagtgctgagcgaggtgcgctgttatcagcagtgccgtattgattaccctatctgggagcccttttgacatcttatctcggctttgactgcctttttgattgaacagtactggcaagtgagggagaaagggctttggagagagacgggagccaggatgtgctgccagggcagttggtgcggagaggggcctgagagcaccttggcctgctcctctcctctcaggccacaccctgggaagggagggtgcagccagctctcatgacctacctgagctttcaggtgaagtccacaacctggtgttggaactgtggttggaatccgtgggagagggccctcgcctggccacctctgtcaggctctgcgctgattgcccggcggtctcacccacacctgccctggttcttctgccccagtcgtcttgccctgttagttgtcttaggggaaagagcacagcccgaaggtgctgctgcttgtgtggttctggacggcagtggcctctgctgagtgcgtgccgtggtggaggtgcggagaggctgcgggtgctcgggcggacggcggccgaggtgggcgatgcagctttggctcccagccccagggatgccagctggcccgagcgtgggaggacacttgtcctcttctccctcccccagtaccatgcggagaccatcaagaacgtgcgcacagccacggaaagctttgcctcagaccccatcctctaccggcccgtcgcggtggctctggacactaagggacccgagatccgaacggggctcatcaagggcgtgagtatccttgggacacggggagcccagggcgtgtctgtggtgtttgcctgggtgctgccatgttttagaattcaggtcaagtgtaaatgtggattccatggtaccacaaaaggatctttttttttttagtctaaaaactgacttctggctttgagaagcagtttctttgtgtgtcttggccgtctttaagtaacgcaacagaacgtgttggcctttgtctttggctgtttcctcggatgtgctaagttagagaagggcatctgttcaccaagggccaagctttgtgattcctctgagattcagacattgtgctggggaggcgggggcgctggctgccagctggactctcgctcactctcctgtccagagcggcacggcggaggtggagctgaagaagggagccacgctcaagatcacgctggacaacgcctacatggagaagtgcgacgagaacatcctgtggctggactacaagaacatttgcaaggtggtggacgtgggcagcaaggtctacgtggacgatggcctcatctccctgcaggtgaagcagaaaggtgtgtatcgccagcctgagcagcaccccggcctcaggacagcaaaggcagagagctcctccggcctcccgacttgcggggctcgtggaaggtagggaggtaggaagcttggttgtctggcggagagatggtggtatggtgagctctgtttatttgagaggtagattgacagaaaggggaagacagattttctgtctgctagttcactccccgggtgcccacggcatccaggaccaaaggcaggagccaggtctccttcgtggatgggccatcagctgtgcctccagctgtgtcagcagggagccggatcagcagctgaacgaggcgctccactatgggatgtaggcgtcccaagtggcggcctaacctgcaccacggcactcacccaaacgagtgagggagcgctggcagacaggctgtgggcggcggttgggcttgtttgcgtggccccggcccccaggtgtgcttccctggtcctccgcgggagggaggcacctgctgcttgctgctcccctgtcccctggggatgggccctggcggctctgcatcccctgctcgctgtgcccacaggtcctgacttcctggtgacggaggtggagaacggtggcttcttgggcagcaagaagggcgtgaacctccccgggctgcggtggacctgcctgccgtgtccgagaaggacatccaggatctgaagttcggcgtggagcaggacgtgacatggtgtttgcctctttcatcnnnnnnnnnnnnnnnnnnnnnnnnnnnnnnnnnnnnnnnnnnnnnnnnnnnnnnnnnnnnnnnnnnnnnnnnnnnnnnnnnnnnnnnnnnnnnnnnnnnnnnnnnnnnnnnnnnnnnnnnnnnnnnnnnnnnnnnnnnnnnnnnnnnnnnnnnnnnnnnnnnnnnnnnnnnnnnnnnnnnnnnnnnnnnnnnnnnnnnnnnnnnnnnnnnnnnnnnnnnnnnnnnnnnnnnnnnnnnnnnnnnnnnnnnnnnnnnnaccgggggacccacaccagagagagcaggcctccggccacaggaaggggggctgcccccgttcctgaccggcgacccatggggaagcgcgagggtcggggtcttggtcttccctcagaagggctggcccgggcgatgagccactcgcccccagagggaagcctggggggtcttcttcaggtccccagggctgccccagcccagcctgaccacctccgccgtctcagtgtggccagctggcccctcctagagcagtagctcgtgaggggcagggcggcagcagccctggggccccacagcctggtgttctggccgtctccggctctgcctgggcgtccttcctaccacatgagctcggctctctgcctttgctgtcctgatgggccgggctgctggctcgggccggtgatgcgcgtgccctcttgcctccccggggcatgcctgtggtgtccttggctagatgaggccgccgaccttggggtgggaagcagccagcagcgtcggtgcccttcctgggaaatgctgactggagcacttgagggcctcacagggtcaggtggagaggcggggcggggcatcccagaaggtgtcgaggcccaggagccgggagcctggccacgtgcacgcatctgtgctgtgtcgggccctccgagttaggggtcgtggccggggcttcctgtctgtcaccatacttgggacccctgtggaatatgacttctgtttcgtccctgccccctctgtcaggtttgatgagatcctggaggccagcgacgggatcatggtggctcgtggtgatcttggcattgagattcctgcagagaaggtcttccttgcccagaagatgataattgggcgatgcaaccgtgctgggaagcctgtcatctgtgccacgcaggcatgtggccctccctggggaccccgtccctgtgcacccccagtccagcagggtctcacccgtgctctgcccctcccagatgctggagagcatgatcaagaagccccgccccacccgcgccgagggcagtgacgtggccaacgcggtcctggatggagccgactgcatcatgctgtctggagagacggccaagggcgactacccgctggaggccgtccgcatgcagcacctggtgagtgcccagggccccgcttccgcggagcctcactgcacgagtgaggcatgtgctgggcgtggggcgccccttctgccccgcctcccagctcctgtccggagaagtcaccccagcttccgagtccttcgcctgagtcctggggtactgctgccctcagcagatgcctgtcgccctcctcagaggtccaggggcttcagcacctttggcctgatctggaagacaccagggctcctgcccccagctgctctgtttggctttgactggactccctgcggggcctgtgtgcacccagcaagctgcctgtgagccggccttgcatggtgcctgcagcgggaccggcttctgtgctgtgggggtgcagctgcctcacttagtccagacgacccagaggggcttgggaaggtggccagccccggtggtcctcacactggagtcatctgcaggagtctggggctgggccatagccgcctgacctcttctgtaggtgggagcccagggctggttgtcaaggccgctcgggcttggtgcaccttgagccccagtcacctggagagtggctccctgtggtctctgacgcccctctgtctgtgtgctgtggtaagctcaagcgggagggtgatgaccttgtctgaagcacacggactacagaaagtgtctctgggcgaagtctccgctctctcaggacctcgtctgtaagctggattagatgagatctacgactgctggctttagttctgataagtccctggtacactgatgtaatcctgacagctcccagcatcaccagggctgtgggacaagaactcccaggacactgacccaaagccggccttctccctgcggttcccctgcccagtaggacttagaacgaggctctgggtcccagagttggttctgggttctgaattctgtgcctctttcccttaactggtctttcccatggacagacagcttagggcgttgcaggctctgggccaggatgtggctgccctgcaggtggtgcaggccactagccggcagccgcctctcagtgtccgtgctcggactgatgcactgacccgtaactcagggctaggccgcaccaggtatggccctggctcctgtccctgtccctgtccctcgggctgcatgcactcattccatcgttaactcggcggtgctccccgcgtctgcttccgctcggagatgaaatgaatggggcggtgctgctgacccttcctcgcccgttgatgactaagccactgggaactgcattgtaatctcgaacgcttccactcgctttctgattctcagtctcacctgagctggtggtctgtggtaactcagctctctcgcgcctgttttaatcagtagctgttaatcaagcgtcctgtgacgtccccgcatgctcccatgggtgtctcttcacatggctgttcagggcggccctcgcgagctggcctgtgctgccagctctcctgcgtggccttggctgctgacgcctgcctcccagccctgttgtctgtttccacggcgggcactggggagagcacccttgtgcctcaagccaagcagcctccatgtggcacaaacacccagacagccaagtgaggaggggcctgctccttcccgaaatctgtgtcacgaggcagcgtggtcaggtccagcctgggcaggtccccatgccacggcgctagagcccgcggccatactggcttccctccactcccagccccggtatcggagggtgaggtgtgaaattctccatgccccacagctggctggacctggaccctctgcctctgcctgacgacccgattaacccggggtgccttcctccctgattaatcccccgttctgtctttccgtgtcttgtcttccctgtctcctcctcctcctctcttccttgccctctcccctaacccttacagatagctcgcgaggctgaggcagccatgttccaccgcaagctgttcgaagaacttgcgcgagcctccagtcactccacagacctcatggaggccatggccatgggcagcgtggaggcttcctataagtgtttagcggcagctttgatagttctgacggagtctggcaggtagggcccgaggccaggtaacgctgcaggggaccctgcctcttgcgccagctgctccaggatgcgcggcctgggcccagagcctctgctcagctgcaggaagacagccagggtggtcaggacagggcaggaccggaggctctgcctcggtaggcagcggcgtctcgggcagccggtggaggaacgccctcggggagtctggctctgctgctcccgggctgcagccctcaggctcgtgttggccttgctgggccgtgtcccccacccgctgtctgtagactcatcccctcccctctgacgaagctctgacgaagctctgtcccctctcgtccccctggacggatgttgctcccctagattgcccgtgaggcagaggctgccatctaccacttgcaattatttgaggagctccgccgcctggcgcccattaccagcgaccccacagaagccgccgccgtgggtgccgtggaggcctccttcaagtgctgcagtggggccataatcgtgctgaccaagtctggcaggtaggaggcgccagcgagcgcctggcagtgccctgctgcgggacacccctgcaggaggggcctgggagcggtcctggcgcagtgcgcagatggtgctgagccaaggtaagcccctctgcccaccacctgcaccctggcagggaaggatgctcccaggcccccgggccaggaccagcagtgagcggagccgggttgtggactcgctgcgtaaggggtagggctgacgacacatacttgttctttaaaagctgctccttggaaacagaagcagggttgccttttctggttcttaggacctctttgcaaacttagtctggaaaatctgaatgctgttcccatctctgccagacacaccagtgggttctgggcccaggaaggtcaccccccctttcccctcattttgtggggctgtggtgccggggttggacttggcctgagttaccctccctcccctgtggccctgggagacagcgggtggggaggaggggctgtagctgggctgccgtgtgcgaccaggagaggtctgcgacgcccactcttgggctttcgggctgacctttgtagaacggccggcttagctctgcactattcttagcggcagtcttctgagatttcacagctctgaccccagcagctgcctcccctgaaggccaagcctgttcctggcacctgttctgtcttcgcagcttgctcccggggcctgctccttcgcgggcccctccccagctcctgcagggcccctggcacagggctcagcagagtccccacctccagggtcccctgacaggcggagctgcccccatgcccacctttctctcatcacgaagcccttacctgaatctacacaatcttaggagttaatctttggttaaaaaatcttttttacttatttgaaaggcagagttggagaaagggagacaggtcttccccggttcacgccccgaatggctgcagcggccagggctgggccaggctgaagccgtgcccgtgtgggatgcccatgtccctatgccacaatgctggcccccccgggaatttttttttttttttttaagatttatttatttatttgaaagagttacacagagaaagaagcagagagagagaggtcttccatcggctggttcactccccaattggccacaatggccagagctgtgccagttcaaagccaggagcttctgggtctcccacgtgggtgcaggggcccaaggacttggggcgtcttccactgcttccccaggccacagcagagagctggatcggaagtggagcagccgagactcaggcagtacccttatgggatgtcggcactgtatgtggcggcttcacctgctatgccacagcactggccctttgggaattcttaagatgcctccggatcttcaagtttgtctgagatctggagcccagttgctggggccgcttgggtggacgagcccggcagtggagggtccgtgtgttgctgggcccagggtctggcagctgtgctgcggctctgcagtcaggctgtgggccacacgctgctccgctgtgcttctgccggccccaagacgaggccctgcactagggctgccaggtggagggagcaggactccctctgccatagtggaaaagtccagggtgtggcaaggcagctgccagccctggccacgtggggtcagtggatgagatggggcggctccctgccctcagaggcaccagagagcaggtgtggaagtggccagagcttcaggctggcgtagtgagttggattagggggtgagctattgccaaaggcccgggggggggggggggctccagggacactgcttaatggtcgtcctgcttgtctcctgtcccaggtctgctcaccaagtggcccggtaccgcccgcgcgcccccatcattgccgtgacacggaaccaccagaccgcccgccaggcccacctgtaccgtgggatcttcccggtggtgtgtaaggatccggtccaggaggcctgggctgaggatgtcgacctccgggtgaacttggccatgaatgtcggtgcgtgctgggagcaagactagagacctgaggggcaggatacctggctactggcttctgggaccctgaagcctggggaacataacggggggaaccccaagaccagagaggccaagagacctagctgagcacccctggtccccactggggatgttccctgaatcccactgcttgccagtcctgagcagcgcccgggaggggaggggtgccatagctcgcagccacagtaaaacgcctcgttctgtggcagtgctctgggggttaaggtttatgtcatttatttgaagggcagagtgcctgagggggagggagggaggcaaagatcttgcatccactggttcagtcctcaaataggcgcaacagccagaaggccagagtcgggcccagagctccatccgggtcccccccatggatggcagaggcaaaggcatttgggccaccttaggatgccttccctggctcgttggtaggaagcaggagcagcctggacaggggatgccggcgtggagtggcagcttaccctgctgcaccacgctgttggccccgctgcccgggtgttgggagaggagaggagcagctggctctgaccttaggcagtcttaggtcgtgtccaagtccctgcccactttgtccccgctgtgaggctggcgccaccttgtggagggtggaagtccctcaccagcttctctcctgcaggcaaggcccgcggtttcttcaagaagggagatgtggtcattgtgctcaccggatggcgccctggctctggcttcaccaacaccatgcgcgtggtgcccgtgccgtga

SEQ ID NO: 52 - DNA, 17257 bp, Gallus gallus
agcggcggcggcgctcgggcaggacaggctttgggcacggcggcggaagcagcagcaggaggtaacggcggcctccggccccgcatagggagggcgttgaaggagggcggcgagcgggcagccgaggccgccgtcgtcatcgccggacccgacgttcaggcgggagtgttacgttcaggacagggcgctgagggggcgctgaggggagggggcggctccacgcggttggggtaacggcggcgctggcggagggatggatgatggatggatgatgggtgggtgggcagatgggtgcccgcagcgctccgcccgcccgggctgagtcagccgtcggcgccacggccacgtgctggggccccgctcggctcttcccgaggctcccggctctcccagccccgaggtcccattcatccccgcgtggccgcccaccccctccccccgccccgccgcgggccctgaagcgctcggggtgcgtgaatggggcttttgttggcgcacggcggccgcccgtcggggcggcgaggcggcgtgcagagcccgcttcgtgccgctccgggtcgcacagcgctctgtggggagcgggtggtgcgcggggccgggttccggcaccctcctcctccagggacggctccagagcacgcgctggcaccgggccgttgtgtgtgtgtgggggggtaaccggagaaccgcaccccaacgcggggccgaaatcgccgccgtcagtacgcggctccaccccgttcccggagcaacgctcggacagctgcgagccgtggaggagcggccgcgcccgcgcacctcgccgtgccccggggctgagcgccgcgaccacgtgctgccctgcgcggggtgggggcggggcggggcgccgcgctgtgcggtcccgcacgtacggcatggactgctgcgggggcttcctggggtacggctccagagcgccgagctctgattgctgccgttgtgcagcgaagctgtctgacctgtgccggcgcagcccgcagcgcggtgaggctggaaggtgtgcacgcttcaactgtactctctcgataagtttgccgtctgttctttaatcgaagcctgctccgtgcccttgtcctccgagaagggcagacgcagcatagcaacacgtagtgaaggtgcccaacgctcatcctccgcctgcaggctcagtggcccatcccggccggccccacgagggctgacgttgggaggccatcttgcagttgcataaggctgcggcgcaacctccctcccgcagtaggagtcatccttcccccccccccctccacccccctctctgcaaggggggttgccgtgttggcagcctgccgtgcgcccagctccatggctgtggggtggggatggcggtggggctgtgcctctttcctgccccggggtacagctggaatgcctcagctagaggttccgtactgcaactcacactgagtcaccccgctgccctgcaacggtcctgcctttctggaacgttcagcggccaagggaggaaccggccatcttgagcgtgccctgcctgaaatggggtgataccttggggggatttaagagttacgccccgagaaaggaaagcagctttgtgcagggaatcaggctttgcaaggtattactccccgcccccttcctggctcagctcagagtgccttcaggtgttcctgagaagctgatttaaaaaacaaaaagtgggaaatgccagacattcctcttagggttataaaaccgccctttgagcatcactccttgcagatgggatgcaggaggaagcacaggaatgtagggctccctgcagcccagcagacggtggctggggtttctttcttctgctgctgcgtttcttctctccccctcgggcaaggtcacagcatcgcggcgcctctcatctccttgaatttgctgaaaaatctcaggggattctgactcaaagcagttttaactctccttcctttttatacaatcgtaaagcctttggggcttgaaaatcacacttacaaatgacttgagtgggtggggagtttccacggggaggaagctgcctccaaagcagggaggctgagttgctgcccatctttctgggaacatatgagtcgcactcagtgcttgtccctccccacaccccattccccacagccacgcgggcccttttgctgctgtttgcagaggcagtttcccagcagaggccttttgcactgtccagcaggtgctccaggatgcgccagcagatgttagagggctgaaacaccgtgttcaggtctgagcagcgggcatccccgtaataaggcgcctttgttgaggcttttatgtgggcaggctttcttgtactgactcgagtgaatcagcagcttctggcagggctgaggtgaaggacgcctgccaggacaaattatggtttctgctggcccgtctttgcgctccatttcgcgcggcgatgaggcgatggtgagtcagggctgcctgcgagaggattggcacgtaggtggggggagcggccggcgggggacctccgtgctcatgctgttcccttctgctcagcccggctttagtggagctgctggtttattaatgccctgtgcagctggaggtgcagcgtgcgcggtgagctccatttttgcgacagatggagtgcatccctgcatggctcagtgtgccgatggcgttctgagcgtgagcggcccccatccaaccgtggggagcaatgcactcgaggtggtggcagcagcacagcaagaagctgagccttgcacaggcacaaagtcctgcctcacctgggtgtaaatgcagaaggaaggtgtgcagggaggggaacatgggcagctttgagctgtattgctgcttgaggacaaaattcctcaattcccccccctcagggagggggaggaggggggggattctcccattgcagcacacgtctgtgggtttcactcagctttcttatagggtcgggaccttccctgctgttctggggatgctttcatctcgtggaggcaagcacggagtttcttactcccagaatcagccagtcttgagccctgtggaggcttcctgccccctgcaaatgcaggggctgcagtagactgcatggtgtcttcgtttggaagagggcacttgaggacattcaaggattctttagccttattcgcgtttgtctgccccggtgttgtgttcaatcaactcaagtctgattatctgtgcaggcttaaaggccgggttaagcctaggtgcacttggtgtgctgaggtgtgtccccgcgtgcagcacgcctgcagtcacgctagcagccggctgcccggtccccaggctgctggcagagatgggctgagagcgggcagggagcgggcagcgcgctgcctgtgcactgaagcgcttgaattttgttgcgttgtgtagctgcaggggaagactggcaatgaagagaagctatgaagggaacttctgcatagaaggcaggtgagctttgggtggcatccgtggggaatgacatttaaatagaagtgtgtcttgcctgtatctaagactctcaagtaggaacataacgatagtctgacccagtagcagctttcttgttacctccatattcatcacgtgggtgtgttggtgtctctgcatggtgagcgagcaggggcaatccctaaacccggcaccgttttcttctcttgcagacaccgaactccagtaaccatgtcgaagcaccacgatgcagggaccgctttcatccagacccagcagctgcacgctgccatggcagacacctttctggagcacatgtgccgcctggacatcgactccgagccaaccattgccagaaacaccggcatcatctgcaccatcggtacgtggctcccagatcccaggaactgtggctcacgttaggctgtgaacgcctgcgttggtgaaactcattgtgggaatgtgggatggcttcagccttcatccgttgccagggttgtgtcttgtctgttgaaacaacacaactttcccatgcctgcctgcccagttttattgctaggggtaaatcgagcgatgtctgaactggttgggttcagatgtgctccctaagacaaggcaaaggagctgctttcgtgttgagcaagtctgtatccactgtgcttcacttatcccctccatgtgaaacagcctgacgtttgtgggttatctcattatttatatgaagttaatattcaaactgtttcctccttttttaggcccagcctcccgctctgtggacaagctgaaggaaatgattaaatctggaatgaatgttgcccgcctcaacttctcgcacggcacccacgaggtaagggtggggatggggctgacgctgccctgaacctgtaactgctcatcccttccttcccttctgtaagaggagaccaagggaaatcgagcttgctgcagagcagctgtggtagtgtaggaagacagaactttagctttatgtgtgggggaagtgtgccagctgtaaataccaagcctgcaagactgctgataagatttcagtgctttctggtagcagcttgagttgtttccacacccttctctgtacctacctctaccttgggagtcaggtagctgatatctgaggcccttcacttctttcccccctcatgggggagtgaacttgcatttcctttacaggactgctgctcctgagttacttgtgcacccctgcaggagtacacaactatcagttgttcaccctgcttcactgttggaggctttgcaagcggtcagtgaatgaccttgtctcaaaatataaatcatttgaagtaattactgtgtgcatttgaaagaattgagcttctggacttgcctggctagccagccgctcaggttatgttcccagtagtcatgaggctggttgcttgtcacttggggggcaataaacctctaagactaaggtcagaagaaatcaacactgcttgtggtggacgagccctttttgatataaatagatgagatcctcagcaatgctgcaggagcaaaggatcccattccagggttgcccagaatgtcatccttagcgttgaggctgagttcttacgctggctgtcctccagctttcaaaatgtcaaactgtaaccaaatgacagctgtcggtggctttacttactgaactgtgagccctgaggtgcgtaacagctcgacctctcaccctcatggcctttaaaggccacagggcactgcagaaatcaaaaggtctagtgtttagctgcgcacagccgttggaccatgactgtattagcctgtggtagcagcagtgtgcaggctacagctgaccaaaattccaatgcagaaagggccgtatggaccaacttcacccctcagtggtcatgtgctgctacacagccagcaggctcagcaaagagttggtggccaagcttgaaccttcttagctgtcttagcacagtgctgtggttggtgtgcttgttagctgaggtgaagggcacggaatgtggcttggctttgggtgtagtgcagctcaattgcgtatttggtttagatggaggttaggtgatggcagttggtcatgctgcaatctcctgcctggtttgactgccagctgtaaccaggcaagtctgagttcccttctggttcctcaagcactccgttgtccgcgacggttgcctggggttttcatgtgctgcgcttgtttcagttccagtgttcatcctaaagcacatcatggggctcgagttagcaactgcaaatagatgctagaccttgaagctctttcatggaggaagtctgctttacttaagcccctgtcagcattcctgtcacatacgtaattctcaaggaagtcacactccctaggagccggtcattgatctgtatcaagtcacaaaatgccccaggtgactgggagcagataagccccatgactctgctcagatatgtttcctgtgctgcccctgttacagctgtgatgtgtggaagggccaggtgcctcttcagtctccggttgtgcccttgatcagtaaacttaattttttctgctcttgagagttaactgtggtgtatttctggctgagggcatgcgcactgacctgagcacagcttgctgcagctgcaccttcctgatcccagggcaggtgatgtgagggcagccaggtgatccaggctgcatgctgtcagcccgtgccacagagaggggaaagggcatttcttatcttgaggagcctgccaagtattgcataactctgtcaagcttatctctagtgttgtttaaactagatagcaacctgacttgatgatcatctgaagcttgtttgagatgattgggttgggaatttccttgtgaaactgtcctgaaattggcagcgctaacaaaatgctcttgcacatgtggaagggttttggactgtggtgtgcagtgacagagccttggacttccggctgcagttgctttagctctcaaaataaaatgcaaatacgtaaagggataatatcctctgagaagatcccttatccctaggggagatttgagccagagttgtaaaagtgtccacccgtatgcctgacagcagagtccttgttttggtcatgcctgtaggactgacagagggggatgaggtcgaaaggctttggggcagtgtggcaccttcacttttaagctctgaggggaagaggacagcagccgtgtgcaactgtcacttagctgtgatgctttctcagtgttcagcccttccacacatgtcagtcctccagctgctgatgttttatcatgcttgagtagtgtttgggctatgtagcacaagcagtggagtagaagtgggctgaaagtttccctttcttttccagtatcatgagggcacaattaagaacgtgcgagaggccacagagagctttgcctctgacccgatcacctacagacctgtggctattgcactggacaccaagggacctgaaatccgaactggactcatcaagggagtaagttgctctttttatttacccccacccccagtgcctgagactagatagtgttgttcccatggcctgcttttcccaaacaaggattatcttatgagaacaaaataactgtttgctgtgtctggcatttgtagcaagagtctgcacagactgctgcaagctgggggacagctgggtgcttggttttttttctgaaatccttgttttgacatgcagagtggcacagcagaggtggagctcaagaagggcgcagctctcaaagtgacgctggacaatgccttcatggagaactgcgatgagaatgtgctgtgggtggactacaagaacctcatcaaagttatagatgtgggcagcaaaatctatgtggatgacggtctcatttccttgctggttaaggagaaaggtgtgtagcaaccctcacaggatttgctagctctgcctgttcattcttccctaagaatctttgtgggtttttttttcacctccagaatggttcattaagttctgtattaaagaaattagcactgagatctaagacttactactgctgtaaaatgttgaaagtttggagaaaaaaaaagttgctcagtttggggtaattagcttgagctgacattcactagtcatccaaaaccccctcttacaggtgaatatgtgggggacacgcttatgcttatttaactatgttaattcatacttccttctcagagttgagcaaattttacaacattaaaacccagtgttttatggttagaagctgaactagctttactggtaatgcaagggaaagttaattccccagtgtttccttcatggtggttcaaaaatctgctctagcctggaggtatctcctgtaaccccagagcgtgcaggtgaggtgctgggatattatgggatgctcatgtgcagaaatgcaacctgctagttcttggagggaggcagcccccgtctcctgcatggggggaaaagaggcatctttcccaaaagcagcacagtgggtttgtgctgtgctgccatgggtacattacaagctcacatgttatgggagtccaaggagagcagtgttgtgcttctgttgtgattgctgtaaacactgtggttctcaggcagctttggcaggagggggtgtgggagctggtggtggggagctcgccctgttatgctctgactgtgggaatacatctgtttcaggcaaggactttgtcatgactgaggttgagaacggtggcatgcttggtagtaagaagggagtgaacctcccaggtgctgcggtcgacctgcctgcagtctcagagaaggacattcaggacctgaaatttggcgtggagcagaatgtggacatggtgttcgcttccttcatccgcaaagctgctgatgtccatgctgtcaggaaggtgctaggggaaaagggaaagcacatcaagattatcagcaagattgagaatcacgagggtgtgcgcaggtgagctctgcacgagtggcactgcaagtccttcactctgtagcagcagaaggacacagccctttaatgctgtagatttctgaggagctacgtcactctttgtaatgagtgtgagttcagacttcagcgttctggatgcggactggtgagctaatgcatggaatcaccaaatctgtgacaaactattagactgaaatgtctcagatgaactcttgctcctcttaatctgtttatatatagcttaagaaactgtcctatggcttgaccttgttttcctacctcctactgtggtattacagggtaccaaaatggcacttggaaggtcagtgtgccgatagggtgtctgcgcatcaggctctagagtggtgcttcctttcagaaaaggggggacagagcagagggtccaccctaagaacaaagggagtaatgaatctctcctcttgttgtcaggtttgatgagatcatggaggccagcgatggcattatggtggcccgtggtgacctgggtattgagatccctgctgaaaaagtcttcctcgcacagaagatgatgattgggcgctgcaacagggctggcaaacccatcatttgtgccactcaggtgctcagaacatgaagctagcttgtataacggctgggtgtttgtgggtctggcagggtgtgagtgtcagcagctgtccttgcacgctgaggagattctgggggcaggtccttgatggcacttgctattgggtgagaagcaagagccaggaggtgttgcggtggctgaacaactcatcttcaggcaattcagggatttaggatcttcctctttaaggtttggctgctgaaggctctaccctttgaaaccttgtactatgcgagccttttgagctgtgaccaaacacattttggggaaaaataacttgcactttgcatctcagagcagcacatctgtgcctaacaaaatgattgctctgagttgctgtgtcccaggtcttttgaaagttgcacccacgctgctgcattagaaggaactgaaaaaacaatataatcttaccttgggagctgcaagtgaggggaggaagctgatgctctgcagctttagtacagatcacaaacaggcagtccttaggcactggcagggctgactttctagaagtacttgctctgggcacaggctgtgggaatgtgtgcttctggtagggtagtgcagactgactccaggcagtcattagttgagattctggatgtaccagccacatgttcccaaccagaacagcacgttagtagcaacctcagaaagggacgggaacatgcactgcaatgcatctccaagttgagttccttggaccaagccctggtgttgggaatttgaatcagaaagtgagaatacagtatctgtggtgctgtgatttaaatcccttcagaaaaggagtaagtgtagagtggggagaaaatgttggcttttcttgctttaattcagaggttgttagggagcaggcccctcttggccctgtaactacaggagaatgctaccagaggtcaggttatatcctgacttctaccttatgtgtgtattgaggggccttagtggaaaatcagccacttcttcctgctgtatcctgactcttggacttgtttatctgcagatgttggaaagcatgatcaagaaacctcgcccgacccgcgctgagggcagtgatgttgccaatgcagttctggatggagcagactgcatcatgctgtctggggagaccgccaagggagactacccactggaggctgtgcgcatgcagcacgctgtgagtagccatcctggtgcaagtggcagtgctctgccttccatctgagtccacacataaagatgtaaatacctggtgctaggtggcagcacctagtagcataaagcagcagttctttagttcaagctctcagcatgaggtttacttcacctagtgtggaaccttggactgaatgctgtgtgctactgtcaggtggagctgagagctgctttgcagtgctcagagacctaaaacctcaattataccacattcattttgatttaaggccacggtaaaggctttttggctgctaccttggtatgaatttctttgagtgccttgtgcattttagtgttttaaatgctttaaacttgcccaaggtcaggacgctgcttgttaagcagtgtatctctagataaaaagtgttagctgactcctctgggttaggggggggagggggtgttgggggttgggagagggtgaggagaaggcttgaggtgttgcatccagcagctgatgcatttggtggtgggaatgtttgttgcacgaatgctgacagcaccatgtttttacatgcctgaactgccagaaagctctgctctgcttcatgttaacccagcttgtgtttcagttcatcaaaaatcctgatgcaaggcatctagaagtactggatttccccacttgctagggctgtgaatcacgttagtttcacctgcagctcaggtgatacatctgaaggcactgagctagcgtttctgtttgcagtgcattatctaaacatcttttacctggtcagtatggagtgctgttttctcatgtggcaaataaagcatgaccttaactactgggcagtgactgctggcttacaagctgaattctaactgtggactcaaaatgttcttccttagtctttcagtcctacattgagggctgaatcttcctaccaaggtttggaaacttagtgccatgaatattgcaattttggcctgaaagcttagttaagtacagcacaacctgtctgagtttgtggctctgtaccccccctgcatctgcaaggaacttttcctgcagggctggggataatggtgttccttctttcaggcccccagagatgaactgtaagtttttacctgctgtgcagaggagcaaatccagatttatcttgtttaatgtacataggcacaggcagcaaggtcatcagcagcactgaaaatgagcagggcctgcacctttgcaccactgaaactctcccagggttttgctgggttgctgcgtggtttcacaaagcaatcactttccagtgagctttgcagcaatgagctttctgtttcctgactggcatctctgcagcaaaagaaagtgcttggagttcggcagcaagtttccaaatgttgggcaggctgattcctacttcttggagtgggcttccttccacttccagctgacgatctgcagttgtcaaatgctgacatggcccttctgtctaacaggactatgatgtgcatagctcttccacttcctttcctctcccttccaccctccagtctcttacctgcatgccaactacaaacacttaaactatttccatgcaagtgaatccagctgtgatgtgcagcgagtaattgctatgccctcctgaagtcattgtcagagcaggcacttgggcacacacactgtgactctttacagtggggaagtagccttcccactaaactcatgttcactctgcatgtagtgcagagctacctgcctctggcctgagcgctgaaggtgtgctgcctgcctgctggtgcctgcagagtttttaggtagagaagtatactccatattccatttgacctaacagtaagtgtgaagccagcagaaacaaaactgtgtgctttaggaccagtgtgttggctctggactcgtgttcctgtctgtcacgtgtcctgttatatttagacataagacacttaactactttggcttaaactgatatcagtggaagagggataattccagcatcacaaaaaataatctattagcaccagagtagcaaaatttctattggaagagggatccaagtacagaaattccatgacaatggcactgcagtctttgctttaacatcagcttgttgtgcagtgtgtggcggctgttcaactttgggagtaaggggatgaagtgtccttgagaagatcggcctttgcatgcttttctagtctctgcaagccttctttatcaggttgtcaaggacgagtgcagccctttgagatgggaattgtcttttaatgtgagtgattctcatgctactgggatgaataaatcatgaagcttgttgcacatgctaaggctgtgaccaggaggcctttaattgtgcacctctggcctgtttgagcctggcataaattcttcactgtacgtggtgagacagccctgtaaggaaggcttgcttctgcttctttcctctgttactgaaagagaagttggtactgcacttggaggtgaaacttctttggctcttagttgaactagatgaaacctggaagggagcacatctccctttccagggaagaactaccaagaagtgaaataagcagccacaagaaagtgcagtctgaggggctatgctgtaagccctgaaaagcgagctgtgtttggttgatctgagaagagtccaaaatacagcaagagtgctgccattaaaacacctgccggctggatggtgcggggcggccagtgcagctgtgctgtgacatgcagcattgcacctgggagccaaagagtgttttgcaccctgaccttgagtatcctcttgcatgcattactatgacaattaagcaaattaacgtgatctcatgttactctggtctacctttccttcttttctttcctcttttcttctctgcccttcttcctcgggcctgcagattgctcgtgaggctgaggccgcaatgttccatcgtcagcagtttgaagaaatcttacgccacagtgtacaccacagggagcctgctgatgccatggcagcaggcgcggtggaggcctcctttaagtgcttagcagcagctctgatagttatgaccgagtctggcaggtagggctcagagaagggagaggcttaggctgcgtacggtaaccgatgctcgctcccagcatgcgggttagatatgtgctgcttgccagtcactgcgtgaatgagaccacgcttaacattgcaggcattcagcaagcagcgtgcagctctggtatctgcagggcagggccgcaggtgggtaggagcagagcaagagtgcctggcagttgggcatgaatggcaattgagtgtgggctcagcagggtgaggtgccgccaactgggggaagaaaaacttggaggatcaaattgcttgttcattaaggtggtgctgaagccaattttggctcattggcaactcttctgaaagcctgaagctggcagcagctgtgtgacacctctgtgacagagcacctcaccctgccctgtgctgagtgactgacacgagtgttgtcttcccgaatgcgtgtcgctcttctagattgcccgtgaggcggaggccgccatctttcacaggcagctgtttgaggagctgcgtcgcctgacctccctgaactgtgatcccaccgaggccgctgctgttggcgctgtggaagcgtccttcaagtgctgcagcggggccattattgtcctcaccaagtctggaaggtaggaggccgcaggctccctcgggtcacgctggctccgtgaccgagttgggggaaggagacccacacagagtgccttgaaataaagctgtagcagcggagcccgggttctggcagcgacgattccttgggaggtgacagacatgtcaaacatctgcgcatacgcagcaccgggttcccgagcctgccagcgtggcatcggcaccaggccctgcctcttcctgttctgcacagcacctctgccagcagcgctggctggaagagttggaggggaaaagtaaactgctgcaacttccaacttcttagcaagaagtcctcaagttagcagtagagttaaaagttcagcagatgcagaatcttttcctttcaatcaaggctttgtcctcttgaaggagctgtagtttggctgctaccctgctgaacctattgggtgccagcccagctcccctaagcacaagaggggtgaagagaaaatgcttaactagaactgtcaggcagggggagtgaatgcgttgcaagttcttacgggcttcctgaggccttcccgtgagtagtcctgcagaagaagcaggcatccagcttctgcactgccagctgagcccagcactgtggtttcaggtgaggtggtgatgcagactgagactatgtagggagggatttctgaccagccgtgctggtaatgctgctcttcctgttgagtgggagcgaagcacagggctgcagcctggctgtgagcagcttttccatctagagaagccatgctcaaagcgtgttggaccataagtctcaagctactttctggaagagaagctgagtatcttacctggagctggcaacagaattagtgctgcaacggaaacacgaccgtgtgcgtgctgggcatggcctacctcaagagcccttgagtgaacccttaacctaaacttacagcttagaatgatttgaagcagccactttgtgcagagatgaggaacgactacatgagcactgagttgtggatacccttctaaagtttctttgtgaaaggttccagtcttacacttgacctttttggaaagatttgaactctggtatttgaatatttttagctgtggattctgttacagccttggagtacctgtgtctgttagagctgctgggaggtttggggaggattgtctgagagctggcacgtgtgactgggggcttctgaaccaggttcttgctgagcttggctccagaaagcaaggtttgcaaaagttggcgaggctgctggcatgcgtgtcagaacgacggagctgtaaatggcatggctgtgcagcttctattcatttatttatttttgcttctacaagcagagcccaagggaggggaggctgtagttgccacccagcgcatgctgcctgctgtatggaggcactggtgtctctggtcactgcatgtgggtggcagcctccttcagagcaacccggtactccctgctctaagaccaaatgaaggcacttgcttcagtgttgctttcagcagtgcttctgcttctggggaggtgggaggatgagcacgtgggattaaatgttggctgctcctctgggacttaaacccattggtgagctgtggtcagacccatttttgggggtgactgcctttccctgacatggattctgccctctggaagcatcctcctcacagtgctgctgacacaggcttgttccacctcacaaagtgggggttgacaagaatggtggaaacttgcagggaccctgctgagattccaaggagagcttgcagaggacagaataaatggcagctagccaccttcacatagcaacagagacaaataaatgcttgtgtttggggccaaagcatgccaatggcactcaggggtgtgacagtctcccccacaagactggttagagtctgttgccttctgctcttgctcagccccattgctaaatagagaaatgagcgttgagctctgctggtgggactcggctcttgcaaaatactgtgccagcatcccctggtcccaacctggcacacttccagaagtggcagagctctccgggatgacgggctgagcctcgtgctgcaggcaggggtgcccctctggttgtgcctgcgctgcagtgccgtgcctcaccctgtgcctgttgtccttcttgcaggtctgcacacctggtgtcccggtaccgcccgcgggctcccatcatcgccgtcacccgcaatgaccaaacagcacgccaggcacacctgtaccgcggcgtcttccccgtgctgtgcaagcagccggcccacgatgcctgggcagaggatgtggatctccgtgtgaacctgggcatgaatgtcggtgagtgctgcgctcctgccttgctctgggggctgcggtggggccgcagcaggacctgcagcacggtgttggcgctgctgttgggatgcgggggaccgaggttgcataagcgcaccgcatctaagggggaaatgggacggtggttttgtcacagcagccttgaaatagctgcctgcagaaaaccaggtttgctttaataagcgagagaaggggggtgtgaggagacctgagtgctgacgctttttcctccttttccccaggcaaagcccgtggattcttcaagaccggggacctggtgatcgtgctgacgggctggcgccccggctccggctacaccaacaccatgcgggtggtgcccgtgccatgagctgccggcgcccccgcctcttccacccccgcgccccttccccatgcattaggccagcagtcgcttgcgatgttctcctcgtccctagcgtggatttaggttgctcaacaccaccgagtgcagcagcgggggaagagaccttaaatcactcagaatacttgaagtgtgtagttgtttccagacctctctccctgtagttagccatgtcagagcggggccctgtgctccccacgtccccctagcttagcactgccctcagggtgtggctgtgcctctccttgccccggctgtggggtgatggggaaggagtgggcgcttatggtaacggttctgctgctgcacaccgcagctcccccaggttggtgccctctgtccatgaggggttataggttgtcccctctgggcttacactccaaaggtgtgctccacggttcctacaagaatcccaaaccagggtgctgctcgttgtccccctgggtgcaggtggagtcctgcgggttgttggggtgcaggatgggtgggggacgcacgcttcatctccatgcagccacctgcccttctatggtgtctgtctgtgttgtcgcctttcctgagagcgttccttttgtctgggcgccctgtttgctccggtgggtgtattgggttgtggagcaccactgtgcacgtcaataaagagctgagcacccctgc

SEQ ID NO: 53 - DNA, 60974 bp, Sus scrofa
cagagtggctcagcgcggccgtgacggaacgacgaggcgtgcgggtgcgcgacctctcccgcccggccccggcccccgccccttggcctgccgctccgcccccgcggggcgtcccgggccgctcgtcccctcagcggcggccgcgcgcggcccggggtcgccgtgagtactcgcgaggccagcttgtggggcggccgccacggggacggggcggggcggccgagccgcgggaagggtgcggggccagggtggaggaagtgaagggtttggacccggtggctctgagaggccttctgagtttaacaggcttcgcttatggccgggcggctggcgacacagatcgggctcagagcttcttccccgggaggcaggtgttgggtgtcttcggggtctccgggggaaaccggagaagagctctaagtgcttccccaagggaggcctcagtgagggcctgttctggaagcacgagtggcggccaatgttgggggctcaccccggcctcttcttccgccgggtacacgagatagcgctgggaagcgggcatcgccgggcggtgggttctcccccgcactctttgttccatggcctaggctttttgaaaggagcacttcgctgcagagcggagtcaccttctttcccaggaccgccaagccgggatcaaacgttgagatcggaggcttctttgactagatgcaaagttgtcacgcggagaagcgcttttggacctaggccaggacatttgtgatccggacttgatgcttatttacttttggcctattcttatgcaaattttttgttagctgctctctagcgctgacacccttctctgggcattcttcatacagtcagtatttgacttggcttttcttgaaagggttcccttgattacctcgtttagataaatcaaataggtctttcttactagttcattaacagctcccttaattgggttgtaatctcatcactggaagagtggatgtcattagaatctgacaaatgtgctatagtccccagttccactgtacgctattatacttctgaccctaagcaagttgcttgacgtccctgcacctgcatactctatctgtagtgtgaaaagtttaaaataggttatatacagcctagtttgaaaaagatggtagtctctaaattgtttcttcactggacaggaaaaattctctctgaactacttttttctccttgtggtaacagcagaaaccaagcagcaacagcccttggagagagactaagctttcttgacctctacagtggcacagtggcaaagagcttgagaaagttggcacttctgggctacaccattgtcatccaggacattaatgcctccctctttgttcctctgagaccgtccagatcagcacctgtttattttcaaatctcacaaaccccaccccagatcttcatagtttggttctcagctgctcttgaaggtgaatggagtcttgctttttaaaatcatttttgtatggttttgtctatgtgtagatgtgtttaggttcttgtatttatctcccctttggcttaggtcacagttcattcattcattcactcattcaattagctatgttatgagggactgacagtacagacagtgaaaatgctcaaagcctctgccaccgtagagcttacattctgatgggaggtaaatacaataaacaaacattttgtcatagagtggtaagtgctgtaggaaaaaataaagcaaggaaagggtttggagagtgctagtgtgttgtgtattgtgattttactgttttatgtaggatagtcaaggtgatcttcaagcagagatctgaaagagtaaaggagcaagcccagtgaatatgggtgaaaagcattccaagaagagtggcaagcaggcacaaagaccctgtggtgggaatatgcttgatatgttggaagaacagcaagttagagagtttcagtgatactcttcatttcacatttagagttgataggagactccttaaaaagtatgaaagtagcctctgggtttgtttgtttttctttttagaatgaaaatttccaactatatacaaaagtagagagtttacaaacccttgtgtacttatcactcagcttcgtttgtaatcaacattttatgattttcatctgaacatttcatctgttccccattttatttgtgctggaatagtattttaaagcaaatcttggcgttcccatcgtggtgcagtggaaacgaatccgactaggaaccatgaggttgtgggttctatccctgcccttgctcagtgggttaaggatctggtgttgccgtgagctgtggtgtagttcgaagacatggctcggatctggcgtggctgtggctgtggtgtaggccagtggttacagctccaattggacccctagcctgggaacctcaatatgctgcaggtgtggccttaaaaagacaataaaaaaggaaatatttaaattaagatttgaatatttaaagatatcaagcatttcatctctaagaacttcagctgcagtttccttgtgcattttgtttgtaatgggtcaggcagcactgttggctgaaggactgctatgttgtttgccctggcattgtgctttaggtccccattctgggtcagttaccaggtttaaattggtatccgaggaacagaccacaagcccttggaacacacaaggatttagaacagtggtctcagattttatcattcatcagaataacttggagggcttgttaaaacatcccatctctgaagtttctagttcagtaggtttcagtatgaggtctgagaatttactcttttttttttttttttttgccttttaggaacacacctggagcccatggaagctccctggctaggggtcgaattggagctccagcttctggcctatgccactgccacagcaacatgggatcccagccatgtctgcaacctacactgcggctcatggcaacaccagatccttaatttactgagcgtggccaggaattgaacccacatcctcatggatactagttgggtttgtttctgctgagccacaaaaggaactccatgaatttacatttttaacaagttcccaggtgatattgattctgcagatccacagaaccaaggatctagtaacctaagattcaatagaaccatgttacagaccaagaacatctctctttaaggttgggatggatgaaactgagataaatgtagagccaagaaggccaaggacagtggtttttagttttgtgaaagggctaggagttagtgtttttctgagcatttctttggatcattattacattaattggggagtgggttccaagatgagtccatggctttattttgactatgacaactcagactatgagtaccagagaatggtcagtgttgttgaggactttttaacttggctctgattgttatatgatgtctttgagggatgctagtgttaaataagagattatgactaaatcaccaggggtaaagactccaaaagagtctgcttctgatgggcgttggtactatgaagaatattctaaaatgaactgactagactgagtagcataagcgtctggttctgccaccatcacttgtggcgtcagaggtttgatgcagcattgtgaactagagcaaggacgtgattcaatcccagccttccagcttaattggaacagtagtatcttatgtttgtatagtgctttcatatttcattatctttaaagaactgtgcgtacatgcattcaagtatgtcttcttatgtgcaggtgcctacatgtgtataataaaaatatatgctaacgtgtacctgtgtatatgccccctagctgttaagtgaggatgaaatcagttgttttctactttccataggacagcgagtgacttattaccaccaccacaacagagcctgccttctccagcagatctccagtcagctcccgacatcatccccacccccttctcccttgtggcctcctaaatgcccatctcgttagcctgggttcatccggtggtatggaggggtgctgcctagcactgacctggaagtgtgtgtgaccctctgacccaatggtgagaactgattgcccacttcttcaactgatcactgggggcagatggaacagactgcagaccaccttttcctagtattttccttcccaccctttgggaaagtagagtggctatttgaagttagagagaaggggcatgggaacagtcttacttggtgtctacagagggagttttcttgggaaggaaggggagagttaaatacttaagggataaaaaaagggaattatgagacgaaagagtttaggtaggctggggagctgccttaggtaatgaccctagaagtggccagtatgtacttgaacctagatatcctagaaattaactctgacatcaaagtgctcctcaccctcagtcatcataccagtatttaaagaaggccaaaattccctgttgttttcttccatgccaccaagtcagtgatgggccatggatgtgaccagatttaggaagagactgagacccttccaaaagataaggtgaagggaacaaggggattagggcttcagttattctgttccaagagacctcccgttctttgtggaaatctgtttcccatcttaatttgactgtgttccctggaataacacggacccagcaaagcattgtacccttatttcttattaggacatcaaaggccagttctggaatgatgatgattcggagggagataatgaatcagaggaatttctctatggagttcaggtgaggtcctagcccccaaaacccatgttgcatgatctaaatgtgtgtttctctcttgatacattggaagtgaaaaagattgttttggagcagagataagatgaagacctaatgttggtgtggtctgaggattgtcatgttagagctaatttcatatctttgctcttgcctgggactcatacttttcccagggtaaactgcatcctctgtatgtggagcttactcatatgtttagttggaaataattattttctgactatttcctcgctagccagtgggagtaattttattcattagcatcagaattttaacagattattctgccagtgattggttaatgctgtcactgtccagtgcatgatcctgaacaggaatgttggacttttaaagtcagaaccaatctgatttaaattctgtactcttcagcatgttctgagttctcatagaaaagatacctaagtatcctggtcaaggtctgagagaagagttgagacttatggatgtgagctccttaagcaaagccctcagttggtctactgaaaattcttagagtggtgatggagatccccatcacctgtctctcagatccccagcaagagccaccaccaagagcaccttcatataagcagctcttgcttatatgtattgctgtagtttgattttcctgttcctgatgtttcttcatgttctattttcatctatttccttctccctgtatctttcctctctccactgtttttgctgctgactcaggggagctgtgcagctgacctctatcgacacccacagcttgatgcagacattgaagccgtgaaggagatctacagtgagaactctgtattcatcaggtgggacttgactttctgggatggcaagggaatcaaccacatctttccaagttgttaaaatgactagaggttttcttctttatggtgtgatgagttgggtgcggtctgtggatattgatgagctacgagcttaatgatagtgggagtggctcagaatatttaaggttggctgacaggaataaatagggaagtgcagccacttttcctagaagttccctcttatcctagactcctctaggctgtttcccctttaagataagaagggcttctggcctggagaagaccttgatcataaaagtgggatgaggctatagctaagagcctaaatacagagttgccttccacccttccctttcccttgtccccaggctcagttctctctccacttcagtctctgttcccttctttctcccttaatgagtctcacctatggtcacctgtatctctatagagaatatggaactatcgatgacgtggacattgacctccacatcaacatcagcttcctcgatgtaagtggtgctagtagctgccaacaacatgtctgttgggcttgtggattggagtttgacttgtaggcttagaatcttgtttctgagtactgtattcagagcacatcctcttcatccttgtctttccttgaccatcagcagacagtggtgtgtgcatgtgtgtcatatagggaaaatgtcaagtccattcctctctgttgccacactggaaactgtttcccttactcttttaggaggaagtttctacagcctggaaggtcctccggacagaacctattgtgttgaggctgcgattttctctctcccagtacctcgatggaccaggtaaaggcagtgacttcaggcaagtgggtgctttgaatgtggtctagtccaaaatcttaagttaactgaggtagagaacatcccttaaaggccctttttattaatgaaattgttttctctagtccctggatattatttattccttctttcccctcaacttctctaaggaaatatttgaaattggtcagttagttcccagattctaccttctgcctcgatgttttccttctccatcattggtgtttagagcatccttagaatctgaggaagctaatccactgaactggagctgtggactcccaagaggatagacacgcatatgtaggagctttctcttctctttgcagaaccatcgattgaagttttccagccatcgaataaggaaggatttgggttgggtcttcagttgaagaagtaagaacttttttttttttttttttttttttaatcttgttttaggggtgcacccacagcatatggagattcccagtctaagggtcaaattggagctgtagccgccagcctctgccacaggcacagcaacctgggatccgagcacatctgtgacctataccacagcacacggtaacactggatccttaaggcactgatcaaggccagggattgaacctgtatcttcatggatactagttggttttgttaactgctaagccatgatgggaactccaggaaaagtaggaactttgatctttctggttatgaactttttttttgcttttcagggccacactttcgacatatggaagtttccaggctaggggttgaattggagctacaggtattggcctatgctacagccacagcagcatgggatctgagctctgtctgtaacctgcaccacagctcatggcaatgccagatccttaaccccactgagcaaggccagggattgaacaggtgtcttatagatactggttgagtttgtttctgctgagccacaacagaaaccccttggttatgaacatttgaggggaagagatgtggatatgtggatggacagacagaaatctcaaatagattatttctttccaaaaatgtatttctgagatatgcccaagaaagagtaaaattaatttgggccaaatttctggttgtgtggggaagcttatgtttttggggtatctgcccttcagacttcttggaggtgagaagataggcttgaggaaaagcacaaccctggaatttgagtcatgctgatcacatttcctgtgtggtttactcagagtagggctctaggagctcagagagttttagctattgaatgtgtggggcaccttactaagtatttggtatacaaagagaagtgaattatagattctcccctcagtcacgttccaaatagagtccagtggatacatgttctaatacaagtgaatatgtaaggtttagaaaggacacagaggaagttataactcagtctggtggcaggtgaatgaatgaaagatgaaaggaggtaattaatggttttcaagaatgggtaagagttgcccatgaagacagtttctgagggtaacatttgcaagggcacagtcatgtgtaggaagcttaaagtagttatatattgctggtaaaatgcaaagggagtaggatctaaagctaaagaagtactaatgagtccaaatcagagaggatcttgaaattttattttgtaggcagtgggaagattgaagggttttaggcaagaaaaggacttgatcagttttagttttaaaaaaatcattttggtagcattgtgcaaagatagaaaggatgagacaagagaccaaaactatttttgtaggcgacatttgttggagtccatccatgagatgatgtaaacctgagctaggtatgactctaggtaagaagaaaggctagagagattatttgcagggtataaaattcataagacttgatgactgagttgggtatattatacatgacaagagccaaggagtagtggaatattactcatgcgtttccagcctggatgtatattgtaataccagtaatctaaataggggcttaagaagagtaagttcataggatgaagattaataattagttccattttaaacatgtagtttaaaggtaactttgggttattcaagtggagaagctcagtagagagatatatagatttgatacttaaaggagaggttcaggttgaagattcgtattagttataagggtcagaattgcagctatcatagaatatggtgctcagagattgctaagggagagcatgatagaatgagaagaaaatagaatcaagggcaaaacaccctttaacatccagacagaatgccaaaagtaggtagagggagagaaacactcaaggtaggacagagaagttggaaaagaacgggaagagaatagtgtcattgaaggcaaggaggagtgtttctacaaggagggccaaaatttctgtttgatttaacatcaaagtgagagcaattgtagcgcagtggtgaaggtagaaaccagactgtactaagtaaaaattcgtcattggcaataaaagagaaacagtaagtatgggttgagaaatttggttgcagataggagaggaaaagagaggtagctaggctgaggtgccaaaagttgaaactttttatagacttgggtaaaggaactgacaggaaagggggatggttgacagatcaaggtccctatagagggtctgagatctagggtacaaatagagcaatttgtccttaataggagggtcaccttgtcttcggagaatggagggatcaaggtaagggtagaaatggattttgtggtagggttgcaaaattttcagttttctttactgagaagaaaggtcattagttgtagggttgtaggtgaagttaggagcttaaaggagatgataggatttagaataacagtgtagaatgatatgagagagaactgatcaaagagaagtgaaaggattgacaagaccagctgagggcccagctcaagttggaaaccataaatttagggatgtaattttttgcccaacaaagtcagtacccctcgtgtcccttgtctttttcttcactgttcacaaggcagtgggtggtactcactatcccaccacttttgttccactctcagtatagttattcttggcaataaattgccaggttcacagccctggaagacacacctctaaaggcagaggatctgagaatttctctggtccattagatgaggcctgctagctagtgggtatatacccactgaggtaaagaggtactttaggacagtacatttccatgtgctaaggttttaacaggggggttctttagatccacattcccttgtaacaactagcttagtggtccctgggtctgaattttagattagttgccttttgtgatcctggtcccccaacccccagatcgggaaacatgtaagatgaagacaggatttcattaccatcttactgcaattttcttttctttctttctttttttttttttttttttttgtctttttgccttttctagggctgctccagcagcatatggaggttcccaggttaggggtcgaatcggagccatagccctaggcctatgccagagccacagcaacgggggatctgagctgcatctgcaacctacaccacagctcactgcgatgctgaatccttagcccactgagcaaggccagggatcgaacctgtaaccttgtggttcctagtcagatttgttaaccactgagccacgacgggaactccttactgcaattttcttatgtgttactagcctacatacctcatgttttctgtaatcacgcagatatgaatagaagtttgaatgattaaataaatgaaaagttcatttactgcagagaatcatttcacaaggcatcacagtcctatgtcttgatcacttccctgcctgggcttccttaagcctgttcctctttgattccttaggatcctgggtatgtttacatcccaacaatggaaacatctcagcaatgatttcctcaagacccagcaggaaaagaggcatagctggttcaaggcaagtggtaccatcaagaagttccgagctggcctcagcatcttctcacccatccccaagtaagtgttcctccataagctgattatctcttatcaccttaatctcctctaagcccctacctcaccttgattatgtaaacttacatattctttcctctcctcaggtcctctgaattctgtgtctttaattattaacaccatccacatggtcctgtcccctatgtgtctttacccttttactcctggcccagtagtcataccttgtcctttatgtaaaacccagtacctagctcatggtatgtatttggagaaatgtatgctaatctctccacctatcctgtctttgaccctcatccttattccctatgctaaggaggcagagtcagagcaccaaatccttgcttttctggaaggatacactgttttattatctaggttctagaaataaattctgctccattctttgaccccaggtctacattttcccctccctggtgccttctgatcttttcagaggcaaaaacaaacccagattgtagttttccttacacaattattgtcagtcaaacattaggctctttggggtccagctgcctcttgcctagtttaatcacatatatacaaatgcatgcgtgtgtgcacacacacacacagtaggtgaactaggcatcctctccttacctggcctagatgccgtagagattgacctaggctttgcctctgcctgcaacttcatgttctaatcttaagaacacacagataatgacataagatgtctggtgatctccttgttttgacaatttgatccaatgaaactttcctcagatatgagttgctctttgacttagcttgtttggtactttcttatctccaggcctcttccagactcatactgaatccccagtttcatcacttctctttactttctcttcaggtctcccagcttccctatcatacaggactccatgctgaaaggcaaactgggtgtaccagagcttcgggttggacgcctcatgaaccgttccatctcctgcaccatgaagaaccccaaagtggaggtgtttggctaccctcccagcccccaggcaggtctcctctgcccccagcacgcaggcctccctcccccagcacggacctctcctttggtacatgggctgagttagggtttgacttgggtatcagaggatgggaggggaaatgtgggaatatgatttctcaagatgaggtggggatctggttgtcaggtatcaaaaaccatgacatgaatcatgagggagtagaatgaagcacatttagtggttgtgaactcatatttaaacagtctggcaagcttctctgatggtaggcaaagagtctggggttgggcagctcagggaaatgtcatgtgtaatattattaggttgtggttaggacttggtagtcagctgctatagagacctattccacgtactttggagagggttaaggacaggtgagcctttttcaagagcctttggccaaaatgtctgaaggtcttctctccagcttggggactacttagactgatcagagctagggcatagctactttaggagaattttaggtaatgggtatgagtgaggtctttctaggcaccagcttcataggaggctcatgggatttgtctttttaatctcatcaggtcagtggtcactgcaagaacatccccactctggaatatggattccttgttcaggtaatcaagtctaaagcttcatgcataagcctttcccgttttctgacccatctaattccccaatacctcccagcttttcagtcagttagcacacatttcctgaattgctctatttctagaactaagtaactgttgttcagataggaaaaaagaaggcacagttcccatcttcaagaagcttgtagcattactgggaagacaacactcacagactacttacaatctaacgtcaaatgaggcactgcaaattttaagtgcacaggtgccaagatgagagttaaaaatgaagctaattttcttagattcccacacatccttgctcatgtgatctttacatttcctcacaaactttccctgcttgaccaccactggtcgcttgcttctttttaaaacctttttactttctggacacagtttcacttttgcatctgcaattcctttgttcatgtcattccctccagtggccttcttccctgtgtctgcctgttgcaatcaaagtctctgatgccaccttttctataaaatcttcccttttacctgaaatatattagctggaaatatgtctcctctcactgaactcacataacactttttgttttatatggcactgatgtgtcatgtgccacatgctgccttggattgtagttaatttgtgtacataccacatctctcctgttggactatagtgtctgagaaaacttttgttactgagtaatcaaggagacctttcaccaagttaggtacatagtaggcattcagtaaatccacattaaaggaatgagtaaaagcccttgtatgtccatttactataccaaaagtttgtgaaatggaaacagtttgatttatacacaaagtatatacgtggttggaatagccatgttaagacagtgtgtaaaaaaatacgttagaatattgctgcatgagctctggatttgtgctgtctgcccagcatagggttttatctatgatattgatcagtttacaggcagattgttcttggtagtaaaaatggctcttctggccccctgacatctaatcatggactgaatactcgtttgccacacagacacagtctttaatgactacagttaaggttaatagtttgattagtacctgtaaatgtttatgaagtatttcaagattcatctcattactcttgatacctctttgaagtgaataatgtgcactttgtaaatgaggaaaccaaggctcaggttaactaaattgcccaaagttatatatgatattaagtagcggaggaggggagttcccattgtggctcagaggaaatgaatctgactagtatccatgaggatgcaggttcaatccctggccttgctcaagtaggttaaggatccagtgttgctgtgagctgtggtgtaggtcgcagatgctgctcgaatctggcattgctgtggctgtggtgtaggccagcggctacacctccgattctacctctagcctgggaacctccatatgccacgagtatggccctaaaaagaaaatagatcgatagattgatagataaagatcagtcaaaaaatcccatactaaagaaaaaatagtagaggagggatcttaaccaaagtcatctaccatgtctggtcttgtttttactataacattcagtcttagctctagagtcaggccatcagtttaactaagtgtagaacctaagaatagattctaccttacttacatgtctgggaggtaggagagtaacagaaagaagtttaaattatttcctgtatttgggtctgtacttctgaaagacttaatagaatctcttctccctccagatcatgaaatatgcagagcagaggattccaacattgaatgagtactgtgtagtgtgtgatgagcagcatgtctttcagaatgggtcaatgctcaaggtaaatgcctcaaatgtgaccctcttccttagacccatggctaagaccgcttcagacctcatctctattttcctttcttcctgggtctgtggtaaaggtagaattctgtctctactccttgagactttagaaatctcatcaatgctacttggaaagataaggattatcattctagagttgtctgaggtcaagattgtccctcactccttaccttcttattgcacacctcttaccaccaccatctcttaatatttccattcagccagctgtttgtactcgcgaactgtgtgttttctccttctacacattgggagtcatgtctggagctgcagaggaggtggccactggagcagaggtatgggggagagaaaagctgctggggacccaggatcaagaaagaccaatgaacctagcagtttcaccgcttggaatttaatgtccagaaatgctttcctatgtcaggatattgactgtaggattgtttataacagcttttttaaaaatggatacaggcccatctgaatgaagtccatttaagttatggtattttcttacactggaaatactatacagctgttatttatggatagaaaattacatataaaagaaaatacaaccgtatgtatagcacagttcttttttgttgtatttcctatataataactatttctctaggaaaactatctggaagagtatatatcaaacttagctgtagttacctgtgaggaatggaatttggggatgaggggatggtttctatctttttaaaatcactcttttaaatattattcttattaggagtttatattttctaatgagaaaatgatacacatatttgcttttgaaaaaaatgctgagagcctccataaggtagacctatgctggctactgtgtgactcccagcactgggaaatcatttcgcttctcatctctttctctccttttccctaaggtggtggatctgctggtggccatgtgtagggcagctctggagtcccctagaaagagcatcatctttgagccttatccttctgtggtggaccccactgatcccaagactctggcctttaaccctaaggtatagttgcttgggaagaaagtcaggacaaaggaacagaaatgctaaagataatgggagactatgggctatcattctagtgtacacaacaggttggaataaggggaactcttaaaccctaaactttggttgttttagtgaataaataagtaaacataacttgcaatataacagaaacaataacgtctgagtttgtcagaagaaagggagaagagttaatattagttttgtcgttataggaaagaatatagactttgattcaagacacactatgattccgtttaggttccgttgcatcctagcttaatggtgttaggcaaatcactgaatatgtctgaacctcagtttccttataatgcctattataaaaataagagataacataaaatactatattagtaagggttctctagacaaacagaaccagtagttaatatatggagatatttattgtaagaaattggcttatgtgattatgaagactgagaataccaagatctgtggtgggcaagctggagattcagaagagctgacggtatagggtccaacccaaaagccagcaggttcaacatctaagaagagctcatttttctgtttcagtttgaaagcagggaaaaaaaaaaccaatgtctcagctctaggcagtcaggcaagaggagttccttcttactcagctgttgtgttctattcaggccttcagctgatttagatgaggcccatctgaagagggaggggtatccgctttcctcagtctaccctcaaacgtttatcccatctagaaatgccttaacagacacacccagaataatgtttgagcaaatgtttgggcagtccatggcccagtcaaattagcacaattaacagttgacaaaattaaccatcatgtgttcccagcagagtgcttcactattactcattgctgtgtatcaggcactataccaggttctttacatatgttaatcttcagaacatctctatgagaatagtgggattttgtgttttcacttacacagagatactgaggtcctaagaggcatataacttaccctattatgctcatttggtaaaagagaacatacatactattctagaacttcctgacactaaatatatgttctttccatgaaatatgctgtttcccaagggcctagtcttcttttgtacatgtcaccctcctttacatcacatctcactctcttcctcttttcttcacctggttcttctcttcccattgattccttgcagaagaagaattatgagcgacttcaaaaagctctggatagtgtgatgtccatccgggagatgacccaggtattctgccctttgcctgtcccctgtgttatgcctgccggctcatgtgccctattctgcttggaattcatgggagtggaatgaagatttagaaatgttactcaaatctctcactgtattttctttagtcttccctttttagccttcccagtctttgttctctgttttgttagctctgttacacctctttctctctcctatgtctctcttaacctttacctttattgctgatttattcgcaagttgttcatatttaatgtttttcccataattcttagggcatcagagaggtgagggaaagccctttgcccagggttgggagggtgaggaggggggcttggaggtaaggaactagatccaggggcctacatcttctatccttctaggggtggggcagccacatggagcagtgatcatcctttgactcaaggctgtccctcaccagacttccccacccctcgtctgcaatctctgcatgaatagacattcatttgtactcacattgacaggtgggcctcttctcagcaaatcctatatatcacaattcagattaacacataagatacacctaggagggataatttacttgtcggaagaattctttgctttatgtcaagttttaccacaggattccttagcctaatctttctgcgacattgattttgtttatttttttgatttatagtaaactttttagggctgtaggaattgcataaaatgagggagacccacctgcatgttgttttgtaagcatcttcagtcattttcatatttatttatttattagtctttgcaacctgactggggtccttgagggtgggaaccccatctcctcttgccttggtgtggccttcagtgcctaccttgccctgggctgatagtctttggaaaatgggagggctcccacctctcctgggagataaccttatggctgttgtcttacagggctcatatctggaaatcaagaagcagatggacaagctggatcccctggcccatcctctcctgcagtggtacgagtagaatggttcatccctcagcgggtgggggagtagggcatagtaccagatgtggagccttctcttcttggcatctttctcttagaggtggtttcagcatccttcccaaggttatatattttatggctgctttttcttggggctttattgatacacctggacttgacaagaactcagatcctgacaaagagcccacaggttctgacatgatgcctcaagttttctgtgggtgtttcctgtttcctagtaggcttttgagtgctgcttacatgtaggaattaatgctgttgaattcaattctttttttatgcatgcagagagatctgtctccctatttctactccctttccctatttcaagcccttccctgttgttgactggttgactggccagagccttttgaagcactatcattacccccgcttccttgcaaggttctggcccttctctactttcctctacccccctgctctctccctgattttgattccgttctctattcctgacagagctttccccttctagactactctctgtctggttagcctttgacattagtactttctcagtgcaacatgctctttcttagcatgaggaatggccaggcatagaccatccaggatggcatcacaggtactggcatgaagcaccaaaaaccaaaccatatccataggagataatgctcccttgctgagccattaatggtttactcctttgttctctcctgtcatctgagttcagcctacatacagctgagtctgtccctgaatcctcaggaaatttgggctaatttcttctgtttctttttccagcccaaagagtaacttttcatcttccccatctcggaggcttcaggcttcctctcaggataaccctgagccctagttctaaatttctaaatcccaagtgtcagttgtcacatcgtaatacagaccccacctttctagtttctttttttttggtagcttacctcttgttcatttctttttttgtttttactttttacgactgtacctatggcatatggaagttcctgagccagggatcaaatctgagctgcagctggggactgtgccataactatagcaacaccagatccgagctgcatatgcaacatatgccacagcttgtgacaatgctggacctgtaacccacaaagtgatgccagggatcaaacttatatcctcattcagacaatgtttggtccttaacccattgagccacagtggaaactctttgttcacttcctttcattgtattctttagtctccctagatataggcagcccatttcccacctctctctttcttttatccattttttaaactaccttgtaactagctagtctctggtcagtaacttcactttttttaagtttttatacacaaacactacccgtaggaatatccgtatagtgacctggacttaattcacacagccctggaatctttgcttgttctcgcagaggcagagcaagctgctactttgttcagagtggcctaaccacacacttattctatcctttttgtttttactctgttttgtcttaggatcatctctagcaacaggtcacacattgtcaaactacctctcagcagggtaagtgactgttctcccgctaaactctttaaatttctggtgagaggcagggaggggctccaaaccagctaaccacattagtcctagacctgcctggttgtcttgtccatcagtaatagtctatgcgcctaagtatatatcctttatttggggtcagtacaagcctgatttgctccctttccccagcccttccctccctgatctcgatttctgttctgttttcctgaccacccccccaccctgggcagcagctgaagttcatgcacacctcacaccagttcctcctgctgagcagccctcctgctaaggaggctcggttccggaccgccaagaagctctatggcagcacctttgccttccagtgaggagtgggggggggctgggcatgggtgctggatgaggcaaaaataatatagggggatgggagggtaggttctcttgaggaatacgagtttatgttacactatgtccatcaaccagtcagtgaacaaatacttattaaatgctattgtgataggtgttgtagagaatagagatacataagataaagtcattactctcaagctacttacagtgttgttgaggagaaatgatatttacatataaaaagatgtggttgaaagaacagattggcaggggtagatttgaaagctactttggaggaaatcactttatgcctaattgtaggaggagagagagggggaaaaaaagagagattaaagataatttcaaggggagtcagtggtacccttccttaggatagatgtgaagtcatgactggaagccatatttggaatcagtgataagcttgttgaattcaagatgattttgtttaatttgaaatagcaggataatagacaaatgaaaatattgaaccagcagttgaggatttaggatgggactagccaaagcacagaaaagagggtgggactgaatattagccacacacacacacatcttgcatgcctgtgatgacacccatgtgcatgtccattgctaggtgtatctgtgtccatcttcatgtcctgcgtgggtgagaatgggtgggagtggcagtcttggaagtgtttttgagaacctcataccatgaggagacatatattctaccctgccttgcagtgggtcccacattgagaactggcattcgatcctgcgcaatgggctggtcaatgcatcctacaccaaactgcaggtgaggctgtgccccttttccctttccactccctgccccctgccccactcagttttggggaagtctgccctagagtacccagctgttttttgcttcagcatcctcaaacctagcctcccgtgaggcttccctagggaggaagttgcagccacgtagaatgaatgtgactgttgtatatttgaccttaagctgtgctttttggtgttgtaggaatgggaatgtagctctaggcaggaatcagctgtaggctgattgcagccactgtgatcaattaacctgttagaacttttctatttatttaactgttcattcagagagttgatataggagacatatttctttgctctgcaagactctaaagaatggttattgtccctcatcctggctgctgtcctatattcctttttggggggtggtaatctgcatatgtcccaaggcctagggacaggagcatggattctgagggaatggattcaacggctctataactcctctccaaggcatcagtatctagtgtttcataggcaaagggttaacctgcatccacttttcagccaagcagcttttcaagagtaggtgcctaagattatctgaatgagtgagaagataaaatggggggacagagggctggataagccttgtggctgcctaatatacagccatgggagggcccaggctcatattgctcatcctggtgtttccctgcaagctgcatggagcagcctatggcaaaggcatctacctgagccccatctccagtatttcctttggatactcaggtaagaaataatctctggccacgttgactctatttacattgcatccattttgtgaatacataatcctatgctgtctcctccatcatggatacttggtctatgtcagttctctccccagtcatggatacataatcttctctactttctctccttagaaatttagattctttgcaaagtgaggccatgtctccctttctcttagatagtcctcttcttcatggggatggttttattcactggagaggcttggctctgagaatgggttatggaataactggtagatgaaactaggctcttttggagaacacatttttggtagtagcctgtcattacaggttgtgtgtgtgtacacatgcgtatcggtttatatatgaaagcttgagtcccttccattggcttatatctctggagacattgttcttctccctgtcaaccaccttttacaatttaaactgtctgtaattacacactattgtattagtcactttaaatataagagaaagcattttatttcaaagataggcatgaacaagtttcatagtttagttaggagatgagttaagctttgtccagttcagaaaatgtatctgacttagagctctgtctttgttccaggtttatgtctgagttccttttcagtcttcttttgttcttattctgtatcgtctgtgtataaaagatagccaccacgtagctgcatgtctaccgtatgaaggggacagtgctagatcctttatagattactatttagtattctccagtaattataactgttacaaagataaggaaacttgggtccagaaacgcaaaaccagaaaattccctaataataggataaaccaaacagtagaagaaaggagataatacaggtaagagccaaaatcagtgaaataaaaacaggtatcaataggagttcccactgtggcagagtgggattgacagtgtctctgtggtgccaggatgcaggtttgatcctctgcctggcacagtgggttgaaggatccggcattactgtagctctggcgtaggtcacagctgcagttcagatctgatccctggcccaggaactccacatgcctcggggtggtgaaaaaagaaaagccagatatattagataggtccaaaaaagccaaaagatgattcttttaaagaactaaccagacagataaacctggttagactgattaagaagaaaaagcacaattaataaaaagtacgattaaataatgaagaaaggaacataactatcgatgtagcagaattttaaaagttaatggtggaaatccatcagctttatgccagtgatttgaaacctttgtcaaaatggatgaatccctagaaaaatataacaacaaaactgattcaagaagaaatagtctgaatagctctaaaattataaaagacattgaaatagtagtttaaaattttctacaacaaaacagaaaaagttaccaacccctgataattttacctagtgagtcttaagtcaaactttcaaagaacatattatcccaatcttaaacaaaatcatccagagaatagaaagaaatggaattgcaaatcataataaattgataaatttaactttattaacactaaaatcttcatcagaagacaccttaagaaagtaaaaagttaagttacagagcaggagaaaacatttgcaacacatataaccgcaaaagattagtagtaaaaatgtgttaaaaaaaaattctttcaggagttcccattgtggctcaacgaaaatgaatgtgactagtatccacgaggatgcaggttcgattcctggcctctcagtgggttaaggatctggcattgccatgagctgtggtgtaggtcgcagacacatttggcgtggctgtggctgtggctatggctatggcttaggccaatggttacagctgcgatgagacccctagcctggggacctctatatgccatgggttaggccctaaaaagacccccccccccaaaaaaaaaatcacaaataataaaaagacaactcagttaaaaaataggcaaacaacatgaacagacatttcactgaagatgtgaccaaggaaacatgagcagctgctcagcttctattaatcaagtaagtaaaacaaaaccaaaatgacttaccatttagcatgtaagtggattggcaaaatttgagaatctgatgcctttgattgtagcagaggtgtagatcagcatgatctcttttattgcatatgggaatataaattggtacaaccactttggaaataatttggtggtaaatttcataaaagtgagaaaattttacccctgcaatccagcattttcatttctgcatatgtccacccaaaggtgtatacatgtatgttcagagtaatactgtttgcgacagcaaatcttagaaacaatgcaaattctcatcatcaggagaatggatagagtttccgttatggctcagtggtgacgaacctaactagtatctatgaggatactggttcagtccttggtctcgctcagtggattaaggatccagtgtttccatgaactatggtgtaggttgcagatgcagtttggatctggcattgctatggatgtggtagctacagctccgatttgacccctagcctgggaacttcaatatgctgcaggtacggccctaaaaagtcaaaaagagagagagaatgggtagatacattttaatatattcttgcatcgggctgtcattcagcagtgaaaatgagccaacaatggcattcaacaacttgggagaaattagcttaggcctgtaggtattcattgtgctattaaataaaagtgtgtaatgaaccaaaggtcatgagtgatccatgaagggtaagtgctcagtgaatatttattgaatgtgtgaatgagtcttactccatgtgcttagggtccaaagtgtgggtggggttggaatagtcttttggctttgtctaggttcttagtttttatctttgtccctgcctgagcttccctctaattaagctcttgttctaagtagtgaggttcctctgcctcccgctacccacagagtttctttttgtctattttctccctattctctctctctcttctctcccattggcctttatttattactgagtgcctgaatgactttagttatcatttgaagccagaaatctctattgactttttaattttcttctttatttactgcttatgtaaaatatcatatggcaccattcttcatcctctccaaaggtcaatttgattatatatacaaaatgacatatgcttttgctgttggagttacaggtcatcttgttcaatctcttattactttacagataagaaagcagatacacagaaaaaaatgactttgtcggggtcatacggcttgaagtagcagagctagaacccagatccagttctcttaacctctaggccagttacaggactgacagggtaggctttgcttgaatgactgagtttccgagggccccatagatatgtgagagtctctaccactgggtgggatgtttggtaatgtccagacttattttagtcactctagcatttggccagctctgtctttgttgtatgtttccttctgctcctttctgctctgattttctttattcttcctcagggtatctgtaggttagtgtcaccgggtaccctctggacatcattataaatagagagcatccatttaactagcggaaactgatgacttggccgtagttgcaggttaaaatgaggcacagtgggagatggtaaactttgtctgtttatttagtcatgtgtagaaacttctcacaagtatatactctggacaccaagtctttagggactgtctttgcctccaggttctcagtgtgcattggaaaactcacagaagatgattgggtcactgcggacaggacagtgtgcaacaggattgaaatgggacaagatttagattatatcataaggaccatctctaagactagtcgtagaaatcagagtgttctctggggtagaacctaagtgggaatttcacttaggaccgtgcactgaaatactcaaatctaaaaatgtcgtaacgtttggacacagagctaaacctagtcaagactaatggagaagttggaaacaggggtggtaggtatcctgtaggaggaaattggaaattcaagtcttgaggctctcattgccctgaattttgtcagggacttcagtatgagtgcatgatgaattgacagcctgagcagtgaagaatgtcagtccagtggttatcatttctacctctataccatgactatcacaaaaccaagacttgcagcagaagttagttggagttagaacgttccagggtgggctgatcagataagggcccctgcttatgacctgcaatgatggcatcattttccatcctcacttatcttcctttcagtgtcatggtctcatatgcacatacacagactcatcccaactgtcataaggctgtgcctgtgatgaagctgaatacagagactgaagtcctaatcataggccagaaagagttggcactctttcatatctaaacaggaagaattggaatgagtctatagttataaacagggctattcagtgaggggtaaggagggtggaggatttatggatctagatagggcgaaaatgagtgaattggcacctctcccttaagtctgggaagactttctgcaggaagcaggactcttcaaggtagttactgttatggttacctgtggaaaatttttcatctcttaatgttgtgctttatccctttaccctgaatgactcttgtcagagctttttatgtaactttgaaactagagtagttctgatttgctctgcttgcttcctctccactcatttcactcagcctggcatttgacatgaggcattgatgtcaccattctcctgggccgctcattcctggctcatttcacgtgttacttcctatcttagaatccttcagtgatgccctgatgttcttaggataaagtccagttgccttaacatggcctacaaggtctgcttgattttatcctagcctacctcttccacatcatctttcaccacttctctaccattgactataccccatacaaactaaggcacaaggctttgcttttcctccaggccattcatgtcatattacctctgcttagaacacttccctaccttcatttaactaattaagtcttcctaatcctatacttctcagcctagctgtcaccaggaagccttcttcaaacccctaggctaggctggttcccctcctctgactccacacagtgttctgtatccttcccatcataacctttagcatgctgtgttgtaattatttgttcctttcctgtaatctctataaaactaaagtctgtgagggcagatacattgttttcttcgctgttgtattaccatgtatctctagcttagtgcctgacacatagtaggcacttcagtaaatatttgattaaggaatgggtgactgaactggtttgttgttctgtgacaggaatgggaaaaggacagcacaggatgccctccaaggatgagctggtccagagatataacagaatgaataccatcccccaggtattattcgttagttgcccttggtccactgaggcagaacccttcctctgggataagtttaggctacaggggtggatggggaaacagtggtagtggtgggatgggtggtttaaagatcattttgaaggaatcagatatgttttaagatgaacacatttccagagtcatttgtggcctcagtcataagtatgaaggcagagactgagtttaaatgcagtgacatgaaactgtaaagatggaagcctggactcatctagactgattatgggaaagcaaaaattttgggggggtgactgggagcccaggatatcccaatacccatccccaaccattacctactaaccagcctctctagggaaagtgtaacagtctacctggctctgctttcctcttccagacccgatccattcagtcaaggttcctgcagagtcggaatctaaactgtatagcactttgtgaaggtatgtagcttacccagcccctgtttttctgggccctctgtctttatttctggtgcccctttggcacatggatccaaccaaggataatgatgatgccatttcttccctgcctaaacattatatctgtaacctctggccctcttcttcccagtgattacatccaaggacctccagaagcatgggaacatctgggtgtgccctgtctctgaccatgtctgcacacggttcttctttgtgtaagtctaggaggttaccttggggactccttggaggagtgagggtgcatgatgggactgggagcatgacgacgtgtgactatggggaaagtctctttctgttatcagagacttgtccctggctacctgagtggtgctagcactgggacttgccccttggaggacagggatgggtatagatcagggtctgtttagaggaaaccagataagctgaatcttttccacactaaagagtaacaagaaagggtttgacttacggggtggtgtggccacacttctgaatgcagttccattggttgacattattctggtattgttctccctcttgcgctcacacttgccctatctttggcagatatgaggatggtcaggtgggcgatgccaacattaatactcaggaccccaagatacagaaggaaatcatgcgtgtgatcggaactcaggtttacacaaactgagggggccccagccctcgtaccacccccattcccccgggatccatccaccctaacaaaaagggctcaggagcagcagacagggctgccctgaggacaaggggccattatcaaggggcaggaaaagaataaaagcggcggccttcatggtggaaattgacccaggaactactccacatttggatggcccagattgactccctactcctgattgtcccagttgacttcaccctgtttgtaaataaaacaataaaatggaaggtgctgtggactggatatgatcactgtggtctgactagccttggcccagcacctgccccaagccccaatggaggtgggggtggggagagtggaacatcacgagggttgggactgtttatgttgtgggaatcagagctgaatctgtctagtatagtatactacagatctgtcaacattttaaccaacaaattagataaaggaaacttatcagttatgcagatgacataaactgaggatatagaataccactgatgactgttcttcacgatttaaaaggactaatggaggccaaaacccctcagatttcctatccttagaacctctactttctgcataaaacctctcccctctcctttgctgtatatatcaggagctgatccctacttgcctcctccttccagctgtttctttttgatagggagatgaggggagagctggcaggtacaggaagtgggttggtctctaattcaaaatctataaagaaatcctaaggaatcagcttcccttagtgaaatgaaatccaaattctccaaggctagcaatgggagggaagacagctgttcctaggagacctaattgtttcagtgaaagccatctccctgatgaaattcccactgccagccttctgctggcctttaggctatgctccatgtacctaaaatcctaaattagttacaagagaccagttggacattacaaaatattttatgaattattaatgaaaaataggaacataagcatagagacaacaaaaagcactgaacaagcctggtttttaagtatagatttttaattctgttataacatcttgatgttggactacctgtttcttttcattatcttcaccctacttcggaaataaccttctttgcctgggtgccttacctgctttgtagttatgactacaaggcctgaacttaacatggaagtaccattcttaaggtccatctcctaggagctgtttcttaaactgctttactccttgaatgagactgctgccattctgactctacatgtctcctaaggctctctcccccaatctggtttcaggtctaggagaatagctcttctctaagtaaatgaccccatcaggtgacccaccctaactgaaaatcctgcctcctgggaagacccttgcagctcatctgtgtagtatcagagatagctactaacattttttagttcttaggtagatcattaagtttataacactttggctttcttaccaagtgcttggtattgttgtaagctctctacttgtattgactaatacaattctcaaaacaagcctgcgaagtagatgtcattattcacattttgcagatgagaaaacaggcacagaggatgagtgatttgctcagattccacggctagtgactgatggggcaacctgactccagaattgctattctggttctatgctatatatcctttcaaacttcacaatttttgtttttttcatttaatcctgacaacaaagatggaagataggtgtttttagagatcataagtaatatgtgcaaggtctcacagttggttagtggccattgctgggtttttaaccagatttgctcaactccaggacttgagctcttaaccattcttttacttccccagcggttctcaaactgttggcactggtgttccaacagttgaacctacgtgcttggctactcaaatggtataacatttttgctcagttttcagaaattattaatagatttttctcagttgtaaccatttcttagtttttctgtatcagtaacatctgacagagcaagtactagcaaacggtggaatgagaagtaatgaacaggagttcccgttgtggctcagtggttaacgaatctgactaggaaccacgaggttgtgggttcgatccctggccttgctcagtgggttggggatccggtgttgccgtgagctgtggtgtgggttgcagacgtggcttggatcccatgttgctatggctctggcgtaggccagtgactacagctccaattagacccctagcctgggaacctccatgtgctgcggaagtggcccaagaaatggcaaaaagataaaaaaaagaagtaatgaacagatagtgtatgtttccagaaaaactcaaaatacctgagctgacctcatggaagtcacttttttaataggatatacacaagtcttttagtgccaataaaattataatgaaattaaatgtaccattttatagtgttctgcataacagcaacaggagttttttaatctgaaaagttagaaagctgtacatgaaaaaattcaggaattccctggtggctcagtgggttatagtctagcattgtcactgctgtggcacaagttcagtccttagcctcagaacttccacatgccgcaggcatggaaaaaaaaaattcaaaacatgtatggtataaaacaaatctaattaaaacccgcagcattcctataacaagaatgcttgcattgcccagaaagttgcacagggccctgaatttctggagaggagtcctcccacagcctggagtggaaattaaaggaccattgcccctttctcccacccagggctggctgccttagaggtgggaggtgaaacctgtgaaagccaagtctgtgccagagattgtccttcaccaaagccaagattgttgcaaatcctacacacagaggttcacctactcctggttcaccctttcagacctggacaggctttgttagtactaggtctgggaaaataactattttcttcaattagttctagggggagagtaaatagctatgatttctggattgagaacttaaaactcctggagtttaaacttccccatccctcttatggtaattttccatccaggcagggtgtggccatgattcagtttgtggtgaggatgtggccatccagagaggaggagccttctgttagattctgcctttcatcttggccagtggggagagggagggaagaggctggtgctgagtcatgactgggtaacttaccaggttctcacaagatggattctgagatggaggtttgggtgctgtctcagtttctggaatcaatttgggagtggcagggaggaagcttcaggggtcacacaattccttcagagccctcttcccccagaaagggtgggaataaagtggttcatctgaagtgacatcagtctctggagtataggaattttcccaagtgtttcagagccaccctgcagtgggcccaaagatgttacctttaagttaaagcattgcctacaaaaattgttttatgtagaaaagagatcaaaatttcctttgtcctagctctccttcctgggacaagtagatcaggctagctggtagccagtgagcatggagtggagactagaaatatggtgctaaggacaatgtgactttgatggaactacagcaggaggacatcctggggaaggaggcatttgatctcttgtttgctgatgcctttcttggtcttccagatcttaattactttggggtaacaaggcctgcatacaattccacttgcatcttagggagcctgagctctggctgtacttgtagggaaaaaggagagagcaccgcagtgggaaaaggtagaggcttggtggataggacaaacccaccctaaggaggctttgtcctgtaagcactagcagttctgggctatagaaaaattgctggaggtcttgttggctggggtaggacttcactggaatgaacaaggacttctcaaaaatcttctctccatctaagtgctgatgaggcatctccttaggagggggacctagatacacagtttgatccagaaaactttttttttttccactcttcctttcctctgaaagggtctttccatacatacattcatgtctccttcccttttcctcacaacctcttccctcactacccttaactccaaaaggccaactttctctttcttccaggatttgtctggaattaagatttttctgccacccttccacctacccctggtgggcctgaagagatcttgggaatctgaaggaaagcaaagaagaaattaaaaaggctacttgttctggctctggaaagggcatataaagtccaaagtgaggagttcctgtcatggctcagtggaaatgaacctgactagtatccatgaggatgcagattcaatctctggcctcactcagtgggttaaggatccggtgttgccgtgagctgtggtgtaggtcgcagacgtggatcggatctggccttgctgtggctgtggtgtagaccagcgactacagctccaattagacccctagcctgggaacctccacaggccatgggtgcggctctgggaaaaaaaaaaaaaaattccaaagtgataagcatttctaaacctgacattcaggccaatgggttgtcctgggaatttatattggcctgagaaaactaactgctgtttcaggcagaagccaagagttaacataacggtaaataaaacttgtaatcttgccctctttgtcagggccaaagtttttctgttggctccagagttgggtcagatattgtttgcttacacacctaccttgccagtgactccaaatgaccatcaagagttaaatcaggagttcccgtcgtggcgcagtggttaacgaatccgactaggaaccatgaggttgcgggttcggtccctgcccttgctcagtgggttaccgatccggcgttgccgtgagctgtggtgtaggttgcagacgcggctcggatcccgcgttgctgtggctctggcgtaggccggtggctacagctccgattcaacccctagcctgggaacctccatatgccgtgggagcggcccaagaaatagcaacaacaacaacaacaaaaaagacaaaagacaaaaaaaaaaataaaataaaaaaaaaaaaaaaagacttaaatcattaaggagttcctgctgtggcgcagcagaaacaaatccaaactagtaaccatgaggtggtgggtttgatccctggcctcactcagtgggttaaggatccagcgttaacatgagctgtggtgtaggtcgcagacatggcttggatcctgtgttgttgtggctgtggctgtggcctgcagctgtagctctgattcaacccctagcctgggaacttccatatgctgagggcacagccctaaaaggggaaaaaacaaaacaaaacaaacaaaaaaatcattaagctccagagtctgatttcctggttaagaatccaaacaggtaacagcaatctataccctcactcacacctctgtccagtgaacctagcagctccccctcctatctgccaggtctgtgagcatagtaggagggctggcttatggaggaggagcctagcttctagttgagtctgtgtccttccttagtttccctagtttcatgcagtcctagggttacctgttgctgagtctaaggaataaaggttcaagaggatggatcagagaatggcagagttacttgaattgagaaagatgttctggtacaagtcacaaggaaaaacctctaggactagtcaattctcaaagaggatgcctgctgggcactggtttttatactcattcacataatcatctaaccaaaccccacccaacaagtatgactttccttcagtttacctttaatgaactggactcacgttcaattacaagatacggtcatagggctagtgagtggaattgtaactaaacaccacagatcccaagcttgcttctgtactctgctccttctcatcaaaataatgacaaccaccttaaactctgtgacagattttcaccatgcatctaatgtgagcaaaattatgatggattggaggagtaggtcacaactaggaactaacccctagtctgggaattccatatgccacagggtggccaggggggaaaaaaaaatccaaaaaactggattagggtctgccagtttcatggacagcattttaaaaaaataactgttggatgatcagtatctgtaactgaagggcaatagtttgccatcagctctctaacttaatgcatatgcttttccatcctgggaatatacctagtttagatctttaaagtgcaacatagtctagcattagccagatttttgccactccattgtggtccaccactgttcttagttcatcattagctcaggggccacagctggtcatttataccattcctttctctggatagggagggatctgattgtccctggtgggacatgtggcttttttcccctctcaacttcatgtgctctcaccatctcaataaccaagcatttacttcctatctgcaaactaaggggatgggaaaagattacagaagaaattataaagtattttatctcaaatttaagttgtcactttctcctcgaagcttatctgagctaacaggaaggcataatgaacgcctgtgattcagctacagcgtgtctgcctgagcgagcaggtcacacccattggtctcattttccaggaagaggaaagaatctaagagaatagcattcacgatttttaacgaggcaacactgtatctgcttttaaaacttggctgaaagtaggcaagagttataggtgtttcgttgataactgcagccatcacttgttgcctaattactgggaaatcagaaaatgctttagagaaaaatgtaaaaaacctccaacaatattgatttaaatgcacaaaattgaaaacagaagtgcttattccagcagagattacgggatctaagtctaactgtatttcctgttggttgagttctgcacgaaaactttgtattcactttctactgtctgctggactccagtccccaccaaagcatttgcctggcccaacttgtcctttgttctagccctaagaacaaaagggcctcgtgctcctgtgctcccgctccacgcaaactccgccctctctatttctccctaccccagttccagtgtcggagccctttcgaaggcggcccattgtctccgtcccttcccacctctgataccctctcaggctcctcaacctgcagctcggcttggtctccagggtgcgcgctggggcgggcacccgggcggagtggggggcggggagtcgcaggacaggacttggggaatgctgtccagggacccataaatttgggtagaccagggtagctcagctggggtggcctgggccaaaggtcaagcgaagagcgctggtccaggatcccaaattggcggcaacaggtggccttgggcgccgggaggtctgggagggaggtcttcggcactccgagggcgggtcctgctcctcgccgcttccccattggtctctacggaatgtcaatgctcagtattttatgtaatgtgtccttccgccacggaatgtagtcctccccaaaagggcaacctgcctgcctgttctgcctcagcggcacttcctgcagaaggtgactgtgccccgcgaggacgcagaggggcggggcactgcgagaggggagccaggattgggtgtggggcggggcggcggagggattgcggcggccctgcagtggagataaccttgaggctgaggcagccgattcccgcattggagcgacgcgtcgtgagcctccagaggtctctgcgagcatcgcatcctaagccggaccacgtcggaggtgagcagggggagacactgggccatctgtccccactagggctccatctgcccggccagtgcggaatcttggcctgcctacgcacacagggcacccatatcggagacagcgcaggaacttgggcatcttggagtcacccggttggggtcggaagagaggaaaaaagctgcttgcgcctagggcctctttttcaaaaccctccagctcctgctttttcggaaagcagatgggttggccagctcctttcctgccgcagtccttcatcttcccccacccccattctggttccaacctctcctccttttccttcccttctgtttctggtcccatcctcatcttcttccccttattctcacctaatttggtcctttcctttcgaccctcctcgtttctcctttctctactctgctcccatgttcgcctcctccccttcccccttaatactcgcatctcgtcttcaacctgactgtgcccccttcattctgatgctttccttgaaactcctctagctccactccctggtccctcctccgttcaggttcggtcccctccacatgcctacccgcattcatgcctggttcctgcccctccccctcctctctggtcacgtcctctcctccgcatccctctcctccgcaccctccttcgcgccacccgcgtcctcgcccctcctcttctgttctagtcacgtccgcctgctttcccgcccccgccccttggcctcacatctagttctgtctcctccatcgcggttcctcactcagtcttgggcactcctgcagccacggacctgcgtcccggggtcactgtgcgaagtacagtggtttgcgggataggctcccgtgtgcggccacgggatgcagaagcggcgcccggcaccgctaaagggttacataacccttggccttctccactgcacaggaagaaagggtggctgccctgtggcgtgttcctgttttgtgcggtccttaataagatggggcgacagcagcgctgcactagctccaagagggttacaagactccatcccgccgcggcggggttgcacgtagcggcccaggacccgccccgccccgcgggatcaccaactactgaccttccggcccgttactggccaggcatcacccctggcctgataagactgtgcatgctgctcgggggcctcttaacattggaggcagtcacctggctcctggcctctgcttcacgttaacagatactcccgattgtagaacatggaggccacggggtggggccaggagcaggttatggggagaggaggaatttgtcaagagtttggtgcccagtactgcatccactcagtatgtaaagtgtgcaaagggctgtttggggaaggggtgtggaaaccaggatggctagaatggtcatagcccagggaagtcacaatctaattaggggacacagtgctaaagtctgtgaggaaggtacacactccctgtggggttgaggggggagggcggccggaggccttataaggtggtatcacattgggtttgaagaagcaggaaagcaccttccaatctgaaggttatgtaaagacccagtaatggaaaggtatgccttggcttcatatctgtgttcttcaaacccagaacattgattctaccccccaccccccagcccttgcacaagcagtgcctgatagttaaggtccagacatgatagtggcattgggaacttggaaataggcttttagagtcagatctaactcattaacatactgctatgggtaatggagggaattcagcctcagcaccacagtttcccacatataaattgtagcattttcctcctgatgaaaggattgctttgtacacaactacatggaaatatgttgactactcagtgcagtatctaatctcttgtgggatggctctaaatgtatacttttcttttctttttttttgctttttatactcctgtgcccggggtaaatggaggttcccaggctaggggtcaaatcagagctgtagctgctgacctaggccacagccacaccagacccgagctgtgtctgcgacctacaccatggctcatggcaatgctggatccttaacccactgagtgaagctaggaatcgaacctgcagcctcaaggatactaatcagattcgtttccactgagccacgatgggaactcctaaatgtattcttttggtcactgagtgcaattgcttaatccataactgagcatgagggttcttcttctccctgccatccccaaaccctcagagttaatctttgagagtcaggctctctaaataccagacatctcctggaaaccagtcccctcagggatcctggtacagtgtttacaaagtaactaataatgttacattgcaactccgcttgcaacagcggctctttggtctcctgaaaatggggacctctggacaaagaaaggcaaggagggggatgattttagcctttgatgtttggctacaagagtagaatcaaatttgcaactggggatggtaatctatcttcaccttccactcccacctactccaggtagggttctaggacctgcttagccagctggtgagtgtgagattaggattggaggcaaaggacagtagctccttgttggctgtgcaagggtgtggccacttcctgaggcacagaggacagtttaggtcaggactctgcagcattgttagcaaataatttgccctcaggctgcctgaggatgctgctgggaatgcagtggggctgttctgaggggaagagtgtaacccatcacctggtctgtgggggagaggggaaggctttggggacaatggctcaacctttgaatatatctgcttttaagagaactgtcttcattgggtgagtggggaaactgcactataggcttccacaggcttaaaaactcccctctcccctttcagtgagtcaaaaaatgaagcatgaatttccctcagttaagtatctcgactaagtggaaaaatgattagtgcaggtccccaggcgctataccgccctaatgcttaggtgcagcacggcagagccccatgcccaggtaatataatctgtgcacctgaattcctgagccttatgcagtgggcatggtaaccctttggggaataaaagttgtagtggatatgaataacaatgactttaagaatgtcctttaactcacttctgaattactggacttgagccaaaatatatggacattagtcttctttctaggacactgctctcttgttaagcactgcattaaaagcagatgattttagtgttgaattcacagtttaaccaagagcactattgggtctttaagaattgcaccctcagtgatttggcaagtgactccaagcagaactagcaccttttgggaggtgcttctttgccctgagtattgtgacataatgcgggggtcacaggaaaagccattttatgtcttaaaactgtttatttcttaatattgaggcagtgggagaaatgaggaaatggttgggagcaggaaggtagaaaagatgtaactcttgcattacgaacttgcactgcagtggttttaacttgcttcagcttttatgaaggcaagctagggtgtgttattttggctaagagttgagacttaggtgaaggtagtgggaaatgactcatctgacattatctttatttctgaatcattcaaaatatccacagtccaatcccagttaactggtacaccacaagaatgagtcatcccatgctagaagcaatagttttcttgtaactttgttgaggatcttgtgagataatataagtgatttatttcataaaagttctcataagaccttgagtcctcactttagcatcaattctggtatgaagaggagcagagctaaatgaagactactaccatactttctgggaactttttttttctttctttctttctttcttttttcttttaaccatgagccagccttagacgataaacaaataggctgattatctggggctttgttagagaaactgctttgggaaggtgatccagagtgggtggtgagtgcaatgtgcagcctctgtcagactttttggcctcctggtatgactgctcagcttaggaggggaggttggcagggccaccaagtggttcagctccgccccttgcagccatttttcctacattggtttgtgccagtctgcacgtaggagggaggccaggctgcagtacttctggtggcctctgggactcacctcccccactctgtccataggcagaactcctggggagctgtaagcctctctttcctgacgccagcaagctgtatttggaagtcagacaaggattctggtgggggagatgccaagagccgctatgatagagcattgagcttgctggtcatagcatttcaaagtaaggaccagctcagctgatccaggggggaaaaaaattctctgaagggagccccagcccttccaaacacttaatcaactggtagataatatttgtttaactttagacaactggtatctcctctgtcttgggtgatgagtttaaaataattagtccgctgagtcaggcttagtataggagacaaagaaaattgcgcattttggaggaatcatggagttttgatctagttaagaggcagaagagtaaaaacttggtaaacaaaaccatcctggtaatctagtatccctcttctgtttttacattagagagcagattaacacatggcacccatcagatgggcaaatgttttaaaagtctgacagtgtcaagtgttggcaaaggtgtagggaggcaagagctccctttactggttgattgtaagtggatataaccactttggagagcagttcggcaatatttagtaaagtagaaagtaaacttaccctgtgacccaggaattcatttctggatgtatagaaactcacgtctggactaggacacatgtactaggagagtattgattaatgaggaaaattttggtttaatgggggaaatgaccaactagtaagggaatgcatagatgaatggactagtcatacaatggactagtatagcagttcgtacaagttaactagatctgtataccaactggatagatcttaaatgtgctggaaaggcaagttgtaggatggtaccttataatacactacttagggtattttatataatataatggagttcagtatagatacagacaccctcaaatgaactggaaaaatacgaagttcatgacagtggttggttatcacagtttatgctggggtgtggaaggactggagggacctggggatggaggaaaatgaacttatttttaagagtctagagaaaatttggctaaatgttaatggtcagttctgggtggtagaaatacagatgttaatatttctttagttcaaagcaaaacaaaatagaagcaaacctacgacagtcactatagggaacaccaggcttactaactaggtcagtgctctcagagctggcactgctctttcttccttccatccccccttctcccaacagctgtgatgccgagcagttcctcctttaaatgctgagccagtgcctcccttttgctgaggccctcaggcatcctggtgttgtacctgacttggaagggctctaaatcagggttgcagatcccttgctgcttccagagtgtaaatatcttgccctcagacaccgccttataattttaagcctcataaggggcacaacacagcaaaaatttcatctaaacttcctcctttagactgaaaccagttctctgctcttagtgtctgtgatcaaaccaggaaatctttgatacctgaggacagcaagatttctgtgacttgggacttcctgccctggagttgagtggtcctgttgggggtgggcccatttagtatcagcttttatgacttattcaacctcagatttgaaatagggccttgggctcctgcttataaagtttaagtcgacttctagccctgaataaaagagcaagggaattttacttgaacctataggtgggctcattttatgtaacctagtaacaccagactttgctttttggtatggggcctgctgagggtagaatggacttaatagtctcatttcttaggctaaaaactgcatgtcctggccccactccatatgcaaatatactgtcatcattactctaactgtatgtgaggatgaacagccattcactcaagaccttactaggttctgtggctggcgcagcacccatgttgatcttagtgctgctgttgtcagattggggccagtcttgggaattatgttctgctccatcatctaggaacagagtccggcacattctgatgcaaactttctagtgaatgctgcagttctgaaggtgtggaaatcgggccttcatgctggcttggagacatggagctgtgggtagcaaattgatgttgcaacaaggaacagctgtggacatcaggtgccgtcatcattgggttagtctctgtggtgagatgggcaacaaagcagaattggtacacagagccctggctagtggaagattggcttaagtagatgcgggctcctaggccatgctggtttactagggcggaatgatttgggcccctataaaggaaagaattggttgagtgaagcatgacttttcccagcacaacctgccaacagtactggctctaagtgacatgctgggtatttttaattaattaatttatttaaaaaaaaattttttttggctgcacctgtggcatctggaagtttcaggccagggattgaatctgagcctcagctgtgacctatgctgcagctgtggtaatgctggatcccctgctctgggccagggattgaacccgagcctccgaagcaacccgagtcactgccgtcggattcttaatccactgcaccgtggcaggaatgctgggcattttttcttatatggttttcaccctttggtttctgaaaagtgaccaaaggattgtgtctgacaacaaaactagtttttgagaaccagcagccacttaagatgaaaggtgggaataggggccgctggagctgagctggctgcctgctctatcgttttggcccccaccaaggcctctgatggtgtctcatttctcacagaggagaaatggctctaaggaagatcctactgcaggggctcaggctcaagaataaggctccctggacagggcacagcatgtgctgccatcagtggatatgcccggcttccactgcgggcttgaggttggctctgcatgtctgtgcctcctgaggaggatgaaggaatgagtcagcctggcgcgggctgggccttgggtgctggcaggcactgtcctgacagctgatgttggggaggggagctctttgcagagacctgccttgagaaaccagggccaaggctgctgtcctggggctgggggagaccccagagggtggtgtaggtggaggaccttggagacaagcaggagagccctgactctccctgtaagggagactctggggtggagtctgaggggagggagacctgtgatgacctgggcatgagtcatgaggtctctggtttggtctgggttttaaggacatgttgagatcttgtaggagtttggactgacttgctgacaagccaggtttttttgattgctggtgtgtaaatccactcaaaggccaaacaaaatttcatttgttgtttttgtccttaatagcctgggtgagcaaaagatgagagcttttagacctcagatttaattcaagatgacgaaatagggttagtgtttgagtgcagtatagttgtatctgctctatgtccttgagacggcccttctgtaccagaacattctttttttttttttttggtctttttgtctttttgtattttctagggccgcacctgcagcatatggaggttcccaggctaggggtcaaataagagctgtagctgccggcctttgccagagccacagcaacgcgggatccaagccacatctgcaacctacaccacagctcacagcaacaccagatccttaacccactgagcaaggccaaggatcgaacccgcaacctcatggttcctcgtcggattcgttaaccactgcgccatgacaggaactcctaccagaacattcttatcacaaatattttcctctgatgcttgaggacagactacgtaagaaaggaagtttgctgggtttgggcacataacaggctttttggcagagaactgtcctatggactgtattaattgtcccccaacccccccacccctttgaggttctgaaagggatcaaggttgaccttcttaagtcagtgaaattatcctgcagtgcctttgtgacctagggcttaaggtgcattattccaccaaggccatgtttaaacggtattcctgaagtgcatagagcagcgatggactaatggaactgggaacttctcattgctttcgcttccaacacttttaccaggatgcttgtaaatctatcatttttggaagaggtacatttgtaatttatcttattatgaaagtatttcacattagtaagctttttttaataagagaagaaaaatttgcaatttacagtgatcctaccacccagataacatgctgatagtaatttggtaactatccttccagtcctgttctgtatgtttaatttagtgacccttcccctactctcccccaaaggggagggaccaggttcttctgagatttttttttttttttgtcttttttcgggccacacccacagcatatggaggttcccaggctaggggtcaaatcagagctgtagctgctggcatacaccacagccacagcaacgccagatctgagctacgtctgtgacctacatacaccacagctcacggcaacgccgggtccttaacccactaagcaaggccagggatcaaacccaagtcctcatggatactagtctggttcgttactgctgagccacaatgggaagtcctaaagagactttaaaggagagcagtctttggagtattaggggagtgataagcctaataccaaagagatggtcccacagaaggaccaataagaactcagttttgcctgcaaattttctgttaatcagtttcttggtattttcttgggaggcttctgtgttttactttataacatggctgaatctctagaagcagctattgccaactactacctggatacctggttattaaggtaatttctctattaccccagagagccttagttgcactcagcttttaccttgatccttgtacagctctgcagggcaaacctttctcagatctgagcagtctttgcaagtggggccaaggagccaccctgaaccaacaaaagagcattatatcaccggaagcccaagccctgagaacacaaggtatgaacagtaatcagtagccccagccaggtctttgcaagagaccctaatgtctcaggtagagcgaagatccaaccgatgagttttaagaagagtggggttggttactttagcctactcattgaggtcacaatacagcccccaggctggatggcttctcccactgggaggccacaccaaggcttgtgtgtctgtagttgaggacttgtagccactggctttcactagcttgcaggagattcactcacaactggtctcaaaacttcttgggctttacctgacttctaggaagtggcagagatcgacttagatgcaggctctgctcaagccacccaaagaggctacaaagttagggatggaggaggagaaaaaggcggggttaaatgtaggggtgccttgatttggagccctgagatttaggaggaggtgggacagggcagaagaagggcttggcttgtttttctgagcctgggtgaagcacccaggcacggggatttgagaaggagtagcccttggtctgagggtttgaggagagagatggtctgctgacgaggcgtgtcaagcttctggctcacatccttgcctgatggttcttcaaatgctgcccagaagcttctcaggtctctgtctataatcagctagctaaccggctgagtgagtttagttgtaagtaatgaagaaaagcaaaggttggggcagttgtcaggagggtgacctgtgctgattaattacctggaacagatggtctttgttactcggggtggtgtgcttgtcagacttagaaaggcaatcgggttggtgcatcagaagatctgctgtggagaggatttaacaagcaaccttcacttcctcgtgttgcaactgtcctgttaatgtaactgtagtaattttagaatcagatagtgccactgtggttatcgttggcttgatgcaaactgcttcgcatgtcctaaagtcctgaccaaaagttacaggatggggttgggtacagattcctgggactggtttttattgcctgtccgtggcctgggacctcctctccagcctagggtgaattgaggaatgtgcttatgtagtcctgtgggttagtgaaaaccttggactccagaactaggaagaatgcctggatggtggttatctccatgattaagaaagtcactttgggtttgggtgtagattgttaagaggcagtgtgggtgccctatcctgtagcaggtatttgtagctttgagacagctttttgtacaaagatctagtttgaccaaggtactaaactaggggtgagttgttgatatcactgggagattggttgcagcttccttcagtgcatttaaaatgatatttataggattagcccagggtgagggtggtatgcttacagtggatgcctgggaagtcccctgtgttggccatgctttttaacttgtttctttgtggtcttttccacttgctcacggtgacaagcctggggacctacctgaggagcacccacacagccagagcgtggcagggctccctgtggcctgtgcacagagcgtgcttgttgagttaatgtgtaagcaggaaacggcttcctgtgccaagctgtatattagccatcccaggcctctcagactgatccctctctctcttcagttcctctggacccaagacctcagaagccatgccgaagccccacagtgatgccgggaccgccttcattcagacccagcagctgcacgcggccatggctgacacgttcctggagcacatgtgccgcctggacattgactcgccacccatcacggcccggaacaccggcatcatctgtaccatcggtgagtgggggtgcccccctcccctggaaacaagggcttcatgagacagggatcttttctctcctggaaagactaaataaatgtagcaaacctgggtgctgagtgagatgctaaaaagatccttatgggtactgaggtcataggaatttacagtgaggtactggtatgctctacgcatgctctatgctttatgataaaggtgaaatttagagggtatcttccttagtggatctttgtaggaacatctcagaaacctacctgggaaagatcttgacatgctgtgtacaactgagactctgtagctggacatctgggtgggcttcagggagtgcagagagcgctggtctagtcttagctaggctttcctaaaagaattaggagttatttgggggaggaaaagtttaaggggagggaaaaaaatttttttttgcttcttatactgaagcaaacttaaagtgttattcttattttgaataattaatacttaatcactttaattttttttaacttaggcccagcttcccgatcagtggagacactgaaggagatgattaagtctggaatgaacgtggctcgtttgaacttctctcacggaactcatgaggtgagcctctgccggacagtttggccactggggcaccttgtgggcaacagggcgggagatgccatgttcatttagccacggtggaccaggcaagaaagattggtttacagccagtgggaaggttgtcttcaccagcccatcctcacgctcctttcccctctcctcctcctgccctctcaagtggccaagtctcctctagcaaacaagacctgctttgtcattggccatggttctcccccacagctgagctccattagccctcagtaaggaacgtgtgggagagtttctctggaaacccctctaagccatggggcttgacattcccaccccagcatttctctaacagcttgtgttgcagtgatgaaccaatggctcaccttgcaggttgattctggccaagtttagacccaagacaaactgggcaggtccaggagaagggtttccactgttgccagtgaaggactgagtctaatgctctaacaccgtctggtgtatcctaccccacttcatctgcattgtgttgccagcctttcccttcccagggattctggtacattgaaataaagaagccagcatgtttccctaggagcctggtaggaatatcttagctggggctgtttatgagcagacttgacctgtgggaccttacctggggtcgaggtagaagctattgggaagcactccctcatgcttctgttcccaagttcagaacaaatttattttgaggagtgtgggagctccctgagggacagtgccttttaaaaagaccttcagtttcaaccacagaccatgggctgatgagagggtaatggatgagataaatttttctcactcttaatctctgtatttcctattcaggataaagaaaatgctaccccataaggtcaagtggtgaggggttgccctctggcatttggcagttggtgttaagtttaaactaaaaataaaggcttagaaggtgcaatccaagagctgaattcctcctttctggaaacatgaggctcttcattggaggttccctaacccatatttcataagcagcctatggtctggcaggtatccagcctccaaatgtcagaagggcctgaccaagtgcagaggaaccgtgctcagcaggcccctcgggcaggttgatacgtctgtggtggcattctgtaattttccaaaggcagggagtcctcagcaggaagtcactgggcattcctgcaagtattagcttagtccacggagagagctgaagacatcagtgaaggtcagttcactattgattgctcctgctggcctgtgtgcaggggaaggagcagaaatagattttaagaagttgacctttagctaggctttatggcttcttccatccagtaaaataacaccacacagctctgaaatggcaagggccagtggtatctggtgcacctgctggaagggggctggctcagggattttggctttttttaactccaagaggcttttgtaggttctctgtgctttaactctcattccaagatgagacgggatttaaacaaaaacccatgcctgccttgtggatttattttgagatttttgaccaggatgaagtgggttgtccctgggatcggcattttagaaactgatctgaaattgttctaatattaattatataacgtaagcagtcttattttgacaagcagttggaacatccttttccagctcatgacagttttcagtattcttctaagcagaacattggaatggctttctctccctcactgtgacaatgggacctccagtgtctgcatctgatctttttgtggggttgttgttgctacagcatctgatcttttgacagctttgccatagcacctctaaaccccacttttggcaagatgtgttcctactgattgtgtggtcccattgtgccatgtgggccagaaatacagacttctgaacaaactaaatgtagaaccttccataaggacagtgttggtttgatggaattcactgccaccccgccccagtcccctcctcgtgcgtgccactctcctggacggtggtggttaaatgacaaggcccataaagtgctgagttgggagacttttatcagcagtgtcatttcaataactcttatctaagagcttttgacttcttgcctctgagtccctttttagtcaagtagttgtggcaaatggaaaaagaaaaaggaatgggagaaaaaattatgtattcatgtatgtgtaactgggtccccattctgtatagtgggggaaaaaaagtgtgttgagggaaataacaataaaaaaagaaaaagagaaagggcttcacaggtgagattaaaaccaggatttgttgcaagtgagaatagcaagggttagttagttcagagaaaggtgtgttcccaccgttgccttttgcactttgagactcgaggaagtgattatcagaaccaggtctgtaggacctctgcaatgagttatttagcttggaccactgttagcttgagtaaataactgagtttgaagtgcggtcataatcaatagaggaacagctcagaattaccaaatctgtcagtctgaccctgatggccaccagactggtattttccaaacataagtcctaggtcttttagcccaagtgtctgctttatttgctgagggtttaggtggcagtctaaaagttcctaagattggccctgagagcgggggagtgctgtggtagaggtgggtggaaggtgcttggtgagtgggcggcgctgagactagccgatggcgacaggggtccagagcgtccgtccacagctctttcctgagtgctcagcttcagctctggtgctccaccctggggcagggaaggtggcttatccttctccctcctttcccccagtaccatgcagagaccatcaagaacgtgcgtgcggctacagaaagctttgcttcagatcccattctctaccggccagtggctgtggccctggacactaaaggacctgagatccgaaccgggctcatcaagggcgtgagtatcctgggggaggggggaaggagctggggccccagagacatcctctgcagcctatcccacccggaagccttgtttctcagagctgaggtctatacatgagttttatccatcactgcaaaaaactttgatctactttgattagaaacaatacccagaaggaatgattttttttactctcaaaacttgcttccaagactctcctaacctttgggatcaacttgtctcttttcccctatcatgaaatagtatcactaaaaccttgtgggtttttcttgggtcatttccttgaaatatactgagttagacaatgggatcatttctttccaaagaaaaaagctttattgttacttccagctgagatttgagccttgctccctggaggaaagcttttcttctcctgccaggagggcctggcttctctggacctgtggcttcctcttgtctgcagagcggcactgctgaggtggagctcaagaaaggagccacgctcaagatcaccctggataatgcctacatggaaaagtgtgacgagaatgtcctgtggctggactataagaacatctgcaaggtggtggatgtgggcagcaaggtctacgtggatgatggacttatttctttgctggtgaagcagaaaggtatatatgggagccagggtctaactgtctagaggcagctcccatctcttttctttggcagaagataggaaggtggtgggttggctggcagcaagattgaatccatgcatcctcaggaattccttttataataaactccttatcctcaaaagcagctctgtcgtacctcttgggaagcagatgagaggatttcttttctccctgtccgcactacttgaggttttctgcttttctcctccatctccccagtgtggcatgtctgggactccagtatgcctgtgattgatagctcacacttcagtgccaggtactactctaagcatttaacatattaatttgtttaaattttaaaacaacacgaattccttggtggcacagcagattaaggatctgtcatcgtggctcaggtcgctcctgtggcacaggtttgattcctggtcccagaactttggcatgtctcaggtgcagccaaaagcaagcaaacaaacaccttatgagtagatattgttattatctctatttaactgaggtatggagaggttaactgacttaaccccaggttacacagctagtggagtgtggatgtgaaccctgcaatgtggctccagcacccaccacgtgctgtcacccagttctgtctcctggagagagcctgcttcctggggaagacgtggcccccatggccctgccaccccacctactccattcccacaggtcctgacttcctggtgacggaggtggagaacggcggcttcctgggcagcaagaaaggtgtgaaccttcctggagctgctgtggacctgcctgccgtgtccgagaaggacatccaggatctgaagtttggggtggagcaggacgtggatatggtgttcgcatctttcatccgtaaggcggccgacgtccatgaagtcaggaaggtcctgggagagaaaggaaagaacatcaagataatcagcaaaatcgagaatcacgagggagttcggaggttagtcctcctgcctctcccctgcctccttcagcccccggcccagctctttgaagagcaagatgtccctgtaaatacctgcctccctgcccatcaacttagaggctctcaagcttatttcagagccactgaatcagaacatcctaagagggggagtggaaagtgttggttttttcaagggggaaaaacaaaccaataacttaggtgattgggatgctggtatcttttttttttttttttagtgatttttatttttttccatcatagctggtttacagtgttctgtcagttgtctacatacagcatggtgacccagtcacacatacattcttttctcacattatcgtatgctccatcacaagtgactagacatagatcccagtgctatacagcaggatctcattgctcatccattccaaaggcaatagtttgcatctatgaaccccaaattcccagtccatcccactcccacctctcccccttggagccacaagcctgttctccatgtccatgattttctcttctgtggaagggttcatttatgaggatgctggtatcttgacattgttcctaggccccaggaccagcaccggagagcccagggccactgcttcccagtttgggagccatcacgctgtgctcctaacacagcctgtgtttgctagaattgggccacccacagggaaggcagcagactcttaggggtgctccctcccctgggagccacgtggaagctcagggcctggggttgacaccaaagcatgtggcctcctagtcttcactggccgtggcttgggatgggccagttctggcatggtatcagcttcctagggggaagcatgccattctcctccaggtccaggttgtcccagctcatctcctccacctccccattgctcaccaggtagagccccatgagcatagccagcttggtggcatcacttcctctttggttcctttctagaaacacagctcagtgctgtgaccccctgacctgcttgtgtgggttcagtatgtgtgtttgcccaccttagctttgtgtagatgtccttagtactgggaaatttggggtcctccctctgccatccagaaaagccatgggtacttgctgaccttgtctccaggccaagcaaagccatatccccttgccttcagaaagctggaggtgccccctgaaggagcagccctcaggtgtccttgggtggaagaggccatgaacctttgtgtcaggagcagtcaaccaccttgggttccctttgctccaaaagcggggactggactggaggtggtagagaaacaccttaagaggggcctcataagaaggagatggagaggaaatgggaccctgggactttggaatagacctcactcccttccatttcccccagtaaagtgtccacactggtgccgacgaatcccagaaagcagaactgtcgaccctctttgaggtactgaggtagctggaagacccaccacctccatgtacccatgatgacttcatgcatgggtgtttgtcttggtgcaaggacggctgagtcagagaatcccaggaaaacgtcctttgtatcaccattcttctggcccctattccatataacttctctctctttccaacttacctgtcagatttgatgagatcctagaagccagcgatggtatcatggtggctcgtggtgatctaggcattgagattcctgcagagaaggtcttccttgcccagaagatgatgattgggcggtgcaaccgagctgggaagcctgtcatctgtgccacgcaggcatgtgcctctcctggagcttacaaccttgcacggggaagcattggcggctaccgggtctctcccatctcttccctgctccacgtctcacataacacacacacataccccctttcccccacatccctacacaaagccattctgtctgcacatacatgctctctaggggggttagcctgcagtcgtttgtgtccggagacagtccaggccacgtctcacgagtactctgtcccctcccagatgctggagagcatgatcaagaagccccgtcccacccgggctgagggcagtgatgtggccaatgcagtcttggatggagctgactgcatcatgctgtctggagagacggccaaaggggactaccccctggaggctgttcgcatgcagcacctggtgagttctcagcctgccatcttcccgctcagctcagcttgggcttgggctgggatggaggtgtgctctggcactgagcaataccttttaggcttctatgcctacagggttttatctgtcaagtcacaagccagagtgaggagatgtgtgctgggggcatggagatgtcttattttttttctgttctaccttcctgcccacacccctctcccagttccttctgttctggaggtggcctccttcagcagacgtagcacaattcactcctgtcttcagggttgtgaattcttcctttggctccagtactgggctatctatctgtccctggacagcccagaggacctgagtacctctgccctattctggaaaaggccacaggctcctgctcccagctgttctttgtttggcttctgttttgactcgacacctgtcccaagccagctgcctccgcctgcaggaggagcctgggcctgcggcctgcactggagtctgttgcccacgctgagtcgactgagctggctttgcatggtgcctgcagcagcgcctgctttgctgagctgttgcactcgcctcagactacaaagtggggtttaagtggtgggtgacagggccacaaatagagacagttggagggatgactgattctggctggctctggggtgagagcatctggaggagccctgagggccactcgtccttttcccctaggacctagcttttcagggctctcccactaagctgtgtcccacagcctggctgcttctcagggcttgaggctgggttcctgtgtctgctcctgctctagagcttactgaagagttagtgcagggatcagctatcagagctgagaaagcaagtgaactttcagagcagtcccaggtcactgtcgatatagctcagtgaatgaacttgcctgttaacctgaaatggtgtttctttaagcttttatttgcttttcagccaacaaaagaccctgtgccctttgtgtgacaccctctcccctgcattccacccaaatttaccccccacacacataccccataggaacccctggactagataggatccttttttccttcactttctgtgtaattattaggctttggtagcttccaaagaagatatgactaaatcattttttacactaaatcgctttttcagtggtgaaacaagacatcttgactaaagaggctctctgggctgtccttggcctcctgggtgggtttgcccataacaaaattgatagagaccaatccctgtccctgggatgcgagatatgtttagttagaaccttagagttaaattttgctgccaaaattttcctgtgtagattgatgtaatcttcataacttcagtgagatagaagtcaccccttgttatagaggagggtccctgatgataggacttgagtctgaacccagatcatctggctctaaaacccgtgttctcctctgcaatatggtgcttcgtctagcaggagatcaggacaggtttccatgtgggggctgtgcagaggccagagacgaggcatcaggctctgggctttgaatccatgtatgtttttccatatccctgtctttcctttgaacagacaccttagaactgcaaggctgggactgaatagcactgctcaggagataagttatggagtctgggccaggcagtgcaggcctctcctgtccatgtcaccagttaacactggccagcagcttcccctcttaactgtccactgctttctcctatatctaaccgaggcagtcaatatcccataactaagggttaggcaataccaggtatggttctctttcctgtcacatcccctgtcctgtgggctgcatgccttccattcttgcagggagaaaacctttaataaccgagcaaattctgccactcatctgcttatcctatctgattaatgagatggcattaccaattgtcccttgtccatcattctctaaggtgctggtaattgcattataacctctaagcttacattttctttctatttcttggtctgagcaggtctgtgaataactcagtggctttctcctgggtgttttaatcacttgattttaatgaaatgtcttgttacacttacctgcatgcttccacaggcacctgtctcttcacatggctgttcagtgtgtcccctcacagctcaccgattttccacctgcctgtttagaacgtggtcaagccacgtggccttggctttgtctgacccagcttcccagcgcagctctgtgtgcttccatggcaggccattgcaaaggctcgtagcgtccctgtgcctgaagccaagcaagtgctccatgaatgcatggaggccggcaggaagcccggttggtaaccagacagccatgtgaggaaggaggcctgttccttcctgtgagctgtgtcatgaggcagcgtggtcaagtcctaccagggagccatgcaggcccagcctatgtatgtttccatgccaaggcgctagggtctgctgccatactgtctcccaccgccagtcaaaaagtccttccaaaatcaaaaggcccaatttcccttctgttggaagggaagcagcagcagtcagtgcttggaccacacctccctgagtgggcttccatcaccctgcctctttgcatctgcctaaaggacagacttagccaattaacctaaggtaccttcctctctgattaattccccattctgtctttccatgttgttgtctctcgttttttttttccccctcctccttccctcttccttgcctcccctcctccttaaaccttacagatagctcgtgaggctgaggcagccatgttccaccgcaagctgtttgaagaacttgtgcgagcctccagtcactccacagacctcatggaagccatggccatgggcagcgtggaggcttcttataagtgtttagcggcagctttgatagttctgacggagtctggcaggtagggccccgagagcaggtaactctgtaggataaccagcctcttgctccagctgctctagaagacagccagggcctagccctctgctcaggacctcttctctcatctgcaggaagccagccagggaggtcagggcacgacaggactgcagggtccttgagccccgtagggacataatgtcacaggcacctggtgaagggctggttcctggggagccttgatctcacttagccccacaccccaatgtttgggctcctcttggcctctgcacccagggacatgttcctcaccagctgtctgtgcgactcttcccctccctctcccgtgtgacatggctctgataaagctctgtccccctctcgtccatccggacggatgttgcccccctagattgcccgtgaggcagaggccgccatctaccatttgcaattatttgaggagctccgccgcctggcgcccattaccagcgaccctaccgaagctgccgccgtgggcgccgtggaggcctccttcaagtgctgcagtggggccataatcgtcctcaccaagtctggcaggtaggaggtggcagcggctccccaggaacgccccgctcagtggcacccttccttgggggtcctgggagcagtgcactgaatggtgctcagatggcactgagccaaggtaagacccctctgcctgcgccccggaccctgcagggaaggagctcccccagccccactggccaggctctgggagcgagcctagcccttgccctgggcctgaaggatgggaccccaggcagcacgcataggatgaccgtttgggtccaaatcaagtttatatcttcatgatgaatcagagacttaattgcataactacagatagatagagtgatgacaaatggttattcaacattaaaagctgttctcaaaaagtaggagataatcagctaccacttttgcttattctagttactacatgctctttaaaaagttcagtttggaaagttagtgctgcttgcttacatgctttggttggtgcactcatcccatctgtctttgagtcccaaagacaagtaattgggtgctgcccaggaaaggtcaccgtgctgtcttgctggcactgtgggactgggcagccacgccgaggcctctgcttgacctcagactcggggtcccttccaaattcgggacattgacttatcaactttgctctggggcctggcgatatgctcctcccagggcagctagggtttcctggaagaggagggtggagaggaaggaacaccgaggagcagcagatggggctgctgtgggaccatgacacaagatgcagatttcctcagcagagggctcagaataaacagttccaaccattagggttgacctttgtgaaaaggtccaacctttgctacttggctatttttaactccagtcttctgggatttcactcagtgggtcctgacttcagcacttgcttccctccgaaagccttgtatggaggccagcccttaagcagggcattctctgctgtgacatggcttaagtttccctgacacctgttgagtgccctcatagcttgccttctggggcccagttccccctgcaagcccttccaacccctaagacacatctgcagctacaagtgcatagtgtcagtgttgaaagaagtgccggcattagggttttaagggggggggccctcacccctccagaggagcctccacaggcaaagccttccctgctaagcactccaatctcctggtcttgactcctgggtagcacctatatttctaaacctcgcttgggttttacttgagctctacagcccagttgctgggactgtttcaggggtcatgtgaggtcgggagagggcacagcagaagggaaggcttgcgttataaagtctcagggggactggtgggctctgctcctgttttatgtagatgtcaagagtcaggtgctattcacatgctgcttggcttgtatgtagtgttgctggcagcaaaagaaatgggtgtggtgaggttgggcagggctgcctccctgtgccagaatggaaaaattcagggaaggggggttctgccaactatgggccctgtgggtaagtgggtgagcctgaccaggctgggtcagcatgatccccaggcccaggcctgtggggaggggtgcagcatagatggagagcacagctgtgaagaagagctatatgctgtggaagataaaggatgaggggctgcccagccttgggagcagatactgaactggtcagagccttaggctggcatggtgagttggattagagggtgagctcttgctaaaggccctgaggggcttcctgggacactgtttaatggtcttgcctgtccctcatctcaggtctgcacatcaggtggctaggtaccgcccccgagcccccatcattgctgtgacccggaatcaccagacagctcgccaggcccacctgtaccgcggcatcttccccgtggtgtgtaaggacccagtgcaggaggcctgggccgaggacgtggacctccgggtgaacttggccatgaatgttggtgcgtggctgggaagcaagggctagaggtgggggttggggaaggtgtccctctctaatgctgaatgttctctctgaatcctccatcccattccctgaagcctctgggctgagaccaggagggtctgatccacccattttctctcctcactctcttctagtctggggtccaaagcaagggatcctggagagctagggttgttcattctttagcatctgctcattattgagatttttcataaatttagccagagctcctgcattgtggggcagcccacatatggcttctgtccagtataagagcagagtgttgtgggatcagaggaagcagctatagctgtgaccttgagctgggctctccaccctctagagtagaaaatgaatgttgtccaaaggtccctgccagctctgctctgaatgataaggaaatatcagggctgtggggctggcgccaccttgtgggtataaggaagtaaaggcctgcctgtccttcttgctatttttgattgtggggccgtcttgcaggtgcataccttcctggcatgatttttactcacccgcctctctcctctttttccccaggcaaagcccgaggcttcttcaagaagggagatgtggtcattgtgctgaccgggtggcgccctggttccggcttcaccaacaccatgcgcgtagtgcctgtgccgtgatgcaccctgcagcccctactccagccccatcccatccccctccctcaatccatccattaggccagaaatgcttgtagtgctcacttggggccgtgtgtggcactggtgggctgggacccagggacacctctgtgaaacatggctgtttttaagaccctgcttgggtggggtagttcagagctggacctcccatcaagtatccccatccaagcaagggatgaaggaagggtgcaggcaggactggagtccccagagggcaacagctcctgcttctcttcctttgtgtactcctgtagttctgtagaaaatggatacccagagaactcccagccctggcctggaatcagcaaagagcaggggccttagggcatggggcatgaagcagtggttccagtttaagcagactctggccctggcccttacttacttctccaacccccttagcctccctcactccccctttgttgtgcactgtgcacttctgttccttcactccatttagctgccgctgcagacaaacactccaccctccacctcccatttccccgactactgcagccgcctccaggcctgttgctatagagtctacctgtatgtcaataaacaacagctgaagcacc

SEQ ID NO: 54 - DNA, 26664 bp, Bos taurus
ggcacttcctactgaaggtgactgtgcccggcgaggacgcggaggggcggggccccgagagccgggagccaggattggatgggaggcggggcggcggagggattgcggcgacccacagtcgggataaccttgaggctaaggcagcggatccccgcattggagcgacgcgtcgcgagccccaggacctgtgtgcagtagccgcgcatcccgagccggaccacgtcggaggtgagcgtggggagagactgggccatccgtccccaccggggctccgtctcccggggcagtgcggaatgctggcccgcctgcgcactcaggatggcgcaggatccgcggcatcgtgggctcacccggttgggatcagaaaagaggagaaaggctgcttgtgcctagggtctccttcaaatcccccagctcccgcttcttccgaaggcagatgggtcagccagcccctttctttccccagtccctgatctcccatccccattctggtcccattctcacctccctattcctccctcctctatctggtctcgctctcgtcttcctccctttattctcctaatttgatagtttcctttcatgcgtcagtctcccccatttccactctgctcctatgcccgtccctttcccatcatccttaatactcgcttcttgttttcaacctgtccatgtccccctcattctgatgctttctgtaacttctccttgaaagtccccaagctccgctcccctgtttctcctccattcagctgctgtccccttcttgtacctaccctcattcacgccctggctcccgcccctcccccgcctctctggtcacgtcgctccagcgcatccctctcctgcgcaccttccttcgcgccaccagcctcctcgcccctccccttctgttctagtcacgtccgcctgcactcacgtccccgcccctcggcctcgcatctcctgccccccttctccatcatagttccccagccctgggctggagttccggggtcagctcccgaagtgcagcggtctgcggatgggcaggctggctcccaggcgacccggagatggatgcagtggcggccggaggagcagttaggttacataacccttgatctaacccaatgcaaaggaagaaagggtggctgcccagtggcgcgttcctgttttgtgctgcccagaatacgatagtgcgaccgctgcgctccgcttgctccagggggccttgggggcggggggggggggtggagggcggtgcgcggtgtcccgggctccatcccgccgaggcggggctgcacgtagcggcgccggacccgccctgccgcgcccgctcctcggcatcacgaaacactgaccttcgggcccgttaccgaccaagcatcatctccggcccgccaagcctctggatgctgctcagaggcctcctcgagttcgaggcactcacctggctccctgcctctgcttcacgttacttaacagcgttgcttaacagatgcgcccgattgtagagcgcggaggccgcgggttggaggagagtagaaatatatcaagagcttggtgccacgtacatgcgctcattcaataaaaactcgtataaagagttgtttgggggagggctgtggagaccagaccaggatgactaaaatcgtcctagcctacggaactcagtctgattagcaaacgaatgtaaaagttaccactgtaagtgccgtgaaaaggtacacacgtgcttccacacgtggagggtacgcacttcctgtccgggtttaggaggcctcaccaggtgtcatcacacggggtttgatgaagcggaaacgcaccttccagtctgaagattatttgaagacccagtaatgggttggcatcccttggcttcttatctgtgttcttcaaacccagaacactgatccttccccgtacaaatgagcctgataactgaggtccgtgacggacagaggcagtgggaagatgaaaacaggctttcagaatcaggtttaactcattacatactgatatgaataatagagggaattcagactcaggacctcagtttcccatgtgaaaattgtaacttttttcatcttggttgttaaaagggtgggtcgctatatacacacttacatagatacatattgagtactgggtgcagtgtttaatctctggtgagatgcccccagatgtattcttttggtcacagtgagcccaatgacttcatccataattgaactcaagcactcctcttcttgctgccatcccaaaacacagactcagttcatctttgggagtcaggctctgtgtaaataccagagatctcctagaaaccagtccgctcagggatcctgctgcagtgttggcaaagtaactaacaatgttactttgctgctctccatttgcaacaggggctctttggtcctctagccaaaggaaggcaagaagagagatggctttcagcctcctgtattatagattttggctattaagattagaaacaaacttgcaaacctaagaccaaaatcttcaggttctattggcacctgctccaggtagcattctgggatttgctcaaccagctggtgtgagattaagataagaggcaaaggacagtagctccttgttggctgtatgcagggtgtggccactccctgggatatagagaaggccctaggtcaggactctagtcattgttagcaaataattcaccctcaggttgcctgaggatgctgttgggaatgcaggggggcctgttctgaggggaggagtatgtaacacctcaccagatctctggggggggtggggtgggggaggatgtagggaagatgactcaacctttgaatttttctgcttttaagagaactgtcttcgttgggtgagtggggaaactgcactgtggtctttgcaggcttaaaaatctcctctcccttttcagtgagtcaaataatgaagtatgcattcttcccaattaaaagtgcctcagctaggtgacaaatggatggtggaggtccccaggctctctggacaatgcttaaatgccacgtggcagagcctcaggccccagagatagtctgcacacctgtcctgagccttgtgcgatggatgtggcaacccttttgggaataagcattgtagggaagatgaataatgatgacttaaagattatgtccttgaactcatttctgcattactagaatggagccaaaatgtagggacattagtcatatataggacagctgctctcattttaagcactgcattagaagtaaataatttcagtgttcacagtttaaccaaaagcattattgggtctttaggaattgcagccccagtgacttggcaagtttggtagctgttactccaaacagagctaacacctaaggggaggtgcttatgtgccctgagtgttgtgacattaatgttgggtcacgggaaatgccattttatttcttaaaactgcttatttcttaatgttgaggcagtgaaagaaatggagaagtgtttgagagcaggaacgttgaaaaacatgcaactcttacgttacagacttgtaatgcaagtctacaggagtttttaaatatttatcttcaggttttatgaaggcaagtaagggtgtgttattttggctaaaagctaagactgaggtgaaggtggggggaaatgactcatttgacattaactttatttctgaatcatttggaatgtccacagtcaaatcccagttaactggtgcaccacaggaatgaggcatccatgggagcagagttgttttgcaacactattgagtgagggtcttgtgagatatgtaagtgatttatttcgtgaccagtcctatgggaccttgaatcatcactttaagcttcagttctgatacagatagaactaaatgaagactactctttgcgggggtggggggggtgttgctttgtgtcacagcttgtgggtccttagtttccccaccaggggtcgaacgtgggccctcagcattgaaagtgcaatgtcttaaccattggaccactggggaattcccaatgaagaccattcttaattctaccatactttttgaaaacttgctttttctctctctctctctttaaccacaaactagccaaggactagataaacgaataggctgattatttggggctttgttaaagaagctgttttgggggaggtgagccaggatgggtggtgagtggcagtgtgtgcagactctgctgaacctttggacctcctcctatgactgctccgcttaggaggggaggtgggcagggccaccaagtggtgcaaccccacccctgcagccgtttttcctatattggtttgtgctggtccgcacgtaggagggagagccaggcttcagtacttctggtggcctctgtgactcccctcccccacttctccctataggcaaaactcctggggacccgtaagccgctctttcctgacgccagcaagctgtttggaagtcagacaagggctttagtcggggagataccaagactagctatgacagggttgttgttcgtggcatttcagagtatggaccagctcggctgatggcagtttatattaaaaaaaaaaaatttttttttccttataaaaattatctgaaaggagccccagcccttccaaacatttaatcagccaacaggtaatatttaactgtaggtgactggtgtcacatcacccctttctcaggtgatgagtgcagtcatggcatatgagaccaagccatacaacgttttggaggagcactgaagttttagtctggttaagagtcaggaaagtaaagactcaaaagaaaactatcctgatatctgatatccctcttgttatttcgtcaaagagcagattaacacatcaccaatcagttgggcaaacgttgtaagagtctgacagtgtcaagtgttggcaaaggtgtgggaaggcaagaactcacttgactggttggttgtaaattaatgtaaccactttggagagcaattaagcactattttgtaaaacagaaagcaagcataccctgtggcccaggaatacacctctggtatagaagccacacctgcacaaagagacatgtactaggagaaatattatagtattgattaatgaggaaaaattgggtttagtgggaaaatggtcaaccagtgagggaatacataaatagtctagtcacacactgggctagtatagcagttcatatgaattaactagagctgtgtgccaactggatagatcttaaatatgctgcgaaagcaagttgtttgataatgcctttcagtgtattacttagcatattatagaagcagcagtatcatagtgttgaatagagatacagacacccttagatgaactataaggatagaaaattcatgaccttggttgggtattaggatgtgatgtgaaagggttggaggaaccacctggggatggaggacaaatgaattggatacaatggtaattttaagtctaaaaatctggattaagaacaatttttttctggccatatctcacagcatcttagttccccaaccaggtttgaacccagcccttggtagtgaaagtgtggagtcctaaccattggactgccagggaattccttggataatattaatggtcagttctgggtggcagaaatatagatgttaatgtttcttccttcagttcaaaacagaagcaaacctatggtggtcactgtagggagaccaggcatactaagtaggtcagtgctcgggagatctggcatgcctttctcctcccatcccctcctcttctccctgcagctatgattgattcagggcagctcctcctctaagtactgagccaaggcctcccttttctgaggctatccctcccctggtgttgtacctgacttggaaggatcctgaatcagggtcccaggtcccttggtgcttccagagtgtcagtcttacgccctgaagcactgtctcataattttaagtttagtaaggagcacaactcagcaaaagctttgtctccacttcctccttcagactgaaaccaggtctcttctctgggcatctgatcgaaccaggaaatcctcagcttttgaaatggtagcagtttctctgactcaggacttcctgccctggagttgagtggtccttataggagtgggctctttagcatcagcttttgtgccctattgcacactcagatttgaaataggaccttgggctcctaggtataatatttaagtcacttagttctaaccctgaataaaagagcaagggaattttacttaaacctacagtgggctcattttgttttgtgtaacatggtaacatcaggctttgctttctgttatgggacctgttgagagaatggacttaatattcccatctcttagctaagaactgcttgtcctggccccactccatacttgagagaatggacttaatattcccatctcttagctaagaactgcttgtcctggccccactccatacgcgtatatactgttatcattactctaactgtgtaggaggatgaagggcttctcaggtggctcagtgtaagggacccatctgccagttcaggagacaatcccgactccttggagtaggaagttgcaacgactctagtattcttgcctggagaattgaatggacagaggagcctggtgggctacagtccatggggtcgcaaaagagtaagatgcgaccgacccacaacaacaaataggatgaacagctgagattcattccggaccttactaggttttgtggctggcctggcacccattttgattttgtcgctgcctttgtcagataagggccagtcttgggaattatatttttctgctccatcgtctactaacagagctcctagaaagcagactgacctgaatgccttgtccagcatttttttaatatttatttatttcaccgggtcaggtcttagttacggtacatgggatctagttccctgaccaaggatcaaacctgggccctctgcattgggagctcggagtcttagccactgggctagcaggaaagtccctgtccaacatactgtgatgaaaactttctaatggttgttagtgtgccaaagatttgggaatcagacctccatgctggcttggaaacgtggagatgtagatcgcaaattggtgtcacaattgtgggcagcaggtgccatcatcattgagtcagcctgtgtagtgagattggcatcagagcacacataggttaaaggttggcttatgcagatgtgggctcacaggccaagctggctttctagggcagaatgatgtgggcttttgggaaactcgaatcggtggagtgaagcgtgagtccttcagcacaccctgccagcagtactggctctcagtgacgtgttgggtagtttttcttttatggtttctaccccctggtttctgaggagtgatccaagacttgtgtctggcatgaacagaactgtggcttcagaagaccaggagccacttggaaaggagaggtcggagctggggcccgtggagctgagctgccacttgtgcctgctctcagtcctttcaactgctctcaggcctctgatggtgtcttgtttctcacagaggagaaatgtctctgaggaggatgctacaacaggggctcgggctcaagattcaggttcccgtacccgggcatggcatttgctgccatcagtggagatgcccagcttccactgctggctggaggttggctctgcatgtctgtgcctcctgaggaggaggatgtaggaatgagccagactggcatgagctggacaacgtgtgctggcaggcactgtcccagtggctagcctgagggtgggggagctcttcccagaagctggccctgagaaaccagggctgaggctgggggagagtccagggggtgttttaggtggggatgggcagcttgtgctctggagaagaggctcatgggaggcttcagggcaaagcttgagggaatggaaacccagctggggacctgggcaggtgacaaggtctctggtttgctagtggactttaaggacatggtgagatctcataggaatctggacagatttgctgacaaaccagcttttttggattgctggtgggtacacacactcaaatagcaagtaaaatttcacttgttatttttgtacttagtagcctgggtgagcaaaagatcagagcttgtagacctcaggcttaatctgagataatgaaatagggctagtggttgagccgagtgtattaattgtatctgctgatagcatctcctgttgttgaggcagcccttctgtaccaggatatccttgtcacaaagattttgctctgatgcttgaaggcagactaaacaggaagataagtttgttggatttgggcatgtaactcagatttggggcacagagttgtcctatggaccatattagctttcctccccaccaacttggaagttctggatgaatcaaggttttacctgcccattgcttctgcaccatcagtacaaataccagcacattaaagaaggcaaataatgtctttgaaagctctgctctcacggaccatcctttggtaaccgctagagttactcagttagagtgactcaggtttcttttttcctcactgtgtcatgtggcttgtgggatcttagtttgccaaccagggattgaacctgggcccagggagtgaaagcgctgagtcctaaacactgaaccaccagagaattcctaaggttgatcgtcttagtcagtgaaactatcctgctgtgagtttatgatctagggcccaagatgcattattctacctctaccatgtttagaatattcctgaggtacatagagtggcagttgaataatggtacaaggaccttcacttttgttttaattccaacatttttaccaggacgcttgtaagtgtgtcatttttgaaagaggtacatttagaatttttcttatgaaagtagtatcagtaaactttttagtaaagagaagaaagaaatttgcttgtaatcctaccacacagataatatgctgataatattttggtaggtatccttccagtccagttatgtatgtttaatttagtgcctcccctcccaaagaaggggtggggggtaatagtgaaatattagtaaacgaaggtttaaagagacgttatagggcaggggataaagcattgcaaaggagccactgacaactcttttacctgagaattttcttgggtgacttctgtgtattaatttataacgtagctgaacctctaggaactaccactgcctggatacctggttattaaggtgatttctccattacccccaagagctttagttgcactcagcttttaccttaatccttgtacagctctgcagggcaaacctttctcagctccgagcagtcttttcaagtggggccaaggagccaccctgagtcaaaaaaagagcattatgtcaccggaagcccaagcccagagaacacaaggtacggcacgataatcagtggccccactcgggggtctttgcaaggagaccctaatgtctcaggtctagagccgatccaactaatgcctcttttgggggccacacacagcagtgggatcttactttcccagctgaggatcagactcatggtccttgcagtggaagtgtggagtcttaaccactggactgccagtgaggtccccaactgatgatttttaagaagagttactttaacccactcattgaggtcacactggatgactccatttgcctggaggcctcagtgagacctgtgtgttcccgtggccttggcgtgccaccaagggaaccatctcttcagtggtgttccctttacagccagacgcaccgcagtaatagtgggtgctactgtgtaagcccagcttccaccctgagtgcacggtgggaccttggctgcccaggccatcctgtcagtgattcagaagttctcagatttggtgggggagggggcatagctataactgcgatttgtcacagaggcattaataggtgctctgaaacatcatttggcaaacaccggactacctccaaggtcatggtgctaagagatatgaaaccactatgtcgtggaggaaaggatgttgttttttggtggagaggatgttgttttcatctcggtacctggtatgttgtggggagttaagagatacatatcgaaaggaacagtgtatatgccacgttggatagttggctggtcttagtttcttgtttttaaaggtgtagttggggatctatagctactggttttcagcagcgtgtaggagcctcacttaatacctggtcacagagcttcttgaagttcaccagactttttgaaagtgtcaggcgggtttagatgtgtgctatgccccagccacctggagaggccactcagtcaaggatgcaggaggggaaagagtaagggttacatggatggggtgccttggtttggagccctgagattttggaggaggtgggacagggcaaaagaaaggcttgttcttgtgcctcggctgcagcacttaggcacaggatttgagaaggagcagcccttggtctgaaaacctgcaaaaaggtttctgatgaggactgcaagtttctggctcacgtgcttacctgatgagtcttcagacactgcctggaagcttctcaagtctcttgtctataatcagctaactaactgactgagtttagttgtaaagtcagcaatgaggaaaaataaaggtctgaaccattgtgccctgggtcaggcttgtgacctgggctgattaattacctggaacagatggtctttgttactgtgagtggtgtgctttccagacttagatagggaatgggtggagggtcagaagatcagcctggaaaggatttgacaagcagtgttaatttcttcatagtgcaataattttagagccaggctaggactattgtggttatccttggtttgacgcaaattgctttgaatgtgcctaagtccttctgactgaaagtaccagatgtagttaattcctggggaaaaaaatattttgcattcttggttctggttggacttaacctgtccagggatgggtttttttgcctctcagtgggctggggcatactgtccagcttatggtgaatcgaggaatggacttatgtgtccctgtgggttagtgaaacctaggactccaggactaggaggctacctgaatagtggtctccacgaccaggaaagtcactttgggtttgggtggggactgtgaagagagagtatgggtaccacaccccatagcagatgtttatagctttgagacagcttttcacaaaaagatctagattgaccatggtactaagctaggggtgagttgtctgtatccctggaagattggcaagagattttgacaaaacttccttttgaggaaactcctgcagtgcatgtaaatggtgccatttacaggattagtaggggagttgtcaagatagacattatcccagtgtgagggaggtgtgtgcttaacatgtgcctgggaagtacattcattgggaatgtggttttgacttattctttggggtctttcctacttgctcatgataatgtgagcccatggcccgacttgagcacccacgtagccagagtgtggcggggctgcctgtggcttgtgcacagagcatgcttgttgagttaatgtgtaagcaggaagcagcttctgtgccaagctatatattagccattcaggcagatcacactctctccagttcctctggacccaagacatcagaagccatgtcgaagcaccacagcgacgccgggacggccttcattcagactcagcagctgcacgcagccatggccgacacattcctggagcacatgtgccgcctggacatcgactcaccgcccattacggcccgaaacaccggcatcatctgtaccatcggtgagcgcgggtgcccactccccctgaaacaagggcttcctgagacagtgatcttttctccccccaaaagactaaatgtagcaaacctgggttctgagcaagatgctacagagagattctcaggggaaatgacgtcatggacttggtcgctcagacctgtccaactctgtgacccatggactgtagcccatgaggcccctctgtccatgggatttgtcagacaggaatactggagtgggttgccatttccttcttcaaactgagttcataggaatttgcaggaaggaattcatatgctttatgtgttctgctaaaggtaaaatttagagggtgttttccatggcagttcttactgtctctgagcatctcagagacctaggaaagatcttgtggacttgctctgttcaaccaaaatgctgtagttggacatctgactgggcttcagggctggctacattttactttggttattaagagttctttaaactgaagcacacttgaagtgttaatcctcttttggataatgaacatttaatgactttcaaacttttgttttgttttttctgaactaggcccagcttcacgagcagtggagacattgaaggagatgattaagtctggaatgaatgtggctcgtttgaacttctctcatggaacccacgaggtgagccttgatggtgtggccccttgggcagcttgtaggaaacagggtgggcatgctgtgtttatttagccacagtggaccaggcaggaagaagtggggaatcaatgggaaggttgtcttcaccagcccatccctaccgttcttccccccagatccctgacatctcaagtggccaagtctccttaagcaaagatgacctgctttgtcattggccatggttctccccaacacctgtgctccgttagcctttgataaggaaagcatggaagggttttcctggaatcccctctaagccatggggcttgacacttctgcaccagggtttctataacagctcataattgcaatgatgaaccagtaagtcaccctgcaggttattctgcctattttcattttagacccatgataaatggggcaggtcccagagaagggtttccactattgcaagtgaaggactgggtcctggtttgtagtaccccacttcatcaacattgtgttcccagcctgtcccttcccaggagttctgggacattaaaataaagtcagcacacttgtctagtgatctgggaggagtatgttagcactggggctgtttatgagctgacttggcccctgggaccaggtgacagctattggaaagtgctccactgtgctgctattcccaagatcggaacaagctcattttgaggagtgtgtgggctgcctgaggaacagtgccatgggatttcatactggcatcaatagaagactagtggaggaggcaagctcttgatcctcttggactctgtatttcctgttcagaataaagaaaatgctgccctgtaaggtcacggggttaaggggttgccctctggcatttggaagttggtgataagtttaaactaaaaataaagcctcagtaaatgcagtccaagaactgtatgcctcctttctggaaacatgagagtgttcctcgtaggttccctaccccatgttccataaacagcttatagccttcaaatgtcacagggacctgaccaagttcagaggaactgcgctcagcaggcaccctggggcaggttaagaagcccacagatggcattcttaattccccaaaggtgaagagtcctccgcaacagtcactaggcattcctgcaggcctgtgcttagcccagagagagagctagagacaccagtgaaggtccattcacaattgatccctcctgctgacttgtgccagggtctgctgtgtgcaggggaaggagcagaaataagaaatagcttttaggaagttgacctttaaccaggctttatggcctcttccatctggtaaaataataccacccagctctgaaatggcagggggagagggtggtatctgcacctgttggagggggctggctcaggggagttggtgttttaaactacaagaagcatttggtgattatctgtgctttgactcttattcccagagttggaatttgttttctttttccacactgtatggcaggatcttagttccccaaccagggatcaaacaaacccagggcccctgccttggaggcacagaatcttaaccactggaccacctgggaagtcccttgtgggtttaatttgaagtttttgaccaggatgaagttatgttgcccctggaatcagttttggaaactgatctgaaatattagttatataatgtaaacagttatagtttgacaaacttccaccttttggccgtttttaatactctactaagcagaacattgggtttgctttctgtccttcactcagacagaggaacatctaccatctgatctctttttttggttttgtttatttggtttattgcatctggccttttgacagctttgccacagtgtctccagcccccgcttttggcagctcttgtgggcaagacgtgtcgtattctccggtgccactcacccggatggtggtggttgaaggatgaggcctacatcctgtgttatcagcagtgtcacactgatagcactaggaacttttgccatcttggctccgagtccctttttagtcaaacagtaatggctaatgggaaagagaaagggcttccagggtgagactgaagccgggatttgttgcaagtgagaaatagcaaaggtcagttagttcagagaagcgtattcctacctctccgtgttccgtttccttttctaatcagactggaggaagtgattgtcagaaccaggcctgcatgacttgagcaacatatttaacttgggctgcgtcagcttaagtaaataactgagtttgaattgcggttgtaatcgatagagaagagctcagaattgtcagatctgtcattctaactctggtggccagagcattattatccagatacaaggtcttttaccccagttgtctgctttgtttgctgagaatgtttgttgaatcctagaggctggagggggaggaaacaagcctcttttatgttgacatgtgttgccaccaaaaaccattaaagatatgggtgtaaatattctaaagttcctaagatttgcccttagagtggatgatggcggtggagaagtgggtgaagagctggtaggaatctgctgtatagcacagggagctcaacttggtgctcggggatgacaagaagtgagtagaggcgaggaggttgatgtaagcaggtagaggatgctcggtgatggaggcagtggtctagaatcctggtgaccagcttcagcgctaatcctagatcccgttgtgtgagatgacagatgtggagcttatcgtctcccctcttttcccctagtaccacgcagagaccatcaagaatgtacgtgaagccacggagagctttgcttcagaccccattctctatcggccagtggcagtggccctggacactaaaggacctgagatccgaactgggctcatcaagggcgtgagtatcttggggagaagcaggagagaaggcataggggaccagaaagcccagaagccacgtttctcaaagtttaggtctataaaggagagttttatccatcagtgtagaaagtcttcctttgacctgctttgctaagaaacagtaccagaaagaaacctcttttacactcaaaatctacttccaagtcttttagggagcagcttatctcttcctctttagtataactgaaacactgcaggttattcttgggttatttccttgaaatatactaagttagaaaaggctttattgttccttccaactgaaatttaatcctggttccctagaggaaaaagctgttctcctgccaggaaggcccagctttggacttgtggcttactctcttgtctgctgcagagcggcaccgctgaggtggagctgaagaagggagccacactgaagatcaccctggacaatgcctacatggaaaagtgtgacgagaacatcctgtggctggactacaagaacatttgcaaggtggtggatgtgggcagcaagatctacgtggatgatgggcttatttctctgctggtgaagcagaaaggtagggacagaagtcggtctgattgtttaaaaccagctcccatctctaatttccttgccagaagataggaaggttgtttggttggcagagagactgaatctatatagtctcaggacttcctttcttttttcaaataatctgtttatttatttatatttattttggctgcgttgggtcttagttgtagcacatggggtctttagttgcaacactggactctgtggcacatgggctcatttttttatggctcgagggcttagtggctgtgcagcctgtgggatcttagttcccccaccagggatcaaactcacttcctatgcattgcaaagtggattcttaaacactggaccaccagggaagtcccaggagttccttttataatgaactcctatcctcaaaaacagatttcactccagttcagttgtactcctggagagcaggtgagaagcgcttttacccatcctcactatttaaagatttgcttccctccttcatccacttaacatggtgtctataggactccagtgtgcctgggaatgatggctaacctttaagtgatctgcagtgttctaagctctttctttacatgtagatttgtttaaattttgaaacaacctaatgagtagatactatcatccctgtggagctgagacactgagaggctgatggacttgctcacagttgaattggagtgtgaaccctggcatgtggctccaccacccaccacgtgccccttcccagttctctcgactggggagagcctgcctcctggtggggacacctgcacccagggctcggcctccccaacctgttccattccatacaggtcctgacttcctggtgacggaggtggagaacggtggctccttgggcagcaagaagggtgtgaacctccctggggctgccgtggacctgcctgctgtgtcagaaaaggacatccaggatctaaagtttggggtggagcagaacgtggatatggtgtttgcgtctttcatccgcaaggcttctgatgtccatgaagtcaggaaggtcctgggagagaaaggaaagaacatcaagataatcagcaaaatcgagaatcatgagggagttcggaggtaagtcccctgcctccttcagccccaaccaagctttctgcagagcaatatgtagcctgccacctgcccattagaaataacgtctcaaacttatttcagacccactgactcagaatatcctatgacattggtgggcttgccagatggccctagtggtaaagaccccacctgccagtgtaggagttgtgagttctgtccttggactgagaagatcccctggtgaagggaatggcaacccactctagtattcttgtctggagtatcccatggacagaggagcctggtgggcaaccatccatggcgtcgcaaaagcagacaaaactgaagtgacttagtgcacacgcctgatactggtattggtatttcaggggggagaaaaaaggcttcacagatgattggggtgccagcaccttgacattgttccagggagcagcactggagagggacagggtcaccaccactcccgggctcaagaaccgtgtgtagtgttcctacactggctacgtttgctggaattgggggccaccaaggggaaagacagcaggctctcaggaggagggggctccttctcttggcaagcagtgggattgttggttggggcagctctggcgtggcatccacctccctggggaaaacatgccgtcttcctctggttctgcgtggtcccaatcctgctccactgcttccccagtgctcaccaggcagagccacacgagtgaggccagctgggtgacatctactcctgcttggcctccctactgacagcccaggcttacatgaggggtcaggtgtgtgcatgggaagagtgggaggagccgtgccgcccactgttgcagccttgccatccttagctttgtgtctgtgtccgttgtacggggaaattcagggccctccctctgccatcctgatgagccatgggcacctgctgactttggcttcaggccaggcaaggccatgttcttgtgccttcaacacactggggagggacctctgaaggagcagccttccagtgtccttgactggaagaggccacggacctttgtgtcaagagcagtcagccaccttgggttccatttctgccccagcggtgatgactgaaatgcagatggtagagacacctcaagagggacctcataagatgcaggtggacactgagaatggacttagggttaccagaggggaacgatgggaggaaggaatggtcagggagtttgggatggacctgtacacgcttctgtatttaaaatggatgacccacaaggactactgtagagcacagggaactctgctcggtgttacatggcaacctgggtgggaggagggtctaggggagagtgggtgcacatatgtgtatggctgagtcgctctgctgtgcatctgaaaccatcaagacatggttaatagctatacctcagtataaaataaaaagttaagggaaaaaagacagatggagaggaagtgaacccatgggattttggaggagacccccctggcccctccccttcccctcagtgaagtgtccatcctggtgctgaaggagtccagcgagcagaactgttggcccctttgggggactgagacagctggaacacccctgtgatgatgtcatgggtacttgtcctggtgcaagaatggccaagtcagagaatcccgggaaactttgtgccaccgtacgcgaggcccctgtttgtataacctctgtctctgcaacttgcctgtcaggtttgacgagatcctggaagccagtgatgggatcatggtggctcgtggtgatctgggcattgagatccctgcagagaaggtcttccttgcccagaagatgatgattggtcggtgcaaccgagctgggaagcccgtcatctgtgccacacaggtgtgtgcctctccctgagcgtgcatccttgtacaaggaagctctggaggctacctggtctcttcccatggaccctgccccacatcatacacaaacctattccccccacctgcccccacacacctacacaaagctggattctgtacatacatgctctccagggggtcaccttgtgtccaaagccctcccaggccacatctcacaaatactgtgtcccctcccagatgctggagagcatgatcaagaagcctcgccctacccgggcggagggcagtgacgtggccaatgccgtcttggatggagccgactgcatcatgctgtccggagagacggccaaaggggactaccccctggaagctgtccgcatgcagcacctggtaagttctcccgctgcgggtggaggcaaactccagcatatgggggcaccttgtagtgtcaccctctgtgccctcgatcttttattgtcctccaagtcacacgcagagtgaggaggtgtgtgctggagtcatgggggtgtcttttttgatgggtttttttttttgctcttctgccttcctgcccacacccatctcctagtcccttctgttctggaggcggcctccttcatcacacgtagcacagttcactcccatcttcggggtgtgaatccttcctttgcttgagtcctgggatatctgtactgcttccccctggacagtctagaggacctgagcccttcttccctgttctggaaaagtccaagagctcctgctcccagctggcctgtgtttggcttccattttgattccccacctgtcccagccagtgcctccccgacggggtcctctgggcctgcactgatttggctgtgagctggccttgcatggtacctgcagcagcgcctgctttgctgagctgttgcactcaccctagcagtggggtttaagggaggggtgacaggcccacaaatagaagcaggtggaaggctggctgatcccagctggccctggggtgagagtgtctggaggagccctagtggccgctcctcattctcctgtgggagctagcttttccagggtcttctgctggaccatgtcccacagcctggctgcctctgctctaaagcatcctaaagaggaacacaggcctggggaaacgagcgctacagatggactttcacaagggtcctaggtggctgttgataatgtatagctcagcaaactgtttctttaaccctcctgttcattttccagccagcaaaggaccccaggccctttgtgtgacatccctccaatgcatcctcccccaaaaaacctctggactagataccatcctttccttcttcactttctaagtgattaggctcaagtggcttccaaagaagacatgacagtcacagtggatactttctcaggggtgaaacaagacatcttgactacagatgttttctggtctgtccttggtgttctgggtggatttgcccctaatgaaatcagtagagaccagtgtctgcccttgggacagctgtgtttttctggctgatggccaccccctgtgtgacatgactgctgtcctgatgctcatgcactgcaggctcacggttcttctcacctgtcccagtgagtacttcctctctcctgggagatagtgaccttgaaccagtcccctctagagtggttgatgttagtgtttatgggtttccatatagaattatatacatatactgtaacgataactgctttgcttagtcatgtggccccacggcctctgagaccttgacacgttagactttagggactttgtgtctttgggcacatcattggacctctcaaggccttatctaagaagtgaattagatgggatatgtttaattacaccctttgcgttaaattgcactgctgttataaaatgtctgctaagaacctcatgcaggttcttaacctcagtgaggtcaatgtcaacccacttctaatggatgagggcacatgataatcgagcttgagtttggacccaggtcagctgactctgaagccagcattccctcttagaacacatctagcagatcaggacaggtgtcctgtggggcctgtcctggggtcagagactaaaccagactccgggctctgcaagcatgtctgtttttccaaacccaatcttttctttgaacaaacaccttagaactgtgagactgggattgcatggccctattcaggaggtgagttctcctggccgtgtcaccagttaacactggccaatagcttcccctcttaactgtccactgctttctcctgtaactgacgcaattgacgttcttaactatgggctaggtagtaccagctgtggttctctttcctgttcatgtgccctgtcctcctgggctgcatgcattccattcttgcaggaagaaaccctttaacctagcaaattcagccactcattggctcatcctgtcagattaatgagatggcgttactgattcttccctcacccatcattgtctaagacgctcataactgcattataaccctctaaagcttaagttttctaattcttggtgttacctgagcaagatggtctgaataacacagtggctttctcatgggtgttttaatcattcaattttaatcaaatgccttggtaagcttacctgtgtgcttccacaggcacctgactcttcacatggctgttcgttgtgccccttacaagcttgccagtttccagctgcccgcttagaatgtggtcaagctgcgtgtccttggctttgaccccagctttctagcgctgctcaatgtgcttctgccgcaggccactggagaggcaggcagcatctctgtgtctgaagccaagcaagcactccatgtgtgcatggaggaggccaggcacgaagccctgtggtaactaggcagccatgtgaggaggggggcctattccttcctgcgagctatgtcatgaggcagtgtggtcgagtcctgccagggagccgtggaggggccccagcctccgcatgtttctatgctgaggcgttagagcctgccgtcatattgtctccctcacccccaccgccagtcatggagacctaccaaaatcaagagatccttccagaatggaagaaccagtttcctctctgatggaggaggaacagtagccattgacgcttgaacttccctgagcaggctttcaccaccctgcctctttgcatctgcctgaaggagagacttagccaattaacctacagtaccttcctctcattaattccccgttctgtctttccatgttgttgtctcttgtttgtttccccccaccctccttcttccctcttccttgcctcccctcctctaaaccttacagatagctcgtgaggctgaggcagccatgttccaccgcaagctgtttgaagaacttgcgcgagcctcaagtcactccacagacctcatggaagccatggccatgggcagcgtggaggcttcatataagtgtttagcagcagctttgatagttctcacggagtctggcaggtagggccccgagggcaggtaactctgtaggataaacagccttttgctccagccactctagacgacagccagggcccagccctgagcctaggacgctcctctcgtctgcaggaagccagccagggaggtcagggcaggacagggccacaggatcctccggctcagaaggcacagccatgtcacaggcacctggtgaggggctggttcctgcaagtctcgatctcactcagctcagaacctccagtgatcgggctgttcttggccactgtacccagggacttgctcctccccagctgtctgtgcgactcttcccctccccgtcccgtgtgacacggctctgacagctctgtccccctcgtccctctggacggatgttgcccctagattgcccgtgaggcagaggctgccatctaccatttgcaattgttcgaggagctccgtcgcctgtcacccattaccagcgaccccaccgaagctgccgctgtgggggccgtggaggcgtccttcaagtgctgcagtggggccataatcgtcctcaccaagtctggcaggtaggaggtggcagcaggtccctgggaatgccccgctcagcggcccctttccttgggggtcctgggagcgtgtactgcacggtgctcagatggcattgagccaaggtaagacccctctgcctgcaccccggaccctgcagggaaggagccccctccccctcccccacccagccccccaggcggcacttagtgggtccaaagcgagttttattaaccctcacaacgagctagacttaatcagataactacaggtagcctgaggacaagtggttatttgatattgaaaagctgttcttaaaaaggaaaggaccaccagttttacttctagctaagtgctctttaaaaaagtccagtttgcaaaatgagtttgcaaaaaaagtccagtttgctgacagtgctatttggttggtgtgcctgtcccatctgtctttgagtcccacagataagtgggtgctgcctaggaaaggtcactgtgctatcttgctggcactcgggccaggcaaccagtctgagacctctacttggcctctggcttgagtcccttccaaatccaggatctcaagttaataccccttgctccctgggtctgggggtatgctgctcctccctggggcagctagggtttcctggaggagggaggtggagaggagcagacaggcacccccgtacgccaaggagcagcagctgggactgcctttaggaccaggacacaagatgtgtgccgagtcccgcagtagagggcttagggtaaaaagctccagccgttagggttgacctttgtgaaaaggtccaacctttgctacttggctatttttagtccagtcttctggggtttcactctcagtgagtcctgacttcagcacttgcttccctcagaaaaccttgtatggaggccaggccttaagcagggcatcctctgctgtgacatggcttaagtttccctgacagctgttgcgtgtcctcacagcttgccttctgagcctcgggtcccctgccagcagccccctccaactcctgagacaccagctcctaccagtgtacagtgtcagtgttgaaggaagcatccagcctttgagtttaaaggggcccagtcccctccaggggatccttcataggcagagcctcccccgctgacactccatcccctagtactgccttctgggtagcacttatatttctaatcctcagcctcgcttagatactcaggtttgactctggggctctacagcccagttgctgggactatttcaggggcctgggggtcatgtggagtcaggagagggcacagcagtaggcaaggcttgtcttgtagatttcccaggcaggctggtggtctctgctcctggtttgggtttttttttttttttttttgcagatgtcaagtgtcaggtggtcttcacatgctgcttggcttgtagctgttgctggcagcaagagaaaaggatgtggtgggcttggacagggctgcttccctgtgccagaatgggaaagttcagggaatggtggggggtctgccaagtatgggccatgtggagtaagtgggtaagactgaccatgctgggtcagtatgatcctgcggccctggcctgtaggaggggtttagggtagcatagctctaaagaatatgctatggcagatacagggtgatgggacacctcagtcttgggagcaaatgttgaaatggtcagagcctcaggctggcagagttggattccagggtgagttgttgctgaaggccctgaggggactgtttaaccatcttgtctgcctaccccatctcaggtctgcacatcaggtggccagataccgcccccgggcccccatcattgctgtgactcggaatcaccagacagctcgccaggcccacctataccgcggcatcttccctgtggtgtgtaaggacccagtgcaggaggcctgggctgaggacgtggatctccgggtgaacttggccatgaatgttggtgcgtgtctgggagagaaagctcccggtggagggctggggaaggtgctagagcactggcttctctgagaccctattgaaagaggaacatgccagcctttgtgggcaagagctggcctcactaggaatgttctctggttccttcccagtccctggagtcctgggctacgctcagggcagggagaggacctttgacgtgtggggctgagcagcccaggttctcacctcacgttctttgggagtgggatccaaagcaaaggatcctggataatcacctttgtccattctttggcacttgctcattattgaggttttttttttcttccctataaaattaaccagatctcctacacttggggccagtacacatttagattatgtactcaaatggcctttgtcacagtataaaagtaggatgtcacaggatgagaggaaacagcgagctgtgaccttgggctgggctctccaccttcttgagtagaaaataaatgatgtccaaaggtccctgctacctctgccatctgagtgataaggaaataataccaaggcctccctcattccctttgcctgggctgtgagcctggcgccaccttgtggtgtaagaaagtaaaggcctgtcagcccttcctcagttgtggggcactccaatactttggccacctcatgtgaagagttgactcattggaaaagactctgatgctgggagggattgggggcaggaggagaaggggatgacagaggatgagatggctggatggcatcgactcgatggacatgagtttgagtgaactccaggagttggtgatggacagggaggcctggcgtgctgcgattcatgaggtcgcaaagagtcggacacgactgagtgactgaactgaactcccaagtgtataccttcttggcttaatttttcatttaccagctctcttctcttcttccaggaaaggcccgaggcttcttcaagaagggagacgtggtcattgtgctgaccgggtggcgccctggttccggcttcaccaacaccatgcgtgtagttcctgtgccatgatggactccgaagcccctcctccagcccctgtcccacccctcttccccaaaccatccgttaggccagcattgcttgtagtgctcacttggggctgtaatgtggcactggtgggctgggacaccagggaagaagatgaatacctctgtgaaacctggctggttttaagactttgcttgggtcgggtagttcagagctgggccactcatcacgtggctgcatccaagcaggggatgcaggagggatgcaggcaggactggaggctccagagcttcacacacagggcaacagctcctgcttcccttcctttgtatacccgattcagctcctgcagaaaatggatatccagagaattcccagccctggcccgtgatcaagagtaggggccttagggcatggggcagtggttccagtttaagtagactctggccctggcccttacttgcttctccaaccccctcagcctccctccccttgtgcaccgtatacttctcttccttcactccacccagccgatgctgcaaacactccaccccccatcttccatttcccccactactgcagctgcctccaggcttgttgctatagagcctacctgtatgtcaataaacaacagctgaagcacc